European Patent Specification EP 3 087 187 B1, published December 11, 2024. Title: A METHOD OF GENERATING ADENOVIRUS CONSTRUCTS, PLASMIDS, VIRUSES AND VECTORS OBTAINED THEREFROM. Applicant: Psioxus Therapeutics. The sequence listing filed with the application follows.

SEQUENCE LISTING (43 sequences)

SEQ ID NO: 1 - DNA, 32322 bp, Artificial Sequence
  ColoAd1 genome
tatctatataatataccttatagatggaatggtgccaatatgtaaatgaggtgattttaaaaagtgtggatcgtgtggtgattggctgtggggttaacggctaaaaggggcggtgcgaccgtgggaaaatgacgttttgtgggggtggagtttttttgcaagttgtcgcgggaaatgtgacgcataaaaaggcttttttctcacggaactacttagttttcccacggtatttaacaggaaatgaggtagttttgaccggatgcaagtgaaaattgttgattttcgcgcgaaaactgaatgaggaagtgtttttctgaataatgtggtatttatggcagggtggagtatttgttcagggccaggtagactttgacccattacgtggaggtttcgattaccgtgttttttacctgaatttccgcgtaccgtgtcaaagtcttctgtttttacgtaggtgtcagctgatcgctagggtatttatacctcagggtttgtgtcaagaggccactcttgagtgccagcgagaagagttttctcctctgcgccggcagtttaataataaaaaaatgagagatttgcgatttctgcctcaggaaataatctctgctgagactggaaatgaaatattggagcttgtggtgcacgccctgatgggagacgatccggagccacctgtgcagctttttgagcctcctacgcttcaggaactgtatgatttagaggtagagggatcggaggattctaatgaggaagctgtaaatggcttttttaccgattctatgcttttagctgctaatgaagggttagaattagatccgcctttggacacttttgatactccaggggtaattgtggaaagcggtacaggtgtaagaaaattacctgatttgagttccgtggactgtgatttgcactgctatgaagacgggtttcctccgagtgatgaggaggaccatgaaaaggagcagtccatgcagactgcagcgggtgagggagtgaaggctgccaatgttggttttcagttggattgcccggagcttcctggacatggctgtaagtcttgtgaatttcacaggaaaaatactggagtaaaggaactgttatgttcgctttgttatatgagaacgcactgccactttatttacagtaagtgtgtttaagttaaaatttaaaggaatatgctgtttttcacatgtatattgagtgtgagttttgtgcttcttattataggtcctgtgtctgatgctgatgaatcaccatctcctgattctactacctcacctcctgagattcaagcacctgttcctgtggacgtgcgcaagcccattcctgtgaagcttaagcctgggaaacgtccagcagtggaaaaacttgaggacttgttacagggtggggacggacctttggacttgagtacacggaaacgtccaagacaataagtgttccatatccgtgtttacttaaggtgacgtcaatatttgtgtgacagtgcaatgtaataaaaatatgttaactgttcactggtttttattgctttttgggcggggactcaggtatataagtagaagcagacctgtgtggttagctcataggagctggctttcatccatggaggtttgggccattttggaagaccttaggaagactaggcaactgttagagaacgcttcggacggagtctccggtttttggagattctggttcgctagtgaattagctagggtagtttttaggataaaacaggactataaacaagaatttgaaaagttgttggtagattgcccaggactttttgaagctcttaatttgggccatcaggttcactttaaagaaaaagttttatcagttttagacttttcaaccccaggtagaactgctgctgctgtggcttttcttacttttatattagataaatggatcccgcagactcatttcagcaggggatacgttttggatttcatagccacagcattgtggagaacatggaaggttcgcaagatgaggacaatcttaggttactggccagtgcagcctttgggtgtagcgggaatcctgaggcatccaccggtcatgccagcggttctggaggaggaacagcaagaggacaacccgagagccggcctggaccctccagtggaggaggcggagtagctgacttgtctcctgaactgcaacgggtgcttactggatctacgtccactggacgggataggggcgttaagagggagagggcatctagtggtactgatgctagatctgagttggctttaagtttaatgagtcgcagacgtcctgaaaccatttggtggcatgaggttcagaaagagggaagggatgaagtttctgtattgcaggagaaatattcactggaacaggtgaaaacatgttggttggagcctgaggatgattgggaggtggccattaaaaattatgccaagatagctttgaggcctgataaacagtataagattactagacggattaatatccggaatgcttgttacatatctggaaatggggctgaggtggtaatagatactcaagacaaggcagttattagatgctgcatgatggatatgtggcctggggtagtcggtatggaagcagtaacttttgtaaatgttaagtttaggggagatggttataatggaatagtgtttatggccaataccaaacttatattgcatggttgtagcttttttggtttcaacaatacctgtgtagatgcctggggacaggttagtgtacggggatgtagtttctatgcgtgttggattgccacagctggcagaaccaagagtcaattgtctctgaagaaatgcatatttcaaagatgtaacctgggcattctgaatgaaggcgaagcaagggtccgccactgcgcttctacagatactggatgttttattttgattaagggaaatgccagcgtaaagcataacatgatttgcggtgcttccgatgagaggccttatcaaatgctcacttgtgctggtgggcattgtaatatgctggctactgtgcatattgtttcccatcaacgcaaaaaatggcctgtttttgatcacaatgtgatgacgaagtgtaccatgcatgcaggtgggcgtagaggaatgtttatgccttaccagtgtaacatgaatcatgtgaaagtgttgttggaaccagatgccttttccagaatgagcctaacaggaatttttgacatgaacatgcaaatctggaagatcctgaggtatgatgatacgagatcgagggtacgcgcatgcgaatgcggaggcaagcatgccaggttccagccggtgtgtgtagatgtgactgaagatctcagaccggatcatttggttattgcccgcactggagcagagttcggatccagtggagaagaaactgactaaggtgagtattgggaaaactttggggtgggattttcagatggacagattgagtaaaaatttgttttttctgtcttgcagctgtcatgagtggaaacgcttcttttaaggggggagtcttcagcccttatctgacagggcgtctcccatcctgggcaggagttcgtcagaatgttatgggatctactgtggatggaagacccgtccaacccgccaattcttcaacgctgacctatgctactttaagttcttcacctttggacgcagctgcagctgccgccgccgcttctgttgccgctaacactgtgcttggaatgggttactatggaagcatcatggctaattccacttcctctaataacccttctaccctgactcaggacaagttacttgtccttttggcccagctggaggctttgacccaacgtctgggtgaactttctcagcaggtggtcgagttgcgagtacaaactgagtctgctgtcggcacggcaaagtctaaataaaaaaatcccagaatcaatgaataaataaacaagcttgttgttgatttaaaatcaagtgtttttatttcatttttcgcgcacggtatgccctagaccaccgatctctatcattgagaactcggtggattttttccaggatcctatagaggtgggattgaatgtttagatacatgggcattaggccgtctttggggtggagatagctccattgaagggattcatgctccggggtagtgttgtaaatcacccagtcataacaaggtcgcagtgcatggtgttgcacaatatcttttagaagtaggctgattgccacagataagcccttggtgtaggtgtttacaaaccggttgagctgggatgggtgcattcggggtgaaattatgtgcattttggattggatttttaagttggcaatattgccgccaagatcccgtcttgggttcatgttatgaaggaccaccaagacggtgtatccggtacatttaggaaatttatcgtgcagcttggatggaaaagcgtggaaaaatttggagacacccttgtgtcctccaagattttccatgcactcatccatgataatagcaatggggccgtgggcagcggcgcgggcaaacacgttccgtgggtctgacacatcatagttatgttcctgagttaaatcatcataagccattttaatgaatttggggcggagagtaccagattggggtatgaatgttccttcgggccccggagcatagttcccctcacagatttgcatttcccaagctttcagttccgagggtggaatcatgtccacctggggggctatgaaaaacaccgtttctggggcgggggtgattaattgtgatgatagcaaatttctgagcaattgagatttgccacatccggtggggccataaatgattccgattacgggttgcaggtggtagtttagggaacggcaactgccgtcttctcgaagcaagggggccacctcgttcatcatttcccttacatgcatattttcccgcaccaaatccattaggaggcgctctcctcctagtgatagaagttcttgtagtgaggaaaagtttttcagcggtttcagaccgtcagccatgggcattttggagagagtttgctgcaaaagttctagtctgttccacagttcagtgatgtgttctatggcatctcgatccagcagacctcctcgtttcgcgggtttggacggctcctggaatagggtatgagacgatgggcgtccagcgctgccagggttcggtccttccagggtctcagtgttcgagtcagggttgtttccgtcacagtgaaggggtgtgcgcctgcttgggcgcttgccagggtgcgcttcagactcatcctgctggtcgaaaacttctgtcgcttggcgccctgtatgtcggccaagtagcagtttaccatgagttcgtagttgagcgcctcggctgcgtggcctttggcgcggagcttacctttggaagttttcttgcataccgggcagtataggcatttcagcgcatacaacttgggcgcaaggaaaacggattctggggagtatgcatctgcgccgcaggaggcgcaaacagtttcacattccaccagccaggttaaatccggttcattggggtcaaaaacaagttttccgccatattttttgatgcgtttcttacctttggtctccatgagttcgtgtcctcgttgagtgacaaacaggctgtccgtgtccccgtagactgattttacaggcctcttctccagtggagtgcctcggtcttcttcgtacaggaactctgaccactctgatacaaaggcgcgcgtccaggccagcacaaaggaggctatgtgggaggggtagcgatcgttgtcaaccagggggtccaccttttccaaagtatgcaaacacatgtcaccctcttcaacatccaggaatgtgattggcttgtaggtgtatttcacgtgacctggggtccccgctgggggggtataaaagggggcggttctttgctcttcctcactgtcttccggatcgctgtccaggaacgtcagctgttggggtaggtattccctctcgaaggcgggcatgacctctgcactcaggttgtcagtttctaagaacgaggaggatttgatattgacagtgccggttgagatgcctttcatgaggttttcgtccatctggtcagaaaacacaatttttttattgtcaagtttggtggcaaatgatccatacagggcgttggataaaagtttggcaatggatcgcatggtttggttcttttccttgtccgcgcgctctttggcggcgatgttgagttggacatactcgcgtgccaggcacttccattcggggaagatagttgttaattcatctggcacgattctcacttgccaccctcgattatgcaaggtaattaaatccacactggtggccacctcgcctcgaaggggttcattggtccaacagagcctacctcctttcctagaacagaaagggggaagtgggtctagcataagttcatcgggagggtctgcatccatggtaaagattcccggaagtaaatccttatcaaaatagctgatgggagtggggtcatctaaggccatttgccattctcgagctgccagtgcgcgctcatatgggttaaggggactgccccatggcatgggatgggtgagtgcagaggcatacatgccacagatgtcatagacgtagatgggatcctcaaagatgcctatgtaggttggatagcatcgcccccctctgatacttgctcgcacatagtcatatagttcatgtgatggcgctagcagccccggacccaagttggtgcgattgggtttttctgttctgtagacgatctggcgaaagatggcgtgagaattggaagagatggtgggtctttgaaaaatgttgaaatgggcatgaggtagacctacagagtctctgacaaagtgggcataagattcttgaagcttggttaccagttcggcggtgacaagtacgtctagggcgcagtagtcaagtgtttcttgaatgatgtcataacctggttggtttttcttttcccacagttcgcggttgagaaggtattcttcgcgatccttccagtactcttctagcggaaacccgtctttgtctgcacggtaagatcctagcatgtagaactgattaactgccttgtaagggcagcagcccttctctacgggtagagagtatgcttgagcagcttttcgtagcgaagcgtgagtaagggcaaaggtgtctctgaccatgactttgaggaattggtatttgaagtcgatgtcgtcacaggctccctgttcccagagttggaagtctacccgtttcttgtaggcggggttgggcaaagcgaaagtaacatcattgaagagaatcttgccggccctgggcatgaaattgcgagtgatgcgaaaaggctgtggtacttccgctcggttattgataacctgggcagctaggacgatctcgtcgaaaccgttgatgttgtgtcctacgatgtataattctatgaaacgcggcgtgcctctgacgtgaggtagcttactgagctcatcaaaggttaggtctgtggggtcagataaggcgtagtgttcgagagcccattcgtgcaggtgaggattcgctttaaggaaggaggaccagaggtccactgccagtgctgtttgtaactggtcccggtactgacgaaaatgccgtccgactgccattttttctggggtgacgcaatagaaggtttgggggtcctgccgccagcgatcccacttgagttttatggcgaggtcataggcgatgttgacgagccgctggtctccagagagtttcatgaccagcatgaaggggattagctgcttgccaaaggaccccatccaggtgtaggtttccacatcgtaggtgagaaagagcctttctgtgcgaggatgagagccaatcgggaagaactggatctcctgccaccagttggaggaatggctgttgatgtgatggaagtagaactccctgcgacgcgccgagcattcatgcttgtgcttgtacagacggccgcagtagtcgcagcgttgcacgggttgtatctcgtgaatgagttgtacctggcttcccttgacgagaaatttcagtgggaagccgaggcctggcgattgtatctcgtgctttactatgttgtctgcatcggcctgttcatcttctgtctcgatggtggtcatgctgacgagccctcgcgggaggcaagtccagacctcggcgcggcaggggcggagctcgaggacgagagcgcgcaggctggagctgtccagggtcctgagacgctgcggactcaggttagtaggcagtgtcaggagattaacttgcatgatcttttggagggcgtgcgggaggttcagatagtacttgatctcaacgggtccgttggtggagatgtcgatggcttgcagggttccgtgtcccttgggcgctaccaccgtgcccttgtttttcattttggacggcggtggctctgttgcttcttgcatgtttagaagcggtgtcgagggcgcgcaccgggcggcaggggcggctcgggacccggcggcatggctggcagtggtacgtcggcgccgcgcgcgggtaggttctggtactgcgccctgagaagactcgcatgcgcgacgacgcggcggttgacatcctggatctgacgcctctgggtgaaagctaccggccccgtgagcttgaacctgaaagagagttcaacagaatcaatctcggtatcgttgacggcggcttgcctaaggatttcttgcacgtcaccagagttgtcctggtaggcgatctccgccatgaactgctcgatctcttcctcttgaagatctccgcggcccgctctctcgacggtggccgcgaggtcgttggagatgcgcccaatgagttgagagaatgcattcatgcccgcctcgttccagacgcggctgtagaccacggcccccacgggatctctcgcgcgcatgaccacctgggcgaggttgagctccacgtggcgggtgaagaccgcatagttgcataggcgctggaaaaggtagttgagtgtggtggcgatgtgctcggtgacgaagaaatacatgatccatcgtctcagcggcatctcgctgacatcgcccagagcttccaagcgctccatggcctcgtagaagtccacggcaaaattaaaaaactgggagtttcgcgcggacacggtcaactcctcttccagaagacggataagttcggcgatggtggtgcgcacctcgcgctcgaaagcccctgggatttcttcctcaatctcttcttcttccactaacatctcttcctcttcaggtggggctgcaggaggagggggaacgcggcgacgccggcggcgcacgggcagacggtcgatgaatctttcaatgacctctccgcggcggcggcgcatggtttcagtgacggcgcggccgttctcgcgcggtcgcagagtaaaaacaccgccgcgcatctccttaaagtggtgactgggaggttctccgtttgggagggagagggcgctgattatacattttattaattggcccgtagggactgcacgcagagatctgatcgtgtcaagatccacgggatctgaaaacctttcgacgaaagcgtctaaccagtcacagtcacaaggtaggctgagtacggcttcttgtgggcgggggtggttatgtgttcggtctgggtcttctgtttcttcttcatctcgggaaggtgagacgatgctgctggtgatgaaattaaagtaggcagttctaagacggcggatggtggcgaggagcaccaggtctttgggtccggcttgctggatacgcaggcgattggccattccccaagcattatcctgacatctagcaagatctttgtagtagtcttgcatgagccgttctacgggcacttcttcctcacccgttctgccatgcatacgtgtgagtccaaatccgcgcattggttgtaccagtgccaagtcagctacgactctttcggcgaggatggcttgctgtacttgggtaagggtggcttgaaagtcatcaaaatccacaaagcggtggtaagctcctgtattaatggtgtaagcacagttggccatgactgaccagttaactgtctggtgaccagggcgcacgagctcggtgtatttaaggcgcgaataggcgcgggtgtcaaagatgtaatcgttgcaggtgcgcaccagatactggtaccctataagaaaatgcggcggtggttggcggtagagaggccatcgttctgtagctggagcgccaggggcgaggtcttccaacataaggcggtgatagccgtagatgtacctggacatccaggtgattcctgcggcggtagtagaagcccgaggaaactcgcgtacgcggttccaaatgttgcgtagcggcatgaagtagttcattgtaggcacggtttgaccagtgaggcgcgcgcagtcattgatgctctatagacacggagaaaatgaaagcgttcagcgactcgactccgtagcctggaggaacgtgaacgggttgggtcgcggtgtaccccggttcgagacttgtactcgagccggccggagccgcggctaacgtggtattggcactcccgtctcgacccagcctacaaaaatccaggatacggaatcgagtcgttttgctggtttccgaatggcagggaagtgagtcctattttttttttttgccgctcagatgcatcccgtgctgcgacagatgcgcccccaacaacagcccccctcgcagcagcagcagcagcaatcacaaaaggctgtccctgcaactactgcaactgccgccgtgagcggtgcgggacagcccgcctatgatctggacttggaagagggcgaaggactggcacgtctaggtgcgccttcacccgagcggcatccgcgagttcaactgaaaaaagattctcgcgaggcgtatgtgccccaacagaacctatttagagacagaagcggcgaggagccggaggagatgcgagcttcccgctttaacgcgggtcgtgagctgcgtcacggtttggaccgaagacgagtgttgcgggacgaggatttcgaagttgatgaaatgacagggatcagtcctgccagggcacacgtggctgcagccaaccttgtatcggcttacgagcagacagtaaaggaagagcgtaacttccaaaagtcttttaataatcatgtgcgaaccctgattgcccgcgaagaagttacccttggtttgatgcatttgtgggatttgatggaagctatcattcagaaccctactagcaaacctctgaccgcccagctgtttctggtggtgcaacacagcagagacaatgaggctttcagagaggcgctgctgaacatcaccgaacccgaggggagatggttgtatgatcttatcaacattctacagagtatcatagtgcaggagcggagcctgggcctggccgagaaggtggctgccatcaattactcggttttgagcttgggaaaatattacgctcgcaaaatctacaagactccatacgttcccatagacaaggaggtgaagatagatgggttctacatgcgcatgacgctcaaggtcttgaccctgagcgatgatcttggggtgtatcgcaatgacagaatgcatcgcgcggttagcgccagcaggaggcgcgagttaagcgacagggaactgatgcacagtttgcaaagagctctgactggagctggaaccgagggtgagaattacttcgacatgggagctgacttgcagtggcagcctagtcgcagggctctgagcgccgcgacggcaggatgtgagcttccttacatagaagaggcggatgaaggcgaggaggaagagggcgagtacttggaagactgatggcacaacccgtgttttttgctagatggaacagcaagcaccggatcccgcaatgcgggcggcgctgcagagccagccgtccggcattaactcctcggacgattggacccaggccatgcaacgtatcatggcgttgacgactcgcaaccccgaagcctttagacagcaaccccaggccaaccgtctatcggccatcatggaagctgtagtgccttcccgctctaatcccactcatgagaaggtcctggccatcgtgaacgcgttggtggagaacaaagctattcgtccagatgaggccggactggtatacaacgctctcttagaacgcgtggctcgctacaacagtagcaatgtgcaaaccaatttggaccgtatgataacagatgtacgcgaagccgtgtctcagcgcgaaaggttccagcgtgatgccaacctgggttcgctggtggcgttaaatgctttcttgagtactcagcctgctaatgtgccgcgtggtcaacaggattatactaactttttaagtgctttgagactgatggtatcagaagtacctcagagcgaagtgtatcagtccggtcctgattacttctttcagactagcagacagggcttgcagacggtaaatctgagccaagcttttaaaaaccttaaaggtttgtggggagtgcatgccccggtaggagaaagagcaaccgtgtctagcttgttaactccgaactcccgcctattattactgttggtagctcctttcaccgacagcggtagcatcgaccgtaattcctatttgggttacctactaaacctgtatcgcgaagccatagggcaaagtcaggtggacgagcagacctatcaagaaattacccaagtcagtcgcgctttgggacaggaagacactggcagtttggaagccactctgaacttcttgcttaccaatcggtctcaaaagatccctcctcaatatgctcttactgcggaggaggagaggatccttagatatgtgcagcagagcgtgggattgtttctgatgcaagagggggcaactccgactgcagcactggacatgacagcgcgaaatatggagcccagcatgtatgccagtaaccgacctttcattaacaaactgctggactacttgcacagagctgccgctatgaactctgattatttcaccaatgccatcttaaacccgcactggctgcccccacctggtttctacacgggcgaatatgacatgcccgaccctaatgacggatttctgtgggacgacgtggacagcgatgttttttcacctctttctgatcatcgcacgtggaaaaaggaaggcggcgatagaatgcattcttctgcatcgctgtccggggtcatgggtgctaccgcggctgagcccgagtctgcaagtccttttcctagtctacccttttctctacacagtgtacgtagcagcgaagtgggtagaataagtcgcccgagtttaatgggcgaagaggagtatctaaacgattccttgctcagaccggcaagagaaaaaaatttcccaaacaatggaatagaaagtttggtggataaaatgagtagatggaagacttatgctcaggatcacagagacgagcctgggatcatggggattacaagtagagcgagccgtagacgccagcgccatgacagacagaggggtcttgtgtgggacgatgaggattcggccgatgatagcagcgtgctggacttgggtgggagaggaaggggcaacccgtttgctcatttgcgccctcgcttgggtggtatgttgtaaaaaaaaataaaaaaaaaactcaccaaggccatggcgacgagcgtacgttcgttcttctttattatctgtgtctagtataatgaggcgagtcgtgctaggcggagcggtggtgtatccggagggtcctcctccttcgtacgagagcgtgatgcagcagcagcaggcgacggcggtgatgcaatccccactggaggctccctttgtgcctccgcgatacctggcacctacggagggcagaaacagcattcgttattcggaactggcacctcagtacgataccaccaggttgtatctggtggacaacaagtcggcggacattgcttctctgaactatcagaatgaccacagcaacttcttgaccacggtggtgcaaaacaatgactttacccctacggaagccagcacccagaccattaactttgatgaacgatcgcggtggggcggtcagctaaagaccatcatgcatactaacatgccaaacgtgaacgagtatatgtttagtaacaagttcaaagcgcgtgtgatggtgtccagaaaacctcccgacggtgctgcagttggggatacttatgatcacaagcaggatattttgaaatatgagtggttcgagtttactttgccagaaggcaacttttcagttactatgactattgatttgatgaacaatgccatcatagataattacttgaaagtgggtagacagaatggagtgcttgaaagtgacattggtgttaagttcgacaccaggaacttcaagctgggatgggatcccgaaaccaagttgatcatgcctggagtgtatacgtatgaagccttccatcctgacattgtcttactgcctggctgcggagtggattttaccgagagtcgtttgagcaaccttcttggtatcagaaaaaaacagccatttcaagagggttttaagattttgtatgaagatttagaaggtggtaatattccggccctcttggatgtagatgcctatgagaacagtaagaaagaacaaaaagccaaaatagaagctgctacagctgctgcagaagctaaggcaaacatagttgccagcgactctacaagggttgctaacgctggagaggtcagaggagacaattttgcgccaacacctgttccgactgcagaatcattattggccgatgtgtctgaaggaacggacgtgaaactcactattcaacctgtagaaaaagatagtaagaatagaagctataatgtgttggaagacaaaatcaacacagcctatcgcagttggtatctttcgtacaattatggcgatcccgaaaaaggagtgcgttcctggacattgctcaccacctcagatgtcacctgcggagcagagcaggtctactggtcgcttccagacatgatgaaggatcctgtcactttccgctccactagacaagtcagtaactaccctgtggtgggtgcagagcttatgcccgtcttctcaaagagcttctacaacgaacaagctgtgtactcccagcagctccgccagtccacctcgcttacgcacgtcttcaaccgctttcctgagaaccagattttaatccgtccgccggcgcccaccattaccaccgtcagtgaaaacgttcctgctctcacagatcacgggaccctgccgttgcgcagcagtatccggggagtccaacgtgtgaccgttactgacgccagacgccgcacctgtccctacgtgtacaaggcactgggcatagtcgcaccgcgcgtcctttcaagccgcactttctaaaaaaaaaaaaaatgtccattcttatctcgcccagtaataacaccggttggggtctgcgcgctccaagcaagatgtacggaggcgcacgcaaacgttctacccaacatcctgtccgtgttcgcggacattttcgcgctccatggggcgccctcaagggccgcactcgcgttcgaaccaccgtcgatgatgtaatcgatcaggtggttgccgacgcccgtaattatactcctactgcgcctacatctactgtggatgcagttattgacagtgtagtggctgacgctcgcaactatgctcgacgtaagagccggcgaaggcgcattgccagacgccaccgagctaccactgccatgcgagccgcaagagctctgctacgaagagctagacgcgtggggcgaagagccatgcttagggcggccagacgtgcagcttcgggcgccagcgccggcaggtcccgcaggcaagcagccgctgtcgcagcggcgactattgccgacatggcccaatcgcgaagaggcaatgtatactgggtgcgtgacgctgccaccggtcaacgtgtacccgtgcgcacccgtccccctcgcacttagaagatactgagcagtctccgatgttgtgtcccagcggcgaggatgtccaagcgcaaatacaaggaagaaatgctgcaggttatcgcacctgaagtctacggccaaccgttgaaggatgaaaaaaaaccccgcaaaatcaagcgggttaaaaaggacaaaaaagaagaggaagatggcgatgatgggctggcggagtttgtgcgcgagtttgccccacggcgacgcgtgcaatggcgtgggcgcaaagttcgacatgtgttgagacctggaacttcggtggtctttacacccggcgagcgttcaagcgctacttttaagcgttcctatgatgaggtgtacggggatgatgatattcttgagcaggcggctgaccgattaggcgagtttgcttatggcaagcgtagtagaataacttccaaggatgagacagtgtcgatacccttggatcatggaaatcccacccctagtcttaaaccggtcactttgcagcaagtgttacccgtaactccgcgaacaggtgttaaacgcgaaggtgaagatttgtatcccactatgcaactgatggtacccaaacgccagaagttggaggacgttttggagaaagtaaaagtggatccagatattcaacctgaggttaaagtgagacccattaagcaggtagcgcctggtctgggggtacaaactgtagacattaagattcccactgaaagtatggaagtgcaaactgaacccgcaaagcctactgccacctccactgaagtgcaaacggatccatggatgcccatgcctattacaactgacgccgccggtcccactcgaagatcccgacgaaagtacggtccagcaagtctgttgatgcccaattatgttgtacacccatctattattcctactcctggttaccgaggcactcgctactatcgcagccgaaacagtacctcccgccgtcgccgcaagacacctgcaaatcgcagtcgtcgccgtagacgcacaagcaaaccgactcccggcgccctggtgcggcaagtgtaccgcaatggtagtgcggaacctttgacactgccgcgtgcgcgttaccatccgagtatcatcacttaatcaatgttgccgctgcctccttgcagatatggccctcacttgtcgccttcgcgttcccatcactggttaccgaggaagaaactcgcgccgtagaagagggatgttgggacgcggaatgcgacgctacaggcgacggcgtgctatccgcaagcaattgcggggtggttttttaccagccttaattccaattatcgctgctgcaattggcgcgataccaggcatagcttccgtggcggttcaggcctcgcaacgacattgacattggaaaaaaacgtataaataaaaaaaaaaaaatacaatggactctgacactcctggtcctgtgactatgttttcttagagatggaagacatcaatttttcatccttggctccgcgacacggcacgaagccgtacatgggcacctggagcgacatcggcacgagccaactgaacgggggcgccttcaattggagcagtatctggagcgggcttaaaaattttggctcaaccataaaaacatacgggaacaaagcttggaacagcagtacaggacaggcgcttagaaataaacttaaagaccagaacttccaacaaaaagtagtcgatgggatagcttccggcatcaatggagtggtagatttggctaaccaggctgtgcagaaaaagataaacagtcgtttggacccgccgccagcaaccccaggtgaaatgcaagtggaggaagaaattcctccgccagaaaaacgaggcgacaagcgtccgcgtcccgatttggaagagacgctggtgacgcgcgtagatgaaccgccttcttatgaggaagcaacgaagcttggaatgcccaccactagaccgatagccccaatggccaccggggtgatgaaaccttctcagttgcatcgacccgtcaccttggatttgccccctccccctgctgctactgctgtacccgcttctaagcctgtcgctgccccgaaaccagtcgccgtagccaggtcacgtcccgggggcgctcctcgtccaaatgcgcactggcaaaatactctgaacagcatcgtgggtctaggcgtgcaaagtgtaaaacgccgtcgctgcttttaattaaatatggagtagcgcttaacttgcctatctgtgtatatgtgtcattacacgccgtcacagcagcagaggaaaaaaggaagaggtcgtgcgtcgacgctgagttactttcaagatggccaccccatcgatgctgccccaatgggcatacatgcacatcgccggacaggatgcttcggagtacctgagtccgggtctggtgcagttcgcccgcgccacagacacctacttcaatctgggaaataagtttagaaatcccaccgtagcgccgacccacgatgtgaccaccgaccgtagccagcggctcatgttgcgcttcgtgcccgttgaccgggaggacaatacatactcttacaaagtgcggtacaccctggccgtgggcgacaacagagtgctggatatggccagcacgttctttgacattaggggtgtgttggacagaggtcccagtttcaaaccctattctggtacggcttacaactccctggctcctaaaggcgctccaaatacatctcagtggattgcagaaggtgtaaaaaatacaactggtgaggaacacgtaacagaagaggaaaccaatactactacttacacttttggcaatgctcctgtaaaagctgaagctgaaattacaaaagaaggactcccagtaggtttggaagtttcagatgaagaaagtaaaccgatttatgctgataaaacatatcagccagaacctcagctgggagatgaaacttggactgaccttgatggaaaaaccgaaaagtatggaggcagggctctcaaacccgatactaagatgaaaccatgctacgggtcctttgccaaacctactaatgtgaaaggcggtcaggcaaaacaaaaaacaacggagcagccaaatcagaaagtcgaatatgatatcgacatggagttttttgatgcggcatcgcagaaaacaaacttaagtcctaaaattgtcatgtatgcagaaaatgtaaatttggaaactccagacactcatgtagtgtacaaacctggaacagaagacacaagttccgaagctaatttgggacaacaatctatgcccaacagacccaactacattggcttcagagataactttattggacttatgtactataacagtactggtaacatgggggtgctggctggtcaagcgtctcagttaaatgcagtggttgacttgcaggacagaaacacagaactttcttaccaactcttgcttgactctctgggcgacagaaccagatactttagcatgtggaatcaggctgtggacagttatgatcctgatgtacgtgttattgaaaatcatggtgtggaagatgaacttcccaactactgttttccactggacggcataggtgttccaacaaccagttacaaatcaatagttccaaatggagacaatgcgcctaattggaaggaacctgaagtaaatggaacaagtgagatcggacagggtaatttgtttgccatggaaattaaccttcaagccaatctatggcgaagtttcctttattccaatgtggctctatatctcccagactcgtacaaatacaccccgtccaatgtcactcttccagaaaacaaaaacacctacgactacatgaacgggcgggtggtgccgccatctctagtagacacctatgtgaacattggtgccaggtggtctctggatgccatggacaatgtcaacccattcaaccaccaccgtaacgctggcttgcgttaccgatccatgcttctgggtaacggacgttatgtgcctttccacatacaagtgcctcaaaaattcttcgctgttaaaaacctgctgcttctcccaggctcctacacttatgagtggaactttaggaaggatgtgaacatggttctacagagttccctcggtaacgacctgcgggtagatggcgccagcatcagtttcacgagcatcaacctctatgctacttttttccccatggctcacaacaccgcttccacccttgaagccatgctgcggaatgacaccaatgatcagtcattcaacgactacctatctgcagctaacatgctctaccccattcctgccaatgcaaccaatattcccatttccattccttctcgcaactgggcggctttcagaggctggtcatttaccagactgaaaaccaaagaaactccctctttggggtctggatttgacccctactttgtctattctggttctattccctacctggatggtaccttctacctgaaccacacttttaagaaggtttccatcatgtttgactcttcagtgagctggcctggaaatgacaggttactatctcctaacgaatttgaaataaagcgcactgtggatggcgaaggctacaacgtagcccaatgcaacatgaccaaagactggttcttggtacagatgctcgccaactacaacatcggctatcagggcttctacattccagaaggatacaaagatcgcatgtattcatttttcagaaacttccagcccatgagcaggcaggtggttgatgaggtcaattacaaagacttcaaggccgtcgccataccctaccaacacaacaactctggctttgtgggttacatggctccgaccatgcgccaaggtcaaccctatcccgctaactatccctatccactcattggaacaactgccgtaaatagtgttacgcagaaaaagttcttgtgtgacagaaccatgtggcgcataccgttctcgagcaacttcatgtctatgggggcccttacagacttgggacagaatatgctctatgccaactcagctcatgctctggacatgacctttgaggtggatcccatggatgagcccaccctgctttatcttctcttcgaagttttcgacgtggtcagagtgcatcagccacaccgcggcatcatcgaggcagtctacctgcgtacaccgttctcggccggtaacgctaccacgtaagaagcttcttgcttcttgcaaatagcagctgcaaccatggcctgcggatcccaaaacggctccagcgagcaagagctcagagccattgtccaagacctgggttgcggaccctattttttgggaacctacgataagcgcttcccggggttcatggcccccgataagctcgcctgtgccattgtaaatacggccggacgtgagacggggggagagcactggttggctttcggttggaacccacgttctaacacctgctacctttttgatccttttggattctcggatgatcgtctcaaacagatttaccagtttgaatatgagggtctcctgcgccgcagcgctcttgctaccaaggaccgctgtattacgctggaaaaatctacccagaccgtgcagggtccccgttctgccgcctgcggacttttctgctgcatgttccttcacgcctttgtgcactggcctgaccgtcccatggacggaaaccccaccatgaaattgctaactggagtgccaaacaacatgcttcattctcctaaagtccagcccaccctgtgtgacaatcaaaaagcactctaccattttcttaatacccattcgccttattttcgctcccatcgtacacacatcgaaagggccactgcgttcgaccgtatggatgttcaataatgactcatgtaaacaacgtgttcaataaacatcactttatttttttacatgtatcaaggctctgcattacttatttatttacaagtcgaatgggttctgacgagaatcagaatgacccgcaggcagtgatacgttgcggaactgatacttgggttgccacttgaattcgggaatcaccaacttgggaaccggtatatcgggcaggatgtcactccacagctttctggtcagctgcaaagctccaagcaggtcaggagccgaaatcttgaaatcacaattaggaccagtgctttgagcgcgagagttgcggtacaccggattgcagcactgaaacaccatcagcgacggatgtctcacgcttgccagcacggtgggatctgcaatcatgcccacatccagatcttcagcattggcaatgctgaacggggtcatcttgcaggtctgcctacccatggcgggcacccaattaggcttgtggttgcaatcgcagtgcagggggatcagtatcatcttggcctgatcctgtctgattcctggatacacggctctcatgaaagcatcatattgcttgaaagcctgctgggctttactaccctcggtataaaacatcccgcaggacctgctcgaaaactggttagctgcacagccggcatcattcacacagcagcgggcgtcattgttagctatttgcaccacacttctgccccagcggttttgggtgattttggttcgctcgggattctcctttaaggctcgttgtccgttctcgctggccacatccatctcgataatctgctccttctgaatcataatattgccatgcaggcacttcagcttgccctcataatcattgcagccatgaggccacaacgcacagcctgtacattcccaattatggtgggcgatctgagaaaaagaatgtatcattccctgcagaaatcttcccatcatcgtgctcagtgtcttgtgactagtgaaagttaactggatgcctcggtgctcctcgtttacgtactggtgacagatgcgcttgtattgttcgtgttgctcaggcattagtttaaaagaggttctaagttcgttatccagcctgtacttctccatcagcagacacatcacttccatgcctttctcccaagcagacaccaggggcaagctaatcggattcttaacagtgcaggcagcagctcctttagccagagggtcatctttagcgatcttctcaatgcttcttttgccatccttctcaacgatgcgcacgggcgggtagctgaaacccactgctacaagttgcgcctcttctctttcttcttcgctgtcttgactgatgtcttgcatggggatatgtttggtcttccttggcttctttttggggggtatcggaggaggaggactgtcgctccgttccggagacagggaggattgtgacgtttcgctcaccattaccaactgactgtcggtagaagaacctgaccccacacggcgacaggtgtttctcttcgggggcagaggtggaggcgattgcgaagggctgcggtccgacctggaaggcggatgactggcagaaccccttccgcgttcgggggtgtgctccctgtggcggtcgcttaactgatttccttcgcggctggccattgtgttctcctaggcagagaaacaacagacatggaaactcagccattgctgtcaacatcgccacgagtgccatcacatctcgtcctcagcgacgaggaaaaggagcagagcttaagcattccaccgcccagtcctgccaccacctctaccctagaagataaggaggtcgacgcatctcatgacatgcagaataaaaaagcgaaagagtctgagacagacatcgagcaagacccgggctatgtgacaccggtggaacacgaggaagagttgaaacgctttctagagagagaggatgaaaactgcccaaaacaacgagcagataactatcaccaagatgctggaaatagggatcagaacaccgactacctcatagggcttgacggggaagacgcgctccttaaacatctagcaagacagtcgctcatagtcaaggatgcattattggacagaactgaagtgcccatcagtgtggaagagctcagccgcgcctacgagcttaacctcttttcacctcgtactccccccaaacgtcagccaaacggcacctgcgagccaaatcctcgcttaaacttttatccagcttttgctgtgccagaagtactggctacctatcacatcttttttaaaaatcaaaaaattccagtctcctgccgcgctaatcgcacccgcgccgatgccctactcaatctgggacctggttcacgcttacctgatatagcttccttggaagaggttccaaagatcttcgagggtctgggcaataatgagactcgggccgcaaatgctctgcaaaagggagaaaatggcatggatgagcatcacagcgttctggtggaattggaaggcgataatgccagactcgcagtactcaagcgaagcatcgaggtcacacacttcgcatatcccgctgtcaacctgccccctaaagtcatgacggcggtcatggaccagttactcattaagcgcgcaagtcccctttcagaagacatgcatgacccagatgcctgtgatgagggtaaaccagtggtcagtgatgagcagctaacccgatggctgggcaccgactctcccagggatttggaagagcgtcgcaagcttatgatggccgtggtgctggttaccgtagaactagagtgtctccgacgtttctttaccgattcagaaaccttgcgcaaactcgaagagaatctgcactacacttttagacacggctttgtgcggcaggcatgcaagatatctaacgtggaactcaccaacctggtttcctacatgggtattctgcatgagaatcgcctaggacaaagcgtgctgcacagcaccctgaagggggaagcccgccgtgattacatccgcgattgtgtctatctgtacctgtgccacacgtggcaaaccggcatgggtgtatggcagcaatgtttagaagaacagaacttgaaagagcttgacaagctcttacagaaatctcttaaggttctgtggacagggttcgacgagcgcaccgtcgcttccgacctggcagacctcatcttcccagagcgtctcagggttactttgcgaaacggattgcctgactttatgagccagagcatgcttaacaattttcgctctttcatcctggaacgctccggtatcctgcccgccacctgctgcgcactgccctccgactttgtgcctctcacctaccgcgagtgccccccgccgctatggagtcactgctacctgttccgtctggccaactatctctcctaccactcggatgtgatcgaggatgtgagcggagacggcttgctggagtgtcactgccgctgcaatctgtgcacgccccaccggtccctagcttgcaacccccagttgatgagcgaaacccagataataggcacctttgaattgcaaggccccagcagccaaggcgatgggtcttctcctgggcaaagtttaaaactgaccccgggactgtggacctccgcctacttgcgcaagtttgctccggaagattaccacccctatgaaatcaagttctatgaggaccaatcacagcctccaaaggccgaactttcggcctgcgtcatcacccagggggcaattctggcccaattgcaagccatccaaaaatcccgccaagaatttctactgaaaaagggtaagggggtctaccttgacccccagaccggcgaggaactcaacacaaggttccctcaggatgtcccaacgacgagaaaacaagaagttgaaggtgcagccgccgcccccagaagatatggaggaagattgggacagtcaggcagaggaggcggaggaggacagtctggaggacagtctggaggaagacagtttggaggaggaaaacgaggaggcagaggaggtggaagaagtaaccgccgacaaacagttatcctcggctgcggagacaagcaacagcgctaccatctccgctccgagtcgaggaacccggcggcgtcccagcagtagatgggacgagaccggacgcttcccgaacccaaccagcgcttccaagaccggtaagaaggatcggcagggatacaagtcctggcgggggcataagaatgccatcatctcctgcttgcatgagtgcgggggcaacatatccttcacgcggcgctacttgctattccaccatggggtgaactttccgcgcaatgttttgcattactaccgtcacctccacagcccctactatagccagcaaatcccggcagtctcgacagataaagacagcggcggcgacctccaacagaaaaccagcagcggcagttagaaaatacacaacaagtgcagcaacaggaggattaaagattacagccaacgagccagcgcaaacccgagagttaagaaatcggatctttccaaccctgtatgccatcttccagcagagtcggggtcaagagcaggaactgaaaataaaaaaccgatctctgcgttcgctcaccagaagttgtttgtatcacaagagcgaagatcaacttcagcgcactctcgaggacgccgaggctctcttcaacaagtactgcgcgctgactcttaaagagtaggcagcgaccgcgcttattcaaaaaaggcgggaattacatcatcctcgacatgagtaaagaaattcccacgccttacatgtggagttatcaaccccaaatgggattggcggcaggcgcctcccaggactactccacccgcatgaattggctcagcgccgggccttctatgatttctcgagttaatgatatacgcgcctaccgaaaccaaatacttttggaacagtcagctcttaccaccacgccccgccaacaccttaatcccagaaattggcccgccgccctagtgtaccaggaaagtcccgctcccaccactgtattacttcctcgagacgcccaggccgaagtccaaatgactaatgcaggtgcgcagttagctggcggctccaccctatgtcgtcacaggcctcggcataatataaaacgcctgatgatcagaggccgaggtatccagctcaacgacgagtcggtgagctctccgcttggtctacgaccagacggaatctttcagattgccggctgcgggagatcttccttcacccctcgtcaggctgttctgactttggaaagttcgtcttcgcaaccccgctcgggcggaatcgggaccgttcaatttgtggaggagtttactccctctgtctacttcaaccccttctccggatctcctgggcattacccggacgagttcataccgaacttcgacgcgattagcgagtcagtggacggctacgattgatgtctggtgacgcggctgagctatctcggctgcgacatctagaccactgccgccgctttcgctgctttgcccgggaactcattgagttcatctacttcgaactccccaaggatcaccctcaaggtccggcccacggagtgcggatttctatcgaaggcaaaatagactctcgcctgcaacgaattttctcccagcggcccgtgctgatcgagcgagaccagggaaacaccacggtttccatctactgcatttgtaatcaccccggattgcatgaaagcctttgctgtcttatgtgtactgagtttaataaaaactgaattaagactctcctacggactgccgcttcttcaacccggattttacaaccagaagaacgaaacttttcctgtcgtccaggactctgttaacttcacctttcctactcacaaactagaagctcaacgactacaccgcttttccagaagcattttccctactaatactactttcaaaaccggaggtgagctccaaggtcttcctacagaaaacccttgggtggaagcgggccttgtagtgctaggaattcttgcgggtgggcttgtgattattctttgctacctatacacaccttgcttcactttcttagtggtgttgtggtattggtttaaaaaatggggcccatactagtcttgcttgttttactttcgcttttggaaccgggttctgccaattacgatccatgtctagacttcgacccagaaaactgcacacttacttttgcacccgacacaagccgcatctgtggagttcatcgcctctcttacgaacttggcccccaacgacaaaaatttacctgcatggtgggaatcaaccccatagttatcacccagcaaagtggagatactaagggttgcattcactgctcctgcgattccatcgagtgcacctacaccctgctgaagaccctatgcggcctaagagacctgctaccaatgaattaaaaaatgattaataaaaaatcacttacttgaaatcagcaataaggtctctgttgaaattttctcccagcagcacctcacttccctcttcccaactctggtattctaaaccccgttcagcggcatactttctccatactttaaaggggatgtcaaattttagctcctctcctgtacccacaatcttcatgtctttcttcccagatgaccaagagagtccggctcagtgactccttcaaccctgtctacccctatgaagatgaaagcacctcccaacacccctttataaacccagggtttatttccccaaatggcttcacacaaagcccaaacggagttcttactttaaaatgtttaaccccactaacaaccacaggcggatctctacagctaaaagtgggagggggacttacagtggatgacaccaacggttttttgaaagaaaacataagtgccaccacaccactcgttaagactggtcactctataggtttaccactaggagccggattgggaacgaatgaaaataaactttgtatcaaattaggacaaggacttacattcaattcaaacaacatttgcattgatgacaatattaacaccttatggacaggagtcaaccccaccgaagccaactgtcaaatcatgaactccagtgaatctaatgattgcaaattaattctaacactagttaaaactggagcactagtcactgcatttgtttatgttataggagtatctaacaattttaatatgctaactacacacagaaatataaattttactgcagagctgtttttcgattctactggtaatttactaactagactctcatccctcaaaactccacttaatcataaatcaggacaaaacatggctactggtgccattactaatgctaaaggtttcatgcccagcacgactgcctatcctttcaatgataattctagagaaaaagaaaactacatttacggaacttgttactacacagctagtgatcgcactgcttttcccattgacatatctgtcatgcttaaccgaagagcaataaatgacgagacatcatattgtattcgtataacttggtcctggaacacaggagatgccccagaggtgcaaacctctgctacaaccctagtcacctccccatttaccttttactacatcagagaagacgactgacaaataaagtttaacttgtttatttgaaaatcaattcacaaaatccgagtagttattttgcctcccccttcccatttaacagaatacaccaatctctccccacgcacagctttaaacatttggataccattagatatagacatggttttagattccacattccaaacagtttcagagcgagccaatctggggtcagtgatagataaaaatccatcgggatagtcttttaaagcgctttcacagtccaactgctgcggatgcgactccggagtctggatcacggtcatctggaagaagaacgatgggaatcataatccgaaaacggtatcggacgattgtgtctcatcaaacccacaagcagccgctgtctgcgtcgctccgtgcgactgctgtttatgggatcagggtccacagtgtcctgaagcatgattttaatagcccttaacatcaactttctggtgcgatgcgcgcagcaacgcattctgatttcactcaaatctttgcagtaggtacaacacattattacaatattgtttaataaaccataattaaaagcgctccagccaaaactcatatctgatataatcgcccctgcatgaccatcataccaaagtttaatataaattaaatgacgttccctcaaaaacacactacccacatacatgatctcttttggcatgtgcatattaacaatctgtctgtaccatggacaacgttggttaatcatgcaacccaatataaccttccggaaccacactgccaacaccgctcccccagccatgcattgaagtgaaccctgctgattacaatgacaatgaagaacccaattctctcgaccgtgaatcacttgagaatgaaaaatatctatagtggcacaacatagacataaatgcatgcatcttctcataatttttaactcctcaggatttagaaacatatcccagggaataggaagctcttgcagaacagtaaagctggcagaacaaggaagaccacgaacacaacttacactatgcatagtcatagtatcacaatctggcaacagcgggtggtcttcagtcatagaagctcgggtttcattttcctcacaacgtggtaactgggctctggtgtaagggtgatgtctggcgcatgatgtcgagcgtgcgcgcaaccttgtcataatggagttgcttcctgacattctcgtattttgtatagcaaaacgcggccctggcagaacacactcttcttcgccttctatcctgccgcttagcgtgttccgtgtgatagttcaagtacaaccacactcttaagttggtcaaaagaatgctggcttcagttgtaatcaaaactccatcgcatctaatcgttctgaggaaatcatccaagcaatgcaactggattgtgtttcaagcaggagaggagagggaagagacggaagaaccatgttaatttttattccaaacgatctcgcagtacttcaaattgtagatcgcgcagatggcatctctcgcccccactgtgttggtgaaaaagcacagctagatcaaaagaaatgcgattttcaaggtgctcaacggtggcttccagcaaagcctccacgcgcacatccaagaacaaaagaataccaaaagaaggagcattttctaactcctcaatcatcatattacattcctgcaccattcccagataattttcagctttccagccttgaattattcgtgtcagttcttgtggtaaatccaatccacacattacaaacaggtcccggagggcgccctccaccaccattcttaaacacaccctcataatgacaaaatatcttgctcctgtgtcacctgtagcgaattgagaatggcaacatcaattgacatgcccttggctctaagttcttctttaagttctagttgtaaaaactctctcatattatcaccaaactgcttagccagaagccccccgggaacaagagcaggggacgctacagtgcagtacaagcgcagacctccccaattggctccagcaaaaacaagattggaataagcatattgggaaccgccagtaatatcatcgaagttgctggaaatataatcaggcagagtttcttgtaaaaattgaataaaagaaaaatttgccaaaaaaacattcaaaacctctgggatgcaaatgcaataggttaccgcgctgcgctccaacattgttagttttgaattagtctgcaaaaataaaaaaaaaaacaagcgtcatatcatagtagcctgacgaacagatggataaatcagtctttccatcacaagacaagccacagggtctccagctcgaccctcgtaaaacctgtcatcatgattaaacaacagcaccgaaagttcctcgcggtgaccagcatgaataattcttgatgaagcatacaatccagacatgttagcatcagttaacgagaaaaaacagccaacatagcctttgggtataattatgcttaatcgtaagtatagcaaagccacccctcgcggatacaaagtaaaaggcacaggagaataaaaaatataattatttctctgctgctgttcaggcaacgtcgcccccggtccctctaaatacacatacaaagcctcatcagccatggcttaccagacaaagtacagcgggcacacaaagcacaagctctaaagtgactctccaacctctccacaatatatatatacacaagccctaaactgacgtaatgggagtaaagtgtaaaaaatcccgccaaacccaacacacaccccgaaactgcgtcaccagggaaaagtacagtttcacttccgcaatcccaacaggcgtaacttcctctttctcacggtacgtgatatcccactaacttgcaacgtcattttcccacggtcgcaccgccccttttagccgttaaccccacagccaatcaccacacgatccacactttttaaaatcacctcatttacatattggcaccattccatctataaggtatattatatagata

SEQ ID NO: 2 - DNA, 11978 bp, Artificial Sequence
  ColoAd1 shuttle vector
ggcgcgcctatctatataatataccttatagatggaatggtgccaatatgtaaatgaggtgattttaaaaagtgtggatcgtgtggtgattggctgtggggttaacggctaaaaggggcggtgcgaccgtgggaaaatgacgttttgtgggggtggagtttttttgcaagttgtcgcgggaaatgtgacgcataaaaaggcttttttctcacggaactacttagttttcccacggtatttaacaggaaatgaggtagttttgaccggatgcaagtgaaaattgttgattttcgcgcgaaaactgaatgaggaagtgtttttctgaataatgtggtatttatggcagggtggagtatttgttcagggccaggtagactttgacccattacgtggaggtttcgattaccgtgttttttacctgaatttccgcgtaccgtgtcaaagtcttctgtttttacgtaggtgtcagctgatcgctagggtatttatacctcagggtttgtgtcaagaggccactcttgagtgccagcgagaagagttttctcctctgcgccggcagtttaataataaaaaaatgagagatttgcgatttctgcctcaggaaataatctctgctgagactggaaatgaaatattggagcttgtggtgcacgccctgatgggagacgatccggagccacctgtgcagctttttgagcctcctacgcttcaggaactgtatgatttagaggtagagggatcggaggattctaatgaggaagctgtaaatggcttttttaccgattctatgcttttagctgctaatgaagggttagaattagatccgcctttggacacttttgatactccaggggtaattgtggaaagcggtacaggtgtaagaaaattacctgatttgagttccgtggactgtgatttgcactgctatgaagacgggtttcctccgagtgatgaggaggaccatgaaaaggagcagtccatgcagactgcagcgggtgagggagtgaaggctgccaatgttggttttcagttggattgcccggagcttcctggacatggctgtaagtcttgtgaatttcacaggaaaaatactggagtaaaggaactgttatgttcgctttgttatatgagaacgcactgccactttatttacagtaagtgtgtttaagttaaaatttaaaggaatatgctgtttttcacatgtatattgagtgtgagttttgtgcttcttattataggtcctgtgtctgatgctgatgaatcaccatctcctgattctactacctcacctcctgagattcaagcacctgttcctgtggacgtgcgcaagcccattcctgtgaagcttaagcctgggaaacgtccagcagtggaaaaacttgaggacttgttacagggtggggacggacctttggacttgagtacacggaaacgtccaagacaataagtgttccatatccgtgtttacttaaggtgacgtcaatatttgtgtgacagtgcaatgtaataaaaatatgttaactgttcactggtttttattgctttttgggcggggactcaggtatataagtagaagcagacctgtgtggttagctcataggagctggctttcatccatggaggtttgggccattttggaagaccttaggaagactaggcaactgttagagaacgcttcggacggagtctccggtttttggagattctggttcgctagtgaattagctagggtagtttttaggataaaacaggactataaacaagaatttgaaaagttgttggtagattgcccaggactttttgaagctcttaatttgggccatcaggttcactttaaagaaaaagttttatcagttttagacttttcaaccccaggtagaactgctgctgctgtggcttttcttacttttatattagataaatggatcccgcagactcatttcagcaggggatacgttttggatttcatagccacagcattgtggagaacatggaaggttcgcaagatgaggacaatcttaggttactggccagtgcagcctttgggtgtagcgggaatcctgaggcatccaccggtcatgccagcggttctggaggaggaacagcaagaggacaacccgagagccggcctggaccctccagtggaggaggcggagtagctgacttgtctcctgaactgcaacgggtgcttactggatctacgtccactggacgggataggggcgttaagagggagagggcatctagtggtactgatgctagatctgagttggctttaagtttaatgagtcgcagacgtcctgaaaccatttggtggcatgaggttcagaaagagggaagggatgaagtttctgtattgcaggagaaatattcactggaacaggtgaaaacatgttggttggagcctgaggatgattgggaggtggccattaaaaattatgccaagatagctttgaggcctgataaacagtataagattactagacggattaatatccggaatgcttgttacatatctggaaatggggctgaggtggtaatagatactcaagacaaggcagttattagatgctgcatgatggatatgtggcctggggtagtcggtatggaagcagtaacttttgtaaatgttaagtttaggggagatggttataatggaatagtgtttatggccaataccaaacttatattgcatggttgtagcttttttggtttcaacaatacctgtgtagatgcctggggacaggttagtgtacggggatgtagtttctatgcgtgttggattgccacagctggcagaaccaagagtcaattgtctctgaagaaatgcatatttcaaagatgtaacctgggcattctgaatgaaggcgaagcaagggtccgccactgcgcttctacagatactggatgttttattttgattaagggaaatgccagcgtaaagcataacatgatttgcggtgcttccgatgagaggccttatcaaatgctcacttgtgctggtgggcattgtaatatgctggctactgtgcatattgtttcccatcaacgcaaaaaatggcctgtttttgatcacaatgtgatgacgaagtgtaccatgcatgcaggtgggcgtagaggaatgtttatgccttaccagtgtaacatgaatcatgtgaaagtgttgttggaaccagatgccttttccagaatgagcctaacaggaatttttgacatgaacatgcaaatctggaagatcctgaggtatgatgatacgagatcgagggtacgcgcatgcgaatgcggaggcaagcatgccaggttccagccggtgtgtgtagatgtgactgaagatctcagaccggatcatttggttattgcccgcactggagcagagttcggatccagtggagaagaaactgactaaggtgagtattgggaaaactttggggtgggattttcagatggacagattgagtaaaaatttgttttttctgtcttgcagctgtcatgagtggaaacgcttcttttaaggggggagtcttcagcccttatctgacagggcgtctcccatcctgggcaggagttcgtcagaatgttatgggatctactgtggatggaagacccgtccaacccgccaattcttcaacgctgacctatgctactttaagttcttcacctttggacgcagctgcagctgccgccgccgcttctgttgccgctaacactgtgcttggaatgggttactatggaagcatcatggctaattccacttcctctaataacccttctaccctgactcaggacaagttacttgtccttttggcccagctggaggctttgacccaacgtctgggtgaactttctcagcaggtggtcgagttgcgagtacaaactgagtctgctgtcggcacggcaaagtctaaataaaaaaatcccagaatcaatgaataaataaacaagcttgttgttgatttaaaatcaagtgtttttatttcatttttcgcgcacggtatgccctagaccaccgatctctatcattgagaactcggtggattttttccaggatcctatagaggtgggattgaatgtttagatacatgggcattaggccgtctttggggtggagatagctccattgaagggattcatgctccggggtagtgttgtaaatcacccagtcataacaaggtcgcagtgcatggtgttgcacaatatcttttagaagtaggctgattgccacagataagcccttggtgtaggtgtttacaaaccggttgagctgggatgggtgcattcggggtgaaattatgtgcattttggattggatttttaagttggcaatattgccgccaagatcccgtcttgggttcatgttatgaaggaccaccaagacggtgtatccggtacatttaggaaatttatcgtgcagcttggatggaaaagcgtggaaaaatttggagacacccttgtgtcctccaagattttccatgcactcatccatgataatagcaatggggccgtgggcagcggcgcgggcaaacacgttccgtgggtctgacacatcatagttatgttcctgagttaaatcatcataagccattttaatgaatttggggcggagagtaccagattggggtatgaatgttccttcgggcccatactagtcttgcttgttttactttcgcttttggaaccgggttctgccaattacgatccatgtctagacttcgacccagaaaactgcacacttacttttgcacccgacacaagccgcatctgtggagttcatcgcctctcttacgaacttggcccccaacgacaaaaatttacctgcatggtgggaatcaaccccatagttatcacccagcaaagtggagatactaagggttgcattcactgctcctgcgattccatcgagtgcacctacaccctgctgaagaccctatgcggcctaagagacctgctaccaatgaattaaaaaatgattaataaaaaatcacttacttgaaatcagcaataaggtctctgttgaaattttctcccagcagcacctcacttccctcttcccaactctggtattctaaaccccgttcagcggcatactttctccatactttaaaggggatgtcaaattttagctcctctcctgtacccacaatcttcatgtctttcttcccagatgaccaagagagtccggctcagtgactccttcaaccctgtctacccctatgaagatgaaagcacctcccaacacccctttataaacccagggtttatttccccaaatggcttcacacaaagcccaaacggagttcttactttaaaatgtttaaccccactaacaaccacaggcggatctctacagctaaaagtgggagggggacttacagtggatgacaccaacggttttttgaaagaaaacataagtgccaccacaccactcgttaagactggtcactctataggtttaccactaggagccggattgggaacgaatgaaaataaactttgtatcaaattaggacaaggacttacattcaattcaaacaacatttgcattgatgacaatattaacaccttatggacaggagtcaaccccaccgaagccaactgtcaaatcatgaactccagtgaatctaatgattgcaaattaattctaacactagttaaaactggagcactagtcactgcatttgtttatgttataggagtatctaacaattttaatatgctaactacacacagaaatataaattttactgcagagctgtttttcgattctactggtaatttactaactagactctcatccctcaaaactccacttaatcataaatcaggacaaaacatggctactggtgccattactaatgctaaaggtttcatgcccagcacgactgcctatcctttcaatgataattctagagaaaaagaaaactacatttacggaacttgttactacacagctagtgatcgcactgcttttcccattgacatatctgtcatgcttaaccgaagagcaataaatgacgagacatcatattgtattcgtataacttggtcctggaacacaggagatgccccagaggtgcaaacctctgctacaaccctagtcacctccccatttaccttttactacatcagagaagacgactgacaaataaagtttaacttgtttatttgaaaatcaattcacaaaatccgagtagttattttgcctcccccttcccatttaacagaatacaccaatctctccccacgcacagctttaaacatttggataccattagatatagacatggttttagattccacattccaaacagtttcagagcgagccaatctggggtcagtgatagataaaaatccatcgggatagtcttttaaagcgctttcacagtccaactgctgcggatgcgactccggagtctggatcacggtcatctggaagaagaacgatgggaatcataatccgaaaacggtatcggacgattgtgtctcatcaaacccacaagcagccgctgtctgcgtcgctccgtgcgactgctgtttatgggatcagggtccacagtgtcctgaagcatgattttaatagcccttaacatcaactttctggtgcgatgcgcgcagcaacgcattctgatttcactcaaatctttgcagtaggtacaacacattattacaatattgtttaataaaccataattaaaagcgctccagccaaaactcatatctgatataatcgcccctgcatgaccatcataccaaagtttaatataaattaaatgacgttccctcaaaaacacactacccacatacatgatctcttttggcatgtgcatattaacaatctgtctgtaccatggacaacgttggttaatcatgcaacccaatataaccttccggaaccacactgccaacaccgctcccccagccatgcattgaagtgaaccctgctgattacaatgacaatgaagaacccaattctctcgaccgtgaatcacttgagaatgaaaaatatctatagtggcacaacatagacataaatgcatgcatcttctcataatttttaactcctcaggatttagaaacatatcccagggaataggaagctcttgcagaacagtaaagctggcagaacaaggaagaccacgaacacaacttacactatgcatagtcatagtatcacaatctggcaacagcgggtggtcttcagtcatagaagctcgggtttcattttcctcacaacgtggtaactgggctctggtgtaagggtgatgtctggcgcatgatgtcgagcgtgcgcgcaaccttgtcataatggagttgcttcctgacattctcgtattttgtatagcaaaacgcggccctggcagaacacactcttcttcgccttctatcctgccgcttagcgtgttccgtgtgatagttcaagtacaaccacactcttaagttggtcaaaagaatgctggcttcagttgtaatcaaaactccatcgcatctaatcgttctgaggaaatcatccaagcaatgcaactggattgtgtttcaagcaggagaggagagggaagagacggaagaaccatgttaatttttattccaaacgatctcgcagtacttcaaattgtagatcgcgcagatggcatctctcgcccccactgtgttggtgaaaaagcacagctagatcaaaagaaatgcgattttcaaggtgctcaacggtggcttccagcaaagcctccacgcgcacatccaagaacaaaagaataccaaaagaaggagcattttctaactcctcaatcatcatattacattcctgcaccattcccagataattttcagctttccagccttgaattattcgtgtcagttcttgtggtaaatccaatccacacattacaaacaggtcccggagggcgccctccaccaccattcttaaacacaccctcataatgacaaaatatcttgctcctgtgtcacctgtagcgaattgagaatggcaacatcaattgacatgcccttggctctaagttcttctttaagttctagttgtaaaaactctctcatattatcaccaaactgcttagccagaagccccccgggaacaagagcaggggacgctacagtgcagtacaagcgcagacctccccaattggctccagcaaaaacaagattggaataagcatattgggaaccgccagtaatatcatcgaagttgctggaaatataatcaggcagagtttcttgtaaaaattgaataaaagaaaaatttgccaaaaaaacattcaaaacctctgggatgcaaatgcaataggttaccgcgctgcgctccaacattgttagttttgaattagtctgcaaaaataaaaaaaaaaacaagcgtcatatcatagtagcctgacgaacagatggataaatcagtctttccatcacaagacaagccacagggtctccagctcgaccctcgtaaaacctgtcatcatgattaaacaacagcaccgaaagttcctcgcggtgaccagcatgaataattcttgatgaagcatacaatccagacatgttagcatcagttaacgagaaaaaacagccaacatagcctttgggtataattatgcttaatcgtaagtatagcaaagccacccctcgcggatacaaagtaaaaggcacaggagaataaaaaatataattatttctctgctgctgttcaggcaacgtcgcccccggtccctctaaatacacatacaaagcctcatcagccatggcttaccagacaaagtacagcgggcacacaaagcacaagctctaaagtgactctccaacctctccacaatatatatatacacaagccctaaactgacgtaatgggagtaaagtgtaaaaaatcccgccaaacccaacacacaccccgaaactgcgtcaccagggaaaagtacagtttcacttccgcaatcccaacaggcgtaacttcctctttctcacggtacgtgatatcccactaacttgcaacgtcattttcccacggtcgcaccgccccttttagccgttaaccccacagccaatcaccacacgatccacactttttaaaatcacctcatttacatattggcaccattccatctataaggtatattatatagataggcgcgccctctcttaaggtagcatcgggatcgagtccctgagagaacatcctcaatcccgatctatccttagatccgaggaatatcgaaatcagttacgctagggataacagggtaatatagcatcccctcggattgctatctaccggctcgtcagctatgatctctcgatttcgatcaagaaatctcattggttaccttgggctatcgaaaccagtcaagtcagctacttggcgagatcgacttgtctgagtttcgactacgctcagaattgcgtcagcgcctatcgccaggtattactccaatcccgaatatccgagcctgagagaacatcctcaatcccgatctatccttagatccgaggaatatcgaaatcgtttaaatcttttcttgatggtaaatcattcgaatataagaatggagagacgaatggggaaacgacaaagatgacattctttggtccttctggtgaggttctcaagtttttggttaatcctgtcaacaacttatatcgtatggggctgacttcaggtgctacatttgaagagataaattgcactgaaatctagtaatattttatctgattaataagatgatcttcttgagatcgttttggtctgcgcgtaatctcttgctctgaaaacgaaaaaaccgccttgcagggcggtttttcgaaggttctctgagctaccaactctttgaaccgaggtaactggcttggcagagcgcagtcaccaaaacttgtcctttcagtttagccttaaccggcgcatgacttcaagactaactctgctaaatcaattaccagtggctgctgccagtggtgcttttgcatgtctttccgggttggactcaagacgatagttaccggataaggcgcagcggtcggactgaacggggggttcgtgcatacagtccagcttggagcgaactgcctacccggaactgagtgtcaggcgtggaatgagacaaacgcggccataacagcggaatgacaccggtaaaccgaaaggcaggaacaggagagcgcacgagggagccgccagggggaaacgcctggtatctttatagtcctgtcgggtttcgccaccactgatttgagcgtcagatttcgtgatgcttgtcaggggggcggagcctatggaaaaacggctttgccgcggccctctcacttccctgttaagtatcttcctggcatcttccaggaaatctccgccccgttcgtaagccatttccgctcgccgcagtcgaacgaccgagcgtagcgagtcagtgagcgaggaagcggaatatatcctgtatcacatattctgctgacgcaccggtgcggccttttttctcctgccacatgaagcacttcactgacaccctcatcagtgccaacatagtaagccagtatacactccgctaatttaaacgtggtgtaccgagaacgatcctctcagtgcgatctcgacgatcagtggtattccgacatatcgttgcttggcagtcagccagtcgatcctagcttgggacccaggaagtccaatcgtcagatattgtactcagcctggtcacggcagcgtaccgatctcgtaactataacggtcctaaggtagcgaactagatattgatagtctgatcggtcaacgtataatcgagtcctagcttttgcaaacatctatcaagagacaggatcagcaggaggctttcgcatgattgaacaagatggattgcacgcaggttctccggcggcttgggtggagaggctattcggctatgactgggcacaacagacaatcggctgctctgatgccgccgtgttccggctgtcagcgcaggggcgtccggttctttttgtcaagaccgacctgtccggtgccctgaatgaactgcaagacgaggcagcgcggctatcgtggctggcgacgacgggcgttccttgcgcggctgtgctcgacgttgtcactgaagcgggaagggactggctgctattgggcgaagtgccggggcaggatctcctgtcatctcaccttgctcctgccgagaaagtatccatcatggctgatgcaatgcggcggctgcatacgcttgatccggctacctgcccattcgaccaccaagcgaaacatcgcatcgagcgagcacgtactcggatggaagccggtcttgtcgatcaggatgatctggacgaagagcatcaggggctcgcgccagccgaactgttcgccaggctcaaggcgtctatgcccgacggcgaggatctcgtcgtgacccacggcgatgcctgcttgccgaatatcatggtggaaaatggccgcttttctggattcatcgactgtggccgtctgggtgtggcggaccgctatcaggacatagcgttggctacccgtgatattgctgaagagcttggcggcgaatgggctgaccgcttccttgtgctttacggtatcgccgcgcccgattcgcagcgcatcgccttctatcgccttcttgacgagttcttctgaccgattctaggtgcattggcgcagaaaaaaatgcctgatgcgacgctgcgcgtcttatactcccacatatgccagattcagcaacggatacggcttccccaacttgcccacttccatacgtgtcctccttaccagaaatttatccttaaggtccgtaactataacggtcctaaggtagcgaatcgacctagctctatcgaatctccctcgtttcgagcttacgcgaactagcctctggcgatagcatccgaggggcaggcatctatgtcgggtgcggagaaagaggtaatgtcaagttcgatctgattgcttggcataaagtccgatggttcgagtagactcagttcaacctctctcttaaggtagc

SEQ ID NO: 3 - DNA, 34 bp, Artificial Sequence
  primer 196
ttataggcgcgccctctcttaaggtagcatcggg

SEQ ID NO: 4 - DNA, 35 bp, Artificial Sequence
  primer 197
ttataggcgcgccgctaccttaagagagaggttga

SEQ ID NO: 5 - DNA, 30 bp, Artificial Sequence
  primer 198
ttggcggcgcgcctatctatataatatacc

SEQ ID NO: 6 - DNA, 19 bp, Artificial Sequence
  primer 199
ttggcggcgcgcctatcta

SEQ ID NO: 7 - DNA, 19 bp, Artificial Sequence
  primer 200
aatgcaaatctgtgagggg

SEQ ID NO: 8 - DNA, 22 bp, Artificial Sequence
  primer 201
cttagtggtgttgtggtattgg

SEQ ID NO: 9 - DNA, 19 bp, Artificial Sequence
  primer 202
atcgccttctatcgccttc

SEQ ID NO: 10 - DNA, 19 bp, Artificial Sequence
  primer 203
agcagtgcaaatcacagtc

SEQ ID NO: 11 - DNA, 19 bp, Artificial Sequence
  primer 204
caaactgagtctgctgtcg

SEQ ID NO: 12 - DNA, 19 bp, Artificial Sequence
  primer 205
ataaaggggtgttgggagg

SEQ ID NO: 13 - DNA, 20 bp, Artificial Sequence
  primer 206
ccctcgtaaaacctgtcatc

SEQ ID NO: 14 - DNA, 19 bp, Artificial Sequence
  primer 207
cccattcgtctctccattc

SEQ ID NO: 15 - DNA, 12105 bp, Artificial Sequence
  ColoAd2.0 shuttle vector
ggcgcgcctatctatataatataccttatagatggaatggtgccaatatgtaaatgaggtgattttaaaaagtgtggatcgtgtggtgattggctgtggggttaacggctaaaaggggcggtgcgaccgtgggaaaatgacgttttgtgggggtggagtttttttgcaagttgtcgcgggaaatgtgacgcataaaaaggcttttttctcacggaactacttagttttcccacggtatttaacaggaaatgaggtagttttgaccggatgcaagtgaaaattgttgattttcgcgcgaaaactgaatgaggaagtgtttttctgaataatgtggtatttatggcagggtggagtatttgttcagggccaggtagactttgacccattacgtggaggtttcgattaccgtgttttttacctgaatttccgcgtaccgtgtcaaagtcttctgtttttacgtaggtgtcagctgatcgctagggtatttatacctcagggtttgtgtcaagaggccactcttgagtgccagcgagaagagttttctcctctgcgccggcagtttaataataaaaaaatgagagatttgcgatttctgcctcaggaaataatctctgctgagactggaaatgaaatattggagcttgtggtgcacgccctgatgggagacgatccggagccacctgtgcagctttttgagcctcctacgcttcaggaactgtatgatttagaggtagagggatcggaggattctaatgaggaagctgtaaatggcttttttaccgattctatgcttttagctgctaatgaagggttagaattagatccgcctttggacacttttgatactccaggggtaattgtggaaagcggtacaggtgtaagaaaattacctgatttgagttccgtggactgtgatttgcactgctatgaagacgggtttcctccgagtgatgaggaggaccatgaaaaggagcagtccatgcagactgcagcgggtgagggagtgaaggctgccaatgttggttttcagttggattgcccggagcttcctggacatggctgtaagtcttgtgaatttcacaggaaaaatactggagtaaaggaactgttatgttcgctttgttatatgagaacgcactgccactttatttacagtaagtgtgtttaagttaaaatttaaaggaatatgctgtttttcacatgtatattgagtgtgagttttgtgcttcttattataggtcctgtgtctgatgctgatgaatcaccatctcctgattctactacctcacctcctgagattcaagcacctgttcctgtggacgtgcgcaagcccattcctgtgaagcttaagcctgggaaacgtccagcagtggaaaaacttgaggacttgttacagggtggggacggacctttggacttgagtacacggaaacgtccaagacaataagtgttccatatccgtgtttacttaaggtgacgtcaatatttgtgtgacagtgcaatgtaataaaaatatgttaactgttcactggtttttattgctttttgggcggggactcaggtatataagtagaagcagacctgtgtggttagctcataggagctggctttcatccatggaggtttgggccattttggaagaccttaggaagactaggcaactgttagagaacgcttcggacggagtctccggtttttggagattctggttcgctagtgaattagctagggtagtttttaggataaaacaggactataaacaagaatttgaaaagttgttggtagattgcccaggactttttgaagctcttaatttgggccatcaggttcactttaaagaaaaagttttatcagttttagacttttcaaccccaggtagaactgctgctgctgtggcttttcttacttttatattagataaatggatcccgcagactcatttcagcaggggatacgttttggatttcatagccacagcattgtggagaacatggaaggttcgcaagatgaggacaatcttaggttactggccagtgcagcctttgggtgtagcgggaatcctgaggcatccaccggtcatgccagcggttctggaggaggaacagcaagaggacaacccgagagccggcctggaccctccagtggaggaggcggagtagctgacttgtctcctgaactgcaacgggtgcttactggatctacgtccactggacgggataggggcgttaagagggagagggcatctagtggtactgatgctagatctgagttggctttaagtttaatgagtcgcagacgtcctgaaaccatttggtggcatgaggttcagaaagagggaagggatgaagtttctgtattgcaggagaaatattcactggaacaggtgaaaacatgttggttggagcctgaggatgattgggaggtggccattaaaaattatgccaagatagctttgaggcctgataaacagtataagattactagacggattaatatccggaatgcttgttacatatctggaaatggggctgaggtggtaatagatactcaagacaaggcagttattagatgctgcatgatggatatgtggcctggggtagtcggtatggaagcagtaacttttgtaaatgttaagtttaggggagatggttataatggaatagtgtttatggccaataccaaacttatattgcatggttgtagcttttttggtttcaacaatacctgtgtagatgcctggggacaggttagtgtacggggatgtagtttctatgcgtgttggattgccacagctggcagaaccaagagtcaattgtctctgaagaaatgcatatttcaaagatgtaacctgggcattctgaatgaaggcgaagcaagggtccgccactgcgcttctacagatactggatgttttattttgattaagggaaatgccagcgtaaagcataacatgatttgcggtgcttccgatgagaggccttatcaaatgctcacttgtgctggtgggcattgtaatatgctggctactgtgcatattgtttcccatcaacgcaaaaaatggcctgtttttgatcacaatgtgatgacgaagtgtaccatgcatgcaggtgggcgtagaggaatgtttatgccttaccagtgtaacatgaatcatgtgaaagtgttgttggaaccagatgccttttccagaatgagcctaacaggaatttttgacatgaacatgcaaatctggaagatcctgaggtatgatgatacgagatcgagggtacgcgcatgcgaatgcggaggcaagcatgccaggttccagccggtgtgtgtagatgtgactgaagatctcagaccggatcatttggttattgcccgcactggagcagagttcggatccagtggagaagaaactgactaaggtgagtattgggaaaactttggggtgggattttcagatggacagattgagtaaaaatttgttttttctgtcttgcagctgtcatgagtggaaacgcttcttttaaggggggagtcttcagcccttatctgacagggcgtctcccatcctgggcaggagttcgtcagaatgttatgggatctactgtggatggaagacccgtccaacccgccaattcttcaacgctgacctatgctactttaagttcttcacctttggacgcagctgcagctgccgccgccgcttctgttgccgctaacactgtgcttggaatgggttactatggaagcatcatggctaattccacttcctctaataacccttctaccctgactcaggacaagttacttgtccttttggcccagctggaggctttgacccaacgtctgggtgaactttctcagcaggtggtcgagttgcgagtacaaactgagtctgctgtcggcacggcaaagtctaaataaaaaaatcccagaatcaatgaataaataaacaagcttgttgttgatttaaaatcaagtgtttttatttcatttttcgcgcacggtatgccctagaccaccgatctctatcattgagaactcggtggattttttccaggatcctatagaggtgggattgaatgtttagatacatgggcattaggccgtctttggggtggagatagctccattgaagggattcatgctccggggtagtgttgtaaatcacccagtcataacaaggtcgcagtgcatggtgttgcacaatatcttttagaagtaggctgattgccacagataagcccttggtgtaggtgtttacaaaccggttgagctgggatgggtgcattcggggtgaaattatgtgcattttggattggatttttaagttggcaatattgccgccaagatcccgtcttgggttcatgttatgaaggaccaccaagacggtgtatccggtacatttaggaaatttatcgtgcagcttggatggaaaagcgtggaaaaatttggagacacccttgtgtcctccaagattttccatgcactcatccatgataatagcaatggggccgtgggcagcggcgcgggcaaacacgttccgtgggtctgacacatcatagttatgttcctgagttaaatcatcataagccattttaatgaatttggggcggagagtaccagattggggtatgaatgttccttcgggcccatactagtcttgcttgttttactttcgcttttggaaccgggttctgccaattacgatccatgtctagacttcgacccagaaaactgcacacttacttttgcacccgacacaagccgcatctgtggagttcatcgcctctcttacgaacttggcccccaacgacaaaaatttacctgcatggtgggaatcaaccccatagttatcacccagcaaagtggagatactaagggttgcattcactgctcctgcgattccatcgagtgcacctacaccctgctgaagaccctatgcggcctaagagacctgctaccaatgaattaaaaaatgattaataaaaaatcacttacttgaaatcagcaataaggtctctgttgaaattttctcccagcagcacctcacttccctcttcccaactctggtattctaaaccccgttcagcggcatactttctccatactttaaaggggatgtcaaattttagctcctctcctgtacccacaatcttcatgtctttcttcccagtggccggccatgaccaagagagtccggctcagtgactccttcaaccctgtctacccctatgaagatgaaagcacctcccaacacccctttataaacccagggtttatttccccaaatggcttcacacaaagcccaaacggagttcttactttaaaatgtttaaccccactaacaaccacaggcggatctctacagctaaaagtgggagggggacttacagtggatgacaccaacggttttttgaaagaaaacataagtgccaccacaccactcgttaagactggtcactctataggtttaccactaggagccggattgggaacgaatgaaaataaactttgtatcaaattaggacaaggacttacattcaattcaaacaacatttgcattgatgacaatattaacaccttatggacaggagtcaaccccaccgaagccaactgtcaaatcatgaactccagtgaatctaatgattgcaaattaattctaacactagttaaaactggagcactagtcactgcatttgtttatgttataggagtatctaacaattttaatatgctaactacacacagaaatataaattttactgcagagctgtttttcgattctactggtaatttactaactagactctcatccctcaaaactccacttaatcataaatcaggacaaaacatggctactggtgccattactaatgctaaaggtttcatgcccagcacgactgcctatcctttcaatgataattctagagaaaaagaaaactacatttacggaacttgttactacacagctagtgatcgcactgcttttcccattgacatatctgtcatgcttaaccgaagagcaataaatgacgagacatcatattgtattcgtataacttggtcctggaacacaggagatgccccagaggtgcaaacctctgctacaaccctagtcacctccccatttaccttttactacatcagagaagacgactgacaaataaaatcgctatccatcgaagatggatgtgtgttggttttttgtgtgatttgtgcgatcgctatgcggccgcttacctgcaggggttaccacacaaaaaaccaacacaccctaaagctcgatctccgacttgtttatttgaaaatcaattcacaaaatccgagtagttattttgcctcccccttcccatttaacagaatacaccaatctctccccacgcacagctttaaacatttggataccattagatatagacatggttttagattccacattccaaacagtttcagagcgagccaatctggggtcagtgatagataaaaatccatcgggatagtcttttaaagcgctttcacagtccaactgctgcggatgcgactccggagtctggatcacggtcatctggaagaagaacgatgggaatcataatccgaaaacggtatcggacgattgtgtctcatcaaacccacaagcagccgctgtctgcgtcgctccgtgcgactgctgtttatgggatcagggtccacagtgtcctgaagcatgattttaatagcccttaacatcaactttctggtgcgatgcgcgcagcaacgcattctgatttcactcaaatctttgcagtaggtacaacacattattacaatattgtttaataaaccataattaaaagcgctccagccaaaactcatatctgatataatcgcccctgcatgaccatcataccaaagtttaatataaattaaatgacgttccctcaaaaacacactacccacatacatgatctcttttggcatgtgcatattaacaatctgtctgtaccatggacaacgttggttaatcatgcaacccaatataaccttccggaaccacactgccaacaccgctcccccagccatgcattgaagtgaaccctgctgattacaatgacaatgaagaacccaattctctcgaccgtgaatcacttgagaatgaaaaatatctatagtggcacaacatagacataaatgcatgcatcttctcataatttttaactcctcaggatttagaaacatatcccagggaataggaagctcttgcagaacagtaaagctggcagaacaaggaagaccacgaacacaacttacactatgcatagtcatagtatcacaatctggcaacagcgggtggtcttcagtcatagaagctcgggtttcattttcctcacaacgtggtaactgggctctggtgtaagggtgatgtctggcgcatgatgtcgagcgtgcgcgcaaccttgtcataatggagttgcttcctgacattctcgtattttgtatagcaaaacgcggccctggcagaacacactcttcttcgccttctatcctgccgcttagcgtgttccgtgtgatagttcaagtacaaccacactcttaagttggtcaaaagaatgctggcttcagttgtaatcaaaactccatcgcatctaatcgttctgaggaaatcatccaagcaatgcaactggattgtgtttcaagcaggagaggagagggaagagacggaagaaccatgttaatttttattccaaacgatctcgcagtacttcaaattgtagatcgcgcagatggcatctctcgcccccactgtgttggtgaaaaagcacagctagatcaaaagaaatgcgattttcaaggtgctcaacggtggcttccagcaaagcctccacgcgcacatccaagaacaaaagaataccaaaagaaggagcattttctaactcctcaatcatcatattacattcctgcaccattcccagataattttcagctttccagccttgaattattcgtgtcagttcttgtggtaaatccaatccacacattacaaacaggtcccggagggcgccctccaccaccattcttaaacacaccctcataatgacaaaatatcttgctcctgtgtcacctgtagcgaattgagaatggcaacatcaattgacatgcccttggctctaagttcttctttaagttctagttgtaaaaactctctcatattatcaccaaactgcttagccagaagccccccgggaacaagagcaggggacgctacagtgcagtacaagcgcagacctccccaattggctccagcaaaaacaagattggaataagcatattgggaaccgccagtaatatcatcgaagttgctggaaatataatcaggcagagtttcttgtaaaaattgaataaaagaaaaatttgccaaaaaaacattcaaaacctctgggatgcaaatgcaataggttaccgcgctgcgctccaacattgttagttttgaattagtctgcaaaaataaaaaaaaaaacaagcgtcatatcatagtagcctgacgaacagatggataaatcagtctttccatcacaagacaagccacagggtctccagctcgaccctcgtaaaacctgtcatcatgattaaacaacagcaccgaaagttcctcgcggtgaccagcatgaataattcttgatgaagcatacaatccagacatgttagcatcagttaacgagaaaaaacagccaacatagcctttgggtataattatgcttaatcgtaagtatagcaaagccacccctcgcggatacaaagtaaaaggcacaggagaataaaaaatataattatttctctgctgctgttcaggcaacgtcgcccccggtccctctaaatacacatacaaagcctcatcagccatggcttaccagacaaagtacagcgggcacacaaagcacaagctctaaagtgactctccaacctctccacaatatatatatacacaagccctaaactgacgtaatgggagtaaagtgtaaaaaatcccgccaaacccaacacacaccccgaaactgcgtcaccagggaaaagtacagtttcacttccgcaatcccaacaggcgtaacttcctctttctcacggtacgtgatatcccactaacttgcaacgtcattttcccacggtcgcaccgccccttttagccgttaaccccacagccaatcaccacacgatccacactttttaaaatcacctcatttacatattggcaccattccatctataaggtatattatatagataggcgcgccctctcttaaggtagcatcgggatcgagtccctgagagaacatcctcaatcccgatctatccttagatccgaggaatatcgaaatcagttacgctagggataacagggtaatatagcatcccctcggattgctatctaccggctcgtcagctatgatctctcgatttcgatcaagaaatctcattggttaccttgggctatcgaaaccagtcaagtcagctacttggcgagatcgacttgtctgagtttcgactacgctcagaattgcgtcagcgcctatcgccaggtattactccaatcccgaatatccgagcctgagagaacatcctcaatcccgatctatccttagatccgaggaatatcgaaatcgtttaaatcttttcttgatggtaaatcattcgaatataagaatggagagacgaatggggaaacgacaaagatgacattctttggtccttctggtgaggttctcaagtttttggttaatcctgtcaacaacttatatcgtatggggctgacttcaggtgctacatttgaagagataaattgcactgaaatctagtaatattttatctgattaataagatgatcttcttgagatcgttttggtctgcgcgtaatctcttgctctgaaaacgaaaaaaccgccttgcagggcggtttttcgaaggttctctgagctaccaactctttgaaccgaggtaactggcttggcagagcgcagtcaccaaaacttgtcctttcagtttagccttaaccggcgcatgacttcaagactaactctgctaaatcaattaccagtggctgctgccagtggtgcttttgcatgtctttccgggttggactcaagacgatagttaccggataaggcgcagcggtcggactgaacggggggttcgtgcatacagtccagcttggagcgaactgcctacccggaactgagtgtcaggcgtggaatgagacaaacgcggccataacagcggaatgacaccggtaaaccgaaaggcaggaacaggagagcgcacgagggagccgccagggggaaacgcctggtatctttatagtcctgtcgggtttcgccaccactgatttgagcgtcagatttcgtgatgcttgtcaggggggcggagcctatggaaaaacggctttgccgcggccctctcacttccctgttaagtatcttcctggcatcttccaggaaatctccgccccgttcgtaagccatttccgctcgccgcagtcgaacgaccgagcgtagcgagtcagtgagcgaggaagcggaatatatcctgtatcacatattctgctgacgcaccggtgcggccttttttctcctgccacatgaagcacttcactgacaccctcatcagtgccaacatagtaagccagtatacactccgctaatttaaacgtggtgtaccgagaacgatcctctcagtgcgatctcgacgatcagtggtattccgacatatcgttgcttggcagtcagccagtcgatcctagcttgggacccaggaagtccaatcgtcagatattgtactcagcctggtcacggcagcgtaccgatctcgtaactataacggtcctaaggtagcgaactagatattgatagtctgatcggtcaacgtataatcgagtcctagcttttgcaaacatctatcaagagacaggatcagcaggaggctttcgcatgattgaacaagatggattgcacgcaggttctccggcggcttgggtggagaggctattcggctatgactgggcacaacagacaatcggctgctctgatgccgccgtgttccggctgtcagcgcaggggcgtccggttctttttgtcaagaccgacctgtccggtgccctgaatgaactgcaagacgaggcagcgcggctatcgtggctggcgacgacgggcgttccttgcgcggctgtgctcgacgttgtcactgaagcgggaagggactggctgctattgggcgaagtgccggggcaggatctcctgtcatctcaccttgctcctgccgagaaagtatccatcatggctgatgcaatgcggcggctgcatacgcttgatccggctacctgcccattcgaccaccaagcgaaacatcgcatcgagcgagcacgtactcggatggaagccggtcttgtcgatcaggatgatctggacgaagagcatcaggggctcgcgccagccgaactgttcgccaggctcaaggcgtctatgcccgacggcgaggatctcgtcgtgacccacggcgatgcctgcttgccgaatatcatggtggaaaatggccgcttttctggattcatcgactgtggccgtctgggtgtggcggaccgctatcaggacatagcgttggctacccgtgatattgctgaagagcttggcggcgaatgggctgaccgcttccttgtgctttacggtatcgccgcgcccgattcgcagcgcatcgccttctatcgccttcttgacgagttcttctgaccgattctaggtgcattggcgcagaaaaaaatgcctgatgcgacgctgcgcgtcttatactcccacatatgccagattcagcaacggatacggcttccccaacttgcccacttccatacgtgtcctccttaccagaaatttatccttaaggtccgtaactataacggtcctaaggtagcgaatcgacctagctctatcgaatctccctcgtttcgagcttacgcgaactagcctctggcgatagcatccgaggggcaggcatctatgtcgggtgcggagaaagaggtaatgtcaagttcgatctgattgcttggcataaagtccgatggttcgagtagactcagttcaacctctctcttaaggtagc

SEQ ID NO: 16 - DNA, 2350 bp, Artificial Sequence
  ColoAd2.0 synthetic fragment
gggcccatactagtcttgcttgttttactttcgcttttggaaccgggttctgccaattacgatccatgtctagacttcgacccagaaaactgcacacttacttttgcacccgacacaagccgcatctgtggagttcatcgcctctcttacgaacttggcccccaacgacaaaaatttacctgcatggtgggaatcaaccccatagttatcacccagcaaagtggagatactaagggttgcattcactgctcctgcgattccatcgagtgcacctacaccctgctgaagaccctatgcggcctaagagacctgctaccaatgaattaaaaaatgattaataaaaaatcacttacttgaaatcagcaataaggtctctgttgaaattttctcccagcagcacctcacttccctcttcccaactctggtattctaaaccccgttcagcggcatactttctccatactttaaaggggatgtcaaattttagctcctctcctgtacccacaatcttcatgtctttcttcccagtggccggccatgaccaagagagtccggctcagtgactccttcaaccctgtctacccctatgaagatgaaagcacctcccaacacccctttataaacccagggtttatttccccaaatggcttcacacaaagcccaaacggagttcttactttaaaatgtttaaccccactaacaaccacaggcggatctctacagctaaaagtgggagggggacttacagtggatgacaccaacggttttttgaaagaaaacataagtgccaccacaccactcgttaagactggtcactctataggtttaccactaggagccggattgggaacgaatgaaaataaactttgtatcaaattaggacaaggacttacattcaattcaaacaacatttgcattgatgacaatattaacaccttatggacaggagtcaaccccaccgaagccaactgtcaaatcatgaactccagtgaatctaatgattgcaaattaattctaacactagttaaaactggagcactagtcactgcatttgtttatgttataggagtatctaacaattttaatatgctaactacacacagaaatataaattttactgcagagctgtttttcgattctactggtaatttactaactagactctcatccctcaaaactccacttaatcataaatcaggacaaaacatggctactggtgccattactaatgctaaaggtttcatgcccagcacgactgcctatcctttcaatgataattctagagaaaaagaaaactacatttacggaacttgttactacacagctagtgatcgcactgcttttcccattgacatatctgtcatgcttaaccgaagagcaataaatgacgagacatcatattgtattcgtataacttggtcctggaacacaggagatgccccagaggtgcaaacctctgctacaaccctagtcacctccccatttaccttttactacatcagagaagacgactgacaaataaaatcgctatccatcgaagatggatgtgtgttggttttttgtgtgatttgtgcgatcgctatgcggccgcttacctgcaggggttaccacacaaaaaaccaacacaccctaaagctcgatctccgacttgtttatttgaaaatcaattcacaaaatccgagtagttattttgcctcccccttcccatttaacagaatacaccaatctctccccacgcacagctttaaacatttggataccattagatatagacatggttttagattccacattccaaacagtttcagagcgagccaatctggggtcagtgatagataaaaatccatcgggatagtcttttaaagcgctttcacagtccaactgctgcggatgcgactccggagtctggatcacggtcatctggaagaagaacgatgggaatcataatccgaaaacggtatcggacgattgtgtctcatcaaacccacaagcagccgctgtctgcgtcgctccgtgcgactgctgtttatgggatcagggtccacagtgtcctgaagcatgattttaatagcccttaacatcaactttctggtgcgatgcgcgcagcaacgcattctgatttcactcaaatctttgcagtaggtacaacacattattacaatattgtttaataaaccataattaaaagcgctccagccaaaactcatatctgatataatcgcccctgcatgaccatcataccaaagtttaatataaattaaatgacgttccctcaaaaacacactacccacatacatgatctcttttggcatgtgcatattaacaatctgtctgtaccatggacaacgtt

SEQ ID NO: 17 - DNA, 11987 bp, Artificial Sequence
  ColoAd2.1 shuttle vector
ggcgcgcctatctatataatataccttatagatggaatggtgccaatatgtaaatgaggtgattttaaaaagtgtggatcgtgtggtgattggctgtggggttaacggctaaaaggggcggtgcgaccgtgggaaaatgacgttttgtgggggtggagtttttttgcaagttgtcgcgggaaatgtgacgcataaaaaggcttttttctcacggaactacttagttttcccacggtatttaacaggaaatgaggtagttttgaccggatgcaagtgaaaattgttgattttcgcgcgaaaactgaatgaggaagtgtttttctgaataatgtggtatttatggcagggtggagtatttgttcagggccaggtagactttgacccattacgtggaggtttcgattaccgtgttttttacctgaatttccgcgtaccgtgtcaaagtcttctgtttttacgtaggtgtcagctgatcgctagggtatttatacctcagggtttgtgtcaagaggccactcttgagtgccagcgagaagagttttctcctctgcgccggcagtttaataataaaaaaatgagagatttgcgatttctgcctcaggaaataatctctgctgagactggaaatgaaatattggagcttgtggtgcacgccctgatgggagacgatccggagccacctgtgcagctttttgagcctcctacgcttcaggaactgtatgatttagaggtagagggatcggaggattctaatgaggaagctgtaaatggcttttttaccgattctatgcttttagctgctaatgaagggttagaattagatccgcctttggacacttttgatactccaggggtaattgtggaaagcggtacaggtgtaagaaaattacctgatttgagttccgtggactgtgatttgcactgctatgaagacgggtttcctccgagtgatgaggaggaccatgaaaaggagcagtccatgcagactgcagcgggtgagggagtgaaggctgccaatgttggttttcagttggattgcccggagcttcctggacatggctgtaagtcttgtgaatttcacaggaaaaatactggagtaaaggaactgttatgttcgctttgttatatgagaacgcactgccactttatttacagtaagtgtgtttaagttaaaatttaaaggaatatgctgtttttcacatgtatattgagtgtgagttttgtgcttcttattataggtcctgtgtctgatgctgatgaatcaccatctcctgattctactacctcacctcctgagattcaagcacctgttcctgtggacgtgcgcaagcccattcctgtgaagcttaagcctgggaaacgtccagcagtggaaaaacttgaggacttgttacagggtggggacggacctttggacttgagtacacggaaacgtccaagacaataagtgttccatatccgtgtttacttaaggtgacgtcaatatttgtgtgacagtgcaatgtaataaaaatatgttaactgttcactggtttttattgctttttgggcggggactcaggtatataagtagaagcagacctgtgtggttagctcataggagctggctttcatccatggaggtttgggccattttggaagaccttaggaagactaggcaactgttagagaacgcttcggacggagtctccggtttttggagattctggttcgctagtgaattagctagggtagtttttaggataaaacaggactataaacaagaatttgaaaagttgttggtagattgcccaggactttttgaagctcttaatttgggccatcaggttcactttaaagaaaaagttttatcagttttagacttttcaaccccaggtagaactgctgctgctgtggcttttcttacttttatattagataaatggatcccgcagactcatttcagcaggggatacgttttggatttcatagccacagcattgtggagaacatggaaggttcgcaagatgaggacaatcttaggttactggccagtgcagcctttgggtgtagcgggaatcctgaggcatccaccggtcatgccagcggttctggaggaggaacagcaagaggacaacccgagagccggcctggaccctccagtggaggaggcggagtagctgacttgtctcctgaactgcaacgggtgcttactggatctacgtccactggacgggataggggcgttaagagggagagggcatctagtggtactgatgctagatctgagttggctttaagtttaatgagtcgcagacgtcctgaaaccatttggtggcatgaggttcagaaagagggaagggatgaagtttctgtattgcaggagaaatattcactggaacaggtgaaaacatgttggttggagcctgaggatgattgggaggtggccattaaaaattatgccaagatagctttgaggcctgataaacagtataagattactagacggattaatatccggaatgcttgttacatatctggaaatggggctgaggtggtaatagatactcaagacaaggcagttattagatgctgcatgatggatatgtggcctggggtagtcggtatggaagcagtaacttttgtaaatgttaagtttaggggagatggttataatggaatagtgtttatggccaataccaaacttatattgcatggttgtagcttttttggtttcaacaatacctgtgtagatgcctggggacaggttagtgtacggggatgtagtttctatgcgtgttggattgccacagctggcagaaccaagagtcaattgtctctgaagaaatgcatatttcaaagatgtaacctgggcattctgaatgaaggcgaagcaagggtccgccactgcgcttctacagatactggatgttttattttgattaagggaaatgccagcgtaaagcataacatgatttgcggtgcttccgatgagaggccttatcaaatgctcacttgtgctggtgggcattgtaatatgctggctactgtgcatattgtttcccatcaacgcaaaaaatggcctgtttttgatcacaatgtgatgacgaagtgtaccatgcatgcaggtgggcgtagaggaatgtttatgccttaccagtgtaacatgaatcatgtgaaagtgttgttggaaccagatgccttttccagaatgagcctaacaggaatttttgacatgaacatgcaaatctggaagatcctgaggtatgatgatacgagatcgagggtacgcgcatgcgaatgcggaggcaagcatgccaggttccagccggtgtgtgtagatgtgactgaagatctcagaccggatcatttggttattgcccgcactggagcagagttcggatccagtggagaagaaactgactaaggtgagtattgggaaaactttggggtgggattttcagatggacagattgagtaaaaatttgttttttctgtcttgcagctgtcatgagtggaaacgcttcttttaaggggggagtcttcagcccttatctgacagggcgtctcccatcctgggcaggagttcgtcagaatgttatgggatctactgtggatggaagacccgtccaacccgccaattcttcaacgctgacctatgctactttaagttcttcacctttggacgcagctgcagctgccgccgccgcttctgttgccgctaacactgtgcttggaatgggttactatggaagcatcatggctaattccacttcctctaataacccttctaccctgactcaggacaagttacttgtccttttggcccagctggaggctttgacccaacgtctgggtgaactttctcagcaggtggtcgagttgcgagtacaaactgagtctgctgtcggcacggcaaagtctaaataaaaaaatcccagaatcaatgaataaataaacaagcttgttgttgatttaaaatcaagtgtttttatttcatttttcgcgcacggtatgccctagaccaccgatctctatcattgagaactcggtggattttttccaggatcctatagaggtgggattgaatgtttagatacatgggcattaggccgtctttggggtggagatagctccattgaagggattcatgctccggggtagtgttgtaaatcacccagtcataacaaggtcgcagtgcatggtgttgcacaatatcttttagaagtaggctgattgccacagataagcccttggtgtaggtgtttacaaaccggttgagctgggatgggtgcattcggggtgaaattatgtgcattttggattggatttttaagttggcaatattgccgccaagatcccgtcttgggttcatgttatgaaggaccaccaagacggtgtatccggtacatttaggaaatttatcgtgcagcttggatggaaaagcgtggaaaaatttggagacacccttgtgtcctccaagattttccatgcactcatccatgataatagcaatggggccgtgggcagcggcgcgggcaaacacgttccgtgggtctgacacatcatagttatgttcctgagttaaatcatcataagccattttaatgaatttggggcggagagtaccagattggggtatgaatgttccttcgggcccatactagtcttgcttgttttactttcgcttttggaaccgggttctgccaattacgatccatgtctagacttcgacccagaaaactgcacacttacttttgcacccgacacaagccgcatctgtggagttcatcgcctctcttacgaacttggcccccaacgacaaaaatttacctgcatggtgggaatcaaccccatagttatcacccagcaaagtggagatactaagggttgcattcactgctcctgcgattccatcgagtgcacctacaccctgctgaagaccctatgcggcctaagagacctgctaccaatgaattaaaaaatgattaataaaaaatcacttacttgaaatcagcaataaggtctctgttgaaattttctcccagcagcacctcacttccctcttcccaactctggtattctaaaccccgttcagcggcatactttctccatactttaaaggggatgtcaaattttagctcctctcctgtacccacaatcttcatgtctttcttcccagagcggccgcatgaccaagagagtccggctcagtgactccttcaaccctgtctacccctatgaagatgaaagcacctcccaacacccctttataaacccagggtttatttccccaaatggcttcacacaaagcccaaacggagttcttactttaaaatgtttaaccccactaacaaccacaggcggatctctacagctaaaagtgggagggggacttacagtggatgacaccaacggttttttgaaagaaaacataagtgccaccacaccactcgttaagactggtcactctataggtttaccactaggagccggattgggaacgaatgaaaataaactttgtatcaaattaggacaaggacttacattcaattcaaacaacatttgcattgatgacaatattaacaccttatggacaggagtcaaccccaccgaagccaactgtcaaatcatgaactccagtgaatctaatgattgcaaattaattctaacactagttaaaactggagcactagtcactgcatttgtttatgttataggagtatctaacaattttaatatgctaactacacacagaaatataaattttactgcagagctgtttttcgattctactggtaatttactaactagactctcatccctcaaaactccacttaatcataaatcaggacaaaacatggctactggtgccattactaatgctaaaggtttcatgcccagcacgactgcctatcctttcaatgataattctagagaaaaagaaaactacatttacggaacttgttactacacagctagtgatcgcactgcttttcccattgacatatctgtcatgcttaaccgaagagcaataaatgacgagacatcatattgtattcgtataacttggtcctggaacacaggagatgccccagaggtgcaaacctctgctacaaccctagtcacctccccatttaccttttactacatcagagaagacgactgacaaataaagtttaacttgtttatttgaaaatcaattcacaaaatccgagtagttattttgcctcccccttcccatttaacagaatacaccaatctctccccacgcacagctttaaacatttggataccattagatatagacatggttttagattccacattccaaacagtttcagagcgagccaatctggggtcagtgatagataaaaatccatcgggatagtcttttaaagcgctttcacagtccaactgctgcggatgcgactccggagtctggatcacggtcatctggaagaagaacgatgggaatcataatccgaaaacggtatcggacgattgtgtctcatcaaacccacaagcagccgctgtctgcgtcgctccgtgcgactgctgtttatgggatcagggtccacagtgtcctgaagcatgattttaatagcccttaacatcaactttctggtgcgatgcgcgcagcaacgcattctgatttcactcaaatctttgcagtaggtacaacacattattacaatattgtttaataaaccataattaaaagcgctccagccaaaactcatatctgatataatcgcccctgcatgaccatcataccaaagtttaatataaattaaatgacgttccctcaaaaacacactacccacatacatgatctcttttggcatgtgcatattaacaatctgtctgtaccatggacaacgttggttaatcatgcaacccaatataaccttccggaaccacactgccaacaccgctcccccagccatgcattgaagtgaaccctgctgattacaatgacaatgaagaacccaattctctcgaccgtgaatcacttgagaatgaaaaatatctatagtggcacaacatagacataaatgcatgcatcttctcataatttttaactcctcaggatttagaaacatatcccagggaataggaagctcttgcagaacagtaaagctggcagaacaaggaagaccacgaacacaacttacactatgcatagtcatagtatcacaatctggcaacagcgggtggtcttcagtcatagaagctcgggtttcattttcctcacaacgtggtaactgggctctggtgtaagggtgatgtctggcgcatgatgtcgagcgtgcgcgcaaccttgtcataatggagttgcttcctgacattctcgtattttgtatagcaaaacgcggccctggcagaacacactcttcttcgccttctatcctgccgcttagcgtgttccgtgtgatagttcaagtacaaccacactcttaagttggtcaaaagaatgctggcttcagttgtaatcaaaactccatcgcatctaatcgttctgaggaaatcatccaagcaatgcaactggattgtgtttcaagcaggagaggagagggaagagacggaagaaccatgttaatttttattccaaacgatctcgcagtacttcaaattgtagatcgcgcagatggcatctctcgcccccactgtgttggtgaaaaagcacagctagatcaaaagaaatgcgattttcaaggtgctcaacggtggcttccagcaaagcctccacgcgcacatccaagaacaaaagaataccaaaagaaggagcattttctaactcctcaatcatcatattacattcctgcaccattcccagataattttcagctttccagccttgaattattcgtgtcagttcttgtggtaaatccaatccacacattacaaacaggtcccggagggcgccctccaccaccattcttaaacacaccctcataatgacaaaatatcttgctcctgtgtcacctgtagcgaattgagaatggcaacatcaattgacatgcccttggctctaagttcttctttaagttctagttgtaaaaactctctcatattatcaccaaactgcttagccagaagccccccgggaacaagagcaggggacgctacagtgcagtacaagcgcagacctccccaattggctccagcaaaaacaagattggaataagcatattgggaaccgccagtaatatcatcgaagttgctggaaatataatcaggcagagtttcttgtaaaaattgaataaaagaaaaatttgccaaaaaaacattcaaaacctctgggatgcaaatgcaataggttaccgcgctgcgctccaacattgttagttttgaattagtctgcaaaaataaaaaaaaaaacaagcgtcatatcatagtagcctgacgaacagatggataaatcagtctttccatcacaagacaagccacagggtctccagctcgaccctcgtaaaacctgtcatcatgattaaacaacagcaccgaaagttcctcgcggtgaccagcatgaataattcttgatgaagcatacaatccagacatgttagcatcagttaacgagaaaaaacagccaacatagcctttgggtataattatgcttaatcgtaagtatagcaaagccacccctcgcggatacaaagtaaaaggcacaggagaataaaaaatataattatttctctgctgctgttcaggcaacgtcgcccccggtccctctaaatacacatacaaagcctcatcagccatggcttaccagacaaagtacagcgggcacacaaagcacaagctctaaagtgactctccaacctctccacaatatatatatacacaagccctaaactgacgtaatgggagtaaagtgtaaaaaatcccgccaaacccaacacacaccccgaaactgcgtcaccagggaaaagtacagtttcacttccgcaatcccaacaggcgtaacttcctctttctcacggtacgtgatatcccactaacttgcaacgtcattttcccacggtcgcaccgccccttttagccgttaaccccacagccaatcaccacacgatccacactttttaaaatcacctcatttacatattggcaccattccatctataaggtatattatatagataggcgcgccctctcttaaggtagcatcgggatcgagtccctgagagaacatcctcaatcccgatctatccttagatccgaggaatatcgaaatcagttacgctagggataacagggtaatatagcatcccctcggattgctatctaccggctcgtcagctatgatctctcgatttcgatcaagaaatctcattggttaccttgggctatcgaaaccagtcaagtcagctacttggcgagatcgacttgtctgagtttcgactacgctcagaattgcgtcagcgcctatcgccaggtattactccaatcccgaatatccgagcctgagagaacatcctcaatcccgatctatccttagatccgaggaatatcgaaatcgtttaaatcttttcttgatggtaaatcattcgaatataagaatggagagacgaatggggaaacgacaaagatgacattctttggtccttctggtgaggttctcaagtttttggttaatcctgtcaacaacttatatcgtatggggctgacttcaggtgctacatttgaagagataaattgcactgaaatctagtaatattttatctgattaataagatgatcttcttgagatcgttttggtctgcgcgtaatctcttgctctgaaaacgaaaaaaccgccttgcagggcggtttttcgaaggttctctgagctaccaactctttgaaccgaggtaactggcttggcagagcgcagtcaccaaaacttgtcctttcagtttagccttaaccggcgcatgacttcaagactaactctgctaaatcaattaccagtggctgctgccagtggtgcttttgcatgtctttccgggttggactcaagacgatagttaccggataaggcgcagcggtcggactgaacggggggttcgtgcatacagtccagcttggagcgaactgcctacccggaactgagtgtcaggcgtggaatgagacaaacgcggccataacagcggaatgacaccggtaaaccgaaaggcaggaacaggagagcgcacgagggagccgccagggggaaacgcctggtatctttatagtcctgtcgggtttcgccaccactgatttgagcgtcagatttcgtgatgcttgtcaggggggcggagcctatggaaaaacggctttgccgcggccctctcacttccctgttaagtatcttcctggcatcttccaggaaatctccgccccgttcgtaagccatttccgctcgccgcagtcgaacgaccgagcgtagcgagtcagtgagcgaggaagcggaatatatcctgtatcacatattctgctgacgcaccggtgcggccttttttctcctgccacatgaagcacttcactgacaccctcatcagtgccaacatagtaagccagtatacactccgctaatttaaacgtggtgtaccgagaacgatcctctcagtgcgatctcgacgatcagtggtattccgacatatcgttgcttggcagtcagccagtcgatcctagcttgggacccaggaagtccaatcgtcagatattgtactcagcctggtcacggcagcgtaccgatctcgtaactataacggtcctaaggtagcgaactagatattgatagtctgatcggtcaacgtataatcgagtcctagcttttgcaaacatctatcaagagacaggatcagcaggaggctttcgcatgattgaacaagatggattgcacgcaggttctccggcggcttgggtggagaggctattcggctatgactgggcacaacagacaatcggctgctctgatgccgccgtgttccggctgtcagcgcaggggcgtccggttctttttgtcaagaccgacctgtccggtgccctgaatgaactgcaagacgaggcagcgcggctatcgtggctggcgacgacgggcgttccttgcgcggctgtgctcgacgttgtcactgaagcgggaagggactggctgctattgggcgaagtgccggggcaggatctcctgtcatctcaccttgctcctgccgagaaagtatccatcatggctgatgcaatgcggcggctgcatacgcttgatccggctacctgcccattcgaccaccaagcgaaacatcgcatcgagcgagcacgtactcggatggaagccggtcttgtcgatcaggatgatctggacgaagagcatcaggggctcgcgccagccgaactgttcgccaggctcaaggcgtctatgcccgacggcgaggatctcgtcgtgacccacggcgatgcctgcttgccgaatatcatggtggaaaatggccgcttttctggattcatcgactgtggccgtctgggtgtggcggaccgctatcaggacatagcgttggctacccgtgatattgctgaagagcttggcggcgaatgggctgaccgcttccttgtgctttacggtatcgccgcgcccgattcgcagcgcatcgccttctatcgccttcttgacgagttcttctgaccgattctaggtgcattggcgcagaaaaaaatgcctgatgcgacgctgcgcgtcttatactcccacatatgccagattcagcaacggatacggcttccccaacttgcccacttccatacgtgtcctccttaccagaaatttatccttaaggtccgtaactataacggtcctaaggtagcgaatcgacctagctctatcgaatctccctcgtttcgagcttacgcgaactagcctctggcgatagcatccgaggggcaggcatctatgtcgggtgcggagaaagaggtaatgtcaagttcgatctgattgcttggcataaagtccgatggttcgagtagactcagttcaacctctctcttaaggtagc

SEQ ID NO: 18 - DNA, 2232 bp, Artificial Sequence
  - ColoAd2.1 DNA (PCR) fragment
gggcccatactagtcttgcttgttttactttcgcttttggaaccgggttctgccaattacgatccatgtctagacttcgacccagaaaactgcacacttacttttgcacccgacacaagccgcatctgtggagttcatcgcctctcttacgaacttggcccccaacgacaaaaatttacctgcatggtgggaatcaaccccatagttatcacccagcaaagtggagatactaagggttgcattcactgctcctgcgattccatcgagtgcacctacaccctgctgaagaccctatgcggcctaagagacctgctaccaatgaattaaaaaatgattaataaaaaatcacttacttgaaatcagcaataaggtctctgttgaaattttctcccagcagcacctcacttccctcttcccaactctggtattctaaaccccgttcagcggcatactttctccatactttaaaggggatgtcaaattttagctcctctcctgtacccacaatcttcatgtctttcttcccagagcggccgcatgaccaagagagtccggctcagtgactccttcaaccctgtctacccctatgaagatgaaagcacctcccaacacccctttataaacccagggtttatttccccaaatggcttcacacaaagcccaaacggagttcttactttaaaatgtttaaccccactaacaaccacaggcggatctctacagctaaaagtgggagggggacttacagtggatgacaccaacggttttttgaaagaaaacataagtgccaccacaccactcgttaagactggtcactctataggtttaccactaggagccggattgggaacgaatgaaaataaactttgtatcaaattaggacaaggacttacattcaattcaaacaacatttgcattgatgacaatattaacaccttatggacaggagtcaaccccaccgaagccaactgtcaaatcatgaactccagtgaatctaatgattgcaaattaattctaacactagttaaaactggagcactagtcactgcatttgtttatgttataggagtatctaacaattttaatatgctaactacacacagaaatataaattttactgcagagctgtttttcgattctactggtaatttactaactagactctcatccctcaaaactccacttaatcataaatcaggacaaaacatggctactggtgccattactaatgctaaaggtttcatgcccagcacgactgcctatcctttcaatgataattctagagaaaaagaaaactacatttacggaacttgttactacacagctagtgatcgcactgcttttcccattgacatatctgtcatgcttaaccgaagagcaataaatgacgagacatcatattgtattcgtataacttggtcctggaacacaggagatgccccagaggtgcaaacctctgctacaaccctagtcacctccccatttaccttttactacatcagagaagacgactgacaaataaagtttaacttgtttatttgaaaatcaattcacaaaatccgagtagttattttgcctcccccttcccatttaacagaatacaccaatctctccccacgcacagctttaaacatttggataccattagatatagacatggttttagattccacattccaaacagtttcagagcgagccaatctggggtcagtgatagataaaaatccatcgggatagtcttttaaagcgctttcacagtccaactgctgcggatgcgactccggagtctggatcacggtcatctggaagaagaacgatgggaatcataatccgaaaacggtatcggacgattgtgtctcatcaaacccacaagcagccgctgtctgcgtcgctccgtgcgactgctgtttatgggatcagggtccacagtgtcctgaagcatgattttaatagcccttaacatcaactttctggtgcgatgcgcgcagcaacgcattctgatttcactcaaatctttgcagtaggtacaacacattattacaatattgtttaataaaccataattaaaagcgctccagccaaaactcatatctgatataatcgcccctgcatgaccatcataccaaagtttaatataaattaaatgacgttccctcaaaaacacactacccacatacatgatctcttttggcatgtgcatattaacaatctgtctgtaccatggacaacgtt

SEQ ID NO: 19 - skipped

SEQ ID NO: 20 - DNA, 28 bp, Artificial Sequence
  primer 274
ttcggatccgggcccatactagtcttgc

SEQ ID NO: 21 - DNA, 33 bp, Artificial Sequence
  primer 275
catgcggccgctctgggaagaaagacatgaaga

SEQ ID NO: 22 - DNA, 28 bp, Artificial Sequence
  primer 276
tatgcggccgcatgaccaagagagtccg

SEQ ID NO: 23 - DNA, 30 bp, Artificial Sequence
  primer 277
tgcgaattcaacgttgtccatggtacagac

SEQ ID NO: 24 - DNA, 543 bp, Artificial Sequence
  ColoAd2.1 PCR 1 fragment
ggatccgggcccatactagtcttgcttgttttactttcgcttttggaaccgggttctgccaattacgatccatgtctagacttcgacccagaaaactgcacacttacttttgcacccgacacaagccgcatctgtggagttcatcgcctctcttacgaacttggcccccaacgacaaaaatttacctgcatggtgggaatcaaccccatagttatcacccagcaaagtggagatactaagggttgcattcactgctcctgcgattccatcgagtgcacctacaccctgctgaagaccctatgcggcctaagagacctgctaccaatgaattaaaaaatgattaataaaaaatcacttacttgaaatcagcaataaggtctctgttgaaattttctcccagcagcacctcacttccctcttcccaactctggtattctaaaccccgttcagcggcatactttctccatactttaaaggggatgtcaaattttagctcctctcctgtacccacaatcttcatgtctttcttcccagagcggccgc

SEQ ID NO: 25 - DNA, 1709 bp, Artificial Sequence
  ColoAd2.1 PCR 2 fragment
gcggccgcatgaccaagagagtccggctcagtgactccttcaaccctgtctacccctatgaagatgaaagcacctcccaacacccctttataaacccagggtttatttccccaaatggcttcacacaaagcccaaacggagttcttactttaaaatgtttaaccccactaacaaccacaggcggatctctacagctaaaagtgggagggggacttacagtggatgacaccaacggttttttgaaagaaaacataagtgccaccacaccactcgttaagactggtcactctataggtttaccactaggagccggattgggaacgaatgaaaataaactttgtatcaaattaggacaaggacttacattcaattcaaacaacatttgcattgatgacaatattaacaccttatggacaggagtcaaccccaccgaagccaactgtcaaatcatgaactccagtgaatctaatgattgcaaattaattctaacactagttaaaactggagcactagtcactgcatttgtttatgttataggagtatctaacaattttaatatgctaactacacacagaaatataaattttactgcagagctgtttttcgattctactggtaatttactaactagactctcatccctcaaaactccacttaatcataaatcaggacaaaacatggctactggtgccattactaatgctaaaggtttcatgcccagcacgactgcctatcctttcaatgataattctagagaaaaagaaaactacatttacggaacttgttactacacagctagtgatcgcactgcttttcccattgacatatctgtcatgcttaaccgaagagcaataaatgacgagacatcatattgtattcgtataacttggtcctggaacacaggagatgccccagaggtgcaaacctctgctacaaccctagtcacctccccatttaccttttactacatcagagaagacgactgacaaataaagtttaacttgtttatttgaaaatcaattcacaaaatccgagtagttattttgcctcccccttcccatttaacagaatacaccaatctctccccacgcacagctttaaacatttggataccattagatatagacatggttttagattccacattccaaacagtttcagagcgagccaatctggggtcagtgatagataaaaatccatcgggatagtcttttaaagcgctttcacagtccaactgctgcggatgcgactccggagtctggatcacggtcatctggaagaagaacgatgggaatcataatccgaaaacggtatcggacgattgtgtctcatcaaacccacaagcagccgctgtctgcgtcgctccgtgcgactgctgtttatgggatcagggtccacagtgtcctgaagcatgattttaatagcccttaacatcaactttctggtgcgatgcgcgcagcaacgcattctgatttcactcaaatctttgcagtaggtacaacacattattacaatattgtttaataaaccataattaaaagcgctccagccaaaactcatatctgatataatcgcccctgcatgaccatcataccaaagtttaatataaattaaatgacgttccctcaaaaacacactacccacatacatgatctcttttggcatgtgcatattaacaatctgtctgtaccatggacaacgttgaattc

SEQ ID NO: 26 - DNA, 11997 bp, Artificial Sequence
  ColoAd2.4 shuttle vector
ggcgcgcctatctatataatataccttatagatggaatggtgccaatatgtaaatgaggtgattttaaaaagtgtggatcgtgtggtgattggctgtggggttaacggctaaaaggggcggtgcgaccgtgggaaaatgacgttttgtgggggtggagtttttttgcaagttgtcgcgggaaatgtgacgcataaaaaggcttttttctcacggaactacttagttttcccacggtatttaacaggaaatgaggtagttttgaccggatgcaagtgaaaattgttgattttcgcgcgaaaactgaatgaggaagtgtttttctgaataatgtggtatttatggcagggtggagtatttgttcagggccaggtagactttgacccattacgtggaggtttcgattaccgtgttttttacctgaatttccgcgtaccgtgtcaaagtcttctgtttttacgtaggtgtcagctgatcgctagggtatttatacctcagggtttgtgtcaagaggccactcttgagtgccagcgagaagagttttctcctctgcgccggcagtttaataataaaaaaatgagagatttgcgatttctgcctcaggaaataatctctgctgagactggaaatgaaatattggagcttgtggtgcacgccctgatgggagacgatccggagccacctgtgcagctttttgagcctcctacgcttcaggaactgtatgatttagaggtagagggatcggaggattctaatgaggaagctgtaaatggcttttttaccgattctatgcttttagctgctaatgaagggttagaattagatccgcctttggacacttttgatactccaggggtaattgtggaaagcggtacaggtgtaagaaaattacctgatttgagttccgtggactgtgatttgcactgctatgaagacgggtttcctccgagtgatgaggaggaccatgaaaaggagcagtccatgcagactgcagcgggtgagggagtgaaggctgccaatgttggttttcagttggattgcccggagcttcctggacatggctgtaagtcttgtgaatttcacaggaaaaatactggagtaaaggaactgttatgttcgctttgttatatgagaacgcactgccactttatttacagtaagtgtgtttaagttaaaatttaaaggaatatgctgtttttcacatgtatattgagtgtgagttttgtgcttcttattataggtcctgtgtctgatgctgatgaatcaccatctcctgattctactacctcacctcctgagattcaagcacctgttcctgtggacgtgcgcaagcccattcctgtgaagcttaagcctgggaaacgtccagcagtggaaaaacttgaggacttgttacagggtggggacggacctttggacttgagtacacggaaacgtccaagacaataagtgttccatatccgtgtttacttaaggtgacgtcaatatttgtgtgacagtgcaatgtaataaaaatatgttaactgttcactggtttttattgctttttgggcggggactcaggtatataagtagaagcagacctgtgtggttagctcataggagctggctttcatccatggaggtttgggccattttggaagaccttaggaagactaggcaactgttagagaacgcttcggacggagtctccggtttttggagattctggttcgctagtgaattagctagggtagtttttaggataaaacaggactataaacaagaatttgaaaagttgttggtagattgcccaggactttttgaagctcttaatttgggccatcaggttcactttaaagaaaaagttttatcagttttagacttttcaaccccaggtagaactgctgctgctgtggcttttcttacttttatattagataaatggatcccgcagactcatttcagcaggggatacgttttggatttcatagccacagcattgtggagaacatggaaggttcgcaagatgaggacaatcttaggttactggccagtgcagcctttgggtgtagcgggaatcctgaggcatccaccggtcatgccagcggttctggaggaggaacagcaagaggacaacccgagagccggcctggaccctccagtggaggaggcggagtagctgacttgtctcctgaactgcaacgggtgcttactggatctacgtccactggacgggataggggcgttaagagggagagggcatctagtggtactgatgctagatctgagttggctttaagtttaatgagtcgcagacgtcctgaaaccatttggtggcatgaggttcagaaagagggaagggatgaagtttctgtattgcaggagaaatattcactggaacaggtgaaaacatgttggttggagcctgaggatgattgggaggtggccattaaaaattatgccaagatagctttgaggcctgataaacagtataagattactagacggattaatatccggaatgcttgttacatatctggaaatggggctgaggtggtaatagatactcaagacaaggcagttattagatgctgcatgatggatatgtggcctggggtagtcggtatggaagcagtaacttttgtaaatgttaagtttaggggagatggttataatggaatagtgtttatggccaataccaaacttatattgcatggttgtagcttttttggtttcaacaatacctgtgtagatgcctggggacaggttagtgtacggggatgtagtttctatgcgtgttggattgccacagctggcagaaccaagagtcaattgtctctgaagaaatgcatatttcaaagatgtaacctgggcattctgaatgaaggcgaagcaagggtccgccactgcgcttctacagatactggatgttttattttgattaagggaaatgccagcgtaaagcataacatgatttgcggtgcttccgatgagaggccttatcaaatgctcacttgtgctggtgggcattgtaatatgctggctactgtgcatattgtttcccatcaacgcaaaaaatggcctgtttttgatcacaatgtgatgacgaagtgtaccatgcatgcaggtgggcgtagaggaatgtttatgccttaccagtgtaacatgaatcatgtgaaagtgttgttggaaccagatgccttttccagaatgagcctaacaggaatttttgacatgaacatgcaaatctggaagatcctgaggtatgatgatacgagatcgagggtacgcgcatgcgaatgcggaggcaagcatgccaggttccagccggtgtgtgtagatgtgactgaagatctcagaccggatcatttggttattgcccgcactggagcagagttcggatccagtggagaagaaactgactaaggtgagtattgggaaaactttggggtgggattttcagatggacagattgagtaaaaatttgttttttctgtcttgcagctgtcatgagtggaaacgcttcttttaaggggggagtcttcagcccttatctgacagggcgtctcccatcctgggcaggagttcgtcagaatgttatgggatctactgtggatggaagacccgtccaacccgccaattcttcaacgctgacctatgctactttaagttcttcacctttggacgcagctgcagctgccgccgccgcttctgttgccgctaacactgtgcttggaatgggttactatggaagcatcatggctaattccacttcctctaataacccttctaccctgactcaggacaagttacttgtccttttggcccagctggaggctttgacccaacgtctgggtgaactttctcagcaggtggtcgagttgcgagtacaaactgagtctgctgtcggcacggcaaagtctaaataaaaaaatcccagaatcaatgaataaataaacaagcttgttgttgatttaaaatcaagtgtttttatttcatttttcgcgcacggtatgccctagaccaccgatctctatcattgagaactcggtggattttttccaggatcctatagaggtgggattgaatgtttagatacatgggcattaggccgtctttggggtggagatagctccattgaagggattcatgctccggggtagtgttgtaaatcacccagtcataacaaggtcgcagtgcatggtgttgcacaatatcttttagaagtaggctgattgccacagataagcccttggtgtaggtgtttacaaaccggttgagctgggatgggtgcattcggggtgaaattatgtgcattttggattggatttttaagttggcaatattgccgccaagatcccgtcttgggttcatgttatgaaggaccaccaagacggtgtatccggtacatttaggaaatttatcgtgcagcttggatggaaaagcgtggaaaaatttggagacacccttgtgtcctccaagattttccatgcactcatccatgataatagcaatggggccgtgggcagcggcgcgggcaaacacgttccgtgggtctgacacatcatagttatgttcctgagttaaatcatcataagccattttaatgaatttggggcggagagtaccagattggggtatgaatgttccttcgggcccatactagtcttgcttgttttactttcgcttttggaaccgggttctgccaattacgatccatgtctagacttcgacccagaaaactgcacacttacttttgcacccgacacaagccgcatctgtggagttcatcgcctctcttacgaacttggcccccaacgacaaaaatttacctgcatggtgggaatcaaccccatagttatcacccagcaaagtggagatactaagggttgcattcactgctcctgcgattccatcgagtgcacctacaccctgctgaagaccctatgcggcctaagagacctgctaccaatgaattaaaaaatgattaataaaaaatcacttacttgaaatcagcaataaggtctctgttgaaattttctcccagcagcacctcacttccctcttcccaactctggtattctaaaccccgttcagcggcatactttctccatactttaaaggggatgtcaaattttagctcctctcctgtacccacaatcttcatgtctttcttcccagatgaccaagagagtccggctcagtgactccttcaaccctgtctacccctatgaagatgaaagcacctcccaacacccctttataaacccagggtttatttccccaaatggcttcacacaaagcccaaacggagttcttactttaaaatgtttaaccccactaacaaccacaggcggatctctacagctaaaagtgggagggggacttacagtggatgacaccaacggttttttgaaagaaaacataagtgccaccacaccactcgttaagactggtcactctataggtttaccactaggagccggattgggaacgaatgaaaataaactttgtatcaaattaggacaaggacttacattcaattcaaacaacatttgcattgatgacaatattaacaccttatggacaggagtcaaccccaccgaagccaactgtcaaatcatgaactccagtgaatctaatgattgcaaattaattctaacactagttaaaactggagcactagtcactgcatttgtttatgttataggagtatctaacaattttaatatgctaactacacacagaaatataaattttactgcagagctgtttttcgattctactggtaatttactaactagactctcatccctcaaaactccacttaatcataaatcaggacaaaacatggctactggtgccattactaatgctaaaggtttcatgcccagcacgactgcctatcctttcaatgataattctagagaaaaagaaaactacatttacggaacttgttactacacagctagtgatcgcactgcttttcccattgacatatctgtcatgcttaaccgaagagcaataaatgacgagacatcatattgtattcgtataacttggtcctggaacacaggagatgccccagaggtgcaaacctctgctacaaccctagtcacctccccatttaccttttactacatcagagaagacgactgacaaataaagtttgcgatcgctaccctgcaggaacttgtttatttgaaaatcaattcacaaaatccgagtagttattttgcctcccccttcccatttaacagaatacaccaatctctccccacgcacagctttaaacatttggataccattagatatagacatggttttagattccacattccaaacagtttcagagcgagccaatctggggtcagtgatagataaaaatccatcgggatagtcttttaaagcgctttcacagtccaactgctgcggatgcgactccggagtctggatcacggtcatctggaagaagaacgatgggaatcataatccgaaaacggtatcggacgattgtgtctcatcaaacccacaagcagccgctgtctgcgtcgctccgtgcgactgctgtttatgggatcagggtccacagtgtcctgaagcatgattttaatagcccttaacatcaactttctggtgcgatgcgcgcagcaacgcattctgatttcactcaaatctttgcagtaggtacaacacattattacaatattgtttaataaaccataattaaaagcgctccagccaaaactcatatctgatataatcgcccctgcatgaccatcataccaaagtttaatataaattaaatgacgttccctcaaaaacacactacccacatacatgatctcttttggcatgtgcatattaacaatctgtctgtaccatggacaacgttggttaatcatgcaacccaatataaccttccggaaccacactgccaacaccgctcccccagccatgcattgaagtgaaccctgctgattacaatgacaatgaagaacccaattctctcgaccgtgaatcacttgagaatgaaaaatatctatagtggcacaacatagacataaatgcatgcatcttctcataatttttaactcctcaggatttagaaacatatcccagggaataggaagctcttgcagaacagtaaagctggcagaacaaggaagaccacgaacacaacttacactatgcatagtcatagtatcacaatctggcaacagcgggtggtcttcagtcatagaagctcgggtttcattttcctcacaacgtggtaactgggctctggtgtaagggtgatgtctggcgcatgatgtcgagcgtgcgcgcaaccttgtcataatggagttgcttcctgacattctcgtattttgtatagcaaaacgcggccctggcagaacacactcttcttcgccttctatcctgccgcttagcgtgttccgtgtgatagttcaagtacaaccacactcttaagttggtcaaaagaatgctggcttcagttgtaatcaaaactccatcgcatctaatcgttctgaggaaatcatccaagcaatgcaactggattgtgtttcaagcaggagaggagagggaagagacggaagaaccatgttaatttttattccaaacgatctcgcagtacttcaaattgtagatcgcgcagatggcatctctcgcccccactgtgttggtgaaaaagcacagctagatcaaaagaaatgcgattttcaaggtgctcaacggtggcttccagcaaagcctccacgcgcacatccaagaacaaaagaataccaaaagaaggagcattttctaactcctcaatcatcatattacattcctgcaccattcccagataattttcagctttccagccttgaattattcgtgtcagttcttgtggtaaatccaatccacacattacaaacaggtcccggagggcgccctccaccaccattcttaaacacaccctcataatgacaaaatatcttgctcctgtgtcacctgtagcgaattgagaatggcaacatcaattgacatgcccttggctctaagttcttctttaagttctagttgtaaaaactctctcatattatcaccaaactgcttagccagaagccccccgggaacaagagcaggggacgctacagtgcagtacaagcgcagacctccccaattggctccagcaaaaacaagattggaataagcatattgggaaccgccagtaatatcatcgaagttgctggaaatataatcaggcagagtttcttgtaaaaattgaataaaagaaaaatttgccaaaaaaacattcaaaacctctgggatgcaaatgcaataggttaccgcgctgcgctccaacattgttagttttgaattagtctgcaaaaataaaaaaaaaaacaagcgtcatatcatagtagcctgacgaacagatggataaatcagtctttccatcacaagacaagccacagggtctccagctcgaccctcgtaaaacctgtcatcatgattaaacaacagcaccgaaagttcctcgcggtgaccagcatgaataattcttgatgaagcatacaatccagacatgttagcatcagttaacgagaaaaaacagccaacatagcctttgggtataattatgcttaatcgtaagtatagcaaagccacccctcgcggatacaaagtaaaaggcacaggagaataaaaaatataattatttctctgctgctgttcaggcaacgtcgcccccggtccctctaaatacacatacaaagcctcatcagccatggcttaccagacaaagtacagcgggcacacaaagcacaagctctaaagtgactctccaacctctccacaatatatatatacacaagccctaaactgacgtaatgggagtaaagtgtaaaaaatcccgccaaacccaacacacaccccgaaactgcgtcaccagggaaaagtacagtttcacttccgcaatcccaacaggcgtaacttcctctttctcacggtacgtgatatcccactaacttgcaacgtcattttcccacggtcgcaccgccccttttagccgttaaccccacagccaatcaccacacgatccacactttttaaaatcacctcatttacatattggcaccattccatctataaggtatattatatagataggcgcgccctctcttaaggtagcatcgggatcgagtccctgagagaacatcctcaatcccgatctatccttagatccgaggaatatcgaaatcagttacgctagggataacagggtaatatagcatcccctcggattgctatctaccggctcgtcagctatgatctctcgatttcgatcaagaaatctcattggttaccttgggctatcgaaaccagtcaagtcagctacttggcgagatcgacttgtctgagtttcgactacgctcagaattgcgtcagcgcctatcgccaggtattactccaatcccgaatatccgagcctgagagaacatcctcaatcccgatctatccttagatccgaggaatatcgaaatcgtttaaatcttttcttgatggtaaatcattcgaatataagaatggagagacgaatggggaaacgacaaagatgacattctttggtccttctggtgaggttctcaagtttttggttaatcctgtcaacaacttatatcgtatggggctgacttcaggtgctacatttgaagagataaattgcactgaaatctagtaatattttatctgattaataagatgatcttcttgagatcgttttggtctgcgcgtaatctcttgctctgaaaacgaaaaaaccgccttgcagggcggtttttcgaaggttctctgagctaccaactctttgaaccgaggtaactggcttggcagagcgcagtcaccaaaacttgtcctttcagtttagccttaaccggcgcatgacttcaagactaactctgctaaatcaattaccagtggctgctgccagtggtgcttttgcatgtctttccgggttggactcaagacgatagttaccggataaggcgcagcggtcggactgaacggggggttcgtgcatacagtccagcttggagcgaactgcctacccggaactgagtgtcaggcgtggaatgagacaaacgcggccataacagcggaatgacaccggtaaaccgaaaggcaggaacaggagagcgcacgagggagccgccagggggaaacgcctggtatctttatagtcctgtcgggtttcgccaccactgatttgagcgtcagatttcgtgatgcttgtcaggggggcggagcctatggaaaaacggctttgccgcggccctctcacttccctgttaagtatcttcctggcatcttccaggaaatctccgccccgttcgtaagccatttccgctcgccgcagtcgaacgaccgagcgtagcgagtcagtgagcgaggaagcggaatatatcctgtatcacatattctgctgacgcaccggtgcggccttttttctcctgccacatgaagcacttcactgacaccctcatcagtgccaacatagtaagccagtatacactccgctaatttaaacgtggtgtaccgagaacgatcctctcagtgcgatctcgacgatcagtggtattccgacatatcgttgcttggcagtcagccagtcgatcctagcttgggacccaggaagtccaatcgtcagatattgtactcagcctggtcacggcagcgtaccgatctcgtaactataacggtcctaaggtagcgaactagatattgatagtctgatcggtcaacgtataatcgagtcctagcttttgcaaacatctatcaagagacaggatcagcaggaggctttcgcatgattgaacaagatggattgcacgcaggttctccggcggcttgggtggagaggctattcggctatgactgggcacaacagacaatcggctgctctgatgccgccgtgttccggctgtcagcgcaggggcgtccggttctttttgtcaagaccgacctgtccggtgccctgaatgaactgcaagacgaggcagcgcggctatcgtggctggcgacgacgggcgttccttgcgcggctgtgctcgacgttgtcactgaagcgggaagggactggctgctattgggcgaagtgccggggcaggatctcctgtcatctcaccttgctcctgccgagaaagtatccatcatggctgatgcaatgcggcggctgcatacgcttgatccggctacctgcccattcgaccaccaagcgaaacatcgcatcgagcgagcacgtactcggatggaagccggtcttgtcgatcaggatgatctggacgaagagcatcaggggctcgcgccagccgaactgttcgccaggctcaaggcgtctatgcccgacggcgaggatctcgtcgtgacccacggcgatgcctgcttgccgaatatcatggtggaaaatggccgcttttctggattcatcgactgtggccgtctgggtgtggcggaccgctatcaggacatagcgttggctacccgtgatattgctgaagagcttggcggcgaatgggctgaccgcttccttgtgctttacggtatcgccgcgcccgattcgcagcgcatcgccttctatcgccttcttgacgagttcttctgaccgattctaggtgcattggcgcagaaaaaaatgcctgatgcgacgctgcgcgtcttatactcccacatatgccagattcagcaacggatacggcttccccaacttgcccacttccatacgtgtcctccttaccagaaatttatccttaaggtccgtaactataacggtcctaaggtagcgaatcgacctagctctatcgaatctccctcgtttcgagcttacgcgaactagcctctggcgatagcatccgaggggcaggcatctatgtcgggtgcggagaaagaggtaatgtcaagttcgatctgattgcttggcataaagtccgatggttcgagtagactcagttcaacctctctcttaaggtagc

SEQ ID NO: 27 - DNA, 2242 bp, Artificial Sequence
  ColoAd2.4 synthetic fragment
gggcccatactagtcttgcttgttttactttcgcttttggaaccgggttctgccaattacgatccatgtctagacttcgacccagaaaactgcacacttacttttgcacccgacacaagccgcatctgtggagttcatcgcctctcttacgaacttggcccccaacgacaaaaatttacctgcatggtgggaatcaaccccatagttatcacccagcaaagtggagatactaagggttgcattcactgctcctgcgattccatcgagtgcacctacaccctgctgaagaccctatgcggcctaagagacctgctaccaatgaattaaaaaatgattaataaaaaatcacttacttgaaatcagcaataaggtctctgttgaaattttctcccagcagcacctcacttccctcttcccaactctggtattctaaaccccgttcagcggcatactttctccatactttaaaggggatgtcaaattttagctcctctcctgtacccacaatcttcatgtctttcttcccagatgaccaagagagtccggctcagtgactccttcaaccctgtctacccctatgaagatgaaagcacctcccaacacccctttataaacccagggtttatttccccaaatggcttcacacaaagcccaaacggagttcttactttaaaatgtttaaccccactaacaaccacaggcggatctctacagctaaaagtgggagggggacttacagtggatgacaccaacggttttttgaaagaaaacataagtgccaccacaccactcgttaagactggtcactctataggtttaccactaggagccggattgggaacgaatgaaaataaactttgtatcaaattaggacaaggacttacattcaattcaaacaacatttgcattgatgacaatattaacaccttatggacaggagtcaaccccaccgaagccaactgtcaaatcatgaactccagtgaatctaatgattgcaaattaattctaacactagttaaaactggagcactagtcactgcatttgtttatgttataggagtatctaacaattttaatatgctaactacacacagaaatataaattttactgcagagctgtttttcgattctactggtaatttactaactagactctcatccctcaaaactccacttaatcataaatcaggacaaaacatggctactggtgccattactaatgctaaaggtttcatgcccagcacgactgcctatcctttcaatgataattctagagaaaaagaaaactacatttacggaacttgttactacacagctagtgatcgcactgcttttcccattgacatatctgtcatgcttaaccgaagagcaataaatgacgagacatcatattgtattcgtataacttggtcctggaacacaggagatgccccagaggtgcaaacctctgctacaaccctagtcacctccccatttaccttttactacatcagagaagacgactgacaaataaagtttgcgatcgctaccctgcaggaacttgtttatttgaaaatcaattcacaaaatccgagtagttattttgcctcccccttcccatttaacagaatacaccaatctctccccacgcacagctttaaacatttggataccattagatatagacatggttttagattccacattccaaacagtttcagagcgagccaatctggggtcagtgatagataaaaatccatcgggatagtcttttaaagcgctttcacagtccaactgctgcggatgcgactccggagtctggatcacggtcatctggaagaagaacgatgggaatcataatccgaaaacggtatcggacgattgtgtctcatcaaacccacaagcagccgctgtctgcgtcgctccgtgcgactgctgtttatgggatcagggtccacagtgtcctgaagcatgattttaatagcccttaacatcaactttctggtgcgatgcgcgcagcaacgcattctgatttcactcaaatctttgcagtaggtacaacacattattacaatattgtttaataaaccataattaaaagcgctccagccaaaactcatatctgatataatcgcccctgcatgaccatcataccaaagtttaatataaattaaatgacgttccctcaaaaacacactacccacatacatgatctcttttggcatgtgcatattaacaatctgtctgtaccatggacaacgtt

SEQ ID NO: 28 - DNA, 35208 bp, Artificial Sequence
  ColoAd2.4 plasmid
ggcgcgcctatctatataatataccttatagatggaatggtgccaatatgtaaatgaggtgattttaaaaagtgtggatcgtgtggtgattggctgtggggttaacggctaaaaggggcggtgcgaccgtgggaaaatgacgttttgtgggggtggagtttttttgcaagttgtcgcgggaaatgtgacgcataaaaaggcttttttctcacggaactacttagttttcccacggtatttaacaggaaatgaggtagttttgaccggatgcaagtgaaaattgttgattttcgcgcgaaaactgaatgaggaagtgtttttctgaataatgtggtatttatggcagggtggagtatttgttcagggccaggtagactttgacccattacgtggaggtttcgattaccgtgttttttacctgaatttccgcgtaccgtgtcaaagtcttctgtttttacgtaggtgtcagctgatcgctagggtatttatacctcagggtttgtgtcaagaggccactcttgagtgccagcgagaagagttttctcctctgcgccggcagtttaataataaaaaaatgagagatttgcgatttctgcctcaggaaataatctctgctgagactggaaatgaaatattggagcttgtggtgcacgccctgatgggagacgatccggagccacctgtgcagctttttgagcctcctacgcttcaggaactgtatgatttagaggtagagggatcggaggattctaatgaggaagctgtaaatggcttttttaccgattctatgcttttagctgctaatgaagggttagaattagatccgcctttggacacttttgatactccaggggtaattgtggaaagcggtacaggtgtaagaaaattacctgatttgagttccgtggactgtgatttgcactgctatgaagacgggtttcctccgagtgatgaggaggaccatgaaaaggagcagtccatgcagactgcagcgggtgagggagtgaaggctgccaatgttggttttcagttggattgcccggagcttcctggacatggctgtaagtcttgtgaatttcacaggaaaaatactggagtaaaggaactgttatgttcgctttgttatatgagaacgcactgccactttatttacagtaagtgtgtttaagttaaaatttaaaggaatatgctgtttttcacatgtatattgagtgtgagttttgtgcttcttattataggtcctgtgtctgatgctgatgaatcaccatctcctgattctactacctcacctcctgagattcaagcacctgttcctgtggacgtgcgcaagcccattcctgtgaagcttaagcctgggaaacgtccagcagtggaaaaacttgaggacttgttacagggtggggacggacctttggacttgagtacacggaaacgtccaagacaataagtgttccatatccgtgtttacttaaggtgacgtcaatatttgtgtgacagtgcaatgtaataaaaatatgttaactgttcactggtttttattgctttttgggcggggactcaggtatataagtagaagcagacctgtgtggttagctcataggagctggctttcatccatggaggtttgggccattttggaagaccttaggaagactaggcaactgttagagaacgcttcggacggagtctccggtttttggagattctggttcgctagtgaattagctagggtagtttttaggataaaacaggactataaacaagaatttgaaaagttgttggtagattgcccaggactttttgaagctcttaatttgggccatcaggttcactttaaagaaaaagttttatcagttttagacttttcaaccccaggtagaactgctgctgctgtggcttttcttacttttatattagataaatggatcccgcagactcatttcagcaggggatacgttttggatttcatagccacagcattgtggagaacatggaaggttcgcaagatgaggacaatcttaggttactggccagtgcagcctttgggtgtagcgggaatcctgaggcatccaccggtcatgccagcggttctggaggaggaacagcaagaggacaacccgagagccggcctggaccctccagtggaggaggcggagtagctgacttgtctcctgaactgcaacgggtgcttactggatctacgtccactggacgggataggggcgttaagagggagagggcatctagtggtactgatgctagatctgagttggctttaagtttaatgagtcgcagacgtcctgaaaccatttggtggcatgaggttcagaaagagggaagggatgaagtttctgtattgcaggagaaatattcactggaacaggtgaaaacatgttggttggagcctgaggatgattgggaggtggccattaaaaattatgccaagatagctttgaggcctgataaacagtataagattactagacggattaatatccggaatgcttgttacatatctggaaatggggctgaggtggtaatagatactcaagacaaggcagttattagatgctgcatgatggatatgtggcctggggtagtcggtatggaagcagtaacttttgtaaatgttaagtttaggggagatggttataatggaatagtgtttatggccaataccaaacttatattgcatggttgtagcttttttggtttcaacaatacctgtgtagatgcctggggacaggttagtgtacggggatgtagtttctatgcgtgttggattgccacagctggcagaaccaagagtcaattgtctctgaagaaatgcatatttcaaagatgtaacctgggcattctgaatgaaggcgaagcaagggtccgccactgcgcttctacagatactggatgttttattttgattaagggaaatgccagcgtaaagcataacatgatttgcggtgcttccgatgagaggccttatcaaatgctcacttgtgctggtgggcattgtaatatgctggctactgtgcatattgtttcccatcaacgcaaaaaatggcctgtttttgatcacaatgtgatgacgaagtgtaccatgcatgcaggtgggcgtagaggaatgtttatgccttaccagtgtaacatgaatcatgtgaaagtgttgttggaaccagatgccttttccagaatgagcctaacaggaatttttgacatgaacatgcaaatctggaagatcctgaggtatgatgatacgagatcgagggtacgcgcatgcgaatgcggaggcaagcatgccaggttccagccggtgtgtgtagatgtgactgaagatctcagaccggatcatttggttattgcccgcactggagcagagttcggatccagtggagaagaaactgactaaggtgagtattgggaaaactttggggtgggattttcagatggacagattgagtaaaaatttgttttttctgtcttgcagctgtcatgagtggaaacgcttcttttaaggggggagtcttcagcccttatctgacagggcgtctcccatcctgggcaggagttcgtcagaatgttatgggatctactgtggatggaagacccgtccaacccgccaattcttcaacgctgacctatgctactttaagttcttcacctttggacgcagctgcagctgccgccgccgcttctgttgccgctaacactgtgcttggaatgggttactatggaagcatcatggctaattccacttcctctaataacccttctaccctgactcaggacaagttacttgtccttttggcccagctggaggctttgacccaacgtctgggtgaactttctcagcaggtggtcgagttgcgagtacaaactgagtctgctgtcggcacggcaaagtctaaataaaaaaatcccagaatcaatgaataaataaacaagcttgttgttgatttaaaatcaagtgtttttatttcatttttcgcgcacggtatgccctagaccaccgatctctatcattgagaactcggtggattttttccaggatcctatagaggtgggattgaatgtttagatacatgggcattaggccgtctttggggtggagatagctccattgaagggattcatgctccggggtagtgttgtaaatcacccagtcataacaaggtcgcagtgcatggtgttgcacaatatcttttagaagtaggctgattgccacagataagcccttggtgtaggtgtttacaaaccggttgagctgggatgggtgcattcggggtgaaattatgtgcattttggattggatttttaagttggcaatattgccgccaagatcccgtcttgggttcatgttatgaaggaccaccaagacggtgtatccggtacatttaggaaatttatcgtgcagcttggatggaaaagcgtggaaaaatttggagacacccttgtgtcctccaagattttccatgcactcatccatgataatagcaatggggccgtgggcagcggcgcgggcaaacacgttccgtgggtctgacacatcatagttatgttcctgagttaaatcatcataagccattttaatgaatttggggcggagagtaccagattggggtatgaatgttccttcgggccccggagcatagttcccctcacagatttgcatttcccaagctttcagttccgagggtggaatcatgtccacctggggggctatgaaaaacaccgtttctggggcgggggtgattaattgtgatgatagcaaatttctgagcaattgagatttgccacatccggtggggccataaatgattccgattacgggttgcaggtggtagtttagggaacggcaactgccgtcttctcgaagcaagggggccacctcgttcatcatttcccttacatgcatattttcccgcaccaaatccattaggaggcgctctcctcctagtgatagaagttcttgtagtgaggaaaagtttttcagcggtttcagaccgtcagccatgggcattttggagagagtttgctgcaaaagttctagtctgttccacagttcagtgatgtgttctatggcatctcgatccagcagacctcctcgtttcgcgggtttggacggctcctggaatagggtatgagacgatgggcgtccagcgctgccagggttcggtccttccagggtctcagtgttcgagtcagggttgtttccgtcacagtgaaggggtgtgcgcctgcttgggcgcttgccagggtgcgcttcagactcatcctgctggtcgaaaacttctgtcgcttggcgccctgtatgtcggccaagtagcagtttaccatgagttcgtagttgagcgcctcggctgcgtggcctttggcgcggagcttacctttggaagttttcttgcataccgggcagtataggcatttcagcgcatacaacttgggcgcaaggaaaacggattctggggagtatgcatctgcgccgcaggaggcgcaaacagtttcacattccaccagccaggttaaatccggttcattggggtcaaaaacaagttttccgccatattttttgatgcgtttcttacctttggtctccatgagttcgtgtcctcgttgagtgacaaacaggctgtccgtgtccccgtagactgattttacaggcctcttctccagtggagtgcctcggtcttcttcgtacaggaactctgaccactctgatacaaaggcgcgcgtccaggccagcacaaaggaggctatgtgggaggggtagcgatcgttgtcaaccagggggtccaccttttccaaagtatgcaaacacatgtcaccctcttcaacatccaggaatgtgattggcttgtaggtgtatttcacgtgacctggggtccccgctgggggggtataaaagggggcggttctttgctcttcctcactgtcttccggatcgctgtccaggaacgtcagctgttggggtaggtattccctctcgaaggcgggcatgacctctgcactcaggttgtcagtttctaagaacgaggaggatttgatattgacagtgccggttgagatgcctttcatgaggttttcgtccatctggtcagaaaacacaatttttttattgtcaagtttggtggcaaatgatccatacagggcgttggataaaagtttggcaatggatcgcatggtttggttcttttccttgtccgcgcgctctttggcggcgatgttgagttggacatactcgcgtgccaggcacttccattcggggaagatagttgttaattcatctggcacgattctcacttgccaccctcgattatgcaaggtaattaaatccacactggtggccacctcgcctcgaaggggttcattggtccaacagagcctacctcctttcctagaacagaaagggggaagtgggtctagcataagttcatcgggagggtctgcatccatggtaaagattcccggaagtaaatccttatcaaaatagctgatgggagtggggtcatctaaggccatttgccattctcgagctgccagtgcgcgctcatatgggttaaggggactgccccatggcatgggatgggtgagtgcagaggcatacatgccacagatgtcatagacgtagatgggatcctcaaagatgcctatgtaggttggatagcatcgcccccctctgatacttgctcgcacatagtcatatagttcatgtgatggcgctagcagccccggacccaagttggtgcgattgggtttttctgttctgtagacgatctggcgaaagatggcgtgagaattggaagagatggtgggtctttgaaaaatgttgaaatgggcatgaggtagacctacagagtctctgacaaagtgggcataagattcttgaagcttggttaccagttcggcggtgacaagtacgtctagggcgcagtagtcaagtgtttcttgaatgatgtcataacctggttggtttttcttttcccacagttcgcggttgagaaggtattcttcgcgatccttccagtactcttctagcggaaacccgtctttgtctgcacggtaagatcctagcatgtagaactgattaactgccttgtaagggcagcagcccttctctacgggtagagagtatgcttgagcagcttttcgtagcgaagcgtgagtaagggcaaaggtgtctctgaccatgactttgaggaattggtatttgaagtcgatgtcgtcacaggctccctgttcccagagttggaagtctacccgtttcttgtaggcggggttgggcaaagcgaaagtaacatcattgaagagaatcttgccggccctgggcatgaaattgcgagtgatgcgaaaaggctgtggtacttccgctcggttattgataacctgggcagctaggacgatctcgtcgaaaccgttgatgttgtgtcctacgatgtataattctatgaaacgcggcgtgcctctgacgtgaggtagcttactgagctcatcaaaggttaggtctgtggggtcagataaggcgtagtgttcgagagcccattcgtgcaggtgaggattcgctttaaggaaggaggaccagaggtccactgccagtgctgtttgtaactggtcccggtactgacgaaaatgccgtccgactgccattttttctggggtgacgcaatagaaggtttgggggtcctgccgccagcgatcccacttgagttttatggcgaggtcataggcgatgttgacgagccgctggtctccagagagtttcatgaccagcatgaaggggattagctgcttgccaaaggaccccatccaggtgtaggtttccacatcgtaggtgagaaagagcctttctgtgcgaggatgagagccaatcgggaagaactggatctcctgccaccagttggaggaatggctgttgatgtgatggaagtagaactccctgcgacgcgccgagcattcatgcttgtgcttgtacagacggccgcagtagtcgcagcgttgcacgggttgtatctcgtgaatgagttgtacctggcttcccttgacgagaaatttcagtgggaagccgaggcctggcgattgtatctcgtgctttactatgttgtctgcatcggcctgttcatcttctgtctcgatggtggtcatgctgacgagccctcgcgggaggcaagtccagacctcggcgcggcaggggcggagctcgaggacgagagcgcgcaggctggagctgtccagggtcctgagacgctgcggactcaggttagtaggcagtgtcaggagattaacttgcatgatcttttggagggcgtgcgggaggttcagatagtacttgatctcaacgggtccgttggtggagatgtcgatggcttgcagggttccgtgtcccttgggcgctaccaccgtgcccttgtttttcattttggacggcggtggctctgttgcttcttgcatgtttagaagcggtgtcgagggcgcgcaccgggcggcaggggcggctcgggacccggcggcatggctggcagtggtacgtcggcgccgcgcgcgggtaggttctggtactgcgccctgagaagactcgcatgcgcgacgacgcggcggttgacatcctggatctgacgcctctgggtgaaagctaccggccccgtgagcttgaacctgaaagagagttcaacagaatcaatctcggtatcgttgacggcggcttgcctaaggatttcttgcacgtcaccagagttgtcctggtaggcgatctccgccatgaactgctcgatctcttcctcttgaagatctccgcggcccgctctctcgacggtggccgcgaggtcgttggagatgcgcccaatgagttgagagaatgcattcatgcccgcctcgttccagacgcggctgtagaccacggcccccacgggatctctcgcgcgcatgaccacctgggcgaggttgagctccacgtggcgggtgaagaccgcatagttgcataggcgctggaaaaggtagttgagtgtggtggcgatgtgctcggtgacgaagaaatacatgatccatcgtctcagcggcatctcgctgacatcgcccagagcttccaagcgctccatggcctcgtagaagtccacggcaaaattaaaaaactgggagtttcgcgcggacacggtcaactcctcttccagaagacggataagttcggcgatggtggtgcgcacctcgcgctcgaaagcccctgggatttcttcctcaatctcttcttcttccactaacatctcttcctcttcaggtggggctgcaggaggagggggaacgcggcgacgccggcggcgcacgggcagacggtcgatgaatctttcaatgacctctccgcggcggcggcgcatggtttcagtgacggcgcggccgttctcgcgcggtcgcagagtaaaaacaccgccgcgcatctccttaaagtggtgactgggaggttctccgtttgggagggagagggcgctgattatacattttattaattggcccgtagggactgcacgcagagatctgatcgtgtcaagatccacgggatctgaaaacctttcgacgaaagcgtctaaccagtcacagtcacaaggtaggctgagtacggcttcttgtgggcgggggtggttatgtgttcggtctgggtcttctgtttcttcttcatctcgggaaggtgagacgatgctgctggtgatgaaattaaagtaggcagttctaagacggcggatggtggcgaggagcaccaggtctttgggtccggcttgctggatacgcaggcgattggccattccccaagcattatcctgacatctagcaagatctttgtagtagtcttgcatgagccgttctacgggcacttcttcctcacccgttctgccatgcatacgtgtgagtccaaatccgcgcattggttgtaccagtgccaagtcagctacgactctttcggcgaggatggcttgctgtacttgggtaagggtggcttgaaagtcatcaaaatccacaaagcggtggtaagctcctgtattaatggtgtaagcacagttggccatgactgaccagttaactgtctggtgaccagggcgcacgagctcggtgtatttaaggcgcgaataggcgcgggtgtcaaagatgtaatcgttgcaggtgcgcaccagatactggtaccctataagaaaatgcggcggtggttggcggtagagaggccatcgttctgtagctggagcgccaggggcgaggtcttccaacataaggcggtgatagccgtagatgtacctggacatccaggtgattcctgcggcggtagtagaagcccgaggaaactcgcgtacgcggttccaaatgttgcgtagcggcatgaagtagttcattgtaggcacggtttgaccagtgaggcgcgcgcagtcattgatgctctatagacacggagaaaatgaaagcgttcagcgactcgactccgtagcctggaggaacgtgaacgggttgggtcgcggtgtaccccggttcgagacttgtactcgagccggccggagccgcggctaacgtggtattggcactcccgtctcgacccagcctacaaaaatccaggatacggaatcgagtcgttttgctggtttccgaatggcagggaagtgagtcctattttttttttttgccgctcagatgcatcccgtgctgcgacagatgcgcccccaacaacagcccccctcgcagcagcagcagcagcaatcacaaaaggctgtccctgcaactactgcaactgccgccgtgagcggtgcgggacagcccgcctatgatctggacttggaagagggcgaaggactggcacgtctaggtgcgccttcacccgagcggcatccgcgagttcaactgaaaaaagattctcgcgaggcgtatgtgccccaacagaacctatttagagacagaagcggcgaggagccggaggagatgcgagcttcccgctttaacgcgggtcgtgagctgcgtcacggtttggaccgaagacgagtgttgcgggacgaggatttcgaagttgatgaaatgacagggatcagtcctgccagggcacacgtggctgcagccaaccttgtatcggcttacgagcagacagtaaaggaagagcgtaacttccaaaagtcttttaataatcatgtgcgaaccctgattgcccgcgaagaagttacccttggtttgatgcatttgtgggatttgatggaagctatcattcagaaccctactagcaaacctctgaccgcccagctgtttctggtggtgcaacacagcagagacaatgaggctttcagagaggcgctgctgaacatcaccgaacccgaggggagatggttgtatgatcttatcaacattctacagagtatcatagtgcaggagcggagcctgggcctggccgagaaggtggctgccatcaattactcggttttgagcttgggaaaatattacgctcgcaaaatctacaagactccatacgttcccatagacaaggaggtgaagatagatgggttctacatgcgcatgacgctcaaggtcttgaccctgagcgatgatcttggggtgtatcgcaatgacagaatgcatcgcgcggttagcgccagcaggaggcgcgagttaagcgacagggaactgatgcacagtttgcaaagagctctgactggagctggaaccgagggtgagaattacttcgacatgggagctgacttgcagtggcagcctagtcgcagggctctgagcgccgcgacggcaggatgtgagcttccttacatagaagaggcggatgaaggcgaggaggaagagggcgagtacttggaagactgatggcacaacccgtgttttttgctagatggaacagcaagcaccggatcccgcaatgcgggcggcgctgcagagccagccgtccggcattaactcctcggacgattggacccaggccatgcaacgtatcatggcgttgacgactcgcaaccccgaagcctttagacagcaaccccaggccaaccgtctatcggccatcatggaagctgtagtgccttcccgctctaatcccactcatgagaaggtcctggccatcgtgaacgcgttggtggagaacaaagctattcgtccagatgaggccggactggtatacaacgctctcttagaacgcgtggctcgctacaacagtagcaatgtgcaaaccaatttggaccgtatgataacagatgtacgcgaagccgtgtctcagcgcgaaaggttccagcgtgatgccaacctgggttcgctggtggcgttaaatgctttcttgagtactcagcctgctaatgtgccgcgtggtcaacaggattatactaactttttaagtgctttgagactgatggtatcagaagtacctcagagcgaagtgtatcagtccggtcctgattacttctttcagactagcagacagggcttgcagacggtaaatctgagccaagcttttaaaaaccttaaaggtttgtggggagtgcatgccccggtaggagaaagagcaaccgtgtctagcttgttaactccgaactcccgcctattattactgttggtagctcctttcaccgacagcggtagcatcgaccgtaattcctatttgggttacctactaaacctgtatcgcgaagccatagggcaaagtcaggtggacgagcagacctatcaagaaattacccaagtcagtcgcgctttgggacaggaagacactggcagtttggaagccactctgaacttcttgcttaccaatcggtctcaaaagatccctcctcaatatgctcttactgcggaggaggagaggatccttagatatgtgcagcagagcgtgggattgtttctgatgcaagagggggcaactccgactgcagcactggacatgacagcgcgaaatatggagcccagcatgtatgccagtaaccgacctttcattaacaaactgctggactacttgcacagagctgccgctatgaactctgattatttcaccaatgccatcttaaacccgcactggctgcccccacctggtttctacacgggcgaatatgacatgcccgaccctaatgacggatttctgtgggacgacgtggacagcgatgttttttcacctctttctgatcatcgcacgtggaaaaaggaaggcggcgatagaatgcattcttctgcatcgctgtccggggtcatgggtgctaccgcggctgagcccgagtctgcaagtccttttcctagtctacccttttctctacacagtgtacgtagcagcgaagtgggtagaataagtcgcccgagtttaatgggcgaagaggagtatctaaacgattccttgctcagaccggcaagagaaaaaaatttcccaaacaatggaatagaaagtttggtggataaaatgagtagatggaagacttatgctcaggatcacagagacgagcctgggatcatggggattacaagtagagcgagccgtagacgccagcgccatgacagacagaggggtcttgtgtgggacgatgaggattcggccgatgatagcagcgtgctggacttgggtgggagaggaaggggcaacccgtttgctcatttgcgccctcgcttgggtggtatgttgtaaaaaaaaataaaaaaaaaactcaccaaggccatggcgacgagcgtacgttcgttcttctttattatctgtgtctagtataatgaggcgagtcgtgctaggcggagcggtggtgtatccggagggtcctcctccttcgtacgagagcgtgatgcagcagcagcaggcgacggcggtgatgcaatccccactggaggctccctttgtgcctccgcgatacctggcacctacggagggcagaaacagcattcgttattcggaactggcacctcagtacgataccaccaggttgtatctggtggacaacaagtcggcggacattgcttctctgaactatcagaatgaccacagcaacttcttgaccacggtggtgcaaaacaatgactttacccctacggaagccagcacccagaccattaactttgatgaacgatcgcggtggggcggtcagctaaagaccatcatgcatactaacatgccaaacgtgaacgagtatatgtttagtaacaagttcaaagcgcgtgtgatggtgtccagaaaacctcccgacggtgctgcagttggggatacttatgatcacaagcaggatattttgaaatatgagtggttcgagtttactttgccagaaggcaacttttcagttactatgactattgatttgatgaacaatgccatcatagataattacttgaaagtgggtagacagaatggagtgcttgaaagtgacattggtgttaagttcgacaccaggaacttcaagctgggatgggatcccgaaaccaagttgatcatgcctggagtgtatacgtatgaagccttccatcctgacattgtcttactgcctggctgcggagtggattttaccgagagtcgtttgagcaaccttcttggtatcagaaaaaaacagccatttcaagagggttttaagattttgtatgaagatttagaaggtggtaatattccggccctcttggatgtagatgcctatgagaacagtaagaaagaacaaaaagccaaaatagaagctgctacagctgctgcagaagctaaggcaaacatagttgccagcgactctacaagggttgctaacgctggagaggtcagaggagacaattttgcgccaacacctgttccgactgcagaatcattattggccgatgtgtctgaaggaacggacgtgaaactcactattcaacctgtagaaaaagatagtaagaatagaagctataatgtgttggaagacaaaatcaacacagcctatcgcagttggtatctttcgtacaattatggcgatcccgaaaaaggagtgcgttcctggacattgctcaccacctcagatgtcacctgcggagcagagcaggtctactggtcgcttccagacatgatgaaggatcctgtcactttccgctccactagacaagtcagtaactaccctgtggtgggtgcagagcttatgcccgtcttctcaaagagcttctacaacgaacaagctgtgtactcccagcagctccgccagtccacctcgcttacgcacgtcttcaaccgctttcctgagaaccagattttaatccgtccgccggcgcccaccattaccaccgtcagtgaaaacgttcctgctctcacagatcacgggaccctgccgttgcgcagcagtatccggggagtccaacgtgtgaccgttactgacgccagacgccgcacctgtccctacgtgtacaaggcactgggcatagtcgcaccgcgcgtcctttcaagccgcactttctaaaaaaaaaaaaaatgtccattcttatctcgcccagtaataacaccggttggggtctgcgcgctccaagcaagatgtacggaggcgcacgcaaacgttctacccaacatcctgtccgtgttcgcggacattttcgcgctccatggggcgccctcaagggccgcactcgcgttcgaaccaccgtcgatgatgtaatcgatcaggtggttgccgacgcccgtaattatactcctactgcgcctacatctactgtggatgcagttattgacagtgtagtggctgacgctcgcaactatgctcgacgtaagagccggcgaaggcgcattgccagacgccaccgagctaccactgccatgcgagccgcaagagctctgctacgaagagctagacgcgtggggcgaagagccatgcttagggcggccagacgtgcagcttcgggcgccagcgccggcaggtcccgcaggcaagcagccgctgtcgcagcggcgactattgccgacatggcccaatcgcgaagaggcaatgtatactgggtgcgtgacgctgccaccggtcaacgtgtacccgtgcgcacccgtccccctcgcacttagaagatactgagcagtctccgatgttgtgtcccagcggcgaggatgtccaagcgcaaatacaaggaagaaatgctgcaggttatcgcacctgaagtctacggccaaccgttgaaggatgaaaaaaaaccccgcaaaatcaagcgggttaaaaaggacaaaaaagaagaggaagatggcgatgatgggctggcggagtttgtgcgcgagtttgccccacggcgacgcgtgcaatggcgtgggcgcaaagttcgacatgtgttgagacctggaacttcggtggtctttacacccggcgagcgttcaagcgctacttttaagcgttcctatgatgaggtgtacggggatgatgatattcttgagcaggcggctgaccgattaggcgagtttgcttatggcaagcgtagtagaataacttccaaggatgagacagtgtcgatacccttggatcatggaaatcccacccctagtcttaaaccggtcactttgcagcaagtgttacccgtaactccgcgaacaggtgttaaacgcgaaggtgaagatttgtatcccactatgcaactgatggtacccaaacgccagaagttggaggacgttttggagaaagtaaaagtggatccagatattcaacctgaggttaaagtgagacccattaagcaggtagcgcctggtctgggggtacaaactgtagacattaagattcccactgaaagtatggaagtgcaaactgaacccgcaaagcctactgccacctccactgaagtgcaaacggatccatggatgcccatgcctattacaactgacgccgccggtcccactcgaagatcccgacgaaagtacggtccagcaagtctgttgatgcccaattatgttgtacacccatctattattcctactcctggttaccgaggcactcgctactatcgcagccgaaacagtacctcccgccgtcgccgcaagacacctgcaaatcgcagtcgtcgccgtagacgcacaagcaaaccgactcccggcgccctggtgcggcaagtgtaccgcaatggtagtgcggaacctttgacactgccgcgtgcgcgttaccatccgagtatcatcacttaatcaatgttgccgctgcctccttgcagatatggccctcacttgtcgccttcgcgttcccatcactggttaccgaggaagaaactcgcgccgtagaagagggatgttgggacgcggaatgcgacgctacaggcgacggcgtgctatccgcaagcaattgcggggtggttttttaccagccttaattccaattatcgctgctgcaattggcgcgataccaggcatagcttccgtggcggttcaggcctcgcaacgacattgacattggaaaaaaacgtataaataaaaaaaaaaaaatacaatggactctgacactcctggtcctgtgactatgttttcttagagatggaagacatcaatttttcatccttggctccgcgacacggcacgaagccgtacatgggcacctggagcgacatcggcacgagccaactgaacgggggcgccttcaattggagcagtatctggagcgggcttaaaaattttggctcaaccataaaaacatacgggaacaaagcttggaacagcagtacaggacaggcgcttagaaataaacttaaagaccagaacttccaacaaaaagtagtcgatgggatagcttccggcatcaatggagtggtagatttggctaaccaggctgtgcagaaaaagataaacagtcgtttggacccgccgccagcaaccccaggtgaaatgcaagtggaggaagaaattcctccgccagaaaaacgaggcgacaagcgtccgcgtcccgatttggaagagacgctggtgacgcgcgtagatgaaccgccttcttatgaggaagcaacgaagcttggaatgcccaccactagaccgatagccccaatggccaccggggtgatgaaaccttctcagttgcatcgacccgtcaccttggatttgccccctccccctgctgctactgctgtacccgcttctaagcctgtcgctgccccgaaaccagtcgccgtagccaggtcacgtcccgggggcgctcctcgtccaaatgcgcactggcaaaatactctgaacagcatcgtgggtctaggcgtgcaaagtgtaaaacgccgtcgctgcttttaattaaatatggagtagcgcttaacttgcctatctgtgtatatgtgtcattacacgccgtcacagcagcagaggaaaaaaggaagaggtcgtgcgtcgacgctgagttactttcaagatggccaccccatcgatgctgccccaatgggcatacatgcacatcgccggacaggatgcttcggagtacctgagtccgggtctggtgcagttcgcccgcgccacagacacctacttcaatctgggaaataagtttagaaatcccaccgtagcgccgacccacgatgtgaccaccgaccgtagccagcggctcatgttgcgcttcgtgcccgttgaccgggaggacaatacatactcttacaaagtgcggtacaccctggccgtgggcgacaacagagtgctggatatggccagcacgttctttgacattaggggtgtgttggacagaggtcccagtttcaaaccctattctggtacggcttacaactccctggctcctaaaggcgctccaaatacatctcagtggattgcagaaggtgtaaaaaatacaactggtgaggaacacgtaacagaagaggaaaccaatactactacttacacttttggcaatgctcctgtaaaagctgaagctgaaattacaaaagaaggactcccagtaggtttggaagtttcagatgaagaaagtaaaccgatttatgctgataaaacatatcagccagaacctcagctgggagatgaaacttggactgaccttgatggaaaaaccgaaaagtatggaggcagggctctcaaacccgatactaagatgaaaccatgctacgggtcctttgccaaacctactaatgtgaaaggcggtcaggcaaaacaaaaaacaacggagcagccaaatcagaaagtcgaatatgatatcgacatggagttttttgatgcggcatcgcagaaaacaaacttaagtcctaaaattgtcatgtatgcagaaaatgtaaatttggaaactccagacactcatgtagtgtacaaacctggaacagaagacacaagttccgaagctaatttgggacaacaatctatgcccaacagacccaactacattggcttcagagataactttattggacttatgtactataacagtactggtaacatgggggtgctggctggtcaagcgtctcagttaaatgcagtggttgacttgcaggacagaaacacagaactttcttaccaactcttgcttgactctctgggcgacagaaccagatactttagcatgtggaatcaggctgtggacagttatgatcctgatgtacgtgttattgaaaatcatggtgtggaagatgaacttcccaactactgttttccactggacggcataggtgttccaacaaccagttacaaatcaatagttccaaatggagacaatgcgcctaattggaaggaacctgaagtaaatggaacaagtgagatcggacagggtaatttgtttgccatggaaattaaccttcaagccaatctatggcgaagtttcctttattccaatgtggctctatatctcccagactcgtacaaatacaccccgtccaatgtcactcttccagaaaacaaaaacacctacgactacatgaacgggcgggtggtgccgccatctctagtagacacctatgtgaacattggtgccaggtggtctctggatgccatggacaatgtcaacccattcaaccaccaccgtaacgctggcttgcgttaccgatccatgcttctgggtaacggacgttatgtgcctttccacatacaagtgcctcaaaaattcttcgctgttaaaaacctgctgcttctcccaggctcctacacttatgagtggaactttaggaaggatgtgaacatggttctacagagttccctcggtaacgacctgcgggtagatggcgccagcatcagtttcacgagcatcaacctctatgctacttttttccccatggctcacaacaccgcttccacccttgaagccatgctgcggaatgacaccaatgatcagtcattcaacgactacctatctgcagctaacatgctctaccccattcctgccaatgcaaccaatattcccatttccattccttctcgcaactgggcggctttcagaggctggtcatttaccagactgaaaaccaaagaaactccctctttggggtctggatttgacccctactttgtctattctggttctattccctacctggatggtaccttctacctgaaccacacttttaagaaggtttccatcatgtttgactcttcagtgagctggcctggaaatgacaggttactatctcctaacgaatttgaaataaagcgcactgtggatggcgaaggctacaacgtagcccaatgcaacatgaccaaagactggttcttggtacagatgctcgccaactacaacatcggctatcagggcttctacattccagaaggatacaaagatcgcatgtattcatttttcagaaacttccagcccatgagcaggcaggtggttgatgaggtcaattacaaagacttcaaggccgtcgccataccctaccaacacaacaactctggctttgtgggttacatggctccgaccatgcgccaaggtcaaccctatcccgctaactatccctatccactcattggaacaactgccgtaaatagtgttacgcagaaaaagttcttgtgtgacagaaccatgtggcgcataccgttctcgagcaacttcatgtctatgggggcccttacagacttgggacagaatatgctctatgccaactcagctcatgctctggacatgacctttgaggtggatcccatggatgagcccaccctgctttatcttctcttcgaagttttcgacgtggtcagagtgcatcagccacaccgcggcatcatcgaggcagtctacctgcgtacaccgttctcggccggtaacgctaccacgtaagaagcttcttgcttcttgcaaatagcagctgcaaccatggcctgcggatcccaaaacggctccagcgagcaagagctcagagccattgtccaagacctgggttgcggaccctattttttgggaacctacgataagcgcttcccggggttcatggcccccgataagctcgcctgtgccattgtaaatacggccggacgtgagacggggggagagcactggttggctttcggttggaacccacgttctaacacctgctacctttttgatccttttggattctcggatgatcgtctcaaacagatttaccagtttgaatatgagggtctcctgcgccgcagcgctcttgctaccaaggaccgctgtattacgctggaaaaatctacccagaccgtgcagggtccccgttctgccgcctgcggacttttctgctgcatgttccttcacgcctttgtgcactggcctgaccgtcccatggacggaaaccccaccatgaaattgctaactggagtgccaaacaacatgcttcattctcctaaagtccagcccaccctgtgtgacaatcaaaaagcactctaccattttcttaatacccattcgccttattttcgctcccatcgtacacacatcgaaagggccactgcgttcgaccgtatggatgttcaataatgactcatgtaaacaacgtgttcaataaacatcactttatttttttacatgtatcaaggctctgcattacttatttatttacaagtcgaatgggttctgacgagaatcagaatgacccgcaggcagtgatacgttgcggaactgatacttgggttgccacttgaattcgggaatcaccaacttgggaaccggtatatcgggcaggatgtcactccacagctttctggtcagctgcaaagctccaagcaggtcaggagccgaaatcttgaaatcacaattaggaccagtgctttgagcgcgagagttgcggtacaccggattgcagcactgaaacaccatcagcgacggatgtctcacgcttgccagcacggtgggatctgcaatcatgcccacatccagatcttcagcattggcaatgctgaacggggtcatcttgcaggtctgcctacccatggcgggcacccaattaggcttgtggttgcaatcgcagtgcagggggatcagtatcatcttggcctgatcctgtctgattcctggatacacggctctcatgaaagcatcatattgcttgaaagcctgctgggctttactaccctcggtataaaacatcccgcaggacctgctcgaaaactggttagctgcacagccggcatcattcacacagcagcgggcgtcattgttagctatttgcaccacacttctgccccagcggttttgggtgattttggttcgctcgggattctcctttaaggctcgttgtccgttctcgctggccacatccatctcgataatctgctccttctgaatcataatattgccatgcaggcacttcagcttgccctcataatcattgcagccatgaggccacaacgcacagcctgtacattcccaattatggtgggcgatctgagaaaaagaatgtatcattccctgcagaaatcttcccatcatcgtgctcagtgtcttgtgactagtgaaagttaactggatgcctcggtgctcctcgtttacgtactggtgacagatgcgcttgtattgttcgtgttgctcaggcattagtttaaaagaggttctaagttcgttatccagcctgtacttctccatcagcagacacatcacttccatgcctttctcccaagcagacaccaggggcaagctaatcggattcttaacagtgcaggcagcagctcctttagccagagggtcatctttagcgatcttctcaatgcttcttttgccatccttctcaacgatgcgcacgggcgggtagctgaaacccactgctacaagttgcgcctcttctctttcttcttcgctgtcttgactgatgtcttgcatggggatatgtttggtcttccttggcttctttttggggggtatcggaggaggaggactgtcgctccgttccggagacagggaggattgtgacgtttcgctcaccattaccaactgactgtcggtagaagaacctgaccccacacggcgacaggtgtttctcttcgggggcagaggtggaggcgattgcgaagggctgcggtccgacctggaaggcggatgactggcagaaccccttccgcgttcgggggtgtgctccctgtggcggtcgcttaactgatttccttcgcggctggccattgtgttctcctaggcagagaaacaacagacatggaaactcagccattgctgtcaacatcgccacgagtgccatcacatctcgtcctcagcgacgaggaaaaggagcagagcttaagcattccaccgcccagtcctgccaccacctctaccctagaagataaggaggtcgacgcatctcatgacatgcagaataaaaaagcgaaagagtctgagacagacatcgagcaagacccgggctatgtgacaccggtggaacacgaggaagagttgaaacgctttctagagagagaggatgaaaactgcccaaaacaacgagcagataactatcaccaagatgctggaaatagggatcagaacaccgactacctcatagggcttgacggggaagacgcgctccttaaacatctagcaagacagtcgctcatagtcaaggatgcattattggacagaactgaagtgcccatcagtgtggaagagctcagccgcgcctacgagcttaacctcttttcacctcgtactccccccaaacgtcagccaaacggcacctgcgagccaaatcctcgcttaaacttttatccagcttttgctgtgccagaagtactggctacctatcacatcttttttaaaaatcaaaaaattccagtctcctgccgcgctaatcgcacccgcgccgatgccctactcaatctgggacctggttcacgcttacctgatatagcttccttggaagaggttccaaagatcttcgagggtctgggcaataatgagactcgggccgcaaatgctctgcaaaagggagaaaatggcatggatgagcatcacagcgttctggtggaattggaaggcgataatgccagactcgcagtactcaagcgaagcatcgaggtcacacacttcgcatatcccgctgtcaacctgccccctaaagtcatgacggcggtcatggaccagttactcattaagcgcgcaagtcccctttcagaagacatgcatgacccagatgcctgtgatgagggtaaaccagtggtcagtgatgagcagctaacccgatggctgggcaccgactctcccagggatttggaagagcgtcgcaagcttatgatggccgtggtgctggttaccgtagaactagagtgtctccgacgtttctttaccgattcagaaaccttgcgcaaactcgaagagaatctgcactacacttttagacacggctttgtgcggcaggcatgcaagatatctaacgtggaactcaccaacctggtttcctacatgggtattctgcatgagaatcgcctaggacaaagcgtgctgcacagcaccctgaagggggaagcccgccgtgattacatccgcgattgtgtctatctgtacctgtgccacacgtggcaaaccggcatgggtgtatggcagcaatgtttagaagaacagaacttgaaagagcttgacaagctcttacagaaatctcttaaggttctgtggacagggttcgacgagcgcaccgtcgcttccgacctggcagacctcatcttcccagagcgtctcagggttactttgcgaaacggattgcctgactttatgagccagagcatgcttaacaattttcgctctttcatcctggaacgctccggtatcctgcccgccacctgctgcgcactgccctccgactttgtgcctctcacctaccgcgagtgccccccgccgctatggagtcactgctacctgttccgtctggccaactatctctcctaccactcggatgtgatcgaggatgtgagcggagacggcttgctggagtgtcactgccgctgcaatctgtgcacgccccaccggtccctagcttgcaacccccagttgatgagcgaaacccagataataggcacctttgaattgcaaggccccagcagccaaggcgatgggtcttctcctgggcaaagtttaaaactgaccccgggactgtggacctccgcctacttgcgcaagtttgctccggaagattaccacccctatgaaatcaagttctatgaggaccaatcacagcctccaaaggccgaactttcggcctgcgtcatcacccagggggcaattctggcccaattgcaagccatccaaaaatcccgccaagaatttctactgaaaaagggtaagggggtctaccttgacccccagaccggcgaggaactcaacacaaggttccctcaggatgtcccaacgacgagaaaacaagaagttgaaggtgcagccgccgcccccagaagatatggaggaagattgggacagtcaggcagaggaggcggaggaggacagtctggaggacagtctggaggaagacagtttggaggaggaaaacgaggaggcagaggaggtggaagaagtaaccgccgacaaacagttatcctcggctgcggagacaagcaacagcgctaccatctccgctccgagtcgaggaacccggcggcgtcccagcagtagatgggacgagaccggacgcttcccgaacccaaccagcgcttccaagaccggtaagaaggatcggcagggatacaagtcctggcgggggcataagaatgccatcatctcctgcttgcatgagtgcgggggcaacatatccttcacgcggcgctacttgctattccaccatggggtgaactttccgcgcaatgttttgcattactaccgtcacctccacagcccctactatagccagcaaatcccggcagtctcgacagataaagacagcggcggcgacctccaacagaaaaccagcagcggcagttagaaaatacacaacaagtgcagcaacaggaggattaaagattacagccaacgagccagcgcaaacccgagagttaagaaatcggatctttccaaccctgtatgccatcttccagcagagtcggggtcaagagcaggaactgaaaataaaaaaccgatctctgcgttcgctcaccagaagttgtttgtatcacaagagcgaagatcaacttcagcgcactctcgaggacgccgaggctctcttcaacaagtactgcgcgctgactcttaaagagtaggcagcgaccgcgcttattcaaaaaaggcgggaattacatcatcctcgacatgagtaaagaaattcccacgccttacatgtggagttatcaaccccaaatgggattggcggcaggcgcctcccaggactactccacccgcatgaattggctcagcgccgggccttctatgatttctcgagttaatgatatacgcgcctaccgaaaccaaatacttttggaacagtcagctcttaccaccacgccccgccaacaccttaatcccagaaattggcccgccgccctagtgtaccaggaaagtcccgctcccaccactgtattacttcctcgagacgcccaggccgaagtccaaatgactaatgcaggtgcgcagttagctggcggctccaccctatgtcgtcacaggcctcggcataatataaaacgcctgatgatcagaggccgaggtatccagctcaacgacgagtcggtgagctctccgcttggtctacgaccagacggaatctttcagattgccggctgcgggagatcttccttcacccctcgtcaggctgttctgactttggaaagttcgtcttcgcaaccccgctcgggcggaatcgggaccgttcaatttgtggaggagtttactccctctgtctacttcaaccccttctccggatctcctgggcattacccggacgagttcataccgaacttcgacgcgattagcgagtcagtggacggctacgattgatgtctggtgacgcggctgagctatctcggctgcgacatctagaccactgccgccgctttcgctgctttgcccgggaactcattgagttcatctacttcgaactccccaaggatcaccctcaaggtccggcccacggagtgcggatttctatcgaaggcaaaatagactctcgcctgcaacgaattttctcccagcggcccgtgctgatcgagcgagaccagggaaacaccacggtttccatctactgcatttgtaatcaccccggattgcatgaaagcctttgctgtcttatgtgtactgagtttaataaaaactgaattaagactctcctacggactgccgcttcttcaacccggattttacaaccagaagaacgaaacttttcctgtcgtccaggactctgttaacttcacctttcctactcacaaactagaagctcaacgactacaccgcttttccagaagcattttccctactaatactactttcaaaaccggaggtgagctccaaggtcttcctacagaaaacccttgggtggaagcgggccttgtagtgctaggaattcttgcgggtgggcttgtgattattctttgctacctatacacaccttgcttcactttcttagtggtgttgtggtattggtttaaaaaatggggcccatactagtcttgcttgttttactttcgcttttggaaccgggttctgccaattacgatccatgtctagacttcgacccagaaaactgcacacttacttttgcacccgacacaagccgcatctgtggagttcatcgcctctcttacgaacttggcccccaacgacaaaaatttacctgcatggtgggaatcaaccccatagttatcacccagcaaagtggagatactaagggttgcattcactgctcctgcgattccatcgagtgcacctacaccctgctgaagaccctatgcggcctaagagacctgctaccaatgaattaaaaaatgattaataaaaaatcacttacttgaaatcagcaataaggtctctgttgaaattttctcccagcagcacctcacttccctcttcccaactctggtattctaaaccccgttcagcggcatactttctccatactttaaaggggatgtcaaattttagctcctctcctgtacccacaatcttcatgtctttcttcccagatgaccaagagagtccggctcagtgactccttcaaccctgtctacccctatgaagatgaaagcacctcccaacacccctttataaacccagggtttatttccccaaatggcttcacacaaagcccaaacggagttcttactttaaaatgtttaaccccactaacaaccacaggcggatctctacagctaaaagtgggagggggacttacagtggatgacaccaacggttttttgaaagaaaacataagtgccaccacaccactcgttaagactggtcactctataggtttaccactaggagccggattgggaacgaatgaaaataaactttgtatcaaattaggacaaggacttacattcaattcaaacaacatttgcattgatgacaatattaacaccttatggacaggagtcaaccccaccgaagccaactgtcaaatcatgaactccagtgaatctaatgattgcaaattaattctaacactagttaaaactggagcactagtcactgcatttgtttatgttataggagtatctaacaattttaatatgctaactacacacagaaatataaattttactgcagagctgtttttcgattctactggtaatttactaactagactctcatccctcaaaactccacttaatcataaatcaggacaaaacatggctactggtgccattactaatgctaaaggtttcatgcccagcacgactgcctatcctttcaatgataattctagagaaaaagaaaactacatttacggaacttgttactacacagctagtgatcgcactgcttttcccattgacatatctgtcatgcttaaccgaagagcaataaatgacgagacatcatattgtattcgtataacttggtcctggaacacaggagatgccccagaggtgcaaacctctgctacaaccctagtcacctccccatttaccttttactacatcagagaagacgactgacaaataaagtttgcgatcgctaccctgcaggaacttgtttatttgaaaatcaattcacaaaatccgagtagttattttgcctcccccttcccatttaacagaatacaccaatctctccccacgcacagctttaaacatttggataccattagatatagacatggttttagattccacattccaaacagtttcagagcgagccaatctggggtcagtgatagataaaaatccatcgggatagtcttttaaagcgctttcacagtccaactgctgcggatgcgactccggagtctggatcacggtcatctggaagaagaacgatgggaatcataatccgaaaacggtatcggacgattgtgtctcatcaaacccacaagcagccgctgtctgcgtcgctccgtgcgactgctgtttatgggatcagggtccacagtgtcctgaagcatgattttaatagcccttaacatcaactttctggtgcgatgcgcgcagcaacgcattctgatttcactcaaatctttgcagtaggtacaacacattattacaatattgtttaataaaccataattaaaagcgctccagccaaaactcatatctgatataatcgcccctgcatgaccatcataccaaagtttaatataaattaaatgacgttccctcaaaaacacactacccacatacatgatctcttttggcatgtgcatattaacaatctgtctgtaccatggacaacgttggttaatcatgcaacccaatataaccttccggaaccacactgccaacaccgctcccccagccatgcattgaagtgaaccctgctgattacaatgacaatgaagaacccaattctctcgaccgtgaatcacttgagaatgaaaaatatctatagtggcacaacatagacataaatgcatgcatcttctcataatttttaactcctcaggatttagaaacatatcccagggaataggaagctcttgcagaacagtaaagctggcagaacaaggaagaccacgaacacaacttacactatgcatagtcatagtatcacaatctggcaacagcgggtggtcttcagtcatagaagctcgggtttcattttcctcacaacgtggtaactgggctctggtgtaagggtgatgtctggcgcatgatgtcgagcgtgcgcgcaaccttgtcataatggagttgcttcctgacattctcgtattttgtatagcaaaacgcggccctggcagaacacactcttcttcgccttctatcctgccgcttagcgtgttccgtgtgatagttcaagtacaaccacactcttaagttggtcaaaagaatgctggcttcagttgtaatcaaaactccatcgcatctaatcgttctgaggaaatcatccaagcaatgcaactggattgtgtttcaagcaggagaggagagggaagagacggaagaaccatgttaatttttattccaaacgatctcgcagtacttcaaattgtagatcgcgcagatggcatctctcgcccccactgtgttggtgaaaaagcacagctagatcaaaagaaatgcgattttcaaggtgctcaacggtggcttccagcaaagcctccacgcgcacatccaagaacaaaagaataccaaaagaaggagcattttctaactcctcaatcatcatattacattcctgcaccattcccagataattttcagctttccagccttgaattattcgtgtcagttcttgtggtaaatccaatccacacattacaaacaggtcccggagggcgccctccaccaccattcttaaacacaccctcataatgacaaaatatcttgctcctgtgtcacctgtagcgaattgagaatggcaacatcaattgacatgcccttggctctaagttcttctttaagttctagttgtaaaaactctctcatattatcaccaaactgcttagccagaagccccccgggaacaagagcaggggacgctacagtgcagtacaagcgcagacctccccaattggctccagcaaaaacaagattggaataagcatattgggaaccgccagtaatatcatcgaagttgctggaaatataatcaggcagagtttcttgtaaaaattgaataaaagaaaaatttgccaaaaaaacattcaaaacctctgggatgcaaatgcaataggttaccgcgctgcgctccaacattgttagttttgaattagtctgcaaaaataaaaaaaaaaacaagcgtcatatcatagtagcctgacgaacagatggataaatcagtctttccatcacaagacaagccacagggtctccagctcgaccctcgtaaaacctgtcatcatgattaaacaacagcaccgaaagttcctcgcggtgaccagcatgaataattcttgatgaagcatacaatccagacatgttagcatcagttaacgagaaaaaacagccaacatagcctttgggtataattatgcttaatcgtaagtatagcaaagccacccctcgcggatacaaagtaaaaggcacaggagaataaaaaatataattatttctctgctgctgttcaggcaacgtcgcccccggtccctctaaatacacatacaaagcctcatcagccatggcttaccagacaaagtacagcgggcacacaaagcacaagctctaaagtgactctccaacctctccacaatatatatatacacaagccctaaactgacgtaatgggagtaaagtgtaaaaaatcccgccaaacccaacacacaccccgaaactgcgtcaccagggaaaagtacagtttcacttccgcaatcccaacaggcgtaacttcctctttctcacggtacgtgatatcccactaacttgcaacgtcattttcccacggtcgcaccgccccttttagccgttaaccccacagccaatcaccacacgatccacactttttaaaatcacctcatttacatattggcaccattccatctataaggtatattatatagataggcgcgccctctcttaaggtagcatcgggatcgagtccctgagagaacatcctcaatcccgatctatccttagatccgaggaatatcgaaatcagttacgctagggataacagggtaatatagcatcccctcggattgctatctaccggctcgtcagctatgatctctcgatttcgatcaagaaatctcattggttaccttgggctatcgaaaccagtcaagtcagctacttggcgagatcgacttgtctgagtttcgactacgctcagaattgcgtcagcgcctatcgccaggtattactccaatcccgaatatccgagcctgagagaacatcctcaatcccgatctatccttagatccgaggaatatcgaaatcgtttaaatcttttcttgatggtaaatcattcgaatataagaatggagagacgaatggggaaacgacaaagatgacattctttggtccttctggtgaggttctcaagtttttggttaatcctgtcaacaacttatatcgtatggggctgacttcaggtgctacatttgaagagataaattgcactgaaatctagtaatattttatctgattaataagatgatcttcttgagatcgttttggtctgcgcgtaatctcttgctctgaaaacgaaaaaaccgccttgcagggcggtttttcgaaggttctctgagctaccaactctttgaaccgaggtaactggcttggcagagcgcagtcaccaaaacttgtcctttcagtttagccttaaccggcgcatgacttcaagactaactctgctaaatcaattaccagtggctgctgccagtggtgcttttgcatgtctttccgggttggactcaagacgatagttaccggataaggcgcagcggtcggactgaacggggggttcgtgcatacagtccagcttggagcgaactgcctacccggaactgagtgtcaggcgtggaatgagacaaacgcggccataacagcggaatgacaccggtaaaccgaaaggcaggaacaggagagcgcacgagggagccgccagggggaaacgcctggtatctttatagtcctgtcgggtttcgccaccactgatttgagcgtcagatttcgtgatgcttgtcaggggggcggagcctatggaaaaacggctttgccgcggccctctcacttccctgttaagtatcttcctggcatcttccaggaaatctccgccccgttcgtaagccatttccgctcgccgcagtcgaacgaccgagcgtagcgagtcagtgagcgaggaagcggaatatatcctgtatcacatattctgctgacgcaccggtgcggccttttttctcctgccacatgaagcacttcactgacaccctcatcagtgccaacatagtaagccagtatacactccgctaatttaaacgtggtgtaccgagaacgatcctctcagtgcgatctcgacgatcagtggtattccgacatatcgttgcttggcagtcagccagtcgatcctagcttgggacccaggaagtccaatcgtcagatattgtactcagcctggtcacggcagcgtaccgatctcgtaactataacggtcctaaggtagcgaactagatattgatagtctgatcggtcaacgtataatcgagtcctagcttttgcaaacatctatcaagagacaggatcagcaggaggctttcgcatgattgaacaagatggattgcacgcaggttctccggcggcttgggtggagaggctattcggctatgactgggcacaacagacaatcggctgctctgatgccgccgtgttccggctgtcagcgcaggggcgtccggttctttttgtcaagaccgacctgtccggtgccctgaatgaactgcaagacgaggcagcgcggctatcgtggctggcgacgacgggcgttccttgcgcggctgtgctcgacgttgtcactgaagcgggaagggactggctgctattgggcgaagtgccggggcaggatctcctgtcatctcaccttgctcctgccgagaaagtatccatcatggctgatgcaatgcggcggctgcatacgcttgatccggctacctgcccattcgaccaccaagcgaaacatcgcatcgagcgagcacgtactcggatggaagccggtcttgtcgatcaggatgatctggacgaagagcatcaggggctcgcgccagccgaactgttcgccaggctcaaggcgtctatgcccgacggcgaggatctcgtcgtgacccacggcgatgcctgcttgccgaatatcatggtggaaaatggccgcttttctggattcatcgactgtggccgtctgggtgtggcggaccgctatcaggacatagcgttggctacccgtgatattgctgaagagcttggcggcgaatgggctgaccgcttccttgtgctttacggtatcgccgcgcccgattcgcagcgcatcgccttctatcgccttcttgacgagttcttctgaccgattctaggtgcattggcgcagaaaaaaatgcctgatgcgacgctgcgcgtcttatactcccacatatgccagattcagcaacggatacggcttccccaacttgcccacttccatacgtgtcctccttaccagaaatttatccttaaggtccgtaactataacggtcctaaggtagcgaatcgacctagctctatcgaatctccctcgtttcgagcttacgcgaactagcctctggcgatagcatccgaggggcaggcatctatgtcgggtgcggagaaagaggtaatgtcaagttcgatctgattgcttggcataaagtccgatggttcgagtagactcagttcaacctctctcttaaggtagc

SEQ ID NO: 29 - DNA, 19 bp, Artificial Sequence
  19bp insert ColoAd2.4
gcgatcgctaccctgcagg

SEQ ID NO: 30 - DNA, 35316 bp, Artificial Sequence
  ColoAd2.0 Plasmid
ggcgcgcctatctatataatataccttatagatggaatggtgccaatatgtaaatgaggtgattttaaaaagtgtggatcgtgtggtgattggctgtggggttaacggctaaaaggggcggtgcgaccgtgggaaaatgacgttttgtgggggtggagtttttttgcaagttgtcgcgggaaatgtgacgcataaaaaggcttttttctcacggaactacttagttttcccacggtatttaacaggaaatgaggtagttttgaccggatgcaagtgaaaattgttgattttcgcgcgaaaactgaatgaggaagtgtttttctgaataatgtggtatttatggcagggtggagtatttgttcagggccaggtagactttgacccattacgtggaggtttcgattaccgtgttttttacctgaatttccgcgtaccgtgtcaaagtcttctgtttttacgtaggtgtcagctgatcgctagggtatttatacctcagggtttgtgtcaagaggccactcttgagtgccagcgagaagagttttctcctctgcgccggcagtttaataataaaaaaatgagagatttgcgatttctgcctcaggaaataatctctgctgagactggaaatgaaatattggagcttgtggtgcacgccctgatgggagacgatccggagccacctgtgcagctttttgagcctcctacgcttcaggaactgtatgatttagaggtagagggatcggaggattctaatgaggaagctgtaaatggcttttttaccgattctatgcttttagctgctaatgaagggttagaattagatccgcctttggacacttttgatactccaggggtaattgtggaaagcggtacaggtgtaagaaaattacctgatttgagttccgtggactgtgatttgcactgctatgaagacgggtttcctccgagtgatgaggaggaccatgaaaaggagcagtccatgcagactgcagcgggtgagggagtgaaggctgccaatgttggttttcagttggattgcccggagcttcctggacatggctgtaagtcttgtgaatttcacaggaaaaatactggagtaaaggaactgttatgttcgctttgttatatgagaacgcactgccactttatttacagtaagtgtgtttaagttaaaatttaaaggaatatgctgtttttcacatgtatattgagtgtgagttttgtgcttcttattataggtcctgtgtctgatgctgatgaatcaccatctcctgattctactacctcacctcctgagattcaagcacctgttcctgtggacgtgcgcaagcccattcctgtgaagcttaagcctgggaaacgtccagcagtggaaaaacttgaggacttgttacagggtggggacggacctttggacttgagtacacggaaacgtccaagacaataagtgttccatatccgtgtttacttaaggtgacgtcaatatttgtgtgacagtgcaatgtaataaaaatatgttaactgttcactggtttttattgctttttgggcggggactcaggtatataagtagaagcagacctgtgtggttagctcataggagctggctttcatccatggaggtttgggccattttggaagaccttaggaagactaggcaactgttagagaacgcttcggacggagtctccggtttttggagattctggttcgctagtgaattagctagggtagtttttaggataaaacaggactataaacaagaatttgaaaagttgttggtagattgcccaggactttttgaagctcttaatttgggccatcaggttcactttaaagaaaaagttttatcagttttagacttttcaaccccaggtagaactgctgctgctgtggcttttcttacttttatattagataaatggatcccgcagactcatttcagcaggggatacgttttggatttcatagccacagcattgtggagaacatggaaggttcgcaagatgaggacaatcttaggttactggccagtgcagcctttgggtgtagcgggaatcctgaggcatccaccggtcatgccagcggttctggaggaggaacagcaagaggacaacccgagagccggcctggaccctccagtggaggaggcggagtagctgacttgtctcctgaactgcaacgggtgcttactggatctacgtccactggacgggataggggcgttaagagggagagggcatctagtggtactgatgctagatctgagttggctttaagtttaatgagtcgcagacgtcctgaaaccatttggtggcatgaggttcagaaagagggaagggatgaagtttctgtattgcaggagaaatattcactggaacaggtgaaaacatgttggttggagcctgaggatgattgggaggtggccattaaaaattatgccaagatagctttgaggcctgataaacagtataagattactagacggattaatatccggaatgcttgttacatatctggaaatggggctgaggtggtaatagatactcaagacaaggcagttattagatgctgcatgatggatatgtggcctggggtagtcggtatggaagcagtaacttttgtaaatgttaagtttaggggagatggttataatggaatagtgtttatggccaataccaaacttatattgcatggttgtagcttttttggtttcaacaatacctgtgtagatgcctggggacaggttagtgtacggggatgtagtttctatgcgtgttggattgccacagctggcagaaccaagagtcaattgtctctgaagaaatgcatatttcaaagatgtaacctgggcattctgaatgaaggcgaagcaagggtccgccactgcgcttctacagatactggatgttttattttgattaagggaaatgccagcgtaaagcataacatgatttgcggtgcttccgatgagaggccttatcaaatgctcacttgtgctggtgggcattgtaatatgctggctactgtgcatattgtttcccatcaacgcaaaaaatggcctgtttttgatcacaatgtgatgacgaagtgtaccatgcatgcaggtgggcgtagaggaatgtttatgccttaccagtgtaacatgaatcatgtgaaagtgttgttggaaccagatgccttttccagaatgagcctaacaggaatttttgacatgaacatgcaaatctggaagatcctgaggtatgatgatacgagatcgagggtacgcgcatgcgaatgcggaggcaagcatgccaggttccagccggtgtgtgtagatgtgactgaagatctcagaccggatcatttggttattgcccgcactggagcagagttcggatccagtggagaagaaactgactaaggtgagtattgggaaaactttggggtgggattttcagatggacagattgagtaaaaatttgttttttctgtcttgcagctgtcatgagtggaaacgcttcttttaaggggggagtcttcagcccttatctgacagggcgtctcccatcctgggcaggagttcgtcagaatgttatgggatctactgtggatggaagacccgtccaacccgccaattcttcaacgctgacctatgctactttaagttcttcacctttggacgcagctgcagctgccgccgccgcttctgttgccgctaacactgtgcttggaatgggttactatggaagcatcatggctaattccacttcctctaataacccttctaccctgactcaggacaagttacttgtccttttggcccagctggaggctttgacccaacgtctgggtgaactttctcagcaggtggtcgagttgcgagtacaaactgagtctgctgtcggcacggcaaagtctaaataaaaaaatcccagaatcaatgaataaataaacaagcttgttgttgatttaaaatcaagtgtttttatttcatttttcgcgcacggtatgccctagaccaccgatctctatcattgagaactcggtggattttttccaggatcctatagaggtgggattgaatgtttagatacatgggcattaggccgtctttggggtggagatagctccattgaagggattcatgctccggggtagtgttgtaaatcacccagtcataacaaggtcgcagtgcatggtgttgcacaatatcttttagaagtaggctgattgccacagataagcccttggtgtaggtgtttacaaaccggttgagctgggatgggtgcattcggggtgaaattatgtgcattttggattggatttttaagttggcaatattgccgccaagatcccgtcttgggttcatgttatgaaggaccaccaagacggtgtatccggtacatttaggaaatttatcgtgcagcttggatggaaaagcgtggaaaaatttggagacacccttgtgtcctccaagattttccatgcactcatccatgataatagcaatggggccgtgggcagcggcgcgggcaaacacgttccgtgggtctgacacatcatagttatgttcctgagttaaatcatcataagccattttaatgaatttggggcggagagtaccagattggggtatgaatgttccttcgggccccggagcatagttcccctcacagatttgcatttcccaagctttcagttccgagggtggaatcatgtccacctggggggctatgaaaaacaccgtttctggggcgggggtgattaattgtgatgatagcaaatttctgagcaattgagatttgccacatccggtggggccataaatgattccgattacgggttgcaggtggtagtttagggaacggcaactgccgtcttctcgaagcaagggggccacctcgttcatcatttcccttacatgcatattttcccgcaccaaatccattaggaggcgctctcctcctagtgatagaagttcttgtagtgaggaaaagtttttcagcggtttcagaccgtcagccatgggcattttggagagagtttgctgcaaaagttctagtctgttccacagttcagtgatgtgttctatggcatctcgatccagcagacctcctcgtttcgcgggtttggacggctcctggaatagggtatgagacgatgggcgtccagcgctgccagggttcggtccttccagggtctcagtgttcgagtcagggttgtttccgtcacagtgaaggggtgtgcgcctgcttgggcgcttgccagggtgcgcttcagactcatcctgctggtcgaaaacttctgtcgcttggcgccctgtatgtcggccaagtagcagtttaccatgagttcgtagttgagcgcctcggctgcgtggcctttggcgcggagcttacctttggaagttttcttgcataccgggcagtataggcatttcagcgcatacaacttgggcgcaaggaaaacggattctggggagtatgcatctgcgccgcaggaggcgcaaacagtttcacattccaccagccaggttaaatccggttcattggggtcaaaaacaagttttccgccatattttttgatgcgtttcttacctttggtctccatgagttcgtgtcctcgttgagtgacaaacaggctgtccgtgtccccgtagactgattttacaggcctcttctccagtggagtgcctcggtcttcttcgtacaggaactctgaccactctgatacaaaggcgcgcgtccaggccagcacaaaggaggctatgtgggaggggtagcgatcgttgtcaaccagggggtccaccttttccaaagtatgcaaacacatgtcaccctcttcaacatccaggaatgtgattggcttgtaggtgtatttcacgtgacctggggtccccgctgggggggtataaaagggggcggttctttgctcttcctcactgtcttccggatcgctgtccaggaacgtcagctgttggggtaggtattccctctcgaaggcgggcatgacctctgcactcaggttgtcagtttctaagaacgaggaggatttgatattgacagtgccggttgagatgcctttcatgaggttttcgtccatctggtcagaaaacacaatttttttattgtcaagtttggtggcaaatgatccatacagggcgttggataaaagtttggcaatggatcgcatggtttggttcttttccttgtccgcgcgctctttggcggcgatgttgagttggacatactcgcgtgccaggcacttccattcggggaagatagttgttaattcatctggcacgattctcacttgccaccctcgattatgcaaggtaattaaatccacactggtggccacctcgcctcgaaggggttcattggtccaacagagcctacctcctttcctagaacagaaagggggaagtgggtctagcataagttcatcgggagggtctgcatccatggtaaagattcccggaagtaaatccttatcaaaatagctgatgggagtggggtcatctaaggccatttgccattctcgagctgccagtgcgcgctcatatgggttaaggggactgccccatggcatgggatgggtgagtgcagaggcatacatgccacagatgtcatagacgtagatgggatcctcaaagatgcctatgtaggttggatagcatcgcccccctctgatacttgctcgcacatagtcatatagttcatgtgatggcgctagcagccccggacccaagttggtgcgattgggtttttctgttctgtagacgatctggcgaaagatggcgtgagaattggaagagatggtgggtctttgaaaaatgttgaaatgggcatgaggtagacctacagagtctctgacaaagtgggcataagattcttgaagcttggttaccagttcggcggtgacaagtacgtctagggcgcagtagtcaagtgtttcttgaatgatgtcataacctggttggtttttcttttcccacagttcgcggttgagaaggtattcttcgcgatccttccagtactcttctagcggaaacccgtctttgtctgcacggtaagatcctagcatgtagaactgattaactgccttgtaagggcagcagcccttctctacgggtagagagtatgcttgagcagcttttcgtagcgaagcgtgagtaagggcaaaggtgtctctgaccatgactttgaggaattggtatttgaagtcgatgtcgtcacaggctccctgttcccagagttggaagtctacccgtttcttgtaggcggggttgggcaaagcgaaagtaacatcattgaagagaatcttgccggccctgggcatgaaattgcgagtgatgcgaaaaggctgtggtacttccgctcggttattgataacctgggcagctaggacgatctcgtcgaaaccgttgatgttgtgtcctacgatgtataattctatgaaacgcggcgtgcctctgacgtgaggtagcttactgagctcatcaaaggttaggtctgtggggtcagataaggcgtagtgttcgagagcccattcgtgcaggtgaggattcgctttaaggaaggaggaccagaggtccactgccagtgctgtttgtaactggtcccggtactgacgaaaatgccgtccgactgccattttttctggggtgacgcaatagaaggtttgggggtcctgccgccagcgatcccacttgagttttatggcgaggtcataggcgatgttgacgagccgctggtctccagagagtttcatgaccagcatgaaggggattagctgcttgccaaaggaccccatccaggtgtaggtttccacatcgtaggtgagaaagagcctttctgtgcgaggatgagagccaatcgggaagaactggatctcctgccaccagttggaggaatggctgttgatgtgatggaagtagaactccctgcgacgcgccgagcattcatgcttgtgcttgtacagacggccgcagtagtcgcagcgttgcacgggttgtatctcgtgaatgagttgtacctggcttcccttgacgagaaatttcagtgggaagccgaggcctggcgattgtatctcgtgctttactatgttgtctgcatcggcctgttcatcttctgtctcgatggtggtcatgctgacgagccctcgcgggaggcaagtccagacctcggcgcggcaggggcggagctcgaggacgagagcgcgcaggctggagctgtccagggtcctgagacgctgcggactcaggttagtaggcagtgtcaggagattaacttgcatgatcttttggagggcgtgcgggaggttcagatagtacttgatctcaacgggtccgttggtggagatgtcgatggcttgcagggttccgtgtcccttgggcgctaccaccgtgcccttgtttttcattttggacggcggtggctctgttgcttcttgcatgtttagaagcggtgtcgagggcgcgcaccgggcggcaggggcggctcgggacccggcggcatggctggcagtggtacgtcggcgccgcgcgcgggtaggttctggtactgcgccctgagaagactcgcatgcgcgacgacgcggcggttgacatcctggatctgacgcctctgggtgaaagctaccggccccgtgagcttgaacctgaaagagagttcaacagaatcaatctcggtatcgttgacggcggcttgcctaaggatttcttgcacgtcaccagagttgtcctggtaggcgatctccgccatgaactgctcgatctcttcctcttgaagatctccgcggcccgctctctcgacggtggccgcgaggtcgttggagatgcgcccaatgagttgagagaatgcattcatgcccgcctcgttccagacgcggctgtagaccacggcccccacgggatctctcgcgcgcatgaccacctgggcgaggttgagctccacgtggcgggtgaagaccgcatagttgcataggcgctggaaaaggtagttgagtgtggtggcgatgtgctcggtgacgaagaaatacatgatccatcgtctcagcggcatctcgctgacatcgcccagagcttccaagcgctccatggcctcgtagaagtccacggcaaaattaaaaaactgggagtttcgcgcggacacggtcaactcctcttccagaagacggataagttcggcgatggtggtgcgcacctcgcgctcgaaagcccctgggatttcttcctcaatctcttcttcttccactaacatctcttcctcttcaggtggggctgcaggaggagggggaacgcggcgacgccggcggcgcacgggcagacggtcgatgaatctttcaatgacctctccgcggcggcggcgcatggtttcagtgacggcgcggccgttctcgcgcggtcgcagagtaaaaacaccgccgcgcatctccttaaagtggtgactgggaggttctccgtttgggagggagagggcgctgattatacattttattaattggcccgtagggactgcacgcagagatctgatcgtgtcaagatccacgggatctgaaaacctttcgacgaaagcgtctaaccagtcacagtcacaaggtaggctgagtacggcttcttgtgggcgggggtggttatgtgttcggtctgggtcttctgtttcttcttcatctcgggaaggtgagacgatgctgctggtgatgaaattaaagtaggcagttctaagacggcggatggtggcgaggagcaccaggtctttgggtccggcttgctggatacgcaggcgattggccattccccaagcattatcctgacatctagcaagatctttgtagtagtcttgcatgagccgttctacgggcacttcttcctcacccgttctgccatgcatacgtgtgagtccaaatccgcgcattggttgtaccagtgccaagtcagctacgactctttcggcgaggatggcttgctgtacttgggtaagggtggcttgaaagtcatcaaaatccacaaagcggtggtaagctcctgtattaatggtgtaagcacagttggccatgactgaccagttaactgtctggtgaccagggcgcacgagctcggtgtatttaaggcgcgaataggcgcgggtgtcaaagatgtaatcgttgcaggtgcgcaccagatactggtaccctataagaaaatgcggcggtggttggcggtagagaggccatcgttctgtagctggagcgccaggggcgaggtcttccaacataaggcggtgatagccgtagatgtacctggacatccaggtgattcctgcggcggtagtagaagcccgaggaaactcgcgtacgcggttccaaatgttgcgtagcggcatgaagtagttcattgtaggcacggtttgaccagtgaggcgcgcgcagtcattgatgctctatagacacggagaaaatgaaagcgttcagcgactcgactccgtagcctggaggaacgtgaacgggttgggtcgcggtgtaccccggttcgagacttgtactcgagccggccggagccgcggctaacgtggtattggcactcccgtctcgacccagcctacaaaaatccaggatacggaatcgagtcgttttgctggtttccgaatggcagggaagtgagtcctattttttttttttgccgctcagatgcatcccgtgctgcgacagatgcgcccccaacaacagcccccctcgcagcagcagcagcagcaatcacaaaaggctgtccctgcaactactgcaactgccgccgtgagcggtgcgggacagcccgcctatgatctggacttggaagagggcgaaggactggcacgtctaggtgcgccttcacccgagcggcatccgcgagttcaactgaaaaaagattctcgcgaggcgtatgtgccccaacagaacctatttagagacagaagcggcgaggagccggaggagatgcgagcttcccgctttaacgcgggtcgtgagctgcgtcacggtttggaccgaagacgagtgttgcgggacgaggatttcgaagttgatgaaatgacagggatcagtcctgccagggcacacgtggctgcagccaaccttgtatcggcttacgagcagacagtaaaggaagagcgtaacttccaaaagtcttttaataatcatgtgcgaaccctgattgcccgcgaagaagttacccttggtttgatgcatttgtgggatttgatggaagctatcattcagaaccctactagcaaacctctgaccgcccagctgtttctggtggtgcaacacagcagagacaatgaggctttcagagaggcgctgctgaacatcaccgaacccgaggggagatggttgtatgatcttatcaacattctacagagtatcatagtgcaggagcggagcctgggcctggccgagaaggtggctgccatcaattactcggttttgagcttgggaaaatattacgctcgcaaaatctacaagactccatacgttcccatagacaaggaggtgaagatagatgggttctacatgcgcatgacgctcaaggtcttgaccctgagcgatgatcttggggtgtatcgcaatgacagaatgcatcgcgcggttagcgccagcaggaggcgcgagttaagcgacagggaactgatgcacagtttgcaaagagctctgactggagctggaaccgagggtgagaattacttcgacatgggagctgacttgcagtggcagcctagtcgcagggctctgagcgccgcgacggcaggatgtgagcttccttacatagaagaggcggatgaaggcgaggaggaagagggcgagtacttggaagactgatggcacaacccgtgttttttgctagatggaacagcaagcaccggatcccgcaatgcgggcggcgctgcagagccagccgtccggcattaactcctcggacgattggacccaggccatgcaacgtatcatggcgttgacgactcgcaaccccgaagcctttagacagcaaccccaggccaaccgtctatcggccatcatggaagctgtagtgccttcccgctctaatcccactcatgagaaggtcctggccatcgtgaacgcgttggtggagaacaaagctattcgtccagatgaggccggactggtatacaacgctctcttagaacgcgtggctcgctacaacagtagcaatgtgcaaaccaatttggaccgtatgataacagatgtacgcgaagccgtgtctcagcgcgaaaggttccagcgtgatgccaacctgggttcgctggtggcgttaaatgctttcttgagtactcagcctgctaatgtgccgcgtggtcaacaggattatactaactttttaagtgctttgagactgatggtatcagaagtacctcagagcgaagtgtatcagtccggtcctgattacttctttcagactagcagacagggcttgcagacggtaaatctgagccaagcttttaaaaaccttaaaggtttgtggggagtgcatgccccggtaggagaaagagcaaccgtgtctagcttgttaactccgaactcccgcctattattactgttggtagctcctttcaccgacagcggtagcatcgaccgtaattcctatttgggttacctactaaacctgtatcgcgaagccatagggcaaagtcaggtggacgagcagacctatcaagaaattacccaagtcagtcgcgctttgggacaggaagacactggcagtttggaagccactctgaacttcttgcttaccaatcggtctcaaaagatccctcctcaatatgctcttactgcggaggaggagaggatccttagatatgtgcagcagagcgtgggattgtttctgatgcaagagggggcaactccgactgcagcactggacatgacagcgcgaaatatggagcccagcatgtatgccagtaaccgacctttcattaacaaactgctggactacttgcacagagctgccgctatgaactctgattatttcaccaatgccatcttaaacccgcactggctgcccccacctggtttctacacgggcgaatatgacatgcccgaccctaatgacggatttctgtgggacgacgtggacagcgatgttttttcacctctttctgatcatcgcacgtggaaaaaggaaggcggcgatagaatgcattcttctgcatcgctgtccggggtcatgggtgctaccgcggctgagcccgagtctgcaagtccttttcctagtctacccttttctctacacagtgtacgtagcagcgaagtgggtagaataagtcgcccgagtttaatgggcgaagaggagtatctaaacgattccttgctcagaccggcaagagaaaaaaatttcccaaacaatggaatagaaagtttggtggataaaatgagtagatggaagacttatgctcaggatcacagagacgagcctgggatcatggggattacaagtagagcgagccgtagacgccagcgccatgacagacagaggggtcttgtgtgggacgatgaggattcggccgatgatagcagcgtgctggacttgggtgggagaggaaggggcaacccgtttgctcatttgcgccctcgcttgggtggtatgttgtaaaaaaaaataaaaaaaaaactcaccaaggccatggcgacgagcgtacgttcgttcttctttattatctgtgtctagtataatgaggcgagtcgtgctaggcggagcggtggtgtatccggagggtcctcctccttcgtacgagagcgtgatgcagcagcagcaggcgacggcggtgatgcaatccccactggaggctccctttgtgcctccgcgatacctggcacctacggagggcagaaacagcattcgttattcggaactggcacctcagtacgataccaccaggttgtatctggtggacaacaagtcggcggacattgcttctctgaactatcagaatgaccacagcaacttcttgaccacggtggtgcaaaacaatgactttacccctacggaagccagcacccagaccattaactttgatgaacgatcgcggtggggcggtcagctaaagaccatcatgcatactaacatgccaaacgtgaacgagtatatgtttagtaacaagttcaaagcgcgtgtgatggtgtccagaaaacctcccgacggtgctgcagttggggatacttatgatcacaagcaggatattttgaaatatgagtggttcgagtttactttgccagaaggcaacttttcagttactatgactattgatttgatgaacaatgccatcatagataattacttgaaagtgggtagacagaatggagtgcttgaaagtgacattggtgttaagttcgacaccaggaacttcaagctgggatgggatcccgaaaccaagttgatcatgcctggagtgtatacgtatgaagccttccatcctgacattgtcttactgcctggctgcggagtggattttaccgagagtcgtttgagcaaccttcttggtatcagaaaaaaacagccatttcaagagggttttaagattttgtatgaagatttagaaggtggtaatattccggccctcttggatgtagatgcctatgagaacagtaagaaagaacaaaaagccaaaatagaagctgctacagctgctgcagaagctaaggcaaacatagttgccagcgactctacaagggttgctaacgctggagaggtcagaggagacaattttgcgccaacacctgttccgactgcagaatcattattggccgatgtgtctgaaggaacggacgtgaaactcactattcaacctgtagaaaaagatagtaagaatagaagctataatgtgttggaagacaaaatcaacacagcctatcgcagttggtatctttcgtacaattatggcgatcccgaaaaaggagtgcgttcctggacattgctcaccacctcagatgtcacctgcggagcagagcaggtctactggtcgcttccagacatgatgaaggatcctgtcactttccgctccactagacaagtcagtaactaccctgtggtgggtgcagagcttatgcccgtcttctcaaagagcttctacaacgaacaagctgtgtactcccagcagctccgccagtccacctcgcttacgcacgtcttcaaccgctttcctgagaaccagattttaatccgtccgccggcgcccaccattaccaccgtcagtgaaaacgttcctgctctcacagatcacgggaccctgccgttgcgcagcagtatccggggagtccaacgtgtgaccgttactgacgccagacgccgcacctgtccctacgtgtacaaggcactgggcatagtcgcaccgcgcgtcctttcaagccgcactttctaaaaaaaaaaaaaatgtccattcttatctcgcccagtaataacaccggttggggtctgcgcgctccaagcaagatgtacggaggcgcacgcaaacgttctacccaacatcctgtccgtgttcgcggacattttcgcgctccatggggcgccctcaagggccgcactcgcgttcgaaccaccgtcgatgatgtaatcgatcaggtggttgccgacgcccgtaattatactcctactgcgcctacatctactgtggatgcagttattgacagtgtagtggctgacgctcgcaactatgctcgacgtaagagccggcgaaggcgcattgccagacgccaccgagctaccactgccatgcgagccgcaagagctctgctacgaagagctagacgcgtggggcgaagagccatgcttagggcggccagacgtgcagcttcgggcgccagcgccggcaggtcccgcaggcaagcagccgctgtcgcagcggcgactattgccgacatggcccaatcgcgaagaggcaatgtatactgggtgcgtgacgctgccaccggtcaacgtgtacccgtgcgcacccgtccccctcgcacttagaagatactgagcagtctccgatgttgtgtcccagcggcgaggatgtccaagcgcaaatacaaggaagaaatgctgcaggttatcgcacctgaagtctacggccaaccgttgaaggatgaaaaaaaaccccgcaaaatcaagcgggttaaaaaggacaaaaaagaagaggaagatggcgatgatgggctggcggagtttgtgcgcgagtttgccccacggcgacgcgtgcaatggcgtgggcgcaaagttcgacatgtgttgagacctggaacttcggtggtctttacacccggcgagcgttcaagcgctacttttaagcgttcctatgatgaggtgtacggggatgatgatattcttgagcaggcggctgaccgattaggcgagtttgcttatggcaagcgtagtagaataacttccaaggatgagacagtgtcgatacccttggatcatggaaatcccacccctagtcttaaaccggtcactttgcagcaagtgttacccgtaactccgcgaacaggtgttaaacgcgaaggtgaagatttgtatcccactatgcaactgatggtacccaaacgccagaagttggaggacgttttggagaaagtaaaagtggatccagatattcaacctgaggttaaagtgagacccattaagcaggtagcgcctggtctgggggtacaaactgtagacattaagattcccactgaaagtatggaagtgcaaactgaacccgcaaagcctactgccacctccactgaagtgcaaacggatccatggatgcccatgcctattacaactgacgccgccggtcccactcgaagatcccgacgaaagtacggtccagcaagtctgttgatgcccaattatgttgtacacccatctattattcctactcctggttaccgaggcactcgctactatcgcagccgaaacagtacctcccgccgtcgccgcaagacacctgcaaatcgcagtcgtcgccgtagacgcacaagcaaaccgactcccggcgccctggtgcggcaagtgtaccgcaatggtagtgcggaacctttgacactgccgcgtgcgcgttaccatccgagtatcatcacttaatcaatgttgccgctgcctccttgcagatatggccctcacttgtcgccttcgcgttcccatcactggttaccgaggaagaaactcgcgccgtagaagagggatgttgggacgcggaatgcgacgctacaggcgacggcgtgctatccgcaagcaattgcggggtggttttttaccagccttaattccaattatcgctgctgcaattggcgcgataccaggcatagcttccgtggcggttcaggcctcgcaacgacattgacattggaaaaaaacgtataaataaaaaaaaaaaaatacaatggactctgacactcctggtcctgtgactatgttttcttagagatggaagacatcaatttttcatccttggctccgcgacacggcacgaagccgtacatgggcacctggagcgacatcggcacgagccaactgaacgggggcgccttcaattggagcagtatctggagcgggcttaaaaattttggctcaaccataaaaacatacgggaacaaagcttggaacagcagtacaggacaggcgcttagaaataaacttaaagaccagaacttccaacaaaaagtagtcgatgggatagcttccggcatcaatggagtggtagatttggctaaccaggctgtgcagaaaaagataaacagtcgtttggacccgccgccagcaaccccaggtgaaatgcaagtggaggaagaaattcctccgccagaaaaacgaggcgacaagcgtccgcgtcccgatttggaagagacgctggtgacgcgcgtagatgaaccgccttcttatgaggaagcaacgaagcttggaatgcccaccactagaccgatagccccaatggccaccggggtgatgaaaccttctcagttgcatcgacccgtcaccttggatttgccccctccccctgctgctactgctgtacccgcttctaagcctgtcgctgccccgaaaccagtcgccgtagccaggtcacgtcccgggggcgctcctcgtccaaatgcgcactggcaaaatactctgaacagcatcgtgggtctaggcgtgcaaagtgtaaaacgccgtcgctgcttttaattaaatatggagtagcgcttaacttgcctatctgtgtatatgtgtcattacacgccgtcacagcagcagaggaaaaaaggaagaggtcgtgcgtcgacgctgagttactttcaagatggccaccccatcgatgctgccccaatgggcatacatgcacatcgccggacaggatgcttcggagtacctgagtccgggtctggtgcagttcgcccgcgccacagacacctacttcaatctgggaaataagtttagaaatcccaccgtagcgccgacccacgatgtgaccaccgaccgtagccagcggctcatgttgcgcttcgtgcccgttgaccgggaggacaatacatactcttacaaagtgcggtacaccctggccgtgggcgacaacagagtgctggatatggccagcacgttctttgacattaggggtgtgttggacagaggtcccagtttcaaaccctattctggtacggcttacaactccctggctcctaaaggcgctccaaatacatctcagtggattgcagaaggtgtaaaaaatacaactggtgaggaacacgtaacagaagaggaaaccaatactactacttacacttttggcaatgctcctgtaaaagctgaagctgaaattacaaaagaaggactcccagtaggtttggaagtttcagatgaagaaagtaaaccgatttatgctgataaaacatatcagccagaacctcagctgggagatgaaacttggactgaccttgatggaaaaaccgaaaagtatggaggcagggctctcaaacccgatactaagatgaaaccatgctacgggtcctttgccaaacctactaatgtgaaaggcggtcaggcaaaacaaaaaacaacggagcagccaaatcagaaagtcgaatatgatatcgacatggagttttttgatgcggcatcgcagaaaacaaacttaagtcctaaaattgtcatgtatgcagaaaatgtaaatttggaaactccagacactcatgtagtgtacaaacctggaacagaagacacaagttccgaagctaatttgggacaacaatctatgcccaacagacccaactacattggcttcagagataactttattggacttatgtactataacagtactggtaacatgggggtgctggctggtcaagcgtctcagttaaatgcagtggttgacttgcaggacagaaacacagaactttcttaccaactcttgcttgactctctgggcgacagaaccagatactttagcatgtggaatcaggctgtggacagttatgatcctgatgtacgtgttattgaaaatcatggtgtggaagatgaacttcccaactactgttttccactggacggcataggtgttccaacaaccagttacaaatcaatagttccaaatggagacaatgcgcctaattggaaggaacctgaagtaaatggaacaagtgagatcggacagggtaatttgtttgccatggaaattaaccttcaagccaatctatggcgaagtttcctttattccaatgtggctctatatctcccagactcgtacaaatacaccccgtccaatgtcactcttccagaaaacaaaaacacctacgactacatgaacgggcgggtggtgccgccatctctagtagacacctatgtgaacattggtgccaggtggtctctggatgccatggacaatgtcaacccattcaaccaccaccgtaacgctggcttgcgttaccgatccatgcttctgggtaacggacgttatgtgcctttccacatacaagtgcctcaaaaattcttcgctgttaaaaacctgctgcttctcccaggctcctacacttatgagtggaactttaggaaggatgtgaacatggttctacagagttccctcggtaacgacctgcgggtagatggcgccagcatcagtttcacgagcatcaacctctatgctacttttttccccatggctcacaacaccgcttccacccttgaagccatgctgcggaatgacaccaatgatcagtcattcaacgactacctatctgcagctaacatgctctaccccattcctgccaatgcaaccaatattcccatttccattccttctcgcaactgggcggctttcagaggctggtcatttaccagactgaaaaccaaagaaactccctctttggggtctggatttgacccctactttgtctattctggttctattccctacctggatggtaccttctacctgaaccacacttttaagaaggtttccatcatgtttgactcttcagtgagctggcctggaaatgacaggttactatctcctaacgaatttgaaataaagcgcactgtggatggcgaaggctacaacgtagcccaatgcaacatgaccaaagactggttcttggtacagatgctcgccaactacaacatcggctatcagggcttctacattccagaaggatacaaagatcgcatgtattcatttttcagaaacttccagcccatgagcaggcaggtggttgatgaggtcaattacaaagacttcaaggccgtcgccataccctaccaacacaacaactctggctttgtgggttacatggctccgaccatgcgccaaggtcaaccctatcccgctaactatccctatccactcattggaacaactgccgtaaatagtgttacgcagaaaaagttcttgtgtgacagaaccatgtggcgcataccgttctcgagcaacttcatgtctatgggggcccttacagacttgggacagaatatgctctatgccaactcagctcatgctctggacatgacctttgaggtggatcccatggatgagcccaccctgctttatcttctcttcgaagttttcgacgtggtcagagtgcatcagccacaccgcggcatcatcgaggcagtctacctgcgtacaccgttctcggccggtaacgctaccacgtaagaagcttcttgcttcttgcaaatagcagctgcaaccatggcctgcggatcccaaaacggctccagcgagcaagagctcagagccattgtccaagacctgggttgcggaccctattttttgggaacctacgataagcgcttcccggggttcatggcccccgataagctcgcctgtgccattgtaaatacggccggacgtgagacggggggagagcactggttggctttcggttggaacccacgttctaacacctgctacctttttgatccttttggattctcggatgatcgtctcaaacagatttaccagtttgaatatgagggtctcctgcgccgcagcgctcttgctaccaaggaccgctgtattacgctggaaaaatctacccagaccgtgcagggtccccgttctgccgcctgcggacttttctgctgcatgttccttcacgcctttgtgcactggcctgaccgtcccatggacggaaaccccaccatgaaattgctaactggagtgccaaacaacatgcttcattctcctaaagtccagcccaccctgtgtgacaatcaaaaagcactctaccattttcttaatacccattcgccttattttcgctcccatcgtacacacatcgaaagggccactgcgttcgaccgtatggatgttcaataatgactcatgtaaacaacgtgttcaataaacatcactttatttttttacatgtatcaaggctctgcattacttatttatttacaagtcgaatgggttctgacgagaatcagaatgacccgcaggcagtgatacgttgcggaactgatacttgggttgccacttgaattcgggaatcaccaacttgggaaccggtatatcgggcaggatgtcactccacagctttctggtcagctgcaaagctccaagcaggtcaggagccgaaatcttgaaatcacaattaggaccagtgctttgagcgcgagagttgcggtacaccggattgcagcactgaaacaccatcagcgacggatgtctcacgcttgccagcacggtgggatctgcaatcatgcccacatccagatcttcagcattggcaatgctgaacggggtcatcttgcaggtctgcctacccatggcgggcacccaattaggcttgtggttgcaatcgcagtgcagggggatcagtatcatcttggcctgatcctgtctgattcctggatacacggctctcatgaaagcatcatattgcttgaaagcctgctgggctttactaccctcggtataaaacatcccgcaggacctgctcgaaaactggttagctgcacagccggcatcattcacacagcagcgggcgtcattgttagctatttgcaccacacttctgccccagcggttttgggtgattttggttcgctcgggattctcctttaaggctcgttgtccgttctcgctggccacatccatctcgataatctgctccttctgaatcataatattgccatgcaggcacttcagcttgccctcataatcattgcagccatgaggccacaacgcacagcctgtacattcccaattatggtgggcgatctgagaaaaagaatgtatcattccctgcagaaatcttcccatcatcgtgctcagtgtcttgtgactagtgaaagttaactggatgcctcggtgctcctcgtttacgtactggtgacagatgcgcttgtattgttcgtgttgctcaggcattagtttaaaagaggttctaagttcgttatccagcctgtacttctccatcagcagacacatcacttccatgcctttctcccaagcagacaccaggggcaagctaatcggattcttaacagtgcaggcagcagctcctttagccagagggtcatctttagcgatcttctcaatgcttcttttgccatccttctcaacgatgcgcacgggcgggtagctgaaacccactgctacaagttgcgcctcttctctttcttcttcgctgtcttgactgatgtcttgcatggggatatgtttggtcttccttggcttctttttggggggtatcggaggaggaggactgtcgctccgttccggagacagggaggattgtgacgtttcgctcaccattaccaactgactgtcggtagaagaacctgaccccacacggcgacaggtgtttctcttcgggggcagaggtggaggcgattgcgaagggctgcggtccgacctggaaggcggatgactggcagaaccccttccgcgttcgggggtgtgctccctgtggcggtcgcttaactgatttccttcgcggctggccattgtgttctcctaggcagagaaacaacagacatggaaactcagccattgctgtcaacatcgccacgagtgccatcacatctcgtcctcagcgacgaggaaaaggagcagagcttaagcattccaccgcccagtcctgccaccacctctaccctagaagataaggaggtcgacgcatctcatgacatgcagaataaaaaagcgaaagagtctgagacagacatcgagcaagacccgggctatgtgacaccggtggaacacgaggaagagttgaaacgctttctagagagagaggatgaaaactgcccaaaacaacgagcagataactatcaccaagatgctggaaatagggatcagaacaccgactacctcatagggcttgacggggaagacgcgctccttaaacatctagcaagacagtcgctcatagtcaaggatgcattattggacagaactgaagtgcccatcagtgtggaagagctcagccgcgcctacgagcttaacctcttttcacctcgtactccccccaaacgtcagccaaacggcacctgcgagccaaatcctcgcttaaacttttatccagcttttgctgtgccagaagtactggctacctatcacatcttttttaaaaatcaaaaaattccagtctcctgccgcgctaatcgcacccgcgccgatgccctactcaatctgggacctggttcacgcttacctgatatagcttccttggaagaggttccaaagatcttcgagggtctgggcaataatgagactcgggccgcaaatgctctgcaaaagggagaaaatggcatggatgagcatcacagcgttctggtggaattggaaggcgataatgccagactcgcagtactcaagcgaagcatcgaggtcacacacttcgcatatcccgctgtcaacctgccccctaaagtcatgacggcggtcatggaccagttactcattaagcgcgcaagtcccctttcagaagacatgcatgacccagatgcctgtgatgagggtaaaccagtggtcagtgatgagcagctaacccgatggctgggcaccgactctcccagggatttggaagagcgtcgcaagcttatgatggccgtggtgctggttaccgtagaactagagtgtctccgacgtttctttaccgattcagaaaccttgcgcaaactcgaagagaatctgcactacacttttagacacggctttgtgcggcaggcatgcaagatatctaacgtggaactcaccaacctggtttcctacatgggtattctgcatgagaatcgcctaggacaaagcgtgctgcacagcaccctgaagggggaagcccgccgtgattacatccgcgattgtgtctatctgtacctgtgccacacgtggcaaaccggcatgggtgtatggcagcaatgtttagaagaacagaacttgaaagagcttgacaagctcttacagaaatctcttaaggttctgtggacagggttcgacgagcgcaccgtcgcttccgacctggcagacctcatcttcccagagcgtctcagggttactttgcgaaacggattgcctgactttatgagccagagcatgcttaacaattttcgctctttcatcctggaacgctccggtatcctgcccgccacctgctgcgcactgccctccgactttgtgcctctcacctaccgcgagtgccccccgccgctatggagtcactgctacctgttccgtctggccaactatctctcctaccactcggatgtgatcgaggatgtgagcggagacggcttgctggagtgtcactgccgctgcaatctgtgcacgccccaccggtccctagcttgcaacccccagttgatgagcgaaacccagataataggcacctttgaattgcaaggccccagcagccaaggcgatgggtcttctcctgggcaaagtttaaaactgaccccgggactgtggacctccgcctacttgcgcaagtttgctccggaagattaccacccctatgaaatcaagttctatgaggaccaatcacagcctccaaaggccgaactttcggcctgcgtcatcacccagggggcaattctggcccaattgcaagccatccaaaaatcccgccaagaatttctactgaaaaagggtaagggggtctaccttgacccccagaccggcgaggaactcaacacaaggttccctcaggatgtcccaacgacgagaaaacaagaagttgaaggtgcagccgccgcccccagaagatatggaggaagattgggacagtcaggcagaggaggcggaggaggacagtctggaggacagtctggaggaagacagtttggaggaggaaaacgaggaggcagaggaggtggaagaagtaaccgccgacaaacagttatcctcggctgcggagacaagcaacagcgctaccatctccgctccgagtcgaggaacccggcggcgtcccagcagtagatgggacgagaccggacgcttcccgaacccaaccagcgcttccaagaccggtaagaaggatcggcagggatacaagtcctggcgggggcataagaatgccatcatctcctgcttgcatgagtgcgggggcaacatatccttcacgcggcgctacttgctattccaccatggggtgaactttccgcgcaatgttttgcattactaccgtcacctccacagcccctactatagccagcaaatcccggcagtctcgacagataaagacagcggcggcgacctccaacagaaaaccagcagcggcagttagaaaatacacaacaagtgcagcaacaggaggattaaagattacagccaacgagccagcgcaaacccgagagttaagaaatcggatctttccaaccctgtatgccatcttccagcagagtcggggtcaagagcaggaactgaaaataaaaaaccgatctctgcgttcgctcaccagaagttgtttgtatcacaagagcgaagatcaacttcagcgcactctcgaggacgccgaggctctcttcaacaagtactgcgcgctgactcttaaagagtaggcagcgaccgcgcttattcaaaaaaggcgggaattacatcatcctcgacatgagtaaagaaattcccacgccttacatgtggagttatcaaccccaaatgggattggcggcaggcgcctcccaggactactccacccgcatgaattggctcagcgccgggccttctatgatttctcgagttaatgatatacgcgcctaccgaaaccaaatacttttggaacagtcagctcttaccaccacgccccgccaacaccttaatcccagaaattggcccgccgccctagtgtaccaggaaagtcccgctcccaccactgtattacttcctcgagacgcccaggccgaagtccaaatgactaatgcaggtgcgcagttagctggcggctccaccctatgtcgtcacaggcctcggcataatataaaacgcctgatgatcagaggccgaggtatccagctcaacgacgagtcggtgagctctccgcttggtctacgaccagacggaatctttcagattgccggctgcgggagatcttccttcacccctcgtcaggctgttctgactttggaaagttcgtcttcgcaaccccgctcgggcggaatcgggaccgttcaatttgtggaggagtttactccctctgtctacttcaaccccttctccggatctcctgggcattacccggacgagttcataccgaacttcgacgcgattagcgagtcagtggacggctacgattgatgtctggtgacgcggctgagctatctcggctgcgacatctagaccactgccgccgctttcgctgctttgcccgggaactcattgagttcatctacttcgaactccccaaggatcaccctcaaggtccggcccacggagtgcggatttctatcgaaggcaaaatagactctcgcctgcaacgaattttctcccagcggcccgtgctgatcgagcgagaccagggaaacaccacggtttccatctactgcatttgtaatcaccccggattgcatgaaagcctttgctgtcttatgtgtactgagtttaataaaaactgaattaagactctcctacggactgccgcttcttcaacccggattttacaaccagaagaacgaaacttttcctgtcgtccaggactctgttaacttcacctttcctactcacaaactagaagctcaacgactacaccgcttttccagaagcattttccctactaatactactttcaaaaccggaggtgagctccaaggtcttcctacagaaaacccttgggtggaagcgggccttgtagtgctaggaattcttgcgggtgggcttgtgattattctttgctacctatacacaccttgcttcactttcttagtggtgttgtggtattggtttaaaaaatggggcccatactagtcttgcttgttttactttcgcttttggaaccgggttctgccaattacgatccatgtctagacttcgacccagaaaactgcacacttacttttgcacccgacacaagccgcatctgtggagttcatcgcctctcttacgaacttggcccccaacgacaaaaatttacctgcatggtgggaatcaaccccatagttatcacccagcaaagtggagatactaagggttgcattcactgctcctgcgattccatcgagtgcacctacaccctgctgaagaccctatgcggcctaagagacctgctaccaatgaattaaaaaatgattaataaaaaatcacttacttgaaatcagcaataaggtctctgttgaaattttctcccagcagcacctcacttccctcttcccaactctggtattctaaaccccgttcagcggcatactttctccatactttaaaggggatgtcaaattttagctcctctcctgtacccacaatcttcatgtctttcttcccagtggccggccatgaccaagagagtccggctcagtgactccttcaaccctgtctacccctatgaagatgaaagcacctcccaacacccctttataaacccagggtttatttccccaaatggcttcacacaaagcccaaacggagttcttactttaaaatgtttaaccccactaacaaccacaggcggatctctacagctaaaagtgggagggggacttacagtggatgacaccaacggttttttgaaagaaaacataagtgccaccacaccactcgttaagactggtcactctataggtttaccactaggagccggattgggaacgaatgaaaataaactttgtatcaaattaggacaaggacttacattcaattcaaacaacatttgcattgatgacaatattaacaccttatggacaggagtcaaccccaccgaagccaactgtcaaatcatgaactccagtgaatctaatgattgcaaattaattctaacactagttaaaactggagcactagtcactgcatttgtttatgttataggagtatctaacaattttaatatgctaactacacacagaaatataaattttactgcagagctgtttttcgattctactggtaatttactaactagactctcatccctcaaaactccacttaatcataaatcaggacaaaacatggctactggtgccattactaatgctaaaggtttcatgcccagcacgactgcctatcctttcaatgataattctagagaaaaagaaaactacatttacggaacttgttactacacagctagtgatcgcactgcttttcccattgacatatctgtcatgcttaaccgaagagcaataaatgacgagacatcatattgtattcgtataacttggtcctggaacacaggagatgccccagaggtgcaaacctctgctacaaccctagtcacctccccatttaccttttactacatcagagaagacgactgacaaataaaatcgctatccatcgaagatggatgtgtgttggttttttgtgtgatttgtgcgatcgctatgcggccgcttacctgcaggggttaccacacaaaaaaccaacacaccctaaagctcgatctccgacttgtttatttgaaaatcaattcacaaaatccgagtagttattttgcctcccccttcccatttaacagaatacaccaatctctccccacgcacagctttaaacatttggataccattagatatagacatggttttagattccacattccaaacagtttcagagcgagccaatctggggtcagtgatagataaaaatccatcgggatagtcttttaaagcgctttcacagtccaactgctgcggatgcgactccggagtctggatcacggtcatctggaagaagaacgatgggaatcataatccgaaaacggtatcggacgattgtgtctcatcaaacccacaagcagccgctgtctgcgtcgctccgtgcgactgctgtttatgggatcagggtccacagtgtcctgaagcatgattttaatagcccttaacatcaactttctggtgcgatgcgcgcagcaacgcattctgatttcactcaaatctttgcagtaggtacaacacattattacaatattgtttaataaaccataattaaaagcgctccagccaaaactcatatctgatataatcgcccctgcatgaccatcataccaaagtttaatataaattaaatgacgttccctcaaaaacacactacccacatacatgatctcttttggcatgtgcatattaacaatctgtctgtaccatggacaacgttggttaatcatgcaacccaatataaccttccggaaccacactgccaacaccgctcccccagccatgcattgaagtgaaccctgctgattacaatgacaatgaagaacccaattctctcgaccgtgaatcacttgagaatgaaaaatatctatagtggcacaacatagacataaatgcatgcatcttctcataatttttaactcctcaggatttagaaacatatcccagggaataggaagctcttgcagaacagtaaagctggcagaacaaggaagaccacgaacacaacttacactatgcatagtcatagtatcacaatctggcaacagcgggtggtcttcagtcatagaagctcgggtttcattttcctcacaacgtggtaactgggctctggtgtaagggtgatgtctggcgcatgatgtcgagcgtgcgcgcaaccttgtcataatggagttgcttcctgacattctcgtattttgtatagcaaaacgcggccctggcagaacacactcttcttcgccttctatcctgccgcttagcgtgttccgtgtgatagttcaagtacaaccacactcttaagttggtcaaaagaatgctggcttcagttgtaatcaaaactccatcgcatctaatcgttctgaggaaatcatccaagcaatgcaactggattgtgtttcaagcaggagaggagagggaagagacggaagaaccatgttaatttttattccaaacgatctcgcagtacttcaaattgtagatcgcgcagatggcatctctcgcccccactgtgttggtgaaaaagcacagctagatcaaaagaaatgcgattttcaaggtgctcaacggtggcttccagcaaagcctccacgcgcacatccaagaacaaaagaataccaaaagaaggagcattttctaactcctcaatcatcatattacattcctgcaccattcccagataattttcagctttccagccttgaattattcgtgtcagttcttgtggtaaatccaatccacacattacaaacaggtcccggagggcgccctccaccaccattcttaaacacaccctcataatgacaaaatatcttgctcctgtgtcacctgtagcgaattgagaatggcaacatcaattgacatgcccttggctctaagttcttctttaagttctagttgtaaaaactctctcatattatcaccaaactgcttagccagaagccccccgggaacaagagcaggggacgctacagtgcagtacaagcgcagacctccccaattggctccagcaaaaacaagattggaataagcatattgggaaccgccagtaatatcatcgaagttgctggaaatataatcaggcagagtttcttgtaaaaattgaataaaagaaaaatttgccaaaaaaacattcaaaacctctgggatgcaaatgcaataggttaccgcgctgcgctccaacattgttagttttgaattagtctgcaaaaataaaaaaaaaaacaagcgtcatatcatagtagcctgacgaacagatggataaatcagtctttccatcacaagacaagccacagggtctccagctcgaccctcgtaaaacctgtcatcatgattaaacaacagcaccgaaagttcctcgcggtgaccagcatgaataattcttgatgaagcatacaatccagacatgttagcatcagttaacgagaaaaaacagccaacatagcctttgggtataattatgcttaatcgtaagtatagcaaagccacccctcgcggatacaaagtaaaaggcacaggagaataaaaaatataattatttctctgctgctgttcaggcaacgtcgcccccggtccctctaaatacacatacaaagcctcatcagccatggcttaccagacaaagtacagcgggcacacaaagcacaagctctaaagtgactctccaacctctccacaatatatatatacacaagccctaaactgacgtaatgggagtaaagtgtaaaaaatcccgccaaacccaacacacaccccgaaactgcgtcaccagggaaaagtacagtttcacttccgcaatcccaacaggcgtaacttcctctttctcacggtacgtgatatcccactaacttgcaacgtcattttcccacggtcgcaccgccccttttagccgttaaccccacagccaatcaccacacgatccacactttttaaaatcacctcatttacatattggcaccattccatctataaggtatattatatagataggcgcgccctctcttaaggtagcatcgggatcgagtccctgagagaacatcctcaatcccgatctatccttagatccgaggaatatcgaaatcagttacgctagggataacagggtaatatagcatcccctcggattgctatctaccggctcgtcagctatgatctctcgatttcgatcaagaaatctcattggttaccttgggctatcgaaaccagtcaagtcagctacttggcgagatcgacttgtctgagtttcgactacgctcagaattgcgtcagcgcctatcgccaggtattactccaatcccgaatatccgagcctgagagaacatcctcaatcccgatctatccttagatccgaggaatatcgaaatcgtttaaatcttttcttgatggtaaatcattcgaatataagaatggagagacgaatggggaaacgacaaagatgacattctttggtccttctggtgaggttctcaagtttttggttaatcctgtcaacaacttatatcgtatggggctgacttcaggtgctacatttgaagagataaattgcactgaaatctagtaatattttatctgattaataagatgatcttcttgagatcgttttggtctgcgcgtaatctcttgctctgaaaacgaaaaaaccgccttgcagggcggtttttcgaaggttctctgagctaccaactctttgaaccgaggtaactggcttggcagagcgcagtcaccaaaacttgtcctttcagtttagccttaaccggcgcatgacttcaagactaactctgctaaatcaattaccagtggctgctgccagtggtgcttttgcatgtctttccgggttggactcaagacgatagttaccggataaggcgcagcggtcggactgaacggggggttcgtgcatacagtccagcttggagcgaactgcctacccggaactgagtgtcaggcgtggaatgagacaaacgcggccataacagcggaatgacaccggtaaaccgaaaggcaggaacaggagagcgcacgagggagccgccagggggaaacgcctggtatctttatagtcctgtcgggtttcgccaccactgatttgagcgtcagatttcgtgatgcttgtcaggggggcggagcctatggaaaaacggctttgccgcggccctctcacttccctgttaagtatcttcctggcatcttccaggaaatctccgccccgttcgtaagccatttccgctcgccgcagtcgaacgaccgagcgtagcgagtcagtgagcgaggaagcggaatatatcctgtatcacatattctgctgacgcaccggtgcggccttttttctcctgccacatgaagcacttcactgacaccctcatcagtgccaacatagtaagccagtatacactccgctaatttaaacgtggtgtaccgagaacgatcctctcagtgcgatctcgacgatcagtggtattccgacatatcgttgcttggcagtcagccagtcgatcctagcttgggacccaggaagtccaatcgtcagatattgtactcagcctggtcacggcagcgtaccgatctcgtaactataacggtcctaaggtagcgaactagatattgatagtctgatcggtcaacgtataatcgagtcctagcttttgcaaacatctatcaagagacaggatcagcaggaggctttcgcatgattgaacaagatggattgcacgcaggttctccggcggcttgggtggagaggctattcggctatgactgggcacaacagacaatcggctgctctgatgccgccgtgttccggctgtcagcgcaggggcgtccggttctttttgtcaagaccgacctgtccggtgccctgaatgaactgcaagacgaggcagcgcggctatcgtggctggcgacgacgggcgttccttgcgcggctgtgctcgacgttgtcactgaagcgggaagggactggctgctattgggcgaagtgccggggcaggatctcctgtcatctcaccttgctcctgccgagaaagtatccatcatggctgatgcaatgcggcggctgcatacgcttgatccggctacctgcccattcgaccaccaagcgaaacatcgcatcgagcgagcacgtactcggatggaagccggtcttgtcgatcaggatgatctggacgaagagcatcaggggctcgcgccagccgaactgttcgccaggctcaaggcgtctatgcccgacggcgaggatctcgtcgtgacccacggcgatgcctgcttgccgaatatcatggtggaaaatggccgcttttctggattcatcgactgtggccgtctgggtgtggcggaccgctatcaggacatagcgttggctacccgtgatattgctgaagagcttggcggcgaatgggctgaccgcttccttgtgctttacggtatcgccgcgcccgattcgcagcgcatcgccttctatcgccttcttgacgagttcttctgaccgattctaggtgcattggcgcagaaaaaaatgcctgatgcgacgctgcgcgtcttatactcccacatatgccagattcagcaacggatacggcttccccaacttgcccacttccatacgtgtcctccttaccagaaatttatccttaaggtccgtaactataacggtcctaaggtagcgaatcgacctagctctatcgaatctccctcgtttcgagcttacgcgaactagcctctggcgatagcatccgaggggcaggcatctatgtcgggtgcggagaaagaggtaatgtcaagttcgatctgattgcttggcataaagtccgatggttcgagtagactcagttcaacctctctcttaaggtagc

SEQ ID NO: 31 - DNA, 35198 bp, Artificial Sequence
  ColoAd2.1 plasmid
ggcgcgcctatctatataatataccttatagatggaatggtgccaatatgtaaatgaggtgattttaaaaagtgtggatcgtgtggtgattggctgtggggttaacggctaaaaggggcggtgcgaccgtgggaaaatgacgttttgtgggggtggagtttttttgcaagttgtcgcgggaaatgtgacgcataaaaaggcttttttctcacggaactacttagttttcccacggtatttaacaggaaatgaggtagttttgaccggatgcaagtgaaaattgttgattttcgcgcgaaaactgaatgaggaagtgtttttctgaataatgtggtatttatggcagggtggagtatttgttcagggccaggtagactttgacccattacgtggaggtttcgattaccgtgttttttacctgaatttccgcgtaccgtgtcaaagtcttctgtttttacgtaggtgtcagctgatcgctagggtatttatacctcagggtttgtgtcaagaggccactcttgagtgccagcgagaagagttttctcctctgcgccggcagtttaataataaaaaaatgagagatttgcgatttctgcctcaggaaataatctctgctgagactggaaatgaaatattggagcttgtggtgcacgccctgatgggagacgatccggagccacctgtgcagctttttgagcctcctacgcttcaggaactgtatgatttagaggtagagggatcggaggattctaatgaggaagctgtaaatggcttttttaccgattctatgcttttagctgctaatgaagggttagaattagatccgcctttggacacttttgatactccaggggtaattgtggaaagcggtacaggtgtaagaaaattacctgatttgagttccgtggactgtgatttgcactgctatgaagacgggtttcctccgagtgatgaggaggaccatgaaaaggagcagtccatgcagactgcagcgggtgagggagtgaaggctgccaatgttggttttcagttggattgcccggagcttcctggacatggctgtaagtcttgtgaatttcacaggaaaaatactggagtaaaggaactgttatgttcgctttgttatatgagaacgcactgccactttatttacagtaagtgtgtttaagttaaaatttaaaggaatatgctgtttttcacatgtatattgagtgtgagttttgtgcttcttattataggtcctgtgtctgatgctgatgaatcaccatctcctgattctactacctcacctcctgagattcaagcacctgttcctgtggacgtgcgcaagcccattcctgtgaagcttaagcctgggaaacgtccagcagtggaaaaacttgaggacttgttacagggtggggacggacctttggacttgagtacacggaaacgtccaagacaataagtgttccatatccgtgtttacttaaggtgacgtcaatatttgtgtgacagtgcaatgtaataaaaatatgttaactgttcactggtttttattgctttttgggcggggactcaggtatataagtagaagcagacctgtgtggttagctcataggagctggctttcatccatggaggtttgggccattttggaagaccttaggaagactaggcaactgttagagaacgcttcggacggagtctccggtttttggagattctggttcgctagtgaattagctagggtagtttttaggataaaacaggactataaacaagaatttgaaaagttgttggtagattgcccaggactttttgaagctcttaatttgggccatcaggttcactttaaagaaaaagttttatcagttttagacttttcaaccccaggtagaactgctgctgctgtggcttttcttacttttatattagataaatggatcccgcagactcatttcagcaggggatacgttttggatttcatagccacagcattgtggagaacatggaaggttcgcaagatgaggacaatcttaggttactggccagtgcagcctttgggtgtagcgggaatcctgaggcatccaccggtcatgccagcggttctggaggaggaacagcaagaggacaacccgagagccggcctggaccctccagtggaggaggcggagtagctgacttgtctcctgaactgcaacgggtgcttactggatctacgtccactggacgggataggggcgttaagagggagagggcatctagtggtactgatgctagatctgagttggctttaagtttaatgagtcgcagacgtcctgaaaccatttggtggcatgaggttcagaaagagggaagggatgaagtttctgtattgcaggagaaatattcactggaacaggtgaaaacatgttggttggagcctgaggatgattgggaggtggccattaaaaattatgccaagatagctttgaggcctgataaacagtataagattactagacggattaatatccggaatgcttgttacatatctggaaatggggctgaggtggtaatagatactcaagacaaggcagttattagatgctgcatgatggatatgtggcctggggtagtcggtatggaagcagtaacttttgtaaatgttaagtttaggggagatggttataatggaatagtgtttatggccaataccaaacttatattgcatggttgtagcttttttggtttcaacaatacctgtgtagatgcctggggacaggttagtgtacggggatgtagtttctatgcgtgttggattgccacagctggcagaaccaagagtcaattgtctctgaagaaatgcatatttcaaagatgtaacctgggcattctgaatgaaggcgaagcaagggtccgccactgcgcttctacagatactggatgttttattttgattaagggaaatgccagcgtaaagcataacatgatttgcggtgcttccgatgagaggccttatcaaatgctcacttgtgctggtgggcattgtaatatgctggctactgtgcatattgtttcccatcaacgcaaaaaatggcctgtttttgatcacaatgtgatgacgaagtgtaccatgcatgcaggtgggcgtagaggaatgtttatgccttaccagtgtaacatgaatcatgtgaaagtgttgttggaaccagatgccttttccagaatgagcctaacaggaatttttgacatgaacatgcaaatctggaagatcctgaggtatgatgatacgagatcgagggtacgcgcatgcgaatgcggaggcaagcatgccaggttccagccggtgtgtgtagatgtgactgaagatctcagaccggatcatttggttattgcccgcactggagcagagttcggatccagtggagaagaaactgactaaggtgagtattgggaaaactttggggtgggattttcagatggacagattgagtaaaaatttgttttttctgtcttgcagctgtcatgagtggaaacgcttcttttaaggggggagtcttcagcccttatctgacagggcgtctcccatcctgggcaggagttcgtcagaatgttatgggatctactgtggatggaagacccgtccaacccgccaattcttcaacgctgacctatgctactttaagttcttcacctttggacgcagctgcagctgccgccgccgcttctgttgccgctaacactgtgcttggaatgggttactatggaagcatcatggctaattccacttcctctaataacccttctaccctgactcaggacaagttacttgtccttttggcccagctggaggctttgacccaacgtctgggtgaactttctcagcaggtggtcgagttgcgagtacaaactgagtctgctgtcggcacggcaaagtctaaataaaaaaatcccagaatcaatgaataaataaacaagcttgttgttgatttaaaatcaagtgtttttatttcatttttcgcgcacggtatgccctagaccaccgatctctatcattgagaactcggtggattttttccaggatcctatagaggtgggattgaatgtttagatacatgggcattaggccgtctttggggtggagatagctccattgaagggattcatgctccggggtagtgttgtaaatcacccagtcataacaaggtcgcagtgcatggtgttgcacaatatcttttagaagtaggctgattgccacagataagcccttggtgtaggtgtttacaaaccggttgagctgggatgggtgcattcggggtgaaattatgtgcattttggattggatttttaagttggcaatattgccgccaagatcccgtcttgggttcatgttatgaaggaccaccaagacggtgtatccggtacatttaggaaatttatcgtgcagcttggatggaaaagcgtggaaaaatttggagacacccttgtgtcctccaagattttccatgcactcatccatgataatagcaatggggccgtgggcagcggcgcgggcaaacacgttccgtgggtctgacacatcatagttatgttcctgagttaaatcatcataagccattttaatgaatttggggcggagagtaccagattggggtatgaatgttccttcgggccccggagcatagttcccctcacagatttgcatttcccaagctttcagttccgagggtggaatcatgtccacctggggggctatgaaaaacaccgtttctggggcgggggtgattaattgtgatgatagcaaatttctgagcaattgagatttgccacatccggtggggccataaatgattccgattacgggttgcaggtggtagtttagggaacggcaactgccgtcttctcgaagcaagggggccacctcgttcatcatttcccttacatgcatattttcccgcaccaaatccattaggaggcgctctcctcctagtgatagaagttcttgtagtgaggaaaagtttttcagcggtttcagaccgtcagccatgggcattttggagagagtttgctgcaaaagttctagtctgttccacagttcagtgatgtgttctatggcatctcgatccagcagacctcctcgtttcgcgggtttggacggctcctggaatagggtatgagacgatgggcgtccagcgctgccagggttcggtccttccagggtctcagtgttcgagtcagggttgtttccgtcacagtgaaggggtgtgcgcctgcttgggcgcttgccagggtgcgcttcagactcatcctgctggtcgaaaacttctgtcgcttggcgccctgtatgtcggccaagtagcagtttaccatgagttcgtagttgagcgcctcggctgcgtggcctttggcgcggagcttacctttggaagttttcttgcataccgggcagtataggcatttcagcgcatacaacttgggcgcaaggaaaacggattctggggagtatgcatctgcgccgcaggaggcgcaaacagtttcacattccaccagccaggttaaatccggttcattggggtcaaaaacaagttttccgccatattttttgatgcgtttcttacctttggtctccatgagttcgtgtcctcgttgagtgacaaacaggctgtccgtgtccccgtagactgattttacaggcctcttctccagtggagtgcctcggtcttcttcgtacaggaactctgaccactctgatacaaaggcgcgcgtccaggccagcacaaaggaggctatgtgggaggggtagcgatcgttgtcaaccagggggtccaccttttccaaagtatgcaaacacatgtcaccctcttcaacatccaggaatgtgattggcttgtaggtgtatttcacgtgacctggggtccccgctgggggggtataaaagggggcggttctttgctcttcctcactgtcttccggatcgctgtccaggaacgtcagctgttggggtaggtattccctctcgaaggcgggcatgacctctgcactcaggttgtcagtttctaagaacgaggaggatttgatattgacagtgccggttgagatgcctttcatgaggttttcgtccatctggtcagaaaacacaatttttttattgtcaagtttggtggcaaatgatccatacagggcgttggataaaagtttggcaatggatcgcatggtttggttcttttccttgtccgcgcgctctttggcggcgatgttgagttggacatactcgcgtgccaggcacttccattcggggaagatagttgttaattcatctggcacgattctcacttgccaccctcgattatgcaaggtaattaaatccacactggtggccacctcgcctcgaaggggttcattggtccaacagagcctacctcctttcctagaacagaaagggggaagtgggtctagcataagttcatcgggagggtctgcatccatggtaaagattcccggaagtaaatccttatcaaaatagctgatgggagtggggtcatctaaggccatttgccattctcgagctgccagtgcgcgctcatatgggttaaggggactgccccatggcatgggatgggtgagtgcagaggcatacatgccacagatgtcatagacgtagatgggatcctcaaagatgcctatgtaggttggatagcatcgcccccctctgatacttgctcgcacatagtcatatagttcatgtgatggcgctagcagccccggacccaagttggtgcgattgggtttttctgttctgtagacgatctggcgaaagatggcgtgagaattggaagagatggtgggtctttgaaaaatgttgaaatgggcatgaggtagacctacagagtctctgacaaagtgggcataagattcttgaagcttggttaccagttcggcggtgacaagtacgtctagggcgcagtagtcaagtgtttcttgaatgatgtcataacctggttggtttttcttttcccacagttcgcggttgagaaggtattcttcgcgatccttccagtactcttctagcggaaacccgtctttgtctgcacggtaagatcctagcatgtagaactgattaactgccttgtaagggcagcagcccttctctacgggtagagagtatgcttgagcagcttttcgtagcgaagcgtgagtaagggcaaaggtgtctctgaccatgactttgaggaattggtatttgaagtcgatgtcgtcacaggctccctgttcccagagttggaagtctacccgtttcttgtaggcggggttgggcaaagcgaaagtaacatcattgaagagaatcttgccggccctgggcatgaaattgcgagtgatgcgaaaaggctgtggtacttccgctcggttattgataacctgggcagctaggacgatctcgtcgaaaccgttgatgttgtgtcctacgatgtataattctatgaaacgcggcgtgcctctgacgtgaggtagcttactgagctcatcaaaggttaggtctgtggggtcagataaggcgtagtgttcgagagcccattcgtgcaggtgaggattcgctttaaggaaggaggaccagaggtccactgccagtgctgtttgtaactggtcccggtactgacgaaaatgccgtccgactgccattttttctggggtgacgcaatagaaggtttgggggtcctgccgccagcgatcccacttgagttttatggcgaggtcataggcgatgttgacgagccgctggtctccagagagtttcatgaccagcatgaaggggattagctgcttgccaaaggaccccatccaggtgtaggtttccacatcgtaggtgagaaagagcctttctgtgcgaggatgagagccaatcgggaagaactggatctcctgccaccagttggaggaatggctgttgatgtgatggaagtagaactccctgcgacgcgccgagcattcatgcttgtgcttgtacagacggccgcagtagtcgcagcgttgcacgggttgtatctcgtgaatgagttgtacctggcttcccttgacgagaaatttcagtgggaagccgaggcctggcgattgtatctcgtgctttactatgttgtctgcatcggcctgttcatcttctgtctcgatggtggtcatgctgacgagccctcgcgggaggcaagtccagacctcggcgcggcaggggcggagctcgaggacgagagcgcgcaggctggagctgtccagggtcctgagacgctgcggactcaggttagtaggcagtgtcaggagattaacttgcatgatcttttggagggcgtgcgggaggttcagatagtacttgatctcaacgggtccgttggtggagatgtcgatggcttgcagggttccgtgtcccttgggcgctaccaccgtgcccttgtttttcattttggacggcggtggctctgttgcttcttgcatgtttagaagcggtgtcgagggcgcgcaccgggcggcaggggcggctcgggacccggcggcatggctggcagtggtacgtcggcgccgcgcgcgggtaggttctggtactgcgccctgagaagactcgcatgcgcgacgacgcggcggttgacatcctggatctgacgcctctgggtgaaagctaccggccccgtgagcttgaacctgaaagagagttcaacagaatcaatctcggtatcgttgacggcggcttgcctaaggatttcttgcacgtcaccagagttgtcctggtaggcgatctccgccatgaactgctcgatctcttcctcttgaagatctccgcggcccgctctctcgacggtggccgcgaggtcgttggagatgcgcccaatgagttgagagaatgcattcatgcccgcctcgttccagacgcggctgtagaccacggcccccacgggatctctcgcgcgcatgaccacctgggcgaggttgagctccacgtggcgggtgaagaccgcatagttgcataggcgctggaaaaggtagttgagtgtggtggcgatgtgctcggtgacgaagaaatacatgatccatcgtctcagcggcatctcgctgacatcgcccagagcttccaagcgctccatggcctcgtagaagtccacggcaaaattaaaaaactgggagtttcgcgcggacacggtcaactcctcttccagaagacggataagttcggcgatggtggtgcgcacctcgcgctcgaaagcccctgggatttcttcctcaatctcttcttcttccactaacatctcttcctcttcaggtggggctgcaggaggagggggaacgcggcgacgccggcggcgcacgggcagacggtcgatgaatctttcaatgacctctccgcggcggcggcgcatggtttcagtgacggcgcggccgttctcgcgcggtcgcagagtaaaaacaccgccgcgcatctccttaaagtggtgactgggaggttctccgtttgggagggagagggcgctgattatacattttattaattggcccgtagggactgcacgcagagatctgatcgtgtcaagatccacgggatctgaaaacctttcgacgaaagcgtctaaccagtcacagtcacaaggtaggctgagtacggcttcttgtgggcgggggtggttatgtgttcggtctgggtcttctgtttcttcttcatctcgggaaggtgagacgatgctgctggtgatgaaattaaagtaggcagttctaagacggcggatggtggcgaggagcaccaggtctttgggtccggcttgctggatacgcaggcgattggccattccccaagcattatcctgacatctagcaagatctttgtagtagtcttgcatgagccgttctacgggcacttcttcctcacccgttctgccatgcatacgtgtgagtccaaatccgcgcattggttgtaccagtgccaagtcagctacgactctttcggcgaggatggcttgctgtacttgggtaagggtggcttgaaagtcatcaaaatccacaaagcggtggtaagctcctgtattaatggtgtaagcacagttggccatgactgaccagttaactgtctggtgaccagggcgcacgagctcggtgtatttaaggcgcgaataggcgcgggtgtcaaagatgtaatcgttgcaggtgcgcaccagatactggtaccctataagaaaatgcggcggtggttggcggtagagaggccatcgttctgtagctggagcgccaggggcgaggtcttccaacataaggcggtgatagccgtagatgtacctggacatccaggtgattcctgcggcggtagtagaagcccgaggaaactcgcgtacgcggttccaaatgttgcgtagcggcatgaagtagttcattgtaggcacggtttgaccagtgaggcgcgcgcagtcattgatgctctatagacacggagaaaatgaaagcgttcagcgactcgactccgtagcctggaggaacgtgaacgggttgggtcgcggtgtaccccggttcgagacttgtactcgagccggccggagccgcggctaacgtggtattggcactcccgtctcgacccagcctacaaaaatccaggatacggaatcgagtcgttttgctggtttccgaatggcagggaagtgagtcctattttttttttttgccgctcagatgcatcccgtgctgcgacagatgcgcccccaacaacagcccccctcgcagcagcagcagcagcaatcacaaaaggctgtccctgcaactactgcaactgccgccgtgagcggtgcgggacagcccgcctatgatctggacttggaagagggcgaaggactggcacgtctaggtgcgccttcacccgagcggcatccgcgagttcaactgaaaaaagattctcgcgaggcgtatgtgccccaacagaacctatttagagacagaagcggcgaggagccggaggagatgcgagcttcccgctttaacgcgggtcgtgagctgcgtcacggtttggaccgaagacgagtgttgcgggacgaggatttcgaagttgatgaaatgacagggatcagtcctgccagggcacacgtggctgcagccaaccttgtatcggcttacgagcagacagtaaaggaagagcgtaacttccaaaagtcttttaataatcatgtgcgaaccctgattgcccgcgaagaagttacccttggtttgatgcatttgtgggatttgatggaagctatcattcagaaccctactagcaaacctctgaccgcccagctgtttctggtggtgcaacacagcagagacaatgaggctttcagagaggcgctgctgaacatcaccgaacccgaggggagatggttgtatgatcttatcaacattctacagagtatcatagtgcaggagcggagcctgggcctggccgagaaggtggctgccatcaattactcggttttgagcttgggaaaatattacgctcgcaaaatctacaagactccatacgttcccatagacaaggaggtgaagatagatgggttctacatgcgcatgacgctcaaggtcttgaccctgagcgatgatcttggggtgtatcgcaatgacagaatgcatcgcgcggttagcgccagcaggaggcgcgagttaagcgacagggaactgatgcacagtttgcaaagagctctgactggagctggaaccgagggtgagaattacttcgacatgggagctgacttgcagtggcagcctagtcgcagggctctgagcgccgcgacggcaggatgtgagcttccttacatagaagaggcggatgaaggcgaggaggaagagggcgagtacttggaagactgatggcacaacccgtgttttttgctagatggaacagcaagcaccggatcccgcaatgcgggcggcgctgcagagccagccgtccggcattaactcctcggacgattggacccaggccatgcaacgtatcatggcgttgacgactcgcaaccccgaagcctttagacagcaaccccaggccaaccgtctatcggccatcatggaagctgtagtgccttcccgctctaatcccactcatgagaaggtcctggccatcgtgaacgcgttggtggagaacaaagctattcgtccagatgaggccggactggtatacaacgctctcttagaacgcgtggctcgctacaacagtagcaatgtgcaaaccaatttggaccgtatgataacagatgtacgcgaagccgtgtctcagcgcgaaaggttccagcgtgatgccaacctgggttcgctggtggcgttaaatgctttcttgagtactcagcctgctaatgtgccgcgtggtcaacaggattatactaactttttaagtgctttgagactgatggtatcagaagtacctcagagcgaagtgtatcagtccggtcctgattacttctttcagactagcagacagggcttgcagacggtaaatctgagccaagcttttaaaaaccttaaaggtttgtggggagtgcatgccccggtaggagaaagagcaaccgtgtctagcttgttaactccgaactcccgcctattattactgttggtagctcctttcaccgacagcggtagcatcgaccgtaattcctatttgggttacctactaaacctgtatcgcgaagccatagggcaaagtcaggtggacgagcagacctatcaagaaattacccaagtcagtcgcgctttgggacaggaagacactggcagtttggaagccactctgaacttcttgcttaccaatcggtctcaaaagatccctcctcaatatgctcttactgcggaggaggagaggatccttagatatgtgcagcagagcgtgggattgtttctgatgcaagagggggcaactccgactgcagcactggacatgacagcgcgaaatatggagcccagcatgtatgccagtaaccgacctttcattaacaaactgctggactacttgcacagagctgccgctatgaactctgattatttcaccaatgccatcttaaacccgcactggctgcccccacctggtttctacacgggcgaatatgacatgcccgaccctaatgacggatttctgtgggacgacgtggacagcgatgttttttcacctctttctgatcatcgcacgtggaaaaaggaaggcggcgatagaatgcattcttctgcatcgctgtccggggtcatgggtgctaccgcggctgagcccgagtctgcaagtccttttcctagtctacccttttctctacacagtgtacgtagcagcgaagtgggtagaataagtcgcccgagtttaatgggcgaagaggagtatctaaacgattccttgctcagaccggcaagagaaaaaaatttcccaaacaatggaatagaaagtttggtggataaaatgagtagatggaagacttatgctcaggatcacagagacgagcctgggatcatggggattacaagtagagcgagccgtagacgccagcgccatgacagacagaggggtcttgtgtgggacgatgaggattcggccgatgatagcagcgtgctggacttgggtgggagaggaaggggcaacccgtttgctcatttgcgccctcgcttgggtggtatgttgtaaaaaaaaataaaaaaaaaactcaccaaggccatggcgacgagcgtacgttcgttcttctttattatctgtgtctagtataatgaggcgagtcgtgctaggcggagcggtggtgtatccggagggtcctcctccttcgtacgagagcgtgatgcagcagcagcaggcgacggcggtgatgcaatccccactggaggctccctttgtgcctccgcgatacctggcacctacggagggcagaaacagcattcgttattcggaactggcacctcagtacgataccaccaggttgtatctggtggacaacaagtcggcggacattgcttctctgaactatcagaatgaccacagcaacttcttgaccacggtggtgcaaaacaatgactttacccctacggaagccagcacccagaccattaactttgatgaacgatcgcggtggggcggtcagctaaagaccatcatgcatactaacatgccaaacgtgaacgagtatatgtttagtaacaagttcaaagcgcgtgtgatggtgtccagaaaacctcccgacggtgctgcagttggggatacttatgatcacaagcaggatattttgaaatatgagtggttcgagtttactttgccagaaggcaacttttcagttactatgactattgatttgatgaacaatgccatcatagataattacttgaaagtgggtagacagaatggagtgcttgaaagtgacattggtgttaagttcgacaccaggaacttcaagctgggatgggatcccgaaaccaagttgatcatgcctggagtgtatacgtatgaagccttccatcctgacattgtcttactgcctggctgcggagtggattttaccgagagtcgtttgagcaaccttcttggtatcagaaaaaaacagccatttcaagagggttttaagattttgtatgaagatttagaaggtggtaatattccggccctcttggatgtagatgcctatgagaacagtaagaaagaacaaaaagccaaaatagaagctgctacagctgctgcagaagctaaggcaaacatagttgccagcgactctacaagggttgctaacgctggagaggtcagaggagacaattttgcgccaacacctgttccgactgcagaatcattattggccgatgtgtctgaaggaacggacgtgaaactcactattcaacctgtagaaaaagatagtaagaatagaagctataatgtgttggaagacaaaatcaacacagcctatcgcagttggtatctttcgtacaattatggcgatcccgaaaaaggagtgcgttcctggacattgctcaccacctcagatgtcacctgcggagcagagcaggtctactggtcgcttccagacatgatgaaggatcctgtcactttccgctccactagacaagtcagtaactaccctgtggtgggtgcagagcttatgcccgtcttctcaaagagcttctacaacgaacaagctgtgtactcccagcagctccgccagtccacctcgcttacgcacgtcttcaaccgctttcctgagaaccagattttaatccgtccgccggcgcccaccattaccaccgtcagtgaaaacgttcctgctctcacagatcacgggaccctgccgttgcgcagcagtatccggggagtccaacgtgtgaccgttactgacgccagacgccgcacctgtccctacgtgtacaaggcactgggcatagtcgcaccgcgcgtcctttcaagccgcactttctaaaaaaaaaaaaaatgtccattcttatctcgcccagtaataacaccggttggggtctgcgcgctccaagcaagatgtacggaggcgcacgcaaacgttctacccaacatcctgtccgtgttcgcggacattttcgcgctccatggggcgccctcaagggccgcactcgcgttcgaaccaccgtcgatgatgtaatcgatcaggtggttgccgacgcccgtaattatactcctactgcgcctacatctactgtggatgcagttattgacagtgtagtggctgacgctcgcaactatgctcgacgtaagagccggcgaaggcgcattgccagacgccaccgagctaccactgccatgcgagccgcaagagctctgctacgaagagctagacgcgtggggcgaagagccatgcttagggcggccagacgtgcagcttcgggcgccagcgccggcaggtcccgcaggcaagcagccgctgtcgcagcggcgactattgccgacatggcccaatcgcgaagaggcaatgtatactgggtgcgtgacgctgccaccggtcaacgtgtacccgtgcgcacccgtccccctcgcacttagaagatactgagcagtctccgatgttgtgtcccagcggcgaggatgtccaagcgcaaatacaaggaagaaatgctgcaggttatcgcacctgaagtctacggccaaccgttgaaggatgaaaaaaaaccccgcaaaatcaagcgggttaaaaaggacaaaaaagaagaggaagatggcgatgatgggctggcggagtttgtgcgcgagtttgccccacggcgacgcgtgcaatggcgtgggcgcaaagttcgacatgtgttgagacctggaacttcggtggtctttacacccggcgagcgttcaagcgctacttttaagcgttcctatgatgaggtgtacggggatgatgatattcttgagcaggcggctgaccgattaggcgagtttgcttatggcaagcgtagtagaataacttccaaggatgagacagtgtcgatacccttggatcatggaaatcccacccctagtcttaaaccggtcactttgcagcaagtgttacccgtaactccgcgaacaggtgttaaacgcgaaggtgaagatttgtatcccactatgcaactgatggtacccaaacgccagaagttggaggacgttttggagaaagtaaaagtggatccagatattcaacctgaggttaaagtgagacccattaagcaggtagcgcctggtctgggggtacaaactgtagacattaagattcccactgaaagtatggaagtgcaaactgaacccgcaaagcctactgccacctccactgaagtgcaaacggatccatggatgcccatgcctattacaactgacgccgccggtcccactcgaagatcccgacgaaagtacggtccagcaagtctgttgatgcccaattatgttgtacacccatctattattcctactcctggttaccgaggcactcgctactatcgcagccgaaacagtacctcccgccgtcgccgcaagacacctgcaaatcgcagtcgtcgccgtagacgcacaagcaaaccgactcccggcgccctggtgcggcaagtgtaccgcaatggtagtgcggaacctttgacactgccgcgtgcgcgttaccatccgagtatcatcacttaatcaatgttgccgctgcctccttgcagatatggccctcacttgtcgccttcgcgttcccatcactggttaccgaggaagaaactcgcgccgtagaagagggatgttgggacgcggaatgcgacgctacaggcgacggcgtgctatccgcaagcaattgcggggtggttttttaccagccttaattccaattatcgctgctgcaattggcgcgataccaggcatagcttccgtggcggttcaggcctcgcaacgacattgacattggaaaaaaacgtataaataaaaaaaaaaaaatacaatggactctgacactcctggtcctgtgactatgttttcttagagatggaagacatcaatttttcatccttggctccgcgacacggcacgaagccgtacatgggcacctggagcgacatcggcacgagccaactgaacgggggcgccttcaattggagcagtatctggagcgggcttaaaaattttggctcaaccataaaaacatacgggaacaaagcttggaacagcagtacaggacaggcgcttagaaataaacttaaagaccagaacttccaacaaaaagtagtcgatgggatagcttccggcatcaatggagtggtagatttggctaaccaggctgtgcagaaaaagataaacagtcgtttggacccgccgccagcaaccccaggtgaaatgcaagtggaggaagaaattcctccgccagaaaaacgaggcgacaagcgtccgcgtcccgatttggaagagacgctggtgacgcgcgtagatgaaccgccttcttatgaggaagcaacgaagcttggaatgcccaccactagaccgatagccccaatggccaccggggtgatgaaaccttctcagttgcatcgacccgtcaccttggatttgccccctccccctgctgctactgctgtacccgcttctaagcctgtcgctgccccgaaaccagtcgccgtagccaggtcacgtcccgggggcgctcctcgtccaaatgcgcactggcaaaatactctgaacagcatcgtgggtctaggcgtgcaaagtgtaaaacgccgtcgctgcttttaattaaatatggagtagcgcttaacttgcctatctgtgtatatgtgtcattacacgccgtcacagcagcagaggaaaaaaggaagaggtcgtgcgtcgacgctgagttactttcaagatggccaccccatcgatgctgccccaatgggcatacatgcacatcgccggacaggatgcttcggagtacctgagtccgggtctggtgcagttcgcccgcgccacagacacctacttcaatctgggaaataagtttagaaatcccaccgtagcgccgacccacgatgtgaccaccgaccgtagccagcggctcatgttgcgcttcgtgcccgttgaccgggaggacaatacatactcttacaaagtgcggtacaccctggccgtgggcgacaacagagtgctggatatggccagcacgttctttgacattaggggtgtgttggacagaggtcccagtttcaaaccctattctggtacggcttacaactccctggctcctaaaggcgctccaaatacatctcagtggattgcagaaggtgtaaaaaatacaactggtgaggaacacgtaacagaagaggaaaccaatactactacttacacttttggcaatgctcctgtaaaagctgaagctgaaattacaaaagaaggactcccagtaggtttggaagtttcagatgaagaaagtaaaccgatttatgctgataaaacatatcagccagaacctcagctgggagatgaaacttggactgaccttgatggaaaaaccgaaaagtatggaggcagggctctcaaacccgatactaagatgaaaccatgctacgggtcctttgccaaacctactaatgtgaaaggcggtcaggcaaaacaaaaaacaacggagcagccaaatcagaaagtcgaatatgatatcgacatggagttttttgatgcggcatcgcagaaaacaaacttaagtcctaaaattgtcatgtatgcagaaaatgtaaatttggaaactccagacactcatgtagtgtacaaacctggaacagaagacacaagttccgaagctaatttgggacaacaatctatgcccaacagacccaactacattggcttcagagataactttattggacttatgtactataacagtactggtaacatgggggtgctggctggtcaagcgtctcagttaaatgcagtggttgacttgcaggacagaaacacagaactttcttaccaactcttgcttgactctctgggcgacagaaccagatactttagcatgtggaatcaggctgtggacagttatgatcctgatgtacgtgttattgaaaatcatggtgtggaagatgaacttcccaactactgttttccactggacggcataggtgttccaacaaccagttacaaatcaatagttccaaatggagacaatgcgcctaattggaaggaacctgaagtaaatggaacaagtgagatcggacagggtaatttgtttgccatggaaattaaccttcaagccaatctatggcgaagtttcctttattccaatgtggctctatatctcccagactcgtacaaatacaccccgtccaatgtcactcttccagaaaacaaaaacacctacgactacatgaacgggcgggtggtgccgccatctctagtagacacctatgtgaacattggtgccaggtggtctctggatgccatggacaatgtcaacccattcaaccaccaccgtaacgctggcttgcgttaccgatccatgcttctgggtaacggacgttatgtgcctttccacatacaagtgcctcaaaaattcttcgctgttaaaaacctgctgcttctcccaggctcctacacttatgagtggaactttaggaaggatgtgaacatggttctacagagttccctcggtaacgacctgcgggtagatggcgccagcatcagtttcacgagcatcaacctctatgctacttttttccccatggctcacaacaccgcttccacccttgaagccatgctgcggaatgacaccaatgatcagtcattcaacgactacctatctgcagctaacatgctctaccccattcctgccaatgcaaccaatattcccatttccattccttctcgcaactgggcggctttcagaggctggtcatttaccagactgaaaaccaaagaaactccctctttggggtctggatttgacccctactttgtctattctggttctattccctacctggatggtaccttctacctgaaccacacttttaagaaggtttccatcatgtttgactcttcagtgagctggcctggaaatgacaggttactatctcctaacgaatttgaaataaagcgcactgtggatggcgaaggctacaacgtagcccaatgcaacatgaccaaagactggttcttggtacagatgctcgccaactacaacatcggctatcagggcttctacattccagaaggatacaaagatcgcatgtattcatttttcagaaacttccagcccatgagcaggcaggtggttgatgaggtcaattacaaagacttcaaggccgtcgccataccctaccaacacaacaactctggctttgtgggttacatggctccgaccatgcgccaaggtcaaccctatcccgctaactatccctatccactcattggaacaactgccgtaaatagtgttacgcagaaaaagttcttgtgtgacagaaccatgtggcgcataccgttctcgagcaacttcatgtctatgggggcccttacagacttgggacagaatatgctctatgccaactcagctcatgctctggacatgacctttgaggtggatcccatggatgagcccaccctgctttatcttctcttcgaagttttcgacgtggtcagagtgcatcagccacaccgcggcatcatcgaggcagtctacctgcgtacaccgttctcggccggtaacgctaccacgtaagaagcttcttgcttcttgcaaatagcagctgcaaccatggcctgcggatcccaaaacggctccagcgagcaagagctcagagccattgtccaagacctgggttgcggaccctattttttgggaacctacgataagcgcttcccggggttcatggcccccgataagctcgcctgtgccattgtaaatacggccggacgtgagacggggggagagcactggttggctttcggttggaacccacgttctaacacctgctacctttttgatccttttggattctcggatgatcgtctcaaacagatttaccagtttgaatatgagggtctcctgcgccgcagcgctcttgctaccaaggaccgctgtattacgctggaaaaatctacccagaccgtgcagggtccccgttctgccgcctgcggacttttctgctgcatgttccttcacgcctttgtgcactggcctgaccgtcccatggacggaaaccccaccatgaaattgctaactggagtgccaaacaacatgcttcattctcctaaagtccagcccaccctgtgtgacaatcaaaaagcactctaccattttcttaatacccattcgccttattttcgctcccatcgtacacacatcgaaagggccactgcgttcgaccgtatggatgttcaataatgactcatgtaaacaacgtgttcaataaacatcactttatttttttacatgtatcaaggctctgcattacttatttatttacaagtcgaatgggttctgacgagaatcagaatgacccgcaggcagtgatacgttgcggaactgatacttgggttgccacttgaattcgggaatcaccaacttgggaaccggtatatcgggcaggatgtcactccacagctttctggtcagctgcaaagctccaagcaggtcaggagccgaaatcttgaaatcacaattaggaccagtgctttgagcgcgagagttgcggtacaccggattgcagcactgaaacaccatcagcgacggatgtctcacgcttgccagcacggtgggatctgcaatcatgcccacatccagatcttcagcattggcaatgctgaacggggtcatcttgcaggtctgcctacccatggcgggcacccaattaggcttgtggttgcaatcgcagtgcagggggatcagtatcatcttggcctgatcctgtctgattcctggatacacggctctcatgaaagcatcatattgcttgaaagcctgctgggctttactaccctcggtataaaacatcccgcaggacctgctcgaaaactggttagctgcacagccggcatcattcacacagcagcgggcgtcattgttagctatttgcaccacacttctgccccagcggttttgggtgattttggttcgctcgggattctcctttaaggctcgttgtccgttctcgctggccacatccatctcgataatctgctccttctgaatcataatattgccatgcaggcacttcagcttgccctcataatcattgcagccatgaggccacaacgcacagcctgtacattcccaattatggtgggcgatctgagaaaaagaatgtatcattccctgcagaaatcttcccatcatcgtgctcagtgtcttgtgactagtgaaagttaactggatgcctcggtgctcctcgtttacgtactggtgacagatgcgcttgtattgttcgtgttgctcaggcattagtttaaaagaggttctaagttcgttatccagcctgtacttctccatcagcagacacatcacttccatgcctttctcccaagcagacaccaggggcaagctaatcggattcttaacagtgcaggcagcagctcctttagccagagggtcatctttagcgatcttctcaatgcttcttttgccatccttctcaacgatgcgcacgggcgggtagctgaaacccactgctacaagttgcgcctcttctctttcttcttcgctgtcttgactgatgtcttgcatggggatatgtttggtcttccttggcttctttttggggggtatcggaggaggaggactgtcgctccgttccggagacagggaggattgtgacgtttcgctcaccattaccaactgactgtcggtagaagaacctgaccccacacggcgacaggtgtttctcttcgggggcagaggtggaggcgattgcgaagggctgcggtccgacctggaaggcggatgactggcagaaccccttccgcgttcgggggtgtgctccctgtggcggtcgcttaactgatttccttcgcggctggccattgtgttctcctaggcagagaaacaacagacatggaaactcagccattgctgtcaacatcgccacgagtgccatcacatctcgtcctcagcgacgaggaaaaggagcagagcttaagcattccaccgcccagtcctgccaccacctctaccctagaagataaggaggtcgacgcatctcatgacatgcagaataaaaaagcgaaagagtctgagacagacatcgagcaagacccgggctatgtgacaccggtggaacacgaggaagagttgaaacgctttctagagagagaggatgaaaactgcccaaaacaacgagcagataactatcaccaagatgctggaaatagggatcagaacaccgactacctcatagggcttgacggggaagacgcgctccttaaacatctagcaagacagtcgctcatagtcaaggatgcattattggacagaactgaagtgcccatcagtgtggaagagctcagccgcgcctacgagcttaacctcttttcacctcgtactccccccaaacgtcagccaaacggcacctgcgagccaaatcctcgcttaaacttttatccagcttttgctgtgccagaagtactggctacctatcacatcttttttaaaaatcaaaaaattccagtctcctgccgcgctaatcgcacccgcgccgatgccctactcaatctgggacctggttcacgcttacctgatatagcttccttggaagaggttccaaagatcttcgagggtctgggcaataatgagactcgggccgcaaatgctctgcaaaagggagaaaatggcatggatgagcatcacagcgttctggtggaattggaaggcgataatgccagactcgcagtactcaagcgaagcatcgaggtcacacacttcgcatatcccgctgtcaacctgccccctaaagtcatgacggcggtcatggaccagttactcattaagcgcgcaagtcccctttcagaagacatgcatgacccagatgcctgtgatgagggtaaaccagtggtcagtgatgagcagctaacccgatggctgggcaccgactctcccagggatttggaagagcgtcgcaagcttatgatggccgtggtgctggttaccgtagaactagagtgtctccgacgtttctttaccgattcagaaaccttgcgcaaactcgaagagaatctgcactacacttttagacacggctttgtgcggcaggcatgcaagatatctaacgtggaactcaccaacctggtttcctacatgggtattctgcatgagaatcgcctaggacaaagcgtgctgcacagcaccctgaagggggaagcccgccgtgattacatccgcgattgtgtctatctgtacctgtgccacacgtggcaaaccggcatgggtgtatggcagcaatgtttagaagaacagaacttgaaagagcttgacaagctcttacagaaatctcttaaggttctgtggacagggttcgacgagcgcaccgtcgcttccgacctggcagacctcatcttcccagagcgtctcagggttactttgcgaaacggattgcctgactttatgagccagagcatgcttaacaattttcgctctttcatcctggaacgctccggtatcctgcccgccacctgctgcgcactgccctccgactttgtgcctctcacctaccgcgagtgccccccgccgctatggagtcactgctacctgttccgtctggccaactatctctcctaccactcggatgtgatcgaggatgtgagcggagacggcttgctggagtgtcactgccgctgcaatctgtgcacgccccaccggtccctagcttgcaacccccagttgatgagcgaaacccagataataggcacctttgaattgcaaggccccagcagccaaggcgatgggtcttctcctgggcaaagtttaaaactgaccccgggactgtggacctccgcctacttgcgcaagtttgctccggaagattaccacccctatgaaatcaagttctatgaggaccaatcacagcctccaaaggccgaactttcggcctgcgtcatcacccagggggcaattctggcccaattgcaagccatccaaaaatcccgccaagaatttctactgaaaaagggtaagggggtctaccttgacccccagaccggcgaggaactcaacacaaggttccctcaggatgtcccaacgacgagaaaacaagaagttgaaggtgcagccgccgcccccagaagatatggaggaagattgggacagtcaggcagaggaggcggaggaggacagtctggaggacagtctggaggaagacagtttggaggaggaaaacgaggaggcagaggaggtggaagaagtaaccgccgacaaacagttatcctcggctgcggagacaagcaacagcgctaccatctccgctccgagtcgaggaacccggcggcgtcccagcagtagatgggacgagaccggacgcttcccgaacccaaccagcgcttccaagaccggtaagaaggatcggcagggatacaagtcctggcgggggcataagaatgccatcatctcctgcttgcatgagtgcgggggcaacatatccttcacgcggcgctacttgctattccaccatggggtgaactttccgcgcaatgttttgcattactaccgtcacctccacagcccctactatagccagcaaatcccggcagtctcgacagataaagacagcggcggcgacctccaacagaaaaccagcagcggcagttagaaaatacacaacaagtgcagcaacaggaggattaaagattacagccaacgagccagcgcaaacccgagagttaagaaatcggatctttccaaccctgtatgccatcttccagcagagtcggggtcaagagcaggaactgaaaataaaaaaccgatctctgcgttcgctcaccagaagttgtttgtatcacaagagcgaagatcaacttcagcgcactctcgaggacgccgaggctctcttcaacaagtactgcgcgctgactcttaaagagtaggcagcgaccgcgcttattcaaaaaaggcgggaattacatcatcctcgacatgagtaaagaaattcccacgccttacatgtggagttatcaaccccaaatgggattggcggcaggcgcctcccaggactactccacccgcatgaattggctcagcgccgggccttctatgatttctcgagttaatgatatacgcgcctaccgaaaccaaatacttttggaacagtcagctcttaccaccacgccccgccaacaccttaatcccagaaattggcccgccgccctagtgtaccaggaaagtcccgctcccaccactgtattacttcctcgagacgcccaggccgaagtccaaatgactaatgcaggtgcgcagttagctggcggctccaccctatgtcgtcacaggcctcggcataatataaaacgcctgatgatcagaggccgaggtatccagctcaacgacgagtcggtgagctctccgcttggtctacgaccagacggaatctttcagattgccggctgcgggagatcttccttcacccctcgtcaggctgttctgactttggaaagttcgtcttcgcaaccccgctcgggcggaatcgggaccgttcaatttgtggaggagtttactccctctgtctacttcaaccccttctccggatctcctgggcattacccggacgagttcataccgaacttcgacgcgattagcgagtcagtggacggctacgattgatgtctggtgacgcggctgagctatctcggctgcgacatctagaccactgccgccgctttcgctgctttgcccgggaactcattgagttcatctacttcgaactccccaaggatcaccctcaaggtccggcccacggagtgcggatttctatcgaaggcaaaatagactctcgcctgcaacgaattttctcccagcggcccgtgctgatcgagcgagaccagggaaacaccacggtttccatctactgcatttgtaatcaccccggattgcatgaaagcctttgctgtcttatgtgtactgagtttaataaaaactgaattaagactctcctacggactgccgcttcttcaacccggattttacaaccagaagaacgaaacttttcctgtcgtccaggactctgttaacttcacctttcctactcacaaactagaagctcaacgactacaccgcttttccagaagcattttccctactaatactactttcaaaaccggaggtgagctccaaggtcttcctacagaaaacccttgggtggaagcgggccttgtagtgctaggaattcttgcgggtgggcttgtgattattctttgctacctatacacaccttgcttcactttcttagtggtgttgtggtattggtttaaaaaatggggcccatactagtcttgcttgttttactttcgcttttggaaccgggttctgccaattacgatccatgtctagacttcgacccagaaaactgcacacttacttttgcacccgacacaagccgcatctgtggagttcatcgcctctcttacgaacttggcccccaacgacaaaaatttacctgcatggtgggaatcaaccccatagttatcacccagcaaagtggagatactaagggttgcattcactgctcctgcgattccatcgagtgcacctacaccctgctgaagaccctatgcggcctaagagacctgctaccaatgaattaaaaaatgattaataaaaaatcacttacttgaaatcagcaataaggtctctgttgaaattttctcccagcagcacctcacttccctcttcccaactctggtattctaaaccccgttcagcggcatactttctccatactttaaaggggatgtcaaattttagctcctctcctgtacccacaatcttcatgtctttcttcccagagcggccgcatgaccaagagagtccggctcagtgactccttcaaccctgtctacccctatgaagatgaaagcacctcccaacacccctttataaacccagggtttatttccccaaatggcttcacacaaagcccaaacggagttcttactttaaaatgtttaaccccactaacaaccacaggcggatctctacagctaaaagtgggagggggacttacagtggatgacaccaacggttttttgaaagaaaacataagtgccaccacaccactcgttaagactggtcactctataggtttaccactaggagccggattgggaacgaatgaaaataaactttgtatcaaattaggacaaggacttacattcaattcaaacaacatttgcattgatgacaatattaacaccttatggacaggagtcaaccccaccgaagccaactgtcaaatcatgaactccagtgaatctaatgattgcaaattaattctaacactagttaaaactggagcactagtcactgcatttgtttatgttataggagtatctaacaattttaatatgctaactacacacagaaatataaattttactgcagagctgtttttcgattctactggtaatttactaactagactctcatccctcaaaactccacttaatcataaatcaggacaaaacatggctactggtgccattactaatgctaaaggtttcatgcccagcacgactgcctatcctttcaatgataattctagagaaaaagaaaactacatttacggaacttgttactacacagctagtgatcgcactgcttttcccattgacatatctgtcatgcttaaccgaagagcaataaatgacgagacatcatattgtattcgtataacttggtcctggaacacaggagatgccccagaggtgcaaacctctgctacaaccctagtcacctccccatttaccttttactacatcagagaagacgactgacaaataaagtttaacttgtttatttgaaaatcaattcacaaaatccgagtagttattttgcctcccccttcccatttaacagaatacaccaatctctccccacgcacagctttaaacatttggataccattagatatagacatggttttagattccacattccaaacagtttcagagcgagccaatctggggtcagtgatagataaaaatccatcgggatagtcttttaaagcgctttcacagtccaactgctgcggatgcgactccggagtctggatcacggtcatctggaagaagaacgatgggaatcataatccgaaaacggtatcggacgattgtgtctcatcaaacccacaagcagccgctgtctgcgtcgctccgtgcgactgctgtttatgggatcagggtccacagtgtcctgaagcatgattttaatagcccttaacatcaactttctggtgcgatgcgcgcagcaacgcattctgatttcactcaaatctttgcagtaggtacaacacattattacaatattgtttaataaaccataattaaaagcgctccagccaaaactcatatctgatataatcgcccctgcatgaccatcataccaaagtttaatataaattaaatgacgttccctcaaaaacacactacccacatacatgatctcttttggcatgtgcatattaacaatctgtctgtaccatggacaacgttggttaatcatgcaacccaatataaccttccggaaccacactgccaacaccgctcccccagccatgcattgaagtgaaccctgctgattacaatgacaatgaagaacccaattctctcgaccgtgaatcacttgagaatgaaaaatatctatagtggcacaacatagacataaatgcatgcatcttctcataatttttaactcctcaggatttagaaacatatcccagggaataggaagctcttgcagaacagtaaagctggcagaacaaggaagaccacgaacacaacttacactatgcatagtcatagtatcacaatctggcaacagcgggtggtcttcagtcatagaagctcgggtttcattttcctcacaacgtggtaactgggctctggtgtaagggtgatgtctggcgcatgatgtcgagcgtgcgcgcaaccttgtcataatggagttgcttcctgacattctcgtattttgtatagcaaaacgcggccctggcagaacacactcttcttcgccttctatcctgccgcttagcgtgttccgtgtgatagttcaagtacaaccacactcttaagttggtcaaaagaatgctggcttcagttgtaatcaaaactccatcgcatctaatcgttctgaggaaatcatccaagcaatgcaactggattgtgtttcaagcaggagaggagagggaagagacggaagaaccatgttaatttttattccaaacgatctcgcagtacttcaaattgtagatcgcgcagatggcatctctcgcccccactgtgttggtgaaaaagcacagctagatcaaaagaaatgcgattttcaaggtgctcaacggtggcttccagcaaagcctccacgcgcacatccaagaacaaaagaataccaaaagaaggagcattttctaactcctcaatcatcatattacattcctgcaccattcccagataattttcagctttccagccttgaattattcgtgtcagttcttgtggtaaatccaatccacacattacaaacaggtcccggagggcgccctccaccaccattcttaaacacaccctcataatgacaaaatatcttgctcctgtgtcacctgtagcgaattgagaatggcaacatcaattgacatgcccttggctctaagttcttctttaagttctagttgtaaaaactctctcatattatcaccaaactgcttagccagaagccccccgggaacaagagcaggggacgctacagtgcagtacaagcgcagacctccccaattggctccagcaaaaacaagattggaataagcatattgggaaccgccagtaatatcatcgaagttgctggaaatataatcaggcagagtttcttgtaaaaattgaataaaagaaaaatttgccaaaaaaacattcaaaacctctgggatgcaaatgcaataggttaccgcgctgcgctccaacattgttagttttgaattagtctgcaaaaataaaaaaaaaaacaagcgtcatatcatagtagcctgacgaacagatggataaatcagtctttccatcacaagacaagccacagggtctccagctcgaccctcgtaaaacctgtcatcatgattaaacaacagcaccgaaagttcctcgcggtgaccagcatgaataattcttgatgaagcatacaatccagacatgttagcatcagttaacgagaaaaaacagccaacatagcctttgggtataattatgcttaatcgtaagtatagcaaagccacccctcgcggatacaaagtaaaaggcacaggagaataaaaaatataattatttctctgctgctgttcaggcaacgtcgcccccggtccctctaaatacacatacaaagcctcatcagccatggcttaccagacaaagtacagcgggcacacaaagcacaagctctaaagtgactctccaacctctccacaatatatatatacacaagccctaaactgacgtaatgggagtaaagtgtaaaaaatcccgccaaacccaacacacaccccgaaactgcgtcaccagggaaaagtacagtttcacttccgcaatcccaacaggcgtaacttcctctttctcacggtacgtgatatcccactaacttgcaacgtcattttcccacggtcgcaccgccccttttagccgttaaccccacagccaatcaccacacgatccacactttttaaaatcacctcatttacatattggcaccattccatctataaggtatattatatagataggcgcgccctctcttaaggtagcatcgggatcgagtccctgagagaacatcctcaatcccgatctatccttagatccgaggaatatcgaaatcagttacgctagggataacagggtaatatagcatcccctcggattgctatctaccggctcgtcagctatgatctctcgatttcgatcaagaaatctcattggttaccttgggctatcgaaaccagtcaagtcagctacttggcgagatcgacttgtctgagtttcgactacgctcagaattgcgtcagcgcctatcgccaggtattactccaatcccgaatatccgagcctgagagaacatcctcaatcccgatctatccttagatccgaggaatatcgaaatcgtttaaatcttttcttgatggtaaatcattcgaatataagaatggagagacgaatggggaaacgacaaagatgacattctttggtccttctggtgaggttctcaagtttttggttaatcctgtcaacaacttatatcgtatggggctgacttcaggtgctacatttgaagagataaattgcactgaaatctagtaatattttatctgattaataagatgatcttcttgagatcgttttggtctgcgcgtaatctcttgctctgaaaacgaaaaaaccgccttgcagggcggtttttcgaaggttctctgagctaccaactctttgaaccgaggtaactggcttggcagagcgcagtcaccaaaacttgtcctttcagtttagccttaaccggcgcatgacttcaagactaactctgctaaatcaattaccagtggctgctgccagtggtgcttttgcatgtctttccgggttggactcaagacgatagttaccggataaggcgcagcggtcggactgaacggggggttcgtgcatacagtccagcttggagcgaactgcctacccggaactgagtgtcaggcgtggaatgagacaaacgcggccataacagcggaatgacaccggtaaaccgaaaggcaggaacaggagagcgcacgagggagccgccagggggaaacgcctggtatctttatagtcctgtcgggtttcgccaccactgatttgagcgtcagatttcgtgatgcttgtcaggggggcggagcctatggaaaaacggctttgccgcggccctctcacttccctgttaagtatcttcctggcatcttccaggaaatctccgccccgttcgtaagccatttccgctcgccgcagtcgaacgaccgagcgtagcgagtcagtgagcgaggaagcggaatatatcctgtatcacatattctgctgacgcaccggtgcggccttttttctcctgccacatgaagcacttcactgacaccctcatcagtgccaacatagtaagccagtatacactccgctaatttaaacgtggtgtaccgagaacgatcctctcagtgcgatctcgacgatcagtggtattccgacatatcgttgcttggcagtcagccagtcgatcctagcttgggacccaggaagtccaatcgtcagatattgtactcagcctggtcacggcagcgtaccgatctcgtaactataacggtcctaaggtagcgaactagatattgatagtctgatcggtcaacgtataatcgagtcctagcttttgcaaacatctatcaagagacaggatcagcaggaggctttcgcatgattgaacaagatggattgcacgcaggttctccggcggcttgggtggagaggctattcggctatgactgggcacaacagacaatcggctgctctgatgccgccgtgttccggctgtcagcgcaggggcgtccggttctttttgtcaagaccgacctgtccggtgccctgaatgaactgcaagacgaggcagcgcggctatcgtggctggcgacgacgggcgttccttgcgcggctgtgctcgacgttgtcactgaagcgggaagggactggctgctattgggcgaagtgccggggcaggatctcctgtcatctcaccttgctcctgccgagaaagtatccatcatggctgatgcaatgcggcggctgcatacgcttgatccggctacctgcccattcgaccaccaagcgaaacatcgcatcgagcgagcacgtactcggatggaagccggtcttgtcgatcaggatgatctggacgaagagcatcaggggctcgcgccagccgaactgttcgccaggctcaaggcgtctatgcccgacggcgaggatctcgtcgtgacccacggcgatgcctgcttgccgaatatcatggtggaaaatggccgcttttctggattcatcgactgtggccgtctgggtgtggcggaccgctatcaggacatagcgttggctacccgtgatattgctgaagagcttggcggcgaatgggctgaccgcttccttgtgctttacggtatcgccgcgcccgattcgcagcgcatcgccttctatcgccttcttgacgagttcttctgaccgattctaggtgcattggcgcagaaaaaaatgcctgatgcgacgctgcgcgtcttatactcccacatatgccagattcagcaacggatacggcttccccaacttgcccacttccatacgtgtcctccttaccagaaatttatccttaaggtccgtaactataacggtcctaaggtagcgaatcgacctagctctatcgaatctccctcgtttcgagcttacgcgaactagcctctggcgatagcatccgaggggcaggcatctatgtcgggtgcggagaaagaggtaatgtcaagttcgatctgattgcttggcataaagtccgatggttcgagtagactcagttcaacctctctcttaaggtagc

SEQ ID NO: 32 - DNA, 32350 bp, Artificial Sequence
  ColoAd2.4 Genome
cgcgcctatctatataatataccttatagatggaatggtgccaatatgtaaatgaggtgattttaaaaagtgtggatcgtgtggtgattggctgtggggttaacggctaaaaggggcggtgcgaccgtgggaaaatgacgttttgtgggggtggagtttttttgcaagttgtcgcgggaaatgtgacgcataaaaaggcttttttctcacggaactacttagttttcccacggtatttaacaggaaatgaggtagttttgaccggatgcaagtgaaaattgttgattttcgcgcgaaaactgaatgaggaagtgtttttctgaataatgtggtatttatggcagggtggagtatttgttcagggccaggtagactttgacccattacgtggaggtttcgattaccgtgttttttacctgaatttccgcgtaccgtgtcaaagtcttctgtttttacgtaggtgtcagctgatcgctagggtatttatacctcagggtttgtgtcaagaggccactcttgagtgccagcgagaagagttttctcctctgcgccggcagtttaataataaaaaaatgagagatttgcgatttctgcctcaggaaataatctctgctgagactggaaatgaaatattggagcttgtggtgcacgccctgatgggagacgatccggagccacctgtgcagctttttgagcctcctacgcttcaggaactgtatgatttagaggtagagggatcggaggattctaatgaggaagctgtaaatggcttttttaccgattctatgcttttagctgctaatgaagggttagaattagatccgcctttggacacttttgatactccaggggtaattgtggaaagcggtacaggtgtaagaaaattacctgatttgagttccgtggactgtgatttgcactgctatgaagacgggtttcctccgagtgatgaggaggaccatgaaaaggagcagtccatgcagactgcagcgggtgagggagtgaaggctgccaatgttggttttcagttggattgcccggagcttcctggacatggctgtaagtcttgtgaatttcacaggaaaaatactggagtaaaggaactgttatgttcgctttgttatatgagaacgcactgccactttatttacagtaagtgtgtttaagttaaaatttaaaggaatatgctgtttttcacatgtatattgagtgtgagttttgtgcttcttattataggtcctgtgtctgatgctgatgaatcaccatctcctgattctactacctcacctcctgagattcaagcacctgttcctgtggacgtgcgcaagcccattcctgtgaagcttaagcctgggaaacgtccagcagtggaaaaacttgaggacttgttacagggtggggacggacctttggacttgagtacacggaaacgtccaagacaataagtgttccatatccgtgtttacttaaggtgacgtcaatatttgtgtgacagtgcaatgtaataaaaatatgttaactgttcactggtttttattgctttttgggcggggactcaggtatataagtagaagcagacctgtgtggttagctcataggagctggctttcatccatggaggtttgggccattttggaagaccttaggaagactaggcaactgttagagaacgcttcggacggagtctccggtttttggagattctggttcgctagtgaattagctagggtagtttttaggataaaacaggactataaacaagaatttgaaaagttgttggtagattgcccaggactttttgaagctcttaatttgggccatcaggttcactttaaagaaaaagttttatcagttttagacttttcaaccccaggtagaactgctgctgctgtggcttttcttacttttatattagataaatggatcccgcagactcatttcagcaggggatacgttttggatttcatagccacagcattgtggagaacatggaaggttcgcaagatgaggacaatcttaggttactggccagtgcagcctttgggtgtagcgggaatcctgaggcatccaccggtcatgccagcggttctggaggaggaacagcaagaggacaacccgagagccggcctggaccctccagtggaggaggcggagtagctgacttgtctcctgaactgcaacgggtgcttactggatctacgtccactggacgggataggggcgttaagagggagagggcatctagtggtactgatgctagatctgagttggctttaagtttaatgagtcgcagacgtcctgaaaccatttggtggcatgaggttcagaaagagggaagggatgaagtttctgtattgcaggagaaatattcactggaacaggtgaaaacatgttggttggagcctgaggatgattgggaggtggccattaaaaattatgccaagatagctttgaggcctgataaacagtataagattactagacggattaatatccggaatgcttgttacatatctggaaatggggctgaggtggtaatagatactcaagacaaggcagttattagatgctgcatgatggatatgtggcctggggtagtcggtatggaagcagtaacttttgtaaatgttaagtttaggggagatggttataatggaatagtgtttatggccaataccaaacttatattgcatggttgtagcttttttggtttcaacaatacctgtgtagatgcctggggacaggttagtgtacggggatgtagtttctatgcgtgttggattgccacagctggcagaaccaagagtcaattgtctctgaagaaatgcatatttcaaagatgtaacctgggcattctgaatgaaggcgaagcaagggtccgccactgcgcttctacagatactggatgttttattttgattaagggaaatgccagcgtaaagcataacatgatttgcggtgcttccgatgagaggccttatcaaatgctcacttgtgctggtgggcattgtaatatgctggctactgtgcatattgtttcccatcaacgcaaaaaatggcctgtttttgatcacaatgtgatgacgaagtgtaccatgcatgcaggtgggcgtagaggaatgtttatgccttaccagtgtaacatgaatcatgtgaaagtgttgttggaaccagatgccttttccagaatgagcctaacaggaatttttgacatgaacatgcaaatctggaagatcctgaggtatgatgatacgagatcgagggtacgcgcatgcgaatgcggaggcaagcatgccaggttccagccggtgtgtgtagatgtgactgaagatctcagaccggatcatttggttattgcccgcactggagcagagttcggatccagtggagaagaaactgactaaggtgagtattgggaaaactttggggtgggattttcagatggacagattgagtaaaaatttgttttttctgtcttgcagctgtcatgagtggaaacgcttcttttaaggggggagtcttcagcccttatctgacagggcgtctcccatcctgggcaggagttcgtcagaatgttatgggatctactgtggatggaagacccgtccaacccgccaattcttcaacgctgacctatgctactttaagttcttcacctttggacgcagctgcagctgccgccgccgcttctgttgccgctaacactgtgcttggaatgggttactatggaagcatcatggctaattccacttcctctaataacccttctaccctgactcaggacaagttacttgtccttttggcccagctggaggctttgacccaacgtctgggtgaactttctcagcaggtggtcgagttgcgagtacaaactgagtctgctgtcggcacggcaaagtctaaataaaaaaatcccagaatcaatgaataaataaacaagcttgttgttgatttaaaatcaagtgtttttatttcatttttcgcgcacggtatgccctagaccaccgatctctatcattgagaactcggtggattttttccaggatcctatagaggtgggattgaatgtttagatacatgggcattaggccgtctttggggtggagatagctccattgaagggattcatgctccggggtagtgttgtaaatcacccagtcataacaaggtcgcagtgcatggtgttgcacaatatcttttagaagtaggctgattgccacagataagcccttggtgtaggtgtttacaaaccggttgagctgggatgggtgcattcggggtgaaattatgtgcattttggattggatttttaagttggcaatattgccgccaagatcccgtcttgggttcatgttatgaaggaccaccaagacggtgtatccggtacatttaggaaatttatcgtgcagcttggatggaaaagcgtggaaaaatttggagacacccttgtgtcctccaagattttccatgcactcatccatgataatagcaatggggccgtgggcagcggcgcgggcaaacacgttccgtgggtctgacacatcatagttatgttcctgagttaaatcatcataagccattttaatgaatttggggcggagagtaccagattggggtatgaatgttccttcgggccccggagcatagttcccctcacagatttgcatttcccaagctttcagttccgagggtggaatcatgtccacctggggggctatgaaaaacaccgtttctggggcgggggtgattaattgtgatgatagcaaatttctgagcaattgagatttgccacatccggtggggccataaatgattccgattacgggttgcaggtggtagtttagggaacggcaactgccgtcttctcgaagcaagggggccacctcgttcatcatttcccttacatgcatattttcccgcaccaaatccattaggaggcgctctcctcctagtgatagaagttcttgtagtgaggaaaagtttttcagcggtttcagaccgtcagccatgggcattttggagagagtttgctgcaaaagttctagtctgttccacagttcagtgatgtgttctatggcatctcgatccagcagacctcctcgtttcgcgggtttggacggctcctggaatagggtatgagacgatgggcgtccagcgctgccagggttcggtccttccagggtctcagtgttcgagtcagggttgtttccgtcacagtgaaggggtgtgcgcctgcttgggcgcttgccagggtgcgcttcagactcatcctgctggtcgaaaacttctgtcgcttggcgccctgtatgtcggccaagtagcagtttaccatgagttcgtagttgagcgcctcggctgcgtggcctttggcgcggagcttacctttggaagttttcttgcataccgggcagtataggcatttcagcgcatacaacttgggcgcaaggaaaacggattctggggagtatgcatctgcgccgcaggaggcgcaaacagtttcacattccaccagccaggttaaatccggttcattggggtcaaaaacaagttttccgccatattttttgatgcgtttcttacctttggtctccatgagttcgtgtcctcgttgagtgacaaacaggctgtccgtgtccccgtagactgattttacaggcctcttctccagtggagtgcctcggtcttcttcgtacaggaactctgaccactctgatacaaaggcgcgcgtccaggccagcacaaaggaggctatgtgggaggggtagcgatcgttgtcaaccagggggtccaccttttccaaagtatgcaaacacatgtcaccctcttcaacatccaggaatgtgattggcttgtaggtgtatttcacgtgacctggggtccccgctgggggggtataaaagggggcggttctttgctcttcctcactgtcttccggatcgctgtccaggaacgtcagctgttggggtaggtattccctctcgaaggcgggcatgacctctgcactcaggttgtcagtttctaagaacgaggaggatttgatattgacagtgccggttgagatgcctttcatgaggttttcgtccatctggtcagaaaacacaatttttttattgtcaagtttggtggcaaatgatccatacagggcgttggataaaagtttggcaatggatcgcatggtttggttcttttccttgtccgcgcgctctttggcggcgatgttgagttggacatactcgcgtgccaggcacttccattcggggaagatagttgttaattcatctggcacgattctcacttgccaccctcgattatgcaaggtaattaaatccacactggtggccacctcgcctcgaaggggttcattggtccaacagagcctacctcctttcctagaacagaaagggggaagtgggtctagcataagttcatcgggagggtctgcatccatggtaaagattcccggaagtaaatccttatcaaaatagctgatgggagtggggtcatctaaggccatttgccattctcgagctgccagtgcgcgctcatatgggttaaggggactgccccatggcatgggatgggtgagtgcagaggcatacatgccacagatgtcatagacgtagatgggatcctcaaagatgcctatgtaggttggatagcatcgcccccctctgatacttgctcgcacatagtcatatagttcatgtgatggcgctagcagccccggacccaagttggtgcgattgggtttttctgttctgtagacgatctggcgaaagatggcgtgagaattggaagagatggtgggtctttgaaaaatgttgaaatgggcatgaggtagacctacagagtctctgacaaagtgggcataagattcttgaagcttggttaccagttcggcggtgacaagtacgtctagggcgcagtagtcaagtgtttcttgaatgatgtcataacctggttggtttttcttttcccacagttcgcggttgagaaggtattcttcgcgatccttccagtactcttctagcggaaacccgtctttgtctgcacggtaagatcctagcatgtagaactgattaactgccttgtaagggcagcagcccttctctacgggtagagagtatgcttgagcagcttttcgtagcgaagcgtgagtaagggcaaaggtgtctctgaccatgactttgaggaattggtatttgaagtcgatgtcgtcacaggctccctgttcccagagttggaagtctacccgtttcttgtaggcggggttgggcaaagcgaaagtaacatcattgaagagaatcttgccggccctgggcatgaaattgcgagtgatgcgaaaaggctgtggtacttccgctcggttattgataacctgggcagctaggacgatctcgtcgaaaccgttgatgttgtgtcctacgatgtataattctatgaaacgcggcgtgcctctgacgtgaggtagcttactgagctcatcaaaggttaggtctgtggggtcagataaggcgtagtgttcgagagcccattcgtgcaggtgaggattcgctttaaggaaggaggaccagaggtccactgccagtgctgtttgtaactggtcccggtactgacgaaaatgccgtccgactgccattttttctggggtgacgcaatagaaggtttgggggtcctgccgccagcgatcccacttgagttttatggcgaggtcataggcgatgttgacgagccgctggtctccagagagtttcatgaccagcatgaaggggattagctgcttgccaaaggaccccatccaggtgtaggtttccacatcgtaggtgagaaagagcctttctgtgcgaggatgagagccaatcgggaagaactggatctcctgccaccagttggaggaatggctgttgatgtgatggaagtagaactccctgcgacgcgccgagcattcatgcttgtgcttgtacagacggccgcagtagtcgcagcgttgcacgggttgtatctcgtgaatgagttgtacctggcttcccttgacgagaaatttcagtgggaagccgaggcctggcgattgtatctcgtgctttactatgttgtctgcatcggcctgttcatcttctgtctcgatggtggtcatgctgacgagccctcgcgggaggcaagtccagacctcggcgcggcaggggcggagctcgaggacgagagcgcgcaggctggagctgtccagggtcctgagacgctgcggactcaggttagtaggcagtgtcaggagattaacttgcatgatcttttggagggcgtgcgggaggttcagatagtacttgatctcaacgggtccgttggtggagatgtcgatggcttgcagggttccgtgtcccttgggcgctaccaccgtgcccttgtttttcattttggacggcggtggctctgttgcttcttgcatgtttagaagcggtgtcgagggcgcgcaccgggcggcaggggcggctcgggacccggcggcatggctggcagtggtacgtcggcgccgcgcgcgggtaggttctggtactgcgccctgagaagactcgcatgcgcgacgacgcggcggttgacatcctggatctgacgcctctgggtgaaagctaccggccccgtgagcttgaacctgaaagagagttcaacagaatcaatctcggtatcgttgacggcggcttgcctaaggatttcttgcacgtcaccagagttgtcctggtaggcgatctccgccatgaactgctcgatctcttcctcttgaagatctccgcggcccgctctctcgacggtggccgcgaggtcgttggagatgcgcccaatgagttgagagaatgcattcatgcccgcctcgttccagacgcggctgtagaccacggcccccacgggatctctcgcgcgcatgaccacctgggcgaggttgagctccacgtggcgggtgaagaccgcatagttgcataggcgctggaaaaggtagttgagtgtggtggcgatgtgctcggtgacgaagaaatacatgatccatcgtctcagcggcatctcgctgacatcgcccagagcttccaagcgctccatggcctcgtagaagtccacggcaaaattaaaaaactgggagtttcgcgcggacacggtcaactcctcttccagaagacggataagttcggcgatggtggtgcgcacctcgcgctcgaaagcccctgggatttcttcctcaatctcttcttcttccactaacatctcttcctcttcaggtggggctgcaggaggagggggaacgcggcgacgccggcggcgcacgggcagacggtcgatgaatctttcaatgacctctccgcggcggcggcgcatggtttcagtgacggcgcggccgttctcgcgcggtcgcagagtaaaaacaccgccgcgcatctccttaaagtggtgactgggaggttctccgtttgggagggagagggcgctgattatacattttattaattggcccgtagggactgcacgcagagatctgatcgtgtcaagatccacgggatctgaaaacctttcgacgaaagcgtctaaccagtcacagtcacaaggtaggctgagtacggcttcttgtgggcgggggtggttatgtgttcggtctgggtcttctgtttcttcttcatctcgggaaggtgagacgatgctgctggtgatgaaattaaagtaggcagttctaagacggcggatggtggcgaggagcaccaggtctttgggtccggcttgctggatacgcaggcgattggccattccccaagcattatcctgacatctagcaagatctttgtagtagtcttgcatgagccgttctacgggcacttcttcctcacccgttctgccatgcatacgtgtgagtccaaatccgcgcattggttgtaccagtgccaagtcagctacgactctttcggcgaggatggcttgctgtacttgggtaagggtggcttgaaagtcatcaaaatccacaaagcggtggtaagctcctgtattaatggtgtaagcacagttggccatgactgaccagttaactgtctggtgaccagggcgcacgagctcggtgtatttaaggcgcgaataggcgcgggtgtcaaagatgtaatcgttgcaggtgcgcaccagatactggtaccctataagaaaatgcggcggtggttggcggtagagaggccatcgttctgtagctggagcgccaggggcgaggtcttccaacataaggcggtgatagccgtagatgtacctggacatccaggtgattcctgcggcggtagtagaagcccgaggaaactcgcgtacgcggttccaaatgttgcgtagcggcatgaagtagttcattgtaggcacggtttgaccagtgaggcgcgcgcagtcattgatgctctatagacacggagaaaatgaaagcgttcagcgactcgactccgtagcctggaggaacgtgaacgggttgggtcgcggtgtaccccggttcgagacttgtactcgagccggccggagccgcggctaacgtggtattggcactcccgtctcgacccagcctacaaaaatccaggatacggaatcgagtcgttttgctggtttccgaatggcagggaagtgagtcctattttttttttttgccgctcagatgcatcccgtgctgcgacagatgcgcccccaacaacagcccccctcgcagcagcagcagcagcaatcacaaaaggctgtccctgcaactactgcaactgccgccgtgagcggtgcgggacagcccgcctatgatctggacttggaagagggcgaaggactggcacgtctaggtgcgccttcacccgagcggcatccgcgagttcaactgaaaaaagattctcgcgaggcgtatgtgccccaacagaacctatttagagacagaagcggcgaggagccggaggagatgcgagcttcccgctttaacgcgggtcgtgagctgcgtcacggtttggaccgaagacgagtgttgcgggacgaggatttcgaagttgatgaaatgacagggatcagtcctgccagggcacacgtggctgcagccaaccttgtatcggcttacgagcagacagtaaaggaagagcgtaacttccaaaagtcttttaataatcatgtgcgaaccctgattgcccgcgaagaagttacccttggtttgatgcatttgtgggatttgatggaagctatcattcagaaccctactagcaaacctctgaccgcccagctgtttctggtggtgcaacacagcagagacaatgaggctttcagagaggcgctgctgaacatcaccgaacccgaggggagatggttgtatgatcttatcaacattctacagagtatcatagtgcaggagcggagcctgggcctggccgagaaggtggctgccatcaattactcggttttgagcttgggaaaatattacgctcgcaaaatctacaagactccatacgttcccatagacaaggaggtgaagatagatgggttctacatgcgcatgacgctcaaggtcttgaccctgagcgatgatcttggggtgtatcgcaatgacagaatgcatcgcgcggttagcgccagcaggaggcgcgagttaagcgacagggaactgatgcacagtttgcaaagagctctgactggagctggaaccgagggtgagaattacttcgacatgggagctgacttgcagtggcagcctagtcgcagggctctgagcgccgcgacggcaggatgtgagcttccttacatagaagaggcggatgaaggcgaggaggaagagggcgagtacttggaagactgatggcacaacccgtgttttttgctagatggaacagcaagcaccggatcccgcaatgcgggcggcgctgcagagccagccgtccggcattaactcctcggacgattggacccaggccatgcaacgtatcatggcgttgacgactcgcaaccccgaagcctttagacagcaaccccaggccaaccgtctatcggccatcatggaagctgtagtgccttcccgctctaatcccactcatgagaaggtcctggccatcgtgaacgcgttggtggagaacaaagctattcgtccagatgaggccggactggtatacaacgctctcttagaacgcgtggctcgctacaacagtagcaatgtgcaaaccaatttggaccgtatgataacagatgtacgcgaagccgtgtctcagcgcgaaaggttccagcgtgatgccaacctgggttcgctggtggcgttaaatgctttcttgagtactcagcctgctaatgtgccgcgtggtcaacaggattatactaactttttaagtgctttgagactgatggtatcagaagtacctcagagcgaagtgtatcagtccggtcctgattacttctttcagactagcagacagggcttgcagacggtaaatctgagccaagcttttaaaaacctttaaaggtttgtggggagtgcatgccccggtaggagaaagagcaaccgtgtctagcttgttaactccgaactcccgcctattattactgttggtagctcctttcaccgacagcggtagcatcgaccgtaattcctatttgggttacctactaaacctgtatcgcgaagccatagggcaaagtcaggtggacgagcagacctatcaagaaattacccaagtcagtcgcgctttgggacaggaagacactggcagtttggaagccactctgaacttcttgcttaccaatcggtctcaaaagatccctcctcaatatgctcttactgcggaggaggagaggatccttagatatgtgcagcagagcgtgggattgtttctgatgcaagagggggcaactccgactgcagcactggacatgacagcgcgaaatatggagcccagcatgtatgccagtaaccgacctttcattaacaaactgctggactacttgcacagagctgccgctatgaactctgattatttcaccaatgccatcttaaacccgcactggctgcccccacctggtttctacacgggcgaatatgacatgcccgaccctaatgacggatttctgtgggacgacgtggacagcgatgttttttcacctctttctgatcatcgcacgtggaaaaaggaaggcggcgatagaatgcattcttctgcatcgctgtccggggtcatgggtgctaccgcggctgagcccgagtctgcaagtccttttcctagtctacccttttctctacacagtgtacgtagcagcgaagtgggtagaataagtcgcccgagtttaatgggcgaagaggagtatctaaacgattccttgctcagaccggcaagagaaaaaaatttcccaaacaatggaatagaaagtttggtggataaaatgagtagatggaagacttatgctcaggatcacagagacgagcctgggatcatggggattacaagtagagcgagccgtagacgccagcgccatgacagacagaggggtcttgtgtgggacgatgaggattcggccgatgatagcagcgtgctggacttgggtgggagaggaaggggcaacccgtttgctcatttgcgccctcgcttgggtggtatgttgtaaaaaaaaataaaaaaaaaactcaccaaggccatggcgacgagcgtacgttcgttcttctttattatctgtgtctagtataatgaggcgagtcgtgctaggcggagcggtggtgtatccggagggtcctcctccttcgtacgagagcgtgatgcagcagcagcaggcgacggcggtgatgcaatccccactggaggctccctttgtgcctccgcgatacctggcacctacggagggcagaaacagcattcgttattcggaactggcacctcagtacgataccaccaggttgtatctggtggacaacaagtcggcggacattgcttctctgaactatcagaatgaccacagcaacttcttgaccacggtggtgcaaaacaatgactttacccctacggaagccagcacccagaccattaactttgatgaacgatcgcggtggggcggtcagctaaagaccatcatgcatactaacatgccaaacgtgaacgagtatatgtttagtaacaagttcaaagcgcgtgtgatggtgtccagaaaacctcccgacggtgctgcagttggggatacttatgatcacaagcaggatattttgaaatatgagtggttcgagtttactttgccagaaggcaacttttcagttactatgactattgatttgatgaacaatgccatcatagataattacttgaaagtgggtagacagaatggagtgcttgaaagtgacattggtgttaagttcgacaccaggaacttcaagctgggatgggatcccgaaaccaagttgatcatgcctggagtgtatacgtatgaagccttccatcctgacattgtcttactgcctggctgcggagtggattttaccgagagtcgtttgagcaaccttcttggtatcagaaaaaaacagccatttcaagagggttttaagattttgtatgaagatttagaaggtggtaatattccggccctcttggatgtagatgcctatgagaacagtaagaaagaacaaaaagccaaaatagaagctgctacagctgctgcagaagctaaggcaaacatagttgccagcgactctacaagggttgctaacgctggagaggtcagaggagacaattttgcgccaacacctgttccgactgcagaatcattattggccgatgtgtctgaaggaacggacgtgaaactcactattcaacctgtagaaaaagatagtaagaatagaagctataatgtgttggaagacaaaatcaacacagcctatcgcagttggtatctttcgtacaattatggcgatcccgaaaaaggagtgcgttcctggacattgctcaccacctcagatgtcacctgcggagcagagcaggtctactggtcgcttccagacatgatgaaggatcctgtcactttccgctccactagacaagtcagtaactaccctgtggtgggtgcagagcttatgcccgtcttctcaaagagcttctacaacgaacaagctgtgtactcccagcagctccgccagtccacctcgcttacgcacgtcttcaaccgctttcctgagaaccagattttaatccgtccgccggcgcccaccattaccaccgtcagtgaaaacgttcctgctctcacagatcacgggaccctgccgttgcgcagcagtatccggggagtccaacgtgtgaccgttactgacgccagacgccgcacctgtccctacgtgtacaaggcactgggcatagtcgcaccgcgcgtcctttcaagccgcactttctaaaaaaaaaaaaaatgtccattcttatctcgcccagtaataacaccggttggggtctgcgcgctccaagcaagatgtacggaggcgcacgcaaacgttctacccaacatcctgtccgtgttcgcggacattttcgcgctccatggggcgccctcaagggccgcactcgcgttcgaaccaccgtcgatgatgtaatcgatcaggtggttgccgacgcccgtaattatactcctactgcgcctacatctactgtggatgcagttattgacagtgtagtggctgacgctcgcaactatgctcgacgtaagagccggcgaaggcgcattgccagacgccaccgagctaccactgccatgcgagccgcaagagctctgctacgaagagctagacgcgtggggcgaagagccatgcttagggcggccagacgtgcagcttcgggcgccagcgccggcaggtcccgcaggcaagcagccgctgtcgcagcggcgactattgccgacatggcccaatcgcgaagaggcaatgtatactgggtgcgtgacgctgccaccggtcaacgtgtacccgtgcgcacccgtccccctcgcacttagaagatactgagcagtctccgatgttgtgtcccagcggcgaggatgtccaagcgcaaatacaaggaagaaatgctgcaggttatcgcacctgaagtctacggccaaccgttgaaggatgaaaaaaaaccccgcaaaatcaagcgggttaaaaaggacaaaaaagaagaggaagatggcgatgatgggctggcggagtttgtgcgcgagtttgccccacggcgacgcgtgcaatggcgtgggcgcaaagttcgacatgtgttgagacctggaacttcggtggtctttacacccggcgagcgttcaagcgctacttttaagcgttcctatgatgaggtgtacggggatgatgatattcttgagcaggcggctgaccgattaggcgagtttgcttatggcaagcgtagtagaataacttccaaggatgagacagtgtcgatacccttggatcatggaaatcccacccctagtcttaaaccggtcactttgcagcaagtgttacccgtaactccgcgaacaggtgttaaacgcgaaggtgaagatttgtatcccactatgcaactgatggtacccaaacgccagaagttggaggacgttttggagaaagtaaaagtggatccagatattcaacctgaggttaaagtgagacccattaagcaggtagcgcctggtctgggggtacaaactgtagacattaagattcccactgaaagtatggaagtgcaaactgaacccgcaaagcctactgccacctccactgaagtgcaaacggatccatggatgcccatgcctattacaactgacgccgccggtcccactcgaagatcccgacgaaagtacggtccagcaagtctgttgatgcccaattatgttgtacacccatctattattcctactcctggttaccgaggcactcgctactatcgcagccgaaacagtacctcccgccgtcgccgcaagacacctgcaaatcgcagtcgtcgccgtagacgcacaagcaaaccgactcccggcgccctggtgcggcaagtgtaccgcaatggtagtgcggaacctttgacactgccgcgtgcgcgttaccatccgagtatcatcacttaatcaatgttgccgctgcctccttgcagatatggccctcacttgtcgccttcgcgttcccatcactggttaccgaggaagaaactcgcgccgtagaagagggatgttgggacgcggaatgcgacgctacaggcgacggcgtgctatccgcaagcaattgcggggtggttttttaccagccttaattccaattatcgctgctgcaattggcgcgataccaggcatagcttccgtggcggttcaggcctcgcaacgacattgacattggaaaaaaacgtataaataaaaaaaaaaaaatacaatggactctgacactcctggtcctgtgactatgttttcttagagatggaagacatcaatttttcatccttggctccgcgacacggcacgaagccgtacatgggcacctggagcgacatcggcacgagccaactgaacgggggcgccttcaattggagcagtatctggagcgggcttaaaaattttggctcaaccataaaaacatacgggaacaaagcttggaacagcagtacaggacaggcgcttagaaataaacttaaagaccagaacttccaacaaaaagtagtcgatgggatagcttccggcatcaatggagtggtagatttggctaaccaggctgtgcagaaaaagataaacagtcgtttggacccgccgccagcaaccccaggtgaaatgcaagtggaggaagaaattcctccgccagaaaaacgaggcgacaagcgtccgcgtcccgatttggaagagacgctggtgacgcgcgtagatgaaccgccttcttatgaggaagcaacgaagcttggaatgcccaccactagaccgatagccccaatggccaccggggtgatgaaaccttctcagttgcatcgacccgtcaccttggatttgccccctccccctgctgctactgctgtacccgcttctaagcctgtcgctgccccgaaaccagtcgccgtagccaggtcacgtcccgggggcgctcctcgtccaaatgcgcactggcaaaatactctgaacagcatcgtgggtctaggcgtgcaaagtgtaaaacgccgtcgctgcttttaattaaatatggagtagcgcttaacttgcctatctgtgtatatgtgtcattacacgccgtcacagcagcagaggaaaaaaggaagaggtcgtgcgtcgacgctgagttactttcaagatggccaccccatcgatgctgccccaatgggcatacatgcacatcgccggacaggatgcttcggagtacctgagtccgggtctggtgcagttcgcccgcgccacagacacctacttcaatctgggaaataagtttagaaatcccaccgtagcgccgacccacgatgtgaccaccgaccgtagccagcggctcatgttgcgcttcgtgcccgttgaccgggaggacaatacatactcttacaaagtgcggtacaccctggccgtgggcgacaacagagtgctggatatggccagcacgttctttgacattaggggtgtgttggacagaggtcccagtttcaaaccctattctggtacggcttacaactccctggctcctaaaggcgctccaaatacatctcagtggattgcagaaggtgtaaaaaatacaactggtgaggaacacgtaacagaagaggaaaccaatactactacttacacttttggcaatgctcctgtaaaagctgaagctgaaattacaaaagaaggactcccagtaggtttggaagtttcagatgaagaaagtaaaccgatttatgctgataaaacatatcagccagaacctcagctgggagatgaaacttggactgaccttgatggaaaaaccgaaaagtatggaggcagggctctcaaacccgatactaagatgaaaccatgctacgggtcctttgccaaacctactaatgtgaaaggcggtcaggcaaaacaaaaaacaacggagcagccaaatcagaaagtcgaatatgatatcgacatggagttttttgatgcggcatcgcagaaaacaaacttaagtcctaaaattgtcatgtatgcagaaaatgtaaatttggaaactccagacactcatgtagtgtacaaacctggaacagaagacacaagttccgaagctaatttgggacaacaatctatgcccaacagacccaactacattggcttcagagataactttattggacttatgtactataacagtactggtaacatgggggtgctggctggtcaagcgtctcagttaaatgcagtggttgacttgcaggacagaaacacagaactttcttaccaactcttgcttgactctctgggcgacagaaccagatactttagcatgtggaatcaggctgtggacagttatgatcctgatgtacgtgttattgaaaatcatggtgtggaagatgaacttcccaactactgttttccactggacggcataggtgttccaacaaccagttacaaatcaatagttccaaatggagacaatgcgcctaattggaaggaacctgaagtaaatggaacaagtgagatcggacagggtaatttgtttgccatggaaattaaccttcaagccaatctatggcgaagtttcctttattccaatgtggctctatatctcccagactcgtacaaatacaccccgtccaatgtcactcttccagaaaacaaaaacacctacgactacatgaacgggcgggtggtgccgccatctctagtagacacctatgtgaacattggtgccaggtggtctctggatgccatggacaatgtcaacccattcaaccaccaccgtaacgctggcttgcgttaccgatccatgcttctgggtaacggacgttatgtgcctttccacatacaagtgcctcaaaaattcttcgctgttaaaaacctgctgcttctcccaggctcctacacttatgagtggaactttaggaaggatgtgaacatggttctacagagttccctcggtaacgacctgcgggtagatggcgccagcatcagtttcacgagcatcaacctctatgctacttttttccccatggctcacaacaccgcttccacccttgaagccatgctgcggaatgacaccaatgatcagtcattcaacgactacctatctgcagctaacatgctctaccccattcctgccaatgcaaccaatattcccatttccattccttctcgcaactgggcggctttcagaggctggtcatttaccagactgaaaaccaaagaaactccctctttggggtctggatttgacccctactttgtctattctggttctattccctacctggatggtaccttctacctgaaccacacttttaagaaggtttccatcatgtttgactcttcagtgagctggcctggaaatgacaggttactatctcctaacgaatttgaaataaagcgcactgtggatggcgaaggctacaacgtagcccaatgcaacatgaccaaagactggttcttggtacagatgctcgccaactacaacatcggctatcagggcttctacattccagaaggatacaaagatcgcatgtattcatttttcagaaacttccagcccatgagcaggcaggtggttgatgaggtcaattacaaagacttcaaggccgtcgccataccctaccaacacaacaactctggctttgtgggttacatggctccgaccatgcgccaaggtcaaccctatcccgctaactatccctatccactcattggaacaactgccgtaaatagtgttacgcagaaaaagttcttgtgtgacagaaccatgtggcgcataccgttctcgagcaacttcatgtctatgggggcccttacagacttgggacagaatatgctctatgccaactcagctcatgctctggacatgacctttgaggtggatcccatggatgagcccaccctgctttatcttctcttcgaagttttcgacgtggtcagagtgcatcagccacaccgcggcatcatcgaggcagtctacctgcgtacaccgttctcggccggtaacgctaccacgtaagaagcttcttgcttcttgcaaatagcagctgcaaccatggcctgcggatcccaaaacggctccagcgagcaagagctcagagccattgtccaagacctgggttgcggaccctattttttgggaacctacgataagcgcttcccggggttcatggcccccgataagctcgcctgtgccattgtaaatacggccggacgtgagacggggggagagcactggttggctttcggttggaacccacgttctaacacctgctacctttttgatccttttggattctcggatgatcgtctcaaacagatttaccagtttgaatatgagggtctcctgcgccgcagcgctcttgctaccaaggaccgctgtattacgctggaaaaatctacccagaccgtgcagggtccccgttctgccgcctgcggacttttctgctgcatgttccttcacgcctttgtgcactggcctgaccgtcccatggacggaaaccccaccatgaaattgctaactggagtgccaaacaacatgcttcattctcctaaagtccagcccaccctgtgtgacaatcaaaaagcactctaccattttcttaatacccattcgccttattttcgctcccatcgtacacacatcgaaagggccactgcgttcgaccgtatggatgttcaataatgactcatgtaaacaacgtgttcaataaacatcactttatttttttacatgtatcaaggctctgcattacttatttatttacaagtcgaatgggttctgacgagaatcagaatgacccgcaggcagtgatacgttgcggaactgatacttgggttgccacttgaattcgggaatcaccaacttgggaaccggtatatcgggcaggatgtcactccacagctttctggtcagctgcaaagctccaagcaggtcaggagccgaaatcttgaaatcacaattaggaccagtgctttgagcgcgagagttgcggtacaccggattgcagcactgaaacaccatcagcgacggatgtctcacgcttgccagcacggtgggatctgcaatcatgcccacatccagatcttcagcattggcaatgctgaacggggtcatcttgcaggtctgcctacccatggcgggcacccaattaggcttgtggttgcaatcgcagtgcagggggatcagtatcatcttggcctgatcctgtctgattcctggatacacggctctcatgaaagcatcatattgcttgaaagcctgctgggctttactaccctcggtataaaacatcccgcaggacctgctcgaaaactggttagctgcacagccggcatcattcacacagcagcgggcgtcattgttagctatttgcaccacacttctgccccagcggttttgggtgattttggttcgctcgggattctcctttaaggctcgttgtccgttctcgctggccacatccatctcgataatctgctccttctgaatcataatattgccatgcaggcacttcagcttgccctcataatcattgcagccatgaggccacaacgcacagcctgtacattcccaattatggtgggcgatctgagaaaaagaatgtatcattccctgcagaaatcttcccatcatcgtgctcagtgtcttgtgactagtgaaagttaactggatgcctcggtgctcctcgtttacgtactggtgacagatgcgcttgtattgttcgtgttgctcaggcattagtttaaaagaggttctaagttcgttatccagcctgtacttctccatcagcagacacatcacttccatgcctttctcccaagcagacaccaggggcaagctaatcggattcttaacagtgcaggcagcagctcctttagccagagggtcatctttagcgatcttctcaatgcttcttttgccatccttctcaacgatgcgcacgggcgggtagctgaaacccactgctacaagttgcgcctcttctctttcttcttcgctgtcttgactgatgtcttgcatggggatatgtttggtcttccttggcttctttttggggggtatcggaggaggaggactgtcgctccgttccggagacagggaggattgtgacgtttcgctcaccattaccaactgactgtcggtagaagaacctgaccccacacggcgacaggtgtttctcttcgggggcagaggtggaggcgattgcgaagggctgcggtccgacctggaaggcggatgactggcagaaccccttccgcgttcgggggtgtgctccctgtggcggtcgcttaactgatttccttcgcggctggccattgtgttctcctaggcagagaaacaacagacatggaaactcagccattgctgtcaacatcgccacgagtgccatcacatctcgtcctcagcgacgaggaaaaggagcagagcttaagcattccaccgcccagtcctgccaccacctctaccctagaagataaggaggtcgacgcatctcatgacatgcagaataaaaaagcgaaagagtctgagacagacatcgagcaagacccgggctatgtgacaccggtggaacacgaggaagagttgaaacgctttctagagagagaggatgaaaactgcccaaaacaacgagcagataactatcaccaagatgctggaaatagggatcagaacaccgactacctcatagggcttgacggggaagacgcgctccttaaacatctagcaagacagtcgctcatagtcaaggatgcattattggacagaactgaagtgcccatcagtgtggaagagctcagccgcgcctacgagcttaacctcttttcacctcgtactccccccaaacgtcagccaaacggcacctgcgagccaaatcctcgcttaaacttttatccagcttttgctgtgccagaagtactggctacctatcacatcttttttaaaaatcaaaaaattccagtctcctgccgcgctaatcgcacccgcgccgatgccctactcaatctgggacctggttcacgcttacctgatatagcttccttggaagaggttccaaagatcttcgagggtctgggcaataatgagactcgggccgcaaatgctctgcaaaagggagaaaatggcatggatgagcatcacagcgttctggtggaattggaaggcgataatgccagactcgcagtactcaagcgaagcatcgaggtcacacacttcgcatatcccgctgtcaacctgccccctaaagtcatgacggcggtcatggaccagttactcattaagcgcgcaagtcccctttcagaagacatgcatgacccagatgcctgtgatgagggtaaaccagtggtcagtgatgagcagctaacccgatggctgggcaccgactctcccagggatttggaagagcgtcgcaagcttatgatggccgtggtgctggttaccgtagaactagagtgtctccgacgtttctttaccgattcagaaaccttgcgcaaactcgaagagaatctgcactacacttttagacacggctttgtgcggcaggcatgcaagatatctaacgtggaactcaccaacctggtttcctacatgggtattctgcatgagaatcgcctaggacaaagcgtgctgcacagcaccctgaagggggaagcccgccgtgattacatccgcgattgtgtctatctgtacctgtgccacacgtggcaaaccggcatgggtgtatggcagcaatgtttagaagaacagaacttgaaagagcttgacaagctcttacagaaatctcttaaggttctgtggacagggttcgacgagcgcaccgtcgcttccgacctggcagacctcatcttcccagagcgtctcagggttactttgcgaaacggattgcctgactttatgagccagagcatgcttaacaattttcgctctttcatcctggaacgctccggtatcctgcccgccacctgctgcgcactgccctccgactttgtgcctctcacctaccgcgagtgccccccgccgctatggagtcactgctacctgttccgtctggccaactatctctcctaccactcggatgtgatcgaggatgtgagcggagacggcttgctggagtgtcactgccgctgcaatctgtgcacgccccaccggtccctagcttgcaacccccagttgatgagcgaaacccagataataggcacctttgaattgcaaggccccagcagccaaggcgatgggtcttctcctgggcaaagtttaaaactgaccccgggactgtggacctccgcctacttgcgcaagtttgctccggaagattaccacccctatgaaatcaagttctatgaggaccaatcacagcctccaaaggccgaactttcggcctgcgtcatcacccagggggcaattctggcccaattgcaagccatccaaaaatcccgccaagaatttctactgaaaaagggtaagggggtctaccttgacccccagaccggcgaggaactcaacacaaggttccctcaggatgtcccaacgacgagaaaacaagaagttgaaggtgcagccgccgcccccagaagatatggaggaagattgggacagtcaggcagaggaggcggaggaggacagtctggaggacagtctggaggaagacagtttggaggaggaaaacgaggaggcagaggaggtggaagaagtaaccgccgacaaacagttatcctcggctgcggagacaagcaacagcgctaccatctccgctccgagtcgaggaacccggcggcgtcccagcagtagatgggacgagaccggacgcttcccgaacccaaccagcgcttccaagaccggtaagaaggatcggcagggatacaagtcctggcgggggcataagaatgccatcatctcctgcttgcatgagtgcgggggcaacatatccttcacgcggcgctacttgctattccaccatggggtgaactttccgcgcaatgttttgcattactaccgtcacctccacagcccctactatagccagcaaatcccggcagtctcgacagataaagacagcggcggcgacctccaacagaaaaccagcagcggcagttagaaaatacacaacaagtgcagcaacaggaggattaaagattacagccaacgagccagcgcaaacccgagagttaagaaatcggatctttccaaccctgtatgccatcttccagcagagtcggggtcaagagcaggaactgaaaataaaaaaccgatctctgcgttcgctcaccagaagttgtttgtatcacaagagcgaagatcaacttcagcgcactctcgaggacgccgaggctctcttcaacaagtactgcgcgctgactcttaaagagtaggcagcgaccgcgcttattcaaaaaaggcgggaattacatcatcctcgacatgagtaaagaaattcccacgccttacatgtggagttatcaaccccaaatgggattggcggcaggcgcctcccaggactactccacccgcatgaattggctcagcgccgggccttctatgatttctcgagttaatgatatacgcgcctaccgaaaccaaatacttttggaacagtcagctcttaccaccacgccccgccaacaccttaatcccagaaattggcccgccgccctagtgtaccaggaaagtcccgctcccaccactgtattacttcctcgagacgcccaggccgaagtccaaatgactaatgcaggtgcgcagttagctggcggctccaccctatgtcgtcacaggcctcggcataatataaaacgcctgatgatcagaggccgaggtatccagctcaacgacgagtcggtgagctctccgcttggtctacgaccagacggaatctttcagattgccggctgcgggagatcttccttcacccctcgtcaggctgttctgactttggaaagttcgtcttcgcaaccccgctcgggcggaatcgggaccgttcaatttgtggaggagtttactccctctgtctacttcaaccccttctccggatctcctgggcattacccggacgagttcataccgaacttcgacgcgattagcgagtcagtggacggctacgattgatgtctggtgacgcggctgagctatctcggctgcgacatctagaccactgccgccgctttcgctgctttgcccgggaactcattgagttcatctacttcgaactccccaaggatcaccctcaaggtccggcccacggagtgcggatttctatcgaaggcaaaatagactctcgcctgcaacgaattttctcccagcggcccgtgctgatcgagcgagaccagggaaacaccacggtttccatctactgcatttgtaatcaccccggattgcatgaaagcctttgctgtcttatgtgtactgagtttaataaaaactgaattaagactctcctacggactgccgcttcttcaacccggattttacaaccagaagaacgaaacttttcctgtcgtccaggactctgttaacttcacctttcctactcacaaactagaagctcaacgactacaccgcttttccagaagcattttccctactaatactactttcaaaaccggaggtgagctccaaggtcttcctacagaaaacccttgggtggaagcgggccttgtagtgctaggaattcttgcgggtgggcttgtgattattctttgctacctatacacaccttgcttcactttcttagtggtgttgtggtattggtttaaaaaatggggcccatactagtcttgcttgttttactttcgcttttggaaccgggttctgccaattacgatccatgtctagacttcgacccagaaaactgcacacttacttttgcacccgacacaagccgcatctgtggagttcatcgcctctcttacgaacttggcccccaacgacaaaaatttacctgcatggtgggaatcaaccccatagttatcacccagcaaagtggagatactaagggttgcattcactgctcctgcgattccatcgagtgcacctacaccctgctgaagaccctatgcggcctaagagacctgctaccaatgaattaaaaaatgattaataaaaaatcacttacttgaaatcagcaataaggtctctgttgaaattttctcccagcagcacctcacttccctcttcccaactctggtattctaaaccccgttcagcggcatactttctccatactttaaaggggatgtcaaattttagctcctctcctgtacccacaatcttcatgtctttcttcccagatgaccaagagagtccggctcagtgactccttcaaccctgtctacccctatgaagatgaaagcacctcccaacacccctttataaacccagggtttatttccccaaatggcttcacacaaagcccaaacggagttcttactttaaaatgtttaaccccactaacaaccacaggcggatctctacagctaaaagtgggagggggacttacagtggatgacaccaacggttttttgaaagaaaacataagtgccaccacaccactcgttaagactggtcactctataggtttaccactaggagccggattgggaacgaatgaaaataaactttgtatcaaattaggacaaggacttacattcaattcaaacaacatttgcattgatgacaatattaacaccttatggacaggagtcaaccccaccgaagccaactgtcaaatcatgaactccagtgaatctaatgattgcaaattaattctaacactagttaaaactggagcactagtcactgcatttgtttatgttataggagtatctaacaattttaatatgctaactacacacagaaatataaattttactgcagagctgtttttcgattctactggtaatttactaactagactctcatccctcaaaactccacttaatcataaatcaggacaaaacatggctactggtgccattactaatgctaaaggtttcatgcccagcacgactgcctatcctttcaatgataattctagagaaaaagaaaactacatttacggaacttgttactacacagctagtgatcgcactgcttttcccattgacatatctgtcatgcttaaccgaagagcaataaatgacgagacatcatattgtattcgtataacttggtcctggaacacaggagatgccccagaggtgcaaacctctgctacaaccctagtcacctccccatttaccttttactacatcagagaagacgactgacaaataaagtttgcgatcgctaccctgcaggaacttgtttatttgaaaatcaattcacaaaatccgagtagttattttgcctcccccttcccatttaacagaatacaccaatctctccccacgcacagctttaaacatttggataccattagatatagacatggttttagattccacattccaaacagtttcagagcgagccaatctggggtcagtgatagataaaaatccatcgggatagtcttttaaagcgctttcacagtccaactgctgcggatgcgactccggagtctggatcacggtcatctggaagaagaacgatgggaatcataatccgaaaacggtatcggacgattgtgtctcatcaaacccacaagcagccgctgtctgcgtcgctccgtgcgactgctgtttatgggatcagggtccacagtgtcctgaagcatgattttaatagcccttaacatcaactttctggtgcgatgcgcgcagcaacgcattctgatttcactcaaatctttgcagtaggtacaacacattattacaatattgtttaataaaccataattaaaagcgctccagccaaaactcatatctgatataatcgcccctgcatgaccatcataccaaagtttaatataaattaaatgacgttccctcaaaaacacactacccacatacatgatctcttttggcatgtgcatattaacaatctgtctgtaccatggacaacgttggttaatcatgcaacccaatataaccttccggaaccacactgccaacaccgctcccccagccatgcattgaagtgaaccctgctgattacaatgacaatgaagaacccaattctctcgaccgtgaatcacttgagaatgaaaaatatctatagtggcacaacatagacataaatgcatgcatcttctcataatttttaactcctcaggatttagaaacatatcccagggaataggaagctcttgcagaacagtaaagctggcagaacaaggaagaccacgaacacaacttacactatgcatagtcatagtatcacaatctggcaacagcgggtggtcttcagtcatagaagctcgggtttcattttcctcacaacgtggtaactgggctctggtgtaagggtgatgtctggcgcatgatgtcgagcgtgcgcgcaaccttgtcataatggagttgcttcctgacattctcgtattttgtatagcaaaacgcggccctggcagaacacactcttcttcgccttctatcctgccgcttagcgtgttccgtgtgatagttcaagtacaaccacactcttaagttggtcaaaagaatgctggcttcagttgtaatcaaaactccatcgcatctaatcgttctgaggaaatcatccaagcaatgcaactggattgtgtttcaagcaggagaggagagggaagagacggaagaaccatgttaatttttattccaaacgatctcgcagtacttcaaattgtagatcgcgcagatggcatctctcgcccccactgtgttggtgaaaaagcacagctagatcaaaagaaatgcgattttcaaggtgctcaacggtggcttccagcaaagcctccacgcgcacatccaagaacaaaagaataccaaaagaaggagcattttctaactcctcaatcatcatattacattcctgcaccattcccagataattttcagctttccagccttgaattattcgtgtcagttcttgtggtaaatccaatccacacattacaaacaggtcccggagggcgccctccaccaccattcttaaacacaccctcataatgacaaaatatcttgctcctgtgtcacctgtagcgaattgagaatggcaacatcaattgacatgcccttggctctaagttcttctttaagttctagttgtaaaaactctctcatattatcaccaaactgcttagccagaagccccccgggaacaagagcaggggacgctacagtgcagtacaagcgcagacctccccaattggctccagcaaaaacaagattggaataagcatattgggaaccgccagtaatatcatcgaagttgctggaaatataatcaggcagagtttcttgtaaaaattgaataaaagaaaaatttgccaaaaaaacattcaaaacctctgggatgcaaatgcaataggttaccgcgctgcgctccaacattgttagttttgaattagtctgcaaaaataaaaaaaaaaacaagcgtcatatcatagtagcctgacgaacagatggataaatcagtctttccatcacaagacaagccacagggtctccagctcgaccctcgtaaaacctgtcatcatgattaaacaacagcaccgaaagttcctcgcggtgaccagcatgaataattcttgatgaagcatacaatccagacatgttagcatcagttaacgagaaaaaacagccaacatagcctttgggtataattatgcttaatcgtaagtatagcaaagccacccctcgcggatacaaagtaaaaggcacaggagaataaaaaatataattatttctctgctgctgttcaggcaacgtcgcccccggtccctctaaatacacatacaaagcctcatcagccatggcttaccagacaaagtacagcgggcacacaaagcacaagctctaaagtgactctccaacctctccacaatatatatatacacaagccctaaactgacgtaatgggagtaaagtgtaaaaaatcccgccaaacccaacacacaccccgaaactgcgtcaccagggaaaagtacagtttcacttccgcaatcccaacaggcgtaacttcctctttctcacggtacgtgatatcccactaacttgcaacgtcattttcccacggtcgcaccgccccttttagccgttaaccccacagccaatcaccacacgatccacactttttaaaatcacctcatttacatattggcaccattccatctataaggtatattatatagatagg

SEQ ID NO: 33 - DNA, 32458 bp, Artificial Sequence
  ColoAd2.0 genome
cgcgcctatctatataatataccttatagatggaatggtgccaatatgtaaatgaggtgattttaaaaagtgtggatcgtgtggtgattggctgtggggttaacggctaaaaggggcggtgcgaccgtgggaaaatgacgttttgtgggggtggagtttttttgcaagttgtcgcgggaaatgtgacgcataaaaaggcttttttctcacggaactacttagttttcccacggtatttaacaggaaatgaggtagttttgaccggatgcaagtgaaaattgttgattttcgcgcgaaaactgaatgaggaagtgtttttctgaataatgtggtatttatggcagggtggagtatttgttcagggccaggtagactttgacccattacgtggaggtttcgattaccgtgttttttacctgaatttccgcgtaccgtgtcaaagtcttctgtttttacgtaggtgtcagctgatcgctagggtatttatacctcagggtttgtgtcaagaggccactcttgagtgccagcgagaagagttttctcctctgcgccggcagtttaataataaaaaaatgagagatttgcgatttctgcctcaggaaataatctctgctgagactggaaatgaaatattggagcttgtggtgcacgccctgatgggagacgatccggagccacctgtgcagctttttgagcctcctacgcttcaggaactgtatgatttagaggtagagggatcggaggattctaatgaggaagctgtaaatggcttttttaccgattctatgcttttagctgctaatgaagggttagaattagatccgcctttggacacttttgatactccaggggtaattgtggaaagcggtacaggtgtaagaaaattacctgatttgagttccgtggactgtgatttgcactgctatgaagacgggtttcctccgagtgatgaggaggaccatgaaaaggagcagtccatgcagactgcagcgggtgagggagtgaaggctgccaatgttggttttcagttggattgcccggagcttcctggacatggctgtaagtcttgtgaatttcacaggaaaaatactggagtaaaggaactgttatgttcgctttgttatatgagaacgcactgccactttatttacagtaagtgtgtttaagttaaaatttaaaggaatatgctgtttttcacatgtatattgagtgtgagttttgtgcttcttattataggtcctgtgtctgatgctgatgaatcaccatctcctgattctactacctcacctcctgagattcaagcacctgttcctgtggacgtgcgcaagcccattcctgtgaagcttaagcctgggaaacgtccagcagtggaaaaacttgaggacttgttacagggtggggacggacctttggacttgagtacacggaaacgtccaagacaataagtgttccatatccgtgtttacttaaggtgacgtcaatatttgtgtgacagtgcaatgtaataaaaatatgttaactgttcactggtttttattgctttttgggcggggactcaggtatataagtagaagcagacctgtgtggttagctcataggagctggctttcatccatggaggtttgggccattttggaagaccttaggaagactaggcaactgttagagaacgcttcggacggagtctccggtttttggagattctggttcgctagtgaattagctagggtagtttttaggataaaacaggactataaacaagaatttgaaaagttgttggtagattgcccaggactttttgaagctcttaatttgggccatcaggttcactttaaagaaaaagttttatcagttttagacttttcaaccccaggtagaactgctgctgctgtggcttttcttacttttatattagataaatggatcccgcagactcatttcagcaggggatacgttttggatttcatagccacagcattgtggagaacatggaaggttcgcaagatgaggacaatcttaggttactggccagtgcagcctttgggtgtagcgggaatcctgaggcatccaccggtcatgccagcggttctggaggaggaacagcaagaggacaacccgagagccggcctggaccctccagtggaggaggcggagtagctgacttgtctcctgaactgcaacgggtgcttactggatctacgtccactggacgggataggggcgttaagagggagagggcatctagtggtactgatgctagatctgagttggctttaagtttaatgagtcgcagacgtcctgaaaccatttggtggcatgaggttcagaaagagggaagggatgaagtttctgtattgcaggagaaatattcactggaacaggtgaaaacatgttggttggagcctgaggatgattgggaggtggccattaaaaattatgccaagatagctttgaggcctgataaacagtataagattactagacggattaatatccggaatgcttgttacatatctggaaatggggctgaggtggtaatagatactcaagacaaggcagttattagatgctgcatgatggatatgtggcctggggtagtcggtatggaagcagtaacttttgtaaatgttaagtttaggggagatggttataatggaatagtgtttatggccaataccaaacttatattgcatggttgtagcttttttggtttcaacaatacctgtgtagatgcctggggacaggttagtgtacggggatgtagtttctatgcgtgttggattgccacagctggcagaaccaagagtcaattgtctctgaagaaatgcatatttcaaagatgtaacctgggcattctgaatgaaggcgaagcaagggtccgccactgcgcttctacagatactggatgttttattttgattaagggaaatgccagcgtaaagcataacatgatttgcggtgcttccgatgagaggccttatcaaatgctcacttgtgctggtgggcattgtaatatgctggctactgtgcatattgtttcccatcaacgcaaaaaatggcctgtttttgatcacaatgtgatgacgaagtgtaccatgcatgcaggtgggcgtagaggaatgtttatgccttaccagtgtaacatgaatcatgtgaaagtgttgttggaaccagatgccttttccagaatgagcctaacaggaatttttgacatgaacatgcaaatctggaagatcctgaggtatgatgatacgagatcgagggtacgcgcatgcgaatgcggaggcaagcatgccaggttccagccggtgtgtgtagatgtgactgaagatctcagaccggatcatttggttattgcccgcactggagcagagttcggatccagtggagaagaaactgactaaggtgagtattgggaaaactttggggtgggattttcagatggacagattgagtaaaaatttgttttttctgtcttgcagctgtcatgagtggaaacgcttcttttaaggggggagtcttcagcccttatctgacagggcgtctcccatcctgggcaggagttcgtcagaatgttatgggatctactgtggatggaagacccgtccaacccgccaattcttcaacgctgacctatgctactttaagttcttcacctttggacgcagctgcagctgccgccgccgcttctgttgccgctaacactgtgcttggaatgggttactatggaagcatcatggctaattccacttcctctaataacccttctaccctgactcaggacaagttacttgtccttttggcccagctggaggctttgacccaacgtctgggtgaactttctcagcaggtggtcgagttgcgagtacaaactgagtctgctgtcggcacggcaaagtctaaataaaaaaatcccagaatcaatgaataaataaacaagcttgttgttgatttaaaatcaagtgtttttatttcatttttcgcgcacggtatgccctagaccaccgatctctatcattgagaactcggtggattttttccaggatcctatagaggtgggattgaatgtttagatacatgggcattaggccgtctttggggtggagatagctccattgaagggattcatgctccggggtagtgttgtaaatcacccagtcataacaaggtcgcagtgcatggtgttgcacaatatcttttagaagtaggctgattgccacagataagcccttggtgtaggtgtttacaaaccggttgagctgggatgggtgcattcggggtgaaattatgtgcattttggattggatttttaagttggcaatattgccgccaagatcccgtcttgggttcatgttatgaaggaccaccaagacggtgtatccggtacatttaggaaatttatcgtgcagcttggatggaaaagcgtggaaaaatttggagacacccttgtgtcctccaagattttccatgcactcatccatgataatagcaatggggccgtgggcagcggcgcgggcaaacacgttccgtgggtctgacacatcatagttatgttcctgagttaaatcatcataagccattttaatgaatttggggcggagagtaccagattggggtatgaatgttccttcgggccccggagcatagttcccctcacagatttgcatttcccaagctttcagttccgagggtggaatcatgtccacctggggggctatgaaaaacaccgtttctggggcgggggtgattaattgtgatgatagcaaatttctgagcaattgagatttgccacatccggtggggccataaatgattccgattacgggttgcaggtggtagtttagggaacggcaactgccgtcttctcgaagcaagggggccacctcgttcatcatttcccttacatgcatattttcccgcaccaaatccattaggaggcgctctcctcctagtgatagaagttcttgtagtgaggaaaagtttttcagcggtttcagaccgtcagccatgggcattttggagagagtttgctgcaaaagttctagtctgttccacagttcagtgatgtgttctatggcatctcgatccagcagacctcctcgtttcgcgggtttggacggctcctggaatagggtatgagacgatgggcgtccagcgctgccagggttcggtccttccagggtctcagtgttcgagtcagggttgtttccgtcacagtgaaggggtgtgcgcctgcttgggcgcttgccagggtgcgcttcagactcatcctgctggtcgaaaacttctgtcgcttggcgccctgtatgtcggccaagtagcagtttaccatgagttcgtagttgagcgcctcggctgcgtggcctttggcgcggagcttacctttggaagttttcttgcataccgggcagtataggcatttcagcgcatacaacttgggcgcaaggaaaacggattctggggagtatgcatctgcgccgcaggaggcgcaaacagtttcacattccaccagccaggttaaatccggttcattggggtcaaaaacaagttttccgccatattttttgatgcgtttcttacctttggtctccatgagttcgtgtcctcgttgagtgacaaacaggctgtccgtgtccccgtagactgattttacaggcctcttctccagtggagtgcctcggtcttcttcgtacaggaactctgaccactctgatacaaaggcgcgcgtccaggccagcacaaaggaggctatgtgggaggggtagcgatcgttgtcaaccagggggtccaccttttccaaagtatgcaaacacatgtcaccctcttcaacatccaggaatgtgattggcttgtaggtgtatttcacgtgacctggggtccccgctgggggggtataaaagggggcggttctttgctcttcctcactgtcttccggatcgctgtccaggaacgtcagctgttggggtaggtattccctctcgaaggcgggcatgacctctgcactcaggttgtcagtttctaagaacgaggaggatttgatattgacagtgccggttgagatgcctttcatgaggttttcgtccatctggtcagaaaacacaatttttttattgtcaagtttggtggcaaatgatccatacagggcgttggataaaagtttggcaatggatcgcatggtttggttcttttccttgtccgcgcgctctttggcggcgatgttgagttggacatactcgcgtgccaggcacttccattcggggaagatagttgttaattcatctggcacgattctcacttgccaccctcgattatgcaaggtaattaaatccacactggtggccacctcgcctcgaaggggttcattggtccaacagagcctacctcctttcctagaacagaaagggggaagtgggtctagcataagttcatcgggagggtctgcatccatggtaaagattcccggaagtaaatccttatcaaaatagctgatgggagtggggtcatctaaggccatttgccattctcgagctgccagtgcgcgctcatatgggttaaggggactgccccatggcatgggatgggtgagtgcagaggcatacatgccacagatgtcatagacgtagatgggatcctcaaagatgcctatgtaggttggatagcatcgcccccctctgatacttgctcgcacatagtcatatagttcatgtgatggcgctagcagccccggacccaagttggtgcgattgggtttttctgttctgtagacgatctggcgaaagatggcgtgagaattggaagagatggtgggtctttgaaaaatgttgaaatgggcatgaggtagacctacagagtctctgacaaagtgggcataagattcttgaagcttggttaccagttcggcggtgacaagtacgtctagggcgcagtagtcaagtgtttcttgaatgatgtcataacctggttggtttttcttttcccacagttcgcggttgagaaggtattcttcgcgatccttccagtactcttctagcggaaacccgtctttgtctgcacggtaagatcctagcatgtagaactgattaactgccttgtaagggcagcagcccttctctacgggtagagagtatgcttgagcagcttttcgtagcgaagcgtgagtaagggcaaaggtgtctctgaccatgactttgaggaattggtatttgaagtcgatgtcgtcacaggctccctgttcccagagttggaagtctacccgtttcttgtaggcggggttgggcaaagcgaaagtaacatcattgaagagaatcttgccggccctgggcatgaaattgcgagtgatgcgaaaaggctgtggtacttccgctcggttattgataacctgggcagctaggacgatctcgtcgaaaccgttgatgttgtgtcctacgatgtataattctatgaaacgcggcgtgcctctgacgtgaggtagcttactgagctcatcaaaggttaggtctgtggggtcagataaggcgtagtgttcgagagcccattcgtgcaggtgaggattcgctttaaggaaggaggaccagaggtccactgccagtgctgtttgtaactggtcccggtactgacgaaaatgccgtccgactgccattttttctggggtgacgcaatagaaggtttgggggtcctgccgccagcgatcccacttgagttttatggcgaggtcataggcgatgttgacgagccgctggtctccagagagtttcatgaccagcatgaaggggattagctgcttgccaaaggaccccatccaggtgtaggtttccacatcgtaggtgagaaagagcctttctgtgcgaggatgagagccaatcgggaagaactggatctcctgccaccagttggaggaatggctgttgatgtgatggaagtagaactccctgcgacgcgccgagcattcatgcttgtgcttgtacagacggccgcagtagtcgcagcgttgcacgggttgtatctcgtgaatgagttgtacctggcttcccttgacgagaaatttcagtgggaagccgaggcctggcgattgtatctcgtgctttactatgttgtctgcatcggcctgttcatcttctgtctcgatggtggtcatgctgacgagccctcgcgggaggcaagtccagacctcggcgcggcaggggcggagctcgaggacgagagcgcgcaggctggagctgtccagggtcctgagacgctgcggactcaggttagtaggcagtgtcaggagattaacttgcatgatcttttggagggcgtgcgggaggttcagatagtacttgatctcaacgggtccgttggtggagatgtcgatggcttgcagggttccgtgtcccttgggcgctaccaccgtgcccttgtttttcattttggacggcggtggctctgttgcttcttgcatgtttagaagcggtgtcgagggcgcgcaccgggcggcaggggcggctcgggacccggcggcatggctggcagtggtacgtcggcgccgcgcgcgggtaggttctggtactgcgccctgagaagactcgcatgcgcgacgacgcggcggttgacatcctggatctgacgcctctgggtgaaagctaccggccccgtgagcttgaacctgaaagagagttcaacagaatcaatctcggtatcgttgacggcggcttgcctaaggatttcttgcacgtcaccagagttgtcctggtaggcgatctccgccatgaactgctcgatctcttcctcttgaagatctccgcggcccgctctctcgacggtggccgcgaggtcgttggagatgcgcccaatgagttgagagaatgcattcatgcccgcctcgttccagacgcggctgtagaccacggcccccacgggatctctcgcgcgcatgaccacctgggcgaggttgagctccacgtggcgggtgaagaccgcatagttgcataggcgctggaaaaggtagttgagtgtggtggcgatgtgctcggtgacgaagaaatacatgatccatcgtctcagcggcatctcgctgacatcgcccagagcttccaagcgctccatggcctcgtagaagtccacggcaaaattaaaaaactgggagtttcgcgcggacacggtcaactcctcttccagaagacggataagttcggcgatggtggtgcgcacctcgcgctcgaaagcccctgggatttcttcctcaatctcttcttcttccactaacatctcttcctcttcaggtggggctgcaggaggagggggaacgcggcgacgccggcggcgcacgggcagacggtcgatgaatctttcaatgacctctccgcggcggcggcgcatggtttcagtgacggcgcggccgttctcgcgcggtcgcagagtaaaaacaccgccgcgcatctccttaaagtggtgactgggaggttctccgtttgggagggagagggcgctgattatacattttattaattggcccgtagggactgcacgcagagatctgatcgtgtcaagatccacgggatctgaaaacctttcgacgaaagcgtctaaccagtcacagtcacaaggtaggctgagtacggcttcttgtgggcgggggtggttatgtgttcggtctgggtcttctgtttcttcttcatctcgggaaggtgagacgatgctgctggtgatgaaattaaagtaggcagttctaagacggcggatggtggcgaggagcaccaggtctttgggtccggcttgctggatacgcaggcgattggccattccccaagcattatcctgacatctagcaagatctttgtagtagtcttgcatgagccgttctacgggcacttcttcctcacccgttctgccatgcatacgtgtgagtccaaatccgcgcattggttgtaccagtgccaagtcagctacgactctttcggcgaggatggcttgctgtacttgggtaagggtggcttgaaagtcatcaaaatccacaaagcggtggtaagctcctgtattaatggtgtaagcacagttggccatgactgaccagttaactgtctggtgaccagggcgcacgagctcggtgtatttaaggcgcgaataggcgcgggtgtcaaagatgtaatcgttgcaggtgcgcaccagatactggtaccctataagaaaatgcggcggtggttggcggtagagaggccatcgttctgtagctggagcgccaggggcgaggtcttccaacataaggcggtgatagccgtagatgtacctggacatccaggtgattcctgcggcggtagtagaagcccgaggaaactcgcgtacgcggttccaaatgttgcgtagcggcatgaagtagttcattgtaggcacggtttgaccagtgaggcgcgcgcagtcattgatgctctatagacacggagaaaatgaaagcgttcagcgactcgactccgtagcctggaggaacgtgaacgggttgggtcgcggtgtaccccggttcgagacttgtactcgagccggccggagccgcggctaacgtggtattggcactcccgtctcgacccagcctacaaaaatccaggatacggaatcgagtcgttttgctggtttccgaatggcagggaagtgagtcctattttttttttttgccgctcagatgcatcccgtgctgcgacagatgcgcccccaacaacagcccccctcgcagcagcagcagcagcaatcacaaaaggctgtccctgcaactactgcaactgccgccgtgagcggtgcgggacagcccgcctatgatctggacttggaagagggcgaaggactggcacgtctaggtgcgccttcacccgagcggcatccgcgagttcaactgaaaaaagattctcgcgaggcgtatgtgccccaacagaacctatttagagacagaagcggcgaggagccggaggagatgcgagcttcccgctttaacgcgggtcgtgagctgcgtcacggtttggaccgaagacgagtgttgcgggacgaggatttcgaagttgatgaaatgacagggatcagtcctgccagggcacacgtggctgcagccaaccttgtatcggcttacgagcagacagtaaaggaagagcgtaacttccaaaagtcttttaataatcatgtgcgaaccctgattgcccgcgaagaagttacccttggtttgatgcatttgtgggatttgatggaagctatcattcagaaccctactagcaaacctctgaccgcccagctgtttctggtggtgcaacacagcagagacaatgaggctttcagagaggcgctgctgaacatcaccgaacccgaggggagatggttgtatgatcttatcaacattctacagagtatcatagtgcaggagcggagcctgggcctggccgagaaggtggctgccatcaattactcggttttgagcttgggaaaatattacgctcgcaaaatctacaagactccatacgttcccatagacaaggaggtgaagatagatgggttctacatgcgcatgacgctcaaggtcttgaccctgagcgatgatcttggggtgtatcgcaatgacagaatgcatcgcgcggttagcgccagcaggaggcgcgagttaagcgacagggaactgatgcacagtttgcaaagagctctgactggagctggaaccgagggtgagaattacttcgacatgggagctgacttgcagtggcagcctagtcgcagggctctgagcgccgcgacggcaggatgtgagcttccttacatagaagaggcggatgaaggcgaggaggaagagggcgagtacttggaagactgatggcacaacccgtgttttttgctagatggaacagcaagcaccggatcccgcaatgcgggcggcgctgcagagccagccgtccggcattaactcctcggacgattggacccaggccatgcaacgtatcatggcgttgacgactcgcaaccccgaagcctttagacagcaaccccaggccaaccgtctatcggccatcatggaagctgtagtgccttcccgctctaatcccactcatgagaaggtcctggccatcgtgaacgcgttggtggagaacaaagctattcgtccagatgaggccggactggtatacaacgctctcttagaacgcgtggctcgctacaacagtagcaatgtgcaaaccaatttggaccgtatgataacagatgtacgcgaagccgtgtctcagcgcgaaaggttccagcgtgatgccaacctgggttcgctggtggcgttaaatgctttcttgagtactcagcctgctaatgtgccgcgtggtcaacaggattatactaactttttaagtgctttgagactgatggtatcagaagtacctcagagcgaagtgtatcagtccggtcctgattacttctttcagactagcagacagggcttgcagacggtaaatctgagccaagcttttaaaaacctttaaaggtttgtggggagtgcatgccccggtaggagaaagagcaaccgtgtctagcttgttaactccgaactcccgcctattattactgttggtagctcctttcaccgacagcggtagcatcgaccgtaattcctatttgggttacctactaaacctgtatcgcgaagccatagggcaaagtcaggtggacgagcagacctatcaagaaattacccaagtcagtcgcgctttgggacaggaagacactggcagtttggaagccactctgaacttcttgcttaccaatcggtctcaaaagatccctcctcaatatgctcttactgcggaggaggagaggatccttagatatgtgcagcagagcgtgggattgtttctgatgcaagagggggcaactccgactgcagcactggacatgacagcgcgaaatatggagcccagcatgtatgccagtaaccgacctttcattaacaaactgctggactacttgcacagagctgccgctatgaactctgattatttcaccaatgccatcttaaacccgcactggctgcccccacctggtttctacacgggcgaatatgacatgcccgaccctaatgacggatttctgtgggacgacgtggacagcgatgttttttcacctctttctgatcatcgcacgtggaaaaaggaaggcggcgatagaatgcattcttctgcatcgctgtccggggtcatgggtgctaccgcggctgagcccgagtctgcaagtccttttcctagtctacccttttctctacacagtgtacgtagcagcgaagtgggtagaataagtcgcccgagtttaatgggcgaagaggagtatctaaacgattccttgctcagaccggcaagagaaaaaaatttcccaaacaatggaatagaaagtttggtggataaaatgagtagatggaagacttatgctcaggatcacagagacgagcctgggatcatggggattacaagtagagcgagccgtagacgccagcgccatgacagacagaggggtcttgtgtgggacgatgaggattcggccgatgatagcagcgtgctggacttgggtgggagaggaaggggcaacccgtttgctcatttgcgccctcgcttgggtggtatgttgtaaaaaaaaataaaaaaaaaactcaccaaggccatggcgacgagcgtacgttcgttcttctttattatctgtgtctagtataatgaggcgagtcgtgctaggcggagcggtggtgtatccggagggtcctcctccttcgtacgagagcgtgatgcagcagcagcaggcgacggcggtgatgcaatccccactggaggctccctttgtgcctccgcgatacctggcacctacggagggcagaaacagcattcgttattcggaactggcacctcagtacgataccaccaggttgtatctggtggacaacaagtcggcggacattgcttctctgaactatcagaatgaccacagcaacttcttgaccacggtggtgcaaaacaatgactttacccctacggaagccagcacccagaccattaactttgatgaacgatcgcggtggggcggtcagctaaagaccatcatgcatactaacatgccaaacgtgaacgagtatatgtttagtaacaagttcaaagcgcgtgtgatggtgtccagaaaacctcccgacggtgctgcagttggggatacttatgatcacaagcaggatattttgaaatatgagtggttcgagtttactttgccagaaggcaacttttcagttactatgactattgatttgatgaacaatgccatcatagataattacttgaaagtgggtagacagaatggagtgcttgaaagtgacattggtgttaagttcgacaccaggaacttcaagctgggatgggatcccgaaaccaagttgatcatgcctggagtgtatacgtatgaagccttccatcctgacattgtcttactgcctggctgcggagtggattttaccgagagtcgtttgagcaaccttcttggtatcagaaaaaaacagccatttcaagagggttttaagattttgtatgaagatttagaaggtggtaatattccggccctcttggatgtagatgcctatgagaacagtaagaaagaacaaaaagccaaaatagaagctgctacagctgctgcagaagctaaggcaaacatagttgccagcgactctacaagggttgctaacgctggagaggtcagaggagacaattttgcgccaacacctgttccgactgcagaatcattattggccgatgtgtctgaaggaacggacgtgaaactcactattcaacctgtagaaaaagatagtaagaatagaagctataatgtgttggaagacaaaatcaacacagcctatcgcagttggtatctttcgtacaattatggcgatcccgaaaaaggagtgcgttcctggacattgctcaccacctcagatgtcacctgcggagcagagcaggtctactggtcgcttccagacatgatgaaggatcctgtcactttccgctccactagacaagtcagtaactaccctgtggtgggtgcagagcttatgcccgtcttctcaaagagcttctacaacgaacaagctgtgtactcccagcagctccgccagtccacctcgcttacgcacgtcttcaaccgctttcctgagaaccagattttaatccgtccgccggcgcccaccattaccaccgtcagtgaaaacgttcctgctctcacagatcacgggaccctgccgttgcgcagcagtatccggggagtccaacgtgtgaccgttactgacgccagacgccgcacctgtccctacgtgtacaaggcactgggcatagtcgcaccgcgcgtcctttcaagccgcactttctaaaaaaaaaaaaaatgtccattcttatctcgcccagtaataacaccggttggggtctgcgcgctccaagcaagatgtacggaggcgcacgcaaacgttctacccaacatcctgtccgtgttcgcggacattttcgcgctccatggggcgccctcaagggccgcactcgcgttcgaaccaccgtcgatgatgtaatcgatcaggtggttgccgacgcccgtaattatactcctactgcgcctacatctactgtggatgcagttattgacagtgtagtggctgacgctcgcaactatgctcgacgtaagagccggcgaaggcgcattgccagacgccaccgagctaccactgccatgcgagccgcaagagctctgctacgaagagctagacgcgtggggcgaagagccatgcttagggcggccagacgtgcagcttcgggcgccagcgccggcaggtcccgcaggcaagcagccgctgtcgcagcggcgactattgccgacatggcccaatcgcgaagaggcaatgtatactgggtgcgtgacgctgccaccggtcaacgtgtacccgtgcgcacccgtccccctcgcacttagaagatactgagcagtctccgatgttgtgtcccagcggcgaggatgtccaagcgcaaatacaaggaagaaatgctgcaggttatcgcacctgaagtctacggccaaccgttgaaggatgaaaaaaaaccccgcaaaatcaagcgggttaaaaaggacaaaaaagaagaggaagatggcgatgatgggctggcggagtttgtgcgcgagtttgccccacggcgacgcgtgcaatggcgtgggcgcaaagttcgacatgtgttgagacctggaacttcggtggtctttacacccggcgagcgttcaagcgctacttttaagcgttcctatgatgaggtgtacggggatgatgatattcttgagcaggcggctgaccgattaggcgagtttgcttatggcaagcgtagtagaataacttccaaggatgagacagtgtcgatacccttggatcatggaaatcccacccctagtcttaaaccggtcactttgcagcaagtgttacccgtaactccgcgaacaggtgttaaacgcgaaggtgaagatttgtatcccactatgcaactgatggtacccaaacgccagaagttggaggacgttttggagaaagtaaaagtggatccagatattcaacctgaggttaaagtgagacccattaagcaggtagcgcctggtctgggggtacaaactgtagacattaagattcccactgaaagtatggaagtgcaaactgaacccgcaaagcctactgccacctccactgaagtgcaaacggatccatggatgcccatgcctattacaactgacgccgccggtcccactcgaagatcccgacgaaagtacggtccagcaagtctgttgatgcccaattatgttgtacacccatctattattcctactcctggttaccgaggcactcgctactatcgcagccgaaacagtacctcccgccgtcgccgcaagacacctgcaaatcgcagtcgtcgccgtagacgcacaagcaaaccgactcccggcgccctggtgcggcaagtgtaccgcaatggtagtgcggaacctttgacactgccgcgtgcgcgttaccatccgagtatcatcacttaatcaatgttgccgctgcctccttgcagatatggccctcacttgtcgccttcgcgttcccatcactggttaccgaggaagaaactcgcgccgtagaagagggatgttgggacgcggaatgcgacgctacaggcgacggcgtgctatccgcaagcaattgcggggtggttttttaccagccttaattccaattatcgctgctgcaattggcgcgataccaggcatagcttccgtggcggttcaggcctcgcaacgacattgacattggaaaaaaacgtataaataaaaaaaaaaaaatacaatggactctgacactcctggtcctgtgactatgttttcttagagatggaagacatcaatttttcatccttggctccgcgacacggcacgaagccgtacatgggcacctggagcgacatcggcacgagccaactgaacgggggcgccttcaattggagcagtatctggagcgggcttaaaaattttggctcaaccataaaaacatacgggaacaaagcttggaacagcagtacaggacaggcgcttagaaataaacttaaagaccagaacttccaacaaaaagtagtcgatgggatagcttccggcatcaatggagtggtagatttggctaaccaggctgtgcagaaaaagataaacagtcgtttggacccgccgccagcaaccccaggtgaaatgcaagtggaggaagaaattcctccgccagaaaaacgaggcgacaagcgtccgcgtcccgatttggaagagacgctggtgacgcgcgtagatgaaccgccttcttatgaggaagcaacgaagcttggaatgcccaccactagaccgatagccccaatggccaccggggtgatgaaaccttctcagttgcatcgacccgtcaccttggatttgccccctccccctgctgctactgctgtacccgcttctaagcctgtcgctgccccgaaaccagtcgccgtagccaggtcacgtcccgggggcgctcctcgtccaaatgcgcactggcaaaatactctgaacagcatcgtgggtctaggcgtgcaaagtgtaaaacgccgtcgctgcttttaattaaatatggagtagcgcttaacttgcctatctgtgtatatgtgtcattacacgccgtcacagcagcagaggaaaaaaggaagaggtcgtgcgtcgacgctgagttactttcaagatggccaccccatcgatgctgccccaatgggcatacatgcacatcgccggacaggatgcttcggagtacctgagtccgggtctggtgcagttcgcccgcgccacagacacctacttcaatctgggaaataagtttagaaatcccaccgtagcgccgacccacgatgtgaccaccgaccgtagccagcggctcatgttgcgcttcgtgcccgttgaccgggaggacaatacatactcttacaaagtgcggtacaccctggccgtgggcgacaacagagtgctggatatggccagcacgttctttgacattaggggtgtgttggacagaggtcccagtttcaaaccctattctggtacggcttacaactccctggctcctaaaggcgctccaaatacatctcagtggattgcagaaggtgtaaaaaatacaactggtgaggaacacgtaacagaagaggaaaccaatactactacttacacttttggcaatgctcctgtaaaagctgaagctgaaattacaaaagaaggactcccagtaggtttggaagtttcagatgaagaaagtaaaccgatttatgctgataaaacatatcagccagaacctcagctgggagatgaaacttggactgaccttgatggaaaaaccgaaaagtatggaggcagggctctcaaacccgatactaagatgaaaccatgctacgggtcctttgccaaacctactaatgtgaaaggcggtcaggcaaaacaaaaaacaacggagcagccaaatcagaaagtcgaatatgatatcgacatggagttttttgatgcggcatcgcagaaaacaaacttaagtcctaaaattgtcatgtatgcagaaaatgtaaatttggaaactccagacactcatgtagtgtacaaacctggaacagaagacacaagttccgaagctaatttgggacaacaatctatgcccaacagacccaactacattggcttcagagataactttattggacttatgtactataacagtactggtaacatgggggtgctggctggtcaagcgtctcagttaaatgcagtggttgacttgcaggacagaaacacagaactttcttaccaactcttgcttgactctctgggcgacagaaccagatactttagcatgtggaatcaggctgtggacagttatgatcctgatgtacgtgttattgaaaatcatggtgtggaagatgaacttcccaactactgttttccactggacggcataggtgttccaacaaccagttacaaatcaatagttccaaatggagacaatgcgcctaattggaaggaacctgaagtaaatggaacaagtgagatcggacagggtaatttgtttgccatggaaattaaccttcaagccaatctatggcgaagtttcctttattccaatgtggctctatatctcccagactcgtacaaatacaccccgtccaatgtcactcttccagaaaacaaaaacacctacgactacatgaacgggcgggtggtgccgccatctctagtagacacctatgtgaacattggtgccaggtggtctctggatgccatggacaatgtcaacccattcaaccaccaccgtaacgctggcttgcgttaccgatccatgcttctgggtaacggacgttatgtgcctttccacatacaagtgcctcaaaaattcttcgctgttaaaaacctgctgcttctcccaggctcctacacttatgagtggaactttaggaaggatgtgaacatggttctacagagttccctcggtaacgacctgcgggtagatggcgccagcatcagtttcacgagcatcaacctctatgctacttttttccccatggctcacaacaccgcttccacccttgaagccatgctgcggaatgacaccaatgatcagtcattcaacgactacctatctgcagctaacatgctctaccccattcctgccaatgcaaccaatattcccatttccattccttctcgcaactgggcggctttcagaggctggtcatttaccagactgaaaaccaaagaaactccctctttggggtctggatttgacccctactttgtctattctggttctattccctacctggatggtaccttctacctgaaccacacttttaagaaggtttccatcatgtttgactcttcagtgagctggcctggaaatgacaggttactatctcctaacgaatttgaaataaagcgcactgtggatggcgaaggctacaacgtagcccaatgcaacatgaccaaagactggttcttggtacagatgctcgccaactacaacatcggctatcagggcttctacattccagaaggatacaaagatcgcatgtattcatttttcagaaacttccagcccatgagcaggcaggtggttgatgaggtcaattacaaagacttcaaggccgtcgccataccctaccaacacaacaactctggctttgtgggttacatggctccgaccatgcgccaaggtcaaccctatcccgctaactatccctatccactcattggaacaactgccgtaaatagtgttacgcagaaaaagttcttgtgtgacagaaccatgtggcgcataccgttctcgagcaacttcatgtctatgggggcccttacagacttgggacagaatatgctctatgccaactcagctcatgctctggacatgacctttgaggtggatcccatggatgagcccaccctgctttatcttctcttcgaagttttcgacgtggtcagagtgcatcagccacaccgcggcatcatcgaggcagtctacctgcgtacaccgttctcggccggtaacgctaccacgtaagaagcttcttgcttcttgcaaatagcagctgcaaccatggcctgcggatcccaaaacggctccagcgagcaagagctcagagccattgtccaagacctgggttgcggaccctattttttgggaacctacgataagcgcttcccggggttcatggcccccgataagctcgcctgtgccattgtaaatacggccggacgtgagacggggggagagcactggttggctttcggttggaacccacgttctaacacctgctacctttttgatccttttggattctcggatgatcgtctcaaacagatttaccagtttgaatatgagggtctcctgcgccgcagcgctcttgctaccaaggaccgctgtattacgctggaaaaatctacccagaccgtgcagggtccccgttctgccgcctgcggacttttctgctgcatgttccttcacgcctttgtgcactggcctgaccgtcccatggacggaaaccccaccatgaaattgctaactggagtgccaaacaacatgcttcattctcctaaagtccagcccaccctgtgtgacaatcaaaaagcactctaccattttcttaatacccattcgccttattttcgctcccatcgtacacacatcgaaagggccactgcgttcgaccgtatggatgttcaataatgactcatgtaaacaacgtgttcaataaacatcactttatttttttacatgtatcaaggctctgcattacttatttatttacaagtcgaatgggttctgacgagaatcagaatgacccgcaggcagtgatacgttgcggaactgatacttgggttgccacttgaattcgggaatcaccaacttgggaaccggtatatcgggcaggatgtcactccacagctttctggtcagctgcaaagctccaagcaggtcaggagccgaaatcttgaaatcacaattaggaccagtgctttgagcgcgagagttgcggtacaccggattgcagcactgaaacaccatcagcgacggatgtctcacgcttgccagcacggtgggatctgcaatcatgcccacatccagatcttcagcattggcaatgctgaacggggtcatcttgcaggtctgcctacccatggcgggcacccaattaggcttgtggttgcaatcgcagtgcagggggatcagtatcatcttggcctgatcctgtctgattcctggatacacggctctcatgaaagcatcatattgcttgaaagcctgctgggctttactaccctcggtataaaacatcccgcaggacctgctcgaaaactggttagctgcacagccggcatcattcacacagcagcgggcgtcattgttagctatttgcaccacacttctgccccagcggttttgggtgattttggttcgctcgggattctcctttaaggctcgttgtccgttctcgctggccacatccatctcgataatctgctccttctgaatcataatattgccatgcaggcacttcagcttgccctcataatcattgcagccatgaggccacaacgcacagcctgtacattcccaattatggtgggcgatctgagaaaaagaatgtatcattccctgcagaaatcttcccatcatcgtgctcagtgtcttgtgactagtgaaagttaactggatgcctcggtgctcctcgtttacgtactggtgacagatgcgcttgtattgttcgtgttgctcaggcattagtttaaaagaggttctaagttcgttatccagcctgtacttctccatcagcagacacatcacttccatgcctttctcccaagcagacaccaggggcaagctaatcggattcttaacagtgcaggcagcagctcctttagccagagggtcatctttagcgatcttctcaatgcttcttttgccatccttctcaacgatgcgcacgggcgggtagctgaaacccactgctacaagttgcgcctcttctctttcttcttcgctgtcttgactgatgtcttgcatggggatatgtttggtcttccttggcttctttttggggggtatcggaggaggaggactgtcgctccgttccggagacagggaggattgtgacgtttcgctcaccattaccaactgactgtcggtagaagaacctgaccccacacggcgacaggtgtttctcttcgggggcagaggtggaggcgattgcgaagggctgcggtccgacctggaaggcggatgactggcagaaccccttccgcgttcgggggtgtgctccctgtggcggtcgcttaactgatttccttcgcggctggccattgtgttctcctaggcagagaaacaacagacatggaaactcagccattgctgtcaacatcgccacgagtgccatcacatctcgtcctcagcgacgaggaaaaggagcagagcttaagcattccaccgcccagtcctgccaccacctctaccctagaagataaggaggtcgacgcatctcatgacatgcagaataaaaaagcgaaagagtctgagacagacatcgagcaagacccgggctatgtgacaccggtggaacacgaggaagagttgaaacgctttctagagagagaggatgaaaactgcccaaaacaacgagcagataactatcaccaagatgctggaaatagggatcagaacaccgactacctcatagggcttgacggggaagacgcgctccttaaacatctagcaagacagtcgctcatagtcaaggatgcattattggacagaactgaagtgcccatcagtgtggaagagctcagccgcgcctacgagcttaacctcttttcacctcgtactccccccaaacgtcagccaaacggcacctgcgagccaaatcctcgcttaaacttttatccagcttttgctgtgccagaagtactggctacctatcacatcttttttaaaaatcaaaaaattccagtctcctgccgcgctaatcgcacccgcgccgatgccctactcaatctgggacctggttcacgcttacctgatatagcttccttggaagaggttccaaagatcttcgagggtctgggcaataatgagactcgggccgcaaatgctctgcaaaagggagaaaatggcatggatgagcatcacagcgttctggtggaattggaaggcgataatgccagactcgcagtactcaagcgaagcatcgaggtcacacacttcgcatatcccgctgtcaacctgccccctaaagtcatgacggcggtcatggaccagttactcattaagcgcgcaagtcccctttcagaagacatgcatgacccagatgcctgtgatgagggtaaaccagtggtcagtgatgagcagctaacccgatggctgggcaccgactctcccagggatttggaagagcgtcgcaagcttatgatggccgtggtgctggttaccgtagaactagagtgtctccgacgtttctttaccgattcagaaaccttgcgcaaactcgaagagaatctgcactacacttttagacacggctttgtgcggcaggcatgcaagatatctaacgtggaactcaccaacctggtttcctacatgggtattctgcatgagaatcgcctaggacaaagcgtgctgcacagcaccctgaagggggaagcccgccgtgattacatccgcgattgtgtctatctgtacctgtgccacacgtggcaaaccggcatgggtgtatggcagcaatgtttagaagaacagaacttgaaagagcttgacaagctcttacagaaatctcttaaggttctgtggacagggttcgacgagcgcaccgtcgcttccgacctggcagacctcatcttcccagagcgtctcagggttactttgcgaaacggattgcctgactttatgagccagagcatgcttaacaattttcgctctttcatcctggaacgctccggtatcctgcccgccacctgctgcgcactgccctccgactttgtgcctctcacctaccgcgagtgccccccgccgctatggagtcactgctacctgttccgtctggccaactatctctcctaccactcggatgtgatcgaggatgtgagcggagacggcttgctggagtgtcactgccgctgcaatctgtgcacgccccaccggtccctagcttgcaacccccagttgatgagcgaaacccagataataggcacctttgaattgcaaggccccagcagccaaggcgatgggtcttctcctgggcaaagtttaaaactgaccccgggactgtggacctccgcctacttgcgcaagtttgctccggaagattaccacccctatgaaatcaagttctatgaggaccaatcacagcctccaaaggccgaactttcggcctgcgtcatcacccagggggcaattctggcccaattgcaagccatccaaaaatcccgccaagaatttctactgaaaaagggtaagggggtctaccttgacccccagaccggcgaggaactcaacacaaggttccctcaggatgtcccaacgacgagaaaacaagaagttgaaggtgcagccgccgcccccagaagatatggaggaagattgggacagtcaggcagaggaggcggaggaggacagtctggaggacagtctggaggaagacagtttggaggaggaaaacgaggaggcagaggaggtggaagaagtaaccgccgacaaacagttatcctcggctgcggagacaagcaacagcgctaccatctccgctccgagtcgaggaacccggcggcgtcccagcagtagatgggacgagaccggacgcttcccgaacccaaccagcgcttccaagaccggtaagaaggatcggcagggatacaagtcctggcgggggcataagaatgccatcatctcctgcttgcatgagtgcgggggcaacatatccttcacgcggcgctacttgctattccaccatggggtgaactttccgcgcaatgttttgcattactaccgtcacctccacagcccctactatagccagcaaatcccggcagtctcgacagataaagacagcggcggcgacctccaacagaaaaccagcagcggcagttagaaaatacacaacaagtgcagcaacaggaggattaaagattacagccaacgagccagcgcaaacccgagagttaagaaatcggatctttccaaccctgtatgccatcttccagcagagtcggggtcaagagcaggaactgaaaataaaaaaccgatctctgcgttcgctcaccagaagttgtttgtatcacaagagcgaagatcaacttcagcgcactctcgaggacgccgaggctctcttcaacaagtactgcgcgctgactcttaaagagtaggcagcgaccgcgcttattcaaaaaaggcgggaattacatcatcctcgacatgagtaaagaaattcccacgccttacatgtggagttatcaaccccaaatgggattggcggcaggcgcctcccaggactactccacccgcatgaattggctcagcgccgggccttctatgatttctcgagttaatgatatacgcgcctaccgaaaccaaatacttttggaacagtcagctcttaccaccacgccccgccaacaccttaatcccagaaattggcccgccgccctagtgtaccaggaaagtcccgctcccaccactgtattacttcctcgagacgcccaggccgaagtccaaatgactaatgcaggtgcgcagttagctggcggctccaccctatgtcgtcacaggcctcggcataatataaaacgcctgatgatcagaggccgaggtatccagctcaacgacgagtcggtgagctctccgcttggtctacgaccagacggaatctttcagattgccggctgcgggagatcttccttcacccctcgtcaggctgttctgactttggaaagttcgtcttcgcaaccccgctcgggcggaatcgggaccgttcaatttgtggaggagtttactccctctgtctacttcaaccccttctccggatctcctgggcattacccggacgagttcataccgaacttcgacgcgattagcgagtcagtggacggctacgattgatgtctggtgacgcggctgagctatctcggctgcgacatctagaccactgccgccgctttcgctgctttgcccgggaactcattgagttcatctacttcgaactccccaaggatcaccctcaaggtccggcccacggagtgcggatttctatcgaaggcaaaatagactctcgcctgcaacgaattttctcccagcggcccgtgctgatcgagcgagaccagggaaacaccacggtttccatctactgcatttgtaatcaccccggattgcatgaaagcctttgctgtcttatgtgtactgagtttaataaaaactgaattaagactctcctacggactgccgcttcttcaacccggattttacaaccagaagaacgaaacttttcctgtcgtccaggactctgttaacttcacctttcctactcacaaactagaagctcaacgactacaccgcttttccagaagcattttccctactaatactactttcaaaaccggaggtgagctccaaggtcttcctacagaaaacccttgggtggaagcgggccttgtagtgctaggaattcttgcgggtgggcttgtgattattctttgctacctatacacaccttgcttcactttcttagtggtgttgtggtattggtttaaaaaatggggcccatactagtcttgcttgttttactttcgcttttggaaccgggttctgccaattacgatccatgtctagacttcgacccagaaaactgcacacttacttttgcacccgacacaagccgcatctgtggagttcatcgcctctcttacgaacttggcccccaacgacaaaaatttacctgcatggtgggaatcaaccccatagttatcacccagcaaagtggagatactaagggttgcattcactgctcctgcgattccatcgagtgcacctacaccctgctgaagaccctatgcggcctaagagacctgctaccaatgaattaaaaaatgattaataaaaaatcacttacttgaaatcagcaataaggtctctgttgaaattttctcccagcagcacctcacttccctcttcccaactctggtattctaaaccccgttcagcggcatactttctccatactttaaaggggatgtcaaattttagctcctctcctgtacccacaatcttcatgtctttcttcccagtggccggccatgaccaagagagtccggctcagtgactccttcaaccctgtctacccctatgaagatgaaagcacctcccaacacccctttataaacccagggtttatttccccaaatggcttcacacaaagcccaaacggagttcttactttaaaatgtttaaccccactaacaaccacaggcggatctctacagctaaaagtgggagggggacttacagtggatgacaccaacggttttttgaaagaaaacataagtgccaccacaccactcgttaagactggtcactctataggtttaccactaggagccggattgggaacgaatgaaaataaactttgtatcaaattaggacaaggacttacattcaattcaaacaacatttgcattgatgacaatattaacaccttatggacaggagtcaaccccaccgaagccaactgtcaaatcatgaactccagtgaatctaatgattgcaaattaattctaacactagttaaaactggagcactagtcactgcatttgtttatgttataggagtatctaacaattttaatatgctaactacacacagaaatataaattttactgcagagctgtttttcgattctactggtaatttactaactagactctcatccctcaaaactccacttaatcataaatcaggacaaaacatggctactggtgccattactaatgctaaaggtttcatgcccagcacgactgcctatcctttcaatgataattctagagaaaaagaaaactacatttacggaacttgttactacacagctagtgatcgcactgcttttcccattgacatatctgtcatgcttaaccgaagagcaataaatgacgagacatcatattgtattcgtataacttggtcctggaacacaggagatgccccagaggtgcaaacctctgctacaaccctagtcacctccccatttaccttttactacatcagagaagacgactgacaaataaaatcgctatccatcgaagatggatgtgtgttggttttttgtgtgatttgtgcgatcgctatgcggccgcttacctgcaggggttaccacacaaaaaaccaacacaccctaaagctcgatctccgacttgtttatttgaaaatcaattcacaaaatccgagtagttattttgcctcccccttcccatttaacagaatacaccaatctctccccacgcacagctttaaacatttggataccattagatatagacatggttttagattccacattccaaacagtttcagagcgagccaatctggggtcagtgatagataaaaatccatcgggatagtcttttaaagcgctttcacagtccaactgctgcggatgcgactccggagtctggatcacggtcatctggaagaagaacgatgggaatcataatccgaaaacggtatcggacgattgtgtctcatcaaacccacaagcagccgctgtctgcgtcgctccgtgcgactgctgtttatgggatcagggtccacagtgtcctgaagcatgattttaatagcccttaacatcaactttctggtgcgatgcgcgcagcaacgcattctgatttcactcaaatctttgcagtaggtacaacacattattacaatattgtttaataaaccataattaaaagcgctccagccaaaactcatatctgatataatcgcccctgcatgaccatcataccaaagtttaatataaattaaatgacgttccctcaaaaacacactacccacatacatgatctcttttggcatgtgcatattaacaatctgtctgtaccatggacaacgttggttaatcatgcaacccaatataaccttccggaaccacactgccaacaccgctcccccagccatgcattgaagtgaaccctgctgattacaatgacaatgaagaacccaattctctcgaccgtgaatcacttgagaatgaaaaatatctatagtggcacaacatagacataaatgcatgcatcttctcataatttttaactcctcaggatttagaaacatatcccagggaataggaagctcttgcagaacagtaaagctggcagaacaaggaagaccacgaacacaacttacactatgcatagtcatagtatcacaatctggcaacagcgggtggtcttcagtcatagaagctcgggtttcattttcctcacaacgtggtaactgggctctggtgtaagggtgatgtctggcgcatgatgtcgagcgtgcgcgcaaccttgtcataatggagttgcttcctgacattctcgtattttgtatagcaaaacgcggccctggcagaacacactcttcttcgccttctatcctgccgcttagcgtgttccgtgtgatagttcaagtacaaccacactcttaagttggtcaaaagaatgctggcttcagttgtaatcaaaactccatcgcatctaatcgttctgaggaaatcatccaagcaatgcaactggattgtgtttcaagcaggagaggagagggaagagacggaagaaccatgttaatttttattccaaacgatctcgcagtacttcaaattgtagatcgcgcagatggcatctctcgcccccactgtgttggtgaaaaagcacagctagatcaaaagaaatgcgattttcaaggtgctcaacggtggcttccagcaaagcctccacgcgcacatccaagaacaaaagaataccaaaagaaggagcattttctaactcctcaatcatcatattacattcctgcaccattcccagataattttcagctttccagccttgaattattcgtgtcagttcttgtggtaaatccaatccacacattacaaacaggtcccggagggcgccctccaccaccattcttaaacacaccctcataatgacaaaatatcttgctcctgtgtcacctgtagcgaattgagaatggcaacatcaattgacatgcccttggctctaagttcttctttaagttctagttgtaaaaactctctcatattatcaccaaactgcttagccagaagccccccgggaacaagagcaggggacgctacagtgcagtacaagcgcagacctccccaattggctccagcaaaaacaagattggaataagcatattgggaaccgccagtaatatcatcgaagttgctggaaatataatcaggcagagtttcttgtaaaaattgaataaaagaaaaatttgccaaaaaaacattcaaaacctctgggatgcaaatgcaataggttaccgcgctgcgctccaacattgttagttttgaattagtctgcaaaaataaaaaaaaaaacaagcgtcatatcatagtagcctgacgaacagatggataaatcagtctttccatcacaagacaagccacagggtctccagctcgaccctcgtaaaacctgtcatcatgattaaacaacagcaccgaaagttcctcgcggtgaccagcatgaataattcttgatgaagcatacaatccagacatgttagcatcagttaacgagaaaaaacagccaacatagcctttgggtataattatgcttaatcgtaagtatagcaaagccacccctcgcggatacaaagtaaaaggcacaggagaataaaaaatataattatttctctgctgctgttcaggcaacgtcgcccccggtccctctaaatacacatacaaagcctcatcagccatggcttaccagacaaagtacagcgggcacacaaagcacaagctctaaagtgactctccaacctctccacaatatatatatacacaagccctaaactgacgtaatgggagtaaagtgtaaaaaatcccgccaaacccaacacacaccccgaaactgcgtcaccagggaaaagtacagtttcacttccgcaatcccaacaggcgtaacttcctctttctcacggtacgtgatatcccactaacttgcaacgtcattttcccacggtcgcaccgccccttttagccgttaaccccacagccaatcaccacacgatccacactttttaaaatcacctcatttacatattggcaccattccatctataaggtatattatatagatagg

SEQ ID NO: 34 - DNA, 32340 bp, Artificial Sequence
  ColoAd2.1 genome
cgcgcctatctatataatataccttatagatggaatggtgccaatatgtaaatgaggtgattttaaaaagtgtggatcgtgtggtgattggctgtggggttaacggctaaaaggggcggtgcgaccgtgggaaaatgacgttttgtgggggtggagtttttttgcaagttgtcgcgggaaatgtgacgcataaaaaggcttttttctcacggaactacttagttttcccacggtatttaacaggaaatgaggtagttttgaccggatgcaagtgaaaattgttgattttcgcgcgaaaactgaatgaggaagtgtttttctgaataatgtggtatttatggcagggtggagtatttgttcagggccaggtagactttgacccattacgtggaggtttcgattaccgtgttttttacctgaatttccgcgtaccgtgtcaaagtcttctgtttttacgtaggtgtcagctgatcgctagggtatttatacctcagggtttgtgtcaagaggccactcttgagtgccagcgagaagagttttctcctctgcgccggcagtttaataataaaaaaatgagagatttgcgatttctgcctcaggaaataatctctgctgagactggaaatgaaatattggagcttgtggtgcacgccctgatgggagacgatccggagccacctgtgcagctttttgagcctcctacgcttcaggaactgtatgatttagaggtagagggatcggaggattctaatgaggaagctgtaaatggcttttttaccgattctatgcttttagctgctaatgaagggttagaattagatccgcctttggacacttttgatactccaggggtaattgtggaaagcggtacaggtgtaagaaaattacctgatttgagttccgtggactgtgatttgcactgctatgaagacgggtttcctccgagtgatgaggaggaccatgaaaaggagcagtccatgcagactgcagcgggtgagggagtgaaggctgccaatgttggttttcagttggattgcccggagcttcctggacatggctgtaagtcttgtgaatttcacaggaaaaatactggagtaaaggaactgttatgttcgctttgttatatgagaacgcactgccactttatttacagtaagtgtgtttaagttaaaatttaaaggaatatgctgtttttcacatgtatattgagtgtgagttttgtgcttcttattataggtcctgtgtctgatgctgatgaatcaccatctcctgattctactacctcacctcctgagattcaagcacctgttcctgtggacgtgcgcaagcccattcctgtgaagcttaagcctgggaaacgtccagcagtggaaaaacttgaggacttgttacagggtggggacggacctttggacttgagtacacggaaacgtccaagacaataagtgttccatatccgtgtttacttaaggtgacgtcaatatttgtgtgacagtgcaatgtaataaaaatatgttaactgttcactggtttttattgctttttgggcggggactcaggtatataagtagaagcagacctgtgtggttagctcataggagctggctttcatccatggaggtttgggccattttggaagaccttaggaagactaggcaactgttagagaacgcttcggacggagtctccggtttttggagattctggttcgctagtgaattagctagggtagtttttaggataaaacaggactataaacaagaatttgaaaagttgttggtagattgcccaggactttttgaagctcttaatttgggccatcaggttcactttaaagaaaaagttttatcagttttagacttttcaaccccaggtagaactgctgctgctgtggcttttcttacttttatattagataaatggatcccgcagactcatttcagcaggggatacgttttggatttcatagccacagcattgtggagaacatggaaggttcgcaagatgaggacaatcttaggttactggccagtgcagcctttgggtgtagcgggaatcctgaggcatccaccggtcatgccagcggttctggaggaggaacagcaagaggacaacccgagagccggcctggaccctccagtggaggaggcggagtagctgacttgtctcctgaactgcaacgggtgcttactggatctacgtccactggacgggataggggcgttaagagggagagggcatctagtggtactgatgctagatctgagttggctttaagtttaatgagtcgcagacgtcctgaaaccatttggtggcatgaggttcagaaagagggaagggatgaagtttctgtattgcaggagaaatattcactggaacaggtgaaaacatgttggttggagcctgaggatgattgggaggtggccattaaaaattatgccaagatagctttgaggcctgataaacagtataagattactagacggattaatatccggaatgcttgttacatatctggaaatggggctgaggtggtaatagatactcaagacaaggcagttattagatgctgcatgatggatatgtggcctggggtagtcggtatggaagcagtaacttttgtaaatgttaagtttaggggagatggttataatggaatagtgtttatggccaataccaaacttatattgcatggttgtagcttttttggtttcaacaatacctgtgtagatgcctggggacaggttagtgtacggggatgtagtttctatgcgtgttggattgccacagctggcagaaccaagagtcaattgtctctgaagaaatgcatatttcaaagatgtaacctgggcattctgaatgaaggcgaagcaagggtccgccactgcgcttctacagatactggatgttttattttgattaagggaaatgccagcgtaaagcataacatgatttgcggtgcttccgatgagaggccttatcaaatgctcacttgtgctggtgggcattgtaatatgctggctactgtgcatattgtttcccatcaacgcaaaaaatggcctgtttttgatcacaatgtgatgacgaagtgtaccatgcatgcaggtgggcgtagaggaatgtttatgccttaccagtgtaacatgaatcatgtgaaagtgttgttggaaccagatgccttttccagaatgagcctaacaggaatttttgacatgaacatgcaaatctggaagatcctgaggtatgatgatacgagatcgagggtacgcgcatgcgaatgcggaggcaagcatgccaggttccagccggtgtgtgtagatgtgactgaagatctcagaccggatcatttggttattgcccgcactggagcagagttcggatccagtggagaagaaactgactaaggtgagtattgggaaaactttggggtgggattttcagatggacagattgagtaaaaatttgttttttctgtcttgcagctgtcatgagtggaaacgcttcttttaaggggggagtcttcagcccttatctgacagggcgtctcccatcctgggcaggagttcgtcagaatgttatgggatctactgtggatggaagacccgtccaacccgccaattcttcaacgctgacctatgctactttaagttcttcacctttggacgcagctgcagctgccgccgccgcttctgttgccgctaacactgtgcttggaatgggttactatggaagcatcatggctaattccacttcctctaataacccttctaccctgactcaggacaagttacttgtccttttggcccagctggaggctttgacccaacgtctgggtgaactttctcagcaggtggtcgagttgcgagtacaaactgagtctgctgtcggcacggcaaagtctaaataaaaaaatcccagaatcaatgaataaataaacaagcttgttgttgatttaaaatcaagtgtttttatttcatttttcgcgcacggtatgccctagaccaccgatctctatcattgagaactcggtggattttttccaggatcctatagaggtgggattgaatgtttagatacatgggcattaggccgtctttggggtggagatagctccattgaagggattcatgctccggggtagtgttgtaaatcacccagtcataacaaggtcgcagtgcatggtgttgcacaatatcttttagaagtaggctgattgccacagataagcccttggtgtaggtgtttacaaaccggttgagctgggatgggtgcattcggggtgaaattatgtgcattttggattggatttttaagttggcaatattgccgccaagatcccgtcttgggttcatgttatgaaggaccaccaagacggtgtatccggtacatttaggaaatttatcgtgcagcttggatggaaaagcgtggaaaaatttggagacacccttgtgtcctccaagattttccatgcactcatccatgataatagcaatggggccgtgggcagcggcgcgggcaaacacgttccgtgggtctgacacatcatagttatgttcctgagttaaatcatcataagccattttaatgaatttggggcggagagtaccagattggggtatgaatgttccttcgggccccggagcatagttcccctcacagatttgcatttcccaagctttcagttccgagggtggaatcatgtccacctggggggctatgaaaaacaccgtttctggggcgggggtgattaattgtgatgatagcaaatttctgagcaattgagatttgccacatccggtggggccataaatgattccgattacgggttgcaggtggtagtttagggaacggcaactgccgtcttctcgaagcaagggggccacctcgttcatcatttcccttacatgcatattttcccgcaccaaatccattaggaggcgctctcctcctagtgatagaagttcttgtagtgaggaaaagtttttcagcggtttcagaccgtcagccatgggcattttggagagagtttgctgcaaaagttctagtctgttccacagttcagtgatgtgttctatggcatctcgatccagcagacctcctcgtttcgcgggtttggacggctcctggaatagggtatgagacgatgggcgtccagcgctgccagggttcggtccttccagggtctcagtgttcgagtcagggttgtttccgtcacagtgaaggggtgtgcgcctgcttgggcgcttgccagggtgcgcttcagactcatcctgctggtcgaaaacttctgtcgcttggcgccctgtatgtcggccaagtagcagtttaccatgagttcgtagttgagcgcctcggctgcgtggcctttggcgcggagcttacctttggaagttttcttgcataccgggcagtataggcatttcagcgcatacaacttgggcgcaaggaaaacggattctggggagtatgcatctgcgccgcaggaggcgcaaacagtttcacattccaccagccaggttaaatccggttcattggggtcaaaaacaagttttccgccatattttttgatgcgtttcttacctttggtctccatgagttcgtgtcctcgttgagtgacaaacaggctgtccgtgtccccgtagactgattttacaggcctcttctccagtggagtgcctcggtcttcttcgtacaggaactctgaccactctgatacaaaggcgcgcgtccaggccagcacaaaggaggctatgtgggaggggtagcgatcgttgtcaaccagggggtccaccttttccaaagtatgcaaacacatgtcaccctcttcaacatccaggaatgtgattggcttgtaggtgtatttcacgtgacctggggtccccgctgggggggtataaaagggggcggttctttgctcttcctcactgtcttccggatcgctgtccaggaacgtcagctgttggggtaggtattccctctcgaaggcgggcatgacctctgcactcaggttgtcagtttctaagaacgaggaggatttgatattgacagtgccggttgagatgcctttcatgaggttttcgtccatctggtcagaaaacacaatttttttattgtcaagtttggtggcaaatgatccatacagggcgttggataaaagtttggcaatggatcgcatggtttggttcttttccttgtccgcgcgctctttggcggcgatgttgagttggacatactcgcgtgccaggcacttccattcggggaagatagttgttaattcatctggcacgattctcacttgccaccctcgattatgcaaggtaattaaatccacactggtggccacctcgcctcgaaggggttcattggtccaacagagcctacctcctttcctagaacagaaagggggaagtgggtctagcataagttcatcgggagggtctgcatccatggtaaagattcccggaagtaaatccttatcaaaatagctgatgggagtggggtcatctaaggccatttgccattctcgagctgccagtgcgcgctcatatgggttaaggggactgccccatggcatgggatgggtgagtgcagaggcatacatgccacagatgtcatagacgtagatgggatcctcaaagatgcctatgtaggttggatagcatcgcccccctctgatacttgctcgcacatagtcatatagttcatgtgatggcgctagcagccccggacccaagttggtgcgattgggtttttctgttctgtagacgatctggcgaaagatggcgtgagaattggaagagatggtgggtctttgaaaaatgttgaaatgggcatgaggtagacctacagagtctctgacaaagtgggcataagattcttgaagcttggttaccagttcggcggtgacaagtacgtctagggcgcagtagtcaagtgtttcttgaatgatgtcataacctggttggtttttcttttcccacagttcgcggttgagaaggtattcttcgcgatccttccagtactcttctagcggaaacccgtctttgtctgcacggtaagatcctagcatgtagaactgattaactgccttgtaagggcagcagcccttctctacgggtagagagtatgcttgagcagcttttcgtagcgaagcgtgagtaagggcaaaggtgtctctgaccatgactttgaggaattggtatttgaagtcgatgtcgtcacaggctccctgttcccagagttggaagtctacccgtttcttgtaggcggggttgggcaaagcgaaagtaacatcattgaagagaatcttgccggccctgggcatgaaattgcgagtgatgcgaaaaggctgtggtacttccgctcggttattgataacctgggcagctaggacgatctcgtcgaaaccgttgatgttgtgtcctacgatgtataattctatgaaacgcggcgtgcctctgacgtgaggtagcttactgagctcatcaaaggttaggtctgtggggtcagataaggcgtagtgttcgagagcccattcgtgcaggtgaggattcgctttaaggaaggaggaccagaggtccactgccagtgctgtttgtaactggtcccggtactgacgaaaatgccgtccgactgccattttttctggggtgacgcaatagaaggtttgggggtcctgccgccagcgatcccacttgagttttatggcgaggtcataggcgatgttgacgagccgctggtctccagagagtttcatgaccagcatgaaggggattagctgcttgccaaaggaccccatccaggtgtaggtttccacatcgtaggtgagaaagagcctttctgtgcgaggatgagagccaatcgggaagaactggatctcctgccaccagttggaggaatggctgttgatgtgatggaagtagaactccctgcgacgcgccgagcattcatgcttgtgcttgtacagacggccgcagtagtcgcagcgttgcacgggttgtatctcgtgaatgagttgtacctggcttcccttgacgagaaatttcagtgggaagccgaggcctggcgattgtatctcgtgctttactatgttgtctgcatcggcctgttcatcttctgtctcgatggtggtcatgctgacgagccctcgcgggaggcaagtccagacctcggcgcggcaggggcggagctcgaggacgagagcgcgcaggctggagctgtccagggtcctgagacgctgcggactcaggttagtaggcagtgtcaggagattaacttgcatgatcttttggagggcgtgcgggaggttcagatagtacttgatctcaacgggtccgttggtggagatgtcgatggcttgcagggttccgtgtcccttgggcgctaccaccgtgcccttgtttttcattttggacggcggtggctctgttgcttcttgcatgtttagaagcggtgtcgagggcgcgcaccgggcggcaggggcggctcgggacccggcggcatggctggcagtggtacgtcggcgccgcgcgcgggtaggttctggtactgcgccctgagaagactcgcatgcgcgacgacgcggcggttgacatcctggatctgacgcctctgggtgaaagctaccggccccgtgagcttgaacctgaaagagagttcaacagaatcaatctcggtatcgttgacggcggcttgcctaaggatttcttgcacgtcaccagagttgtcctggtaggcgatctccgccatgaactgctcgatctcttcctcttgaagatctccgcggcccgctctctcgacggtggccgcgaggtcgttggagatgcgcccaatgagttgagagaatgcattcatgcccgcctcgttccagacgcggctgtagaccacggcccccacgggatctctcgcgcgcatgaccacctgggcgaggttgagctccacgtggcgggtgaagaccgcatagttgcataggcgctggaaaaggtagttgagtgtggtggcgatgtgctcggtgacgaagaaatacatgatccatcgtctcagcggcatctcgctgacatcgcccagagcttccaagcgctccatggcctcgtagaagtccacggcaaaattaaaaaactgggagtttcgcgcggacacggtcaactcctcttccagaagacggataagttcggcgatggtggtgcgcacctcgcgctcgaaagcccctgggatttcttcctcaatctcttcttcttccactaacatctcttcctcttcaggtggggctgcaggaggagggggaacgcggcgacgccggcggcgcacgggcagacggtcgatgaatctttcaatgacctctccgcggcggcggcgcatggtttcagtgacggcgcggccgttctcgcgcggtcgcagagtaaaaacaccgccgcgcatctccttaaagtggtgactgggaggttctccgtttgggagggagagggcgctgattatacattttattaattggcccgtagggactgcacgcagagatctgatcgtgtcaagatccacgggatctgaaaacctttcgacgaaagcgtctaaccagtcacagtcacaaggtaggctgagtacggcttcttgtgggcgggggtggttatgtgttcggtctgggtcttctgtttcttcttcatctcgggaaggtgagacgatgctgctggtgatgaaattaaagtaggcagttctaagacggcggatggtggcgaggagcaccaggtctttgggtccggcttgctggatacgcaggcgattggccattccccaagcattatcctgacatctagcaagatctttgtagtagtcttgcatgagccgttctacgggcacttcttcctcacccgttctgccatgcatacgtgtgagtccaaatccgcgcattggttgtaccagtgccaagtcagctacgactctttcggcgaggatggcttgctgtacttgggtaagggtggcttgaaagtcatcaaaatccacaaagcggtggtaagctcctgtattaatggtgtaagcacagttggccatgactgaccagttaactgtctggtgaccagggcgcacgagctcggtgtatttaaggcgcgaataggcgcgggtgtcaaagatgtaatcgttgcaggtgcgcaccagatactggtaccctataagaaaatgcggcggtggttggcggtagagaggccatcgttctgtagctggagcgccaggggcgaggtcttccaacataaggcggtgatagccgtagatgtacctggacatccaggtgattcctgcggcggtagtagaagcccgaggaaactcgcgtacgcggttccaaatgttgcgtagcggcatgaagtagttcattgtaggcacggtttgaccagtgaggcgcgcgcagtcattgatgctctatagacacggagaaaatgaaagcgttcagcgactcgactccgtagcctggaggaacgtgaacgggttgggtcgcggtgtaccccggttcgagacttgtactcgagccggccggagccgcggctaacgtggtattggcactcccgtctcgacccagcctacaaaaatccaggatacggaatcgagtcgttttgctggtttccgaatggcagggaagtgagtcctattttttttttttgccgctcagatgcatcccgtgctgcgacagatgcgcccccaacaacagcccccctcgcagcagcagcagcagcaatcacaaaaggctgtccctgcaactactgcaactgccgccgtgagcggtgcgggacagcccgcctatgatctggacttggaagagggcgaaggactggcacgtctaggtgcgccttcacccgagcggcatccgcgagttcaactgaaaaaagattctcgcgaggcgtatgtgccccaacagaacctatttagagacagaagcggcgaggagccggaggagatgcgagcttcccgctttaacgcgggtcgtgagctgcgtcacggtttggaccgaagacgagtgttgcgggacgaggatttcgaagttgatgaaatgacagggatcagtcctgccagggcacacgtggctgcagccaaccttgtatcggcttacgagcagacagtaaaggaagagcgtaacttccaaaagtcttttaataatcatgtgcgaaccctgattgcccgcgaagaagttacccttggtttgatgcatttgtgggatttgatggaagctatcattcagaaccctactagcaaacctctgaccgcccagctgtttctggtggtgcaacacagcagagacaatgaggctttcagagaggcgctgctgaacatcaccgaacccgaggggagatggttgtatgatcttatcaacattctacagagtatcatagtgcaggagcggagcctgggcctggccgagaaggtggctgccatcaattactcggttttgagcttgggaaaatattacgctcgcaaaatctacaagactccatacgttcccatagacaaggaggtgaagatagatgggttctacatgcgcatgacgctcaaggtcttgaccctgagcgatgatcttggggtgtatcgcaatgacagaatgcatcgcgcggttagcgccagcaggaggcgcgagttaagcgacagggaactgatgcacagtttgcaaagagctctgactggagctggaaccgagggtgagaattacttcgacatgggagctgacttgcagtggcagcctagtcgcagggctctgagcgccgcgacggcaggatgtgagcttccttacatagaagaggcggatgaaggcgaggaggaagagggcgagtacttggaagactgatggcacaacccgtgttttttgctagatggaacagcaagcaccggatcccgcaatgcgggcggcgctgcagagccagccgtccggcattaactcctcggacgattggacccaggccatgcaacgtatcatggcgttgacgactcgcaaccccgaagcctttagacagcaaccccaggccaaccgtctatcggccatcatggaagctgtagtgccttcccgctctaatcccactcatgagaaggtcctggccatcgtgaacgcgttggtggagaacaaagctattcgtccagatgaggccggactggtatacaacgctctcttagaacgcgtggctcgctacaacagtagcaatgtgcaaaccaatttggaccgtatgataacagatgtacgcgaagccgtgtctcagcgcgaaaggttccagcgtgatgccaacctgggttcgctggtggcgttaaatgctttcttgagtactcagcctgctaatgtgccgcgtggtcaacaggattatactaactttttaagtgctttgagactgatggtatcagaagtacctcagagcgaagtgtatcagtccggtcctgattacttctttcagactagcagacagggcttgcagacggtaaatctgagccaagcttttaaaaacctttaaaggtttgtggggagtgcatgccccggtaggagaaagagcaaccgtgtctagcttgttaactccgaactcccgcctattattactgttggtagctcctttcaccgacagcggtagcatcgaccgtaattcctatttgggttacctactaaacctgtatcgcgaagccatagggcaaagtcaggtggacgagcagacctatcaagaaattacccaagtcagtcgcgctttgggacaggaagacactggcagtttggaagccactctgaacttcttgcttaccaatcggtctcaaaagatccctcctcaatatgctcttactgcggaggaggagaggatccttagatatgtgcagcagagcgtgggattgtttctgatgcaagagggggcaactccgactgcagcactggacatgacagcgcgaaatatggagcccagcatgtatgccagtaaccgacctttcattaacaaactgctggactacttgcacagagctgccgctatgaactctgattatttcaccaatgccatcttaaacccgcactggctgcccccacctggtttctacacgggcgaatatgacatgcccgaccctaatgacggatttctgtgggacgacgtggacagcgatgttttttcacctctttctgatcatcgcacgtggaaaaaggaaggcggcgatagaatgcattcttctgcatcgctgtccggggtcatgggtgctaccgcggctgagcccgagtctgcaagtccttttcctagtctacccttttctctacacagtgtacgtagcagcgaagtgggtagaataagtcgcccgagtttaatgggcgaagaggagtatctaaacgattccttgctcagaccggcaagagaaaaaaatttcccaaacaatggaatagaaagtttggtggataaaatgagtagatggaagacttatgctcaggatcacagagacgagcctgggatcatggggattacaagtagagcgagccgtagacgccagcgccatgacagacagaggggtcttgtgtgggacgatgaggattcggccgatgatagcagcgtgctggacttgggtgggagaggaaggggcaacccgtttgctcatttgcgccctcgcttgggtggtatgttgtaaaaaaaaataaaaaaaaaactcaccaaggccatggcgacgagcgtacgttcgttcttctttattatctgtgtctagtataatgaggcgagtcgtgctaggcggagcggtggtgtatccggagggtcctcctccttcgtacgagagcgtgatgcagcagcagcaggcgacggcggtgatgcaatccccactggaggctccctttgtgcctccgcgatacctggcacctacggagggcagaaacagcattcgttattcggaactggcacctcagtacgataccaccaggttgtatctggtggacaacaagtcggcggacattgcttctctgaactatcagaatgaccacagcaacttcttgaccacggtggtgcaaaacaatgactttacccctacggaagccagcacccagaccattaactttgatgaacgatcgcggtggggcggtcagctaaagaccatcatgcatactaacatgccaaacgtgaacgagtatatgtttagtaacaagttcaaagcgcgtgtgatggtgtccagaaaacctcccgacggtgctgcagttggggatacttatgatcacaagcaggatattttgaaatatgagtggttcgagtttactttgccagaaggcaacttttcagttactatgactattgatttgatgaacaatgccatcatagataattacttgaaagtgggtagacagaatggagtgcttgaaagtgacattggtgttaagttcgacaccaggaacttcaagctgggatgggatcccgaaaccaagttgatcatgcctggagtgtatacgtatgaagccttccatcctgacattgtcttactgcctggctgcggagtggattttaccgagagtcgtttgagcaaccttcttggtatcagaaaaaaacagccatttcaagagggttttaagattttgtatgaagatttagaaggtggtaatattccggccctcttggatgtagatgcctatgagaacagtaagaaagaacaaaaagccaaaatagaagctgctacagctgctgcagaagctaaggcaaacatagttgccagcgactctacaagggttgctaacgctggagaggtcagaggagacaattttgcgccaacacctgttccgactgcagaatcattattggccgatgtgtctgaaggaacggacgtgaaactcactattcaacctgtagaaaaagatagtaagaatagaagctataatgtgttggaagacaaaatcaacacagcctatcgcagttggtatctttcgtacaattatggcgatcccgaaaaaggagtgcgttcctggacattgctcaccacctcagatgtcacctgcggagcagagcaggtctactggtcgcttccagacatgatgaaggatcctgtcactttccgctccactagacaagtcagtaactaccctgtggtgggtgcagagcttatgcccgtcttctcaaagagcttctacaacgaacaagctgtgtactcccagcagctccgccagtccacctcgcttacgcacgtcttcaaccgctttcctgagaaccagattttaatccgtccgccggcgcccaccattaccaccgtcagtgaaaacgttcctgctctcacagatcacgggaccctgccgttgcgcagcagtatccggggagtccaacgtgtgaccgttactgacgccagacgccgcacctgtccctacgtgtacaaggcactgggcatagtcgcaccgcgcgtcctttcaagccgcactttctaaaaaaaaaaaaaatgtccattcttatctcgcccagtaataacaccggttggggtctgcgcgctccaagcaagatgtacggaggcgcacgcaaacgttctacccaacatcctgtccgtgttcgcggacattttcgcgctccatggggcgccctcaagggccgcactcgcgttcgaaccaccgtcgatgatgtaatcgatcaggtggttgccgacgcccgtaattatactcctactgcgcctacatctactgtggatgcagttattgacagtgtagtggctgacgctcgcaactatgctcgacgtaagagccggcgaaggcgcattgccagacgccaccgagctaccactgccatgcgagccgcaagagctctgctacgaagagctagacgcgtggggcgaagagccatgcttagggcggccagacgtgcagcttcgggcgccagcgccggcaggtcccgcaggcaagcagccgctgtcgcagcggcgactattgccgacatggcccaatcgcgaagaggcaatgtatactgggtgcgtgacgctgccaccggtcaacgtgtacccgtgcgcacccgtccccctcgcacttagaagatactgagcagtctccgatgttgtgtcccagcggcgaggatgtccaagcgcaaatacaaggaagaaatgctgcaggttatcgcacctgaagtctacggccaaccgttgaaggatgaaaaaaaaccccgcaaaatcaagcgggttaaaaaggacaaaaaagaagaggaagatggcgatgatgggctggcggagtttgtgcgcgagtttgccccacggcgacgcgtgcaatggcgtgggcgcaaagttcgacatgtgttgagacctggaacttcggtggtctttacacccggcgagcgttcaagcgctacttttaagcgttcctatgatgaggtgtacggggatgatgatattcttgagcaggcggctgaccgattaggcgagtttgcttatggcaagcgtagtagaataacttccaaggatgagacagtgtcgatacccttggatcatggaaatcccacccctagtcttaaaccggtcactttgcagcaagtgttacccgtaactccgcgaacaggtgttaaacgcgaaggtgaagatttgtatcccactatgcaactgatggtacccaaacgccagaagttggaggacgttttggagaaagtaaaagtggatccagatattcaacctgaggttaaagtgagacccattaagcaggtagcgcctggtctgggggtacaaactgtagacattaagattcccactgaaagtatggaagtgcaaactgaacccgcaaagcctactgccacctccactgaagtgcaaacggatccatggatgcccatgcctattacaactgacgccgccggtcccactcgaagatcccgacgaaagtacggtccagcaagtctgttgatgcccaattatgttgtacacccatctattattcctactcctggttaccgaggcactcgctactatcgcagccgaaacagtacctcccgccgtcgccgcaagacacctgcaaatcgcagtcgtcgccgtagacgcacaagcaaaccgactcccggcgccctggtgcggcaagtgtaccgcaatggtagtgcggaacctttgacactgccgcgtgcgcgttaccatccgagtatcatcacttaatcaatgttgccgctgcctccttgcagatatggccctcacttgtcgccttcgcgttcccatcactggttaccgaggaagaaactcgcgccgtagaagagggatgttgggacgcggaatgcgacgctacaggcgacggcgtgctatccgcaagcaattgcggggtggttttttaccagccttaattccaattatcgctgctgcaattggcgcgataccaggcatagcttccgtggcggttcaggcctcgcaacgacattgacattggaaaaaaacgtataaataaaaaaaaaaaaatacaatggactctgacactcctggtcctgtgactatgttttcttagagatggaagacatcaatttttcatccttggctccgcgacacggcacgaagccgtacatgggcacctggagcgacatcggcacgagccaactgaacgggggcgccttcaattggagcagtatctggagcgggcttaaaaattttggctcaaccataaaaacatacgggaacaaagcttggaacagcagtacaggacaggcgcttagaaataaacttaaagaccagaacttccaacaaaaagtagtcgatgggatagcttccggcatcaatggagtggtagatttggctaaccaggctgtgcagaaaaagataaacagtcgtttggacccgccgccagcaaccccaggtgaaatgcaagtggaggaagaaattcctccgccagaaaaacgaggcgacaagcgtccgcgtcccgatttggaagagacgctggtgacgcgcgtagatgaaccgccttcttatgaggaagcaacgaagcttggaatgcccaccactagaccgatagccccaatggccaccggggtgatgaaaccttctcagttgcatcgacccgtcaccttggatttgccccctccccctgctgctactgctgtacccgcttctaagcctgtcgctgccccgaaaccagtcgccgtagccaggtcacgtcccgggggcgctcctcgtccaaatgcgcactggcaaaatactctgaacagcatcgtgggtctaggcgtgcaaagtgtaaaacgccgtcgctgcttttaattaaatatggagtagcgcttaacttgcctatctgtgtatatgtgtcattacacgccgtcacagcagcagaggaaaaaaggaagaggtcgtgcgtcgacgctgagttactttcaagatggccaccccatcgatgctgccccaatgggcatacatgcacatcgccggacaggatgcttcggagtacctgagtccgggtctggtgcagttcgcccgcgccacagacacctacttcaatctgggaaataagtttagaaatcccaccgtagcgccgacccacgatgtgaccaccgaccgtagccagcggctcatgttgcgcttcgtgcccgttgaccgggaggacaatacatactcttacaaagtgcggtacaccctggccgtgggcgacaacagagtgctggatatggccagcacgttctttgacattaggggtgtgttggacagaggtcccagtttcaaaccctattctggtacggcttacaactccctggctcctaaaggcgctccaaatacatctcagtggattgcagaaggtgtaaaaaatacaactggtgaggaacacgtaacagaagaggaaaccaatactactacttacacttttggcaatgctcctgtaaaagctgaagctgaaattacaaaagaaggactcccagtaggtttggaagtttcagatgaagaaagtaaaccgatttatgctgataaaacatatcagccagaacctcagctgggagatgaaacttggactgaccttgatggaaaaaccgaaaagtatggaggcagggctctcaaacccgatactaagatgaaaccatgctacgggtcctttgccaaacctactaatgtgaaaggcggtcaggcaaaacaaaaaacaacggagcagccaaatcagaaagtcgaatatgatatcgacatggagttttttgatgcggcatcgcagaaaacaaacttaagtcctaaaattgtcatgtatgcagaaaatgtaaatttggaaactccagacactcatgtagtgtacaaacctggaacagaagacacaagttccgaagctaatttgggacaacaatctatgcccaacagacccaactacattggcttcagagataactttattggacttatgtactataacagtactggtaacatgggggtgctggctggtcaagcgtctcagttaaatgcagtggttgacttgcaggacagaaacacagaactttcttaccaactcttgcttgactctctgggcgacagaaccagatactttagcatgtggaatcaggctgtggacagttatgatcctgatgtacgtgttattgaaaatcatggtgtggaagatgaacttcccaactactgttttccactggacggcataggtgttccaacaaccagttacaaatcaatagttccaaatggagacaatgcgcctaattggaaggaacctgaagtaaatggaacaagtgagatcggacagggtaatttgtttgccatggaaattaaccttcaagccaatctatggcgaagtttcctttattccaatgtggctctatatctcccagactcgtacaaatacaccccgtccaatgtcactcttccagaaaacaaaaacacctacgactacatgaacgggcgggtggtgccgccatctctagtagacacctatgtgaacattggtgccaggtggtctctggatgccatggacaatgtcaacccattcaaccaccaccgtaacgctggcttgcgttaccgatccatgcttctgggtaacggacgttatgtgcctttccacatacaagtgcctcaaaaattcttcgctgttaaaaacctgctgcttctcccaggctcctacacttatgagtggaactttaggaaggatgtgaacatggttctacagagttccctcggtaacgacctgcgggtagatggcgccagcatcagtttcacgagcatcaacctctatgctacttttttccccatggctcacaacaccgcttccacccttgaagccatgctgcggaatgacaccaatgatcagtcattcaacgactacctatctgcagctaacatgctctaccccattcctgccaatgcaaccaatattcccatttccattccttctcgcaactgggcggctttcagaggctggtcatttaccagactgaaaaccaaagaaactccctctttggggtctggatttgacccctactttgtctattctggttctattccctacctggatggtaccttctacctgaaccacacttttaagaaggtttccatcatgtttgactcttcagtgagctggcctggaaatgacaggttactatctcctaacgaatttgaaataaagcgcactgtggatggcgaaggctacaacgtagcccaatgcaacatgaccaaagactggttcttggtacagatgctcgccaactacaacatcggctatcagggcttctacattccagaaggatacaaagatcgcatgtattcatttttcagaaacttccagcccatgagcaggcaggtggttgatgaggtcaattacaaagacttcaaggccgtcgccataccctaccaacacaacaactctggctttgtgggttacatggctccgaccatgcgccaaggtcaaccctatcccgctaactatccctatccactcattggaacaactgccgtaaatagtgttacgcagaaaaagttcttgtgtgacagaaccatgtggcgcataccgttctcgagcaacttcatgtctatgggggcccttacagacttgggacagaatatgctctatgccaactcagctcatgctctggacatgacctttgaggtggatcccatggatgagcccaccctgctttatcttctcttcgaagttttcgacgtggtcagagtgcatcagccacaccgcggcatcatcgaggcagtctacctgcgtacaccgttctcggccggtaacgctaccacgtaagaagcttcttgcttcttgcaaatagcagctgcaaccatggcctgcggatcccaaaacggctccagcgagcaagagctcagagccattgtccaagacctgggttgcggaccctattttttgggaacctacgataagcgcttcccggggttcatggcccccgataagctcgcctgtgccattgtaaatacggccggacgtgagacggggggagagcactggttggctttcggttggaacccacgttctaacacctgctacctttttgatccttttggattctcggatgatcgtctcaaacagatttaccagtttgaatatgagggtctcctgcgccgcagcgctcttgctaccaaggaccgctgtattacgctggaaaaatctacccagaccgtgcagggtccccgttctgccgcctgcggacttttctgctgcatgttccttcacgcctttgtgcactggcctgaccgtcccatggacggaaaccccaccatgaaattgctaactggagtgccaaacaacatgcttcattctcctaaagtccagcccaccctgtgtgacaatcaaaaagcactctaccattttcttaatacccattcgccttattttcgctcccatcgtacacacatcgaaagggccactgcgttcgaccgtatggatgttcaataatgactcatgtaaacaacgtgttcaataaacatcactttatttttttacatgtatcaaggctctgcattacttatttatttacaagtcgaatgggttctgacgagaatcagaatgacccgcaggcagtgatacgttgcggaactgatacttgggttgccacttgaattcgggaatcaccaacttgggaaccggtatatcgggcaggatgtcactccacagctttctggtcagctgcaaagctccaagcaggtcaggagccgaaatcttgaaatcacaattaggaccagtgctttgagcgcgagagttgcggtacaccggattgcagcactgaaacaccatcagcgacggatgtctcacgcttgccagcacggtgggatctgcaatcatgcccacatccagatcttcagcattggcaatgctgaacggggtcatcttgcaggtctgcctacccatggcgggcacccaattaggcttgtggttgcaatcgcagtgcagggggatcagtatcatcttggcctgatcctgtctgattcctggatacacggctctcatgaaagcatcatattgcttgaaagcctgctgggctttactaccctcggtataaaacatcccgcaggacctgctcgaaaactggttagctgcacagccggcatcattcacacagcagcgggcgtcattgttagctatttgcaccacacttctgccccagcggttttgggtgattttggttcgctcgggattctcctttaaggctcgttgtccgttctcgctggccacatccatctcgataatctgctccttctgaatcataatattgccatgcaggcacttcagcttgccctcataatcattgcagccatgaggccacaacgcacagcctgtacattcccaattatggtgggcgatctgagaaaaagaatgtatcattccctgcagaaatcttcccatcatcgtgctcagtgtcttgtgactagtgaaagttaactggatgcctcggtgctcctcgtttacgtactggtgacagatgcgcttgtattgttcgtgttgctcaggcattagtttaaaagaggttctaagttcgttatccagcctgtacttctccatcagcagacacatcacttccatgcctttctcccaagcagacaccaggggcaagctaatcggattcttaacagtgcaggcagcagctcctttagccagagggtcatctttagcgatcttctcaatgcttcttttgccatccttctcaacgatgcgcacgggcgggtagctgaaacccactgctacaagttgcgcctcttctctttcttcttcgctgtcttgactgatgtcttgcatggggatatgtttggtcttccttggcttctttttggggggtatcggaggaggaggactgtcgctccgttccggagacagggaggattgtgacgtttcgctcaccattaccaactgactgtcggtagaagaacctgaccccacacggcgacaggtgtttctcttcgggggcagaggtggaggcgattgcgaagggctgcggtccgacctggaaggcggatgactggcagaaccccttccgcgttcgggggtgtgctccctgtggcggtcgcttaactgatttccttcgcggctggccattgtgttctcctaggcagagaaacaacagacatggaaactcagccattgctgtcaacatcgccacgagtgccatcacatctcgtcctcagcgacgaggaaaaggagcagagcttaagcattccaccgcccagtcctgccaccacctctaccctagaagataaggaggtcgacgcatctcatgacatgcagaataaaaaagcgaaagagtctgagacagacatcgagcaagacccgggctatgtgacaccggtggaacacgaggaagagttgaaacgctttctagagagagaggatgaaaactgcccaaaacaacgagcagataactatcaccaagatgctggaaatagggatcagaacaccgactacctcatagggcttgacggggaagacgcgctccttaaacatctagcaagacagtcgctcatagtcaaggatgcattattggacagaactgaagtgcccatcagtgtggaagagctcagccgcgcctacgagcttaacctcttttcacctcgtactccccccaaacgtcagccaaacggcacctgcgagccaaatcctcgcttaaacttttatccagcttttgctgtgccagaagtactggctacctatcacatcttttttaaaaatcaaaaaattccagtctcctgccgcgctaatcgcacccgcgccgatgccctactcaatctgggacctggttcacgcttacctgatatagcttccttggaagaggttccaaagatcttcgagggtctgggcaataatgagactcgggccgcaaatgctctgcaaaagggagaaaatggcatggatgagcatcacagcgttctggtggaattggaaggcgataatgccagactcgcagtactcaagcgaagcatcgaggtcacacacttcgcatatcccgctgtcaacctgccccctaaagtcatgacggcggtcatggaccagttactcattaagcgcgcaagtcccctttcagaagacatgcatgacccagatgcctgtgatgagggtaaaccagtggtcagtgatgagcagctaacccgatggctgggcaccgactctcccagggatttggaagagcgtcgcaagcttatgatggccgtggtgctggttaccgtagaactagagtgtctccgacgtttctttaccgattcagaaaccttgcgcaaactcgaagagaatctgcactacacttttagacacggctttgtgcggcaggcatgcaagatatctaacgtggaactcaccaacctggtttcctacatgggtattctgcatgagaatcgcctaggacaaagcgtgctgcacagcaccctgaagggggaagcccgccgtgattacatccgcgattgtgtctatctgtacctgtgccacacgtggcaaaccggcatgggtgtatggcagcaatgtttagaagaacagaacttgaaagagcttgacaagctcttacagaaatctcttaaggttctgtggacagggttcgacgagcgcaccgtcgcttccgacctggcagacctcatcttcccagagcgtctcagggttactttgcgaaacggattgcctgactttatgagccagagcatgcttaacaattttcgctctttcatcctggaacgctccggtatcctgcccgccacctgctgcgcactgccctccgactttgtgcctctcacctaccgcgagtgccccccgccgctatggagtcactgctacctgttccgtctggccaactatctctcctaccactcggatgtgatcgaggatgtgagcggagacggcttgctggagtgtcactgccgctgcaatctgtgcacgccccaccggtccctagcttgcaacccccagttgatgagcgaaacccagataataggcacctttgaattgcaaggccccagcagccaaggcgatgggtcttctcctgggcaaagtttaaaactgaccccgggactgtggacctccgcctacttgcgcaagtttgctccggaagattaccacccctatgaaatcaagttctatgaggaccaatcacagcctccaaaggccgaactttcggcctgcgtcatcacccagggggcaattctggcccaattgcaagccatccaaaaatcccgccaagaatttctactgaaaaagggtaagggggtctaccttgacccccagaccggcgaggaactcaacacaaggttccctcaggatgtcccaacgacgagaaaacaagaagttgaaggtgcagccgccgcccccagaagatatggaggaagattgggacagtcaggcagaggaggcggaggaggacagtctggaggacagtctggaggaagacagtttggaggaggaaaacgaggaggcagaggaggtggaagaagtaaccgccgacaaacagttatcctcggctgcggagacaagcaacagcgctaccatctccgctccgagtcgaggaacccggcggcgtcccagcagtagatgggacgagaccggacgcttcccgaacccaaccagcgcttccaagaccggtaagaaggatcggcagggatacaagtcctggcgggggcataagaatgccatcatctcctgcttgcatgagtgcgggggcaacatatccttcacgcggcgctacttgctattccaccatggggtgaactttccgcgcaatgttttgcattactaccgtcacctccacagcccctactatagccagcaaatcccggcagtctcgacagataaagacagcggcggcgacctccaacagaaaaccagcagcggcagttagaaaatacacaacaagtgcagcaacaggaggattaaagattacagccaacgagccagcgcaaacccgagagttaagaaatcggatctttccaaccctgtatgccatcttccagcagagtcggggtcaagagcaggaactgaaaataaaaaaccgatctctgcgttcgctcaccagaagttgtttgtatcacaagagcgaagatcaacttcagcgcactctcgaggacgccgaggctctcttcaacaagtactgcgcgctgactcttaaagagtaggcagcgaccgcgcttattcaaaaaaggcgggaattacatcatcctcgacatgagtaaagaaattcccacgccttacatgtggagttatcaaccccaaatgggattggcggcaggcgcctcccaggactactccacccgcatgaattggctcagcgccgggccttctatgatttctcgagttaatgatatacgcgcctaccgaaaccaaatacttttggaacagtcagctcttaccaccacgccccgccaacaccttaatcccagaaattggcccgccgccctagtgtaccaggaaagtcccgctcccaccactgtattacttcctcgagacgcccaggccgaagtccaaatgactaatgcaggtgcgcagttagctggcggctccaccctatgtcgtcacaggcctcggcataatataaaacgcctgatgatcagaggccgaggtatccagctcaacgacgagtcggtgagctctccgcttggtctacgaccagacggaatctttcagattgccggctgcgggagatcttccttcacccctcgtcaggctgttctgactttggaaagttcgtcttcgcaaccccgctcgggcggaatcgggaccgttcaatttgtggaggagtttactccctctgtctacttcaaccccttctccggatctcctgggcattacccggacgagttcataccgaacttcgacgcgattagcgagtcagtggacggctacgattgatgtctggtgacgcggctgagctatctcggctgcgacatctagaccactgccgccgctttcgctgctttgcccgggaactcattgagttcatctacttcgaactccccaaggatcaccctcaaggtccggcccacggagtgcggatttctatcgaaggcaaaatagactctcgcctgcaacgaattttctcccagcggcccgtgctgatcgagcgagaccagggaaacaccacggtttccatctactgcatttgtaatcaccccggattgcatgaaagcctttgctgtcttatgtgtactgagtttaataaaaactgaattaagactctcctacggactgccgcttcttcaacccggattttacaaccagaagaacgaaacttttcctgtcgtccaggactctgttaacttcacctttcctactcacaaactagaagctcaacgactacaccgcttttccagaagcattttccctactaatactactttcaaaaccggaggtgagctccaaggtcttcctacagaaaacccttgggtggaagcgggccttgtagtgctaggaattcttgcgggtgggcttgtgattattctttgctacctatacacaccttgcttcactttcttagtggtgttgtggtattggtttaaaaaatggggcccatactagtcttgcttgttttactttcgcttttggaaccgggttctgccaattacgatccatgtctagacttcgacccagaaaactgcacacttacttttgcacccgacacaagccgcatctgtggagttcatcgcctctcttacgaacttggcccccaacgacaaaaatttacctgcatggtgggaatcaaccccatagttatcacccagcaaagtggagatactaagggttgcattcactgctcctgcgattccatcgagtgcacctacaccctgctgaagaccctatgcggcctaagagacctgctaccaatgaattaaaaaatgattaataaaaaatcacttacttgaaatcagcaataaggtctctgttgaaattttctcccagcagcacctcacttccctcttcccaactctggtattctaaaccccgttcagcggcatactttctccatactttaaaggggatgtcaaattttagctcctctcctgtacccacaatcttcatgtctttcttcccagagcggccgcatgaccaagagagtccggctcagtgactccttcaaccctgtctacccctatgaagatgaaagcacctcccaacacccctttataaacccagggtttatttccccaaatggcttcacacaaagcccaaacggagttcttactttaaaatgtttaaccccactaacaaccacaggcggatctctacagctaaaagtgggagggggacttacagtggatgacaccaacggttttttgaaagaaaacataagtgccaccacaccactcgttaagactggtcactctataggtttaccactaggagccggattgggaacgaatgaaaataaactttgtatcaaattaggacaaggacttacattcaattcaaacaacatttgcattgatgacaatattaacaccttatggacaggagtcaaccccaccgaagccaactgtcaaatcatgaactccagtgaatctaatgattgcaaattaattctaacactagttaaaactggagcactagtcactgcatttgtttatgttataggagtatctaacaattttaatatgctaactacacacagaaatataaattttactgcagagctgtttttcgattctactggtaatttactaactagactctcatccctcaaaactccacttaatcataaatcaggacaaaacatggctactggtgccattactaatgctaaaggtttcatgcccagcacgactgcctatcctttcaatgataattctagagaaaaagaaaactacatttacggaacttgttactacacagctagtgatcgcactgcttttcccattgacatatctgtcatgcttaaccgaagagcaataaatgacgagacatcatattgtattcgtataacttggtcctggaacacaggagatgccccagaggtgcaaacctctgctacaaccctagtcacctccccatttaccttttactacatcagagaagacgactgacaaataaagtttaacttgtttatttgaaaatcaattcacaaaatccgagtagttattttgcctcccccttcccatttaacagaatacaccaatctctccccacgcacagctttaaacatttggataccattagatatagacatggttttagattccacattccaaacagtttcagagcgagccaatctggggtcagtgatagataaaaatccatcgggatagtcttttaaagcgctttcacagtccaactgctgcggatgcgactccggagtctggatcacggtcatctggaagaagaacgatgggaatcataatccgaaaacggtatcggacgattgtgtctcatcaaacccacaagcagccgctgtctgcgtcgctccgtgcgactgctgtttatgggatcagggtccacagtgtcctgaagcatgattttaatagcccttaacatcaactttctggtgcgatgcgcgcagcaacgcattctgatttcactcaaatctttgcagtaggtacaacacattattacaatattgtttaataaaccataattaaaagcgctccagccaaaactcatatctgatataatcgcccctgcatgaccatcataccaaagtttaatataaattaaatgacgttccctcaaaaacacactacccacatacatgatctcttttggcatgtgcatattaacaatctgtctgtaccatggacaacgttggttaatcatgcaacccaatataaccttccggaaccacactgccaacaccgctcccccagccatgcattgaagtgaaccctgctgattacaatgacaatgaagaacccaattctctcgaccgtgaatcacttgagaatgaaaaatatctatagtggcacaacatagacataaatgcatgcatcttctcataatttttaactcctcaggatttagaaacatatcccagggaataggaagctcttgcagaacagtaaagctggcagaacaaggaagaccacgaacacaacttacactatgcatagtcatagtatcacaatctggcaacagcgggtggtcttcagtcatagaagctcgggtttcattttcctcacaacgtggtaactgggctctggtgtaagggtgatgtctggcgcatgatgtcgagcgtgcgcgcaaccttgtcataatggagttgcttcctgacattctcgtattttgtatagcaaaacgcggccctggcagaacacactcttcttcgccttctatcctgccgcttagcgtgttccgtgtgatagttcaagtacaaccacactcttaagttggtcaaaagaatgctggcttcagttgtaatcaaaactccatcgcatctaatcgttctgaggaaatcatccaagcaatgcaactggattgtgtttcaagcaggagaggagagggaagagacggaagaaccatgttaatttttattccaaacgatctcgcagtacttcaaattgtagatcgcgcagatggcatctctcgcccccactgtgttggtgaaaaagcacagctagatcaaaagaaatgcgattttcaaggtgctcaacggtggcttccagcaaagcctccacgcgcacatccaagaacaaaagaataccaaaagaaggagcattttctaactcctcaatcatcatattacattcctgcaccattcccagataattttcagctttccagccttgaattattcgtgtcagttcttgtggtaaatccaatccacacattacaaacaggtcccggagggcgccctccaccaccattcttaaacacaccctcataatgacaaaatatcttgctcctgtgtcacctgtagcgaattgagaatggcaacatcaattgacatgcccttggctctaagttcttctttaagttctagttgtaaaaactctctcatattatcaccaaactgcttagccagaagccccccgggaacaagagcaggggacgctacagtgcagtacaagcgcagacctccccaattggctccagcaaaaacaagattggaataagcatattgggaaccgccagtaatatcatcgaagttgctggaaatataatcaggcagagtttcttgtaaaaattgaataaaagaaaaatttgccaaaaaaacattcaaaacctctgggatgcaaatgcaataggttaccgcgctgcgctccaacattgttagttttgaattagtctgcaaaaataaaaaaaaaaacaagcgtcatatcatagtagcctgacgaacagatggataaatcagtctttccatcacaagacaagccacagggtctccagctcgaccctcgtaaaacctgtcatcatgattaaacaacagcaccgaaagttcctcgcggtgaccagcatgaataattcttgatgaagcatacaatccagacatgttagcatcagttaacgagaaaaaacagccaacatagcctttgggtataattatgcttaatcgtaagtatagcaaagccacccctcgcggatacaaagtaaaaggcacaggagaataaaaaatataattatttctctgctgctgttcaggcaacgtcgcccccggtccctctaaatacacatacaaagcctcatcagccatggcttaccagacaaagtacagcgggcacacaaagcacaagctctaaagtgactctccaacctctccacaatatatatatacacaagccctaaactgacgtaatgggagtaaagtgtaaaaaatcccgccaaacccaacacacaccccgaaactgcgtcaccagggaaaagtacagtttcacttccgcaatcccaacaggcgtaacttcctctttctcacggtacgtgatatcccactaacttgcaacgtcattttcccacggtcgcaccgccccttttagccgttaaccccacagccaatcaccacacgatccacactttttaaaatcacctcatttacatattggcaccattccatctataaggtatattatatagatagg

SEQ ID NO: 35 - DNA, 36280 bp, Artificial Sequence
  Plasmid pNG-62
ggcgcgcctatctatataatataccttatagatggaatggtgccaatatgtaaatgaggtgattttaaaaagtgtggatcgtgtggtgattggctgtggggttaacggctaaaaggggcggtgcgaccgtgggaaaatgacgttttgtgggggtggagtttttttgcaagttgtcgcgggaaatgtgacgcataaaaaggcttttttctcacggaactacttagttttcccacggtatttaacaggaaatgaggtagttttgaccggatgcaagtgaaaattgttgattttcgcgcgaaaactgaatgaggaagtgtttttctgaataatgtggtatttatggcagggtggagtatttgttcagggccaggtagactttgacccattacgtggaggtttcgattaccgtgttttttacctgaatttccgcgtaccgtgtcaaagtcttctgtttttacgtaggtgtcagctgatcgctagggtatttatacctcagggtttgtgtcaagaggccactcttgagtgccagcgagaagagttttctcctctgcgccggcagtttaataataaaaaaatgagagatttgcgatttctgcctcaggaaataatctctgctgagactggaaatgaaatattggagcttgtggtgcacgccctgatgggagacgatccggagccacctgtgcagctttttgagcctcctacgcttcaggaactgtatgatttagaggtagagggatcggaggattctaatgaggaagctgtaaatggcttttttaccgattctatgcttttagctgctaatgaagggttagaattagatccgcctttggacacttttgatactccaggggtaattgtggaaagcggtacaggtgtaagaaaattacctgatttgagttccgtggactgtgatttgcactgctatgaagacgggtttcctccgagtgatgaggaggaccatgaaaaggagcagtccatgcagactgcagcgggtgagggagtgaaggctgccaatgttggttttcagttggattgcccggagcttcctggacatggctgtaagtcttgtgaatttcacaggaaaaatactggagtaaaggaactgttatgttcgctttgttatatgagaacgcactgccactttatttacagtaagtgtgtttaagttaaaatttaaaggaatatgctgtttttcacatgtatattgagtgtgagttttgtgcttcttattataggtcctgtgtctgatgctgatgaatcaccatctcctgattctactacctcacctcctgagattcaagcacctgttcctgtggacgtgcgcaagcccattcctgtgaagcttaagcctgggaaacgtccagcagtggaaaaacttgaggacttgttacagggtggggacggacctttggacttgagtacacggaaacgtccaagacaataagtgttccatatccgtgtttacttaaggtgacgtcaatatttgtgtgacagtgcaatgtaataaaaatatgttaactgttcactggtttttattgctttttgggcggggactcaggtatataagtagaagcagacctgtgtggttagctcataggagctggctttcatccatggaggtttgggccattttggaagaccttaggaagactaggcaactgttagagaacgcttcggacggagtctccggtttttggagattctggttcgctagtgaattagctagggtagtttttaggataaaacaggactataaacaagaatttgaaaagttgttggtagattgcccaggactttttgaagctcttaatttgggccatcaggttcactttaaagaaaaagttttatcagttttagacttttcaaccccaggtagaactgctgctgctgtggcttttcttacttttatattagataaatggatcccgcagactcatttcagcaggggatacgttttggatttcatagccacagcattgtggagaacatggaaggttcgcaagatgaggacaatcttaggttactggccagtgcagcctttgggtgtagcgggaatcctgaggcatccaccggtcatgccagcggttctggaggaggaacagcaagaggacaacccgagagccggcctggaccctccagtggaggaggcggagtagctgacttgtctcctgaactgcaacgggtgcttactggatctacgtccactggacgggataggggcgttaagagggagagggcatctagtggtactgatgctagatctgagttggctttaagtttaatgagtcgcagacgtcctgaaaccatttggtggcatgaggttcagaaagagggaagggatgaagtttctgtattgcaggagaaatattcactggaacaggtgaaaacatgttggttggagcctgaggatgattgggaggtggccattaaaaattatgccaagatagctttgaggcctgataaacagtataagattactagacggattaatatccggaatgcttgttacatatctggaaatggggctgaggtggtaatagatactcaagacaaggcagttattagatgctgcatgatggatatgtggcctggggtagtcggtatggaagcagtaacttttgtaaatgttaagtttaggggagatggttataatggaatagtgtttatggccaataccaaacttatattgcatggttgtagcttttttggtttcaacaatacctgtgtagatgcctggggacaggttagtgtacggggatgtagtttctatgcgtgttggattgccacagctggcagaaccaagagtcaattgtctctgaagaaatgcatatttcaaagatgtaacctgggcattctgaatgaaggcgaagcaagggtccgccactgcgcttctacagatactggatgttttattttgattaagggaaatgccagcgtaaagcataacatgatttgcggtgcttccgatgagaggccttatcaaatgctcacttgtgctggtgggcattgtaatatgctggctactgtgcatattgtttcccatcaacgcaaaaaatggcctgtttttgatcacaatgtgatgacgaagtgtaccatgcatgcaggtgggcgtagaggaatgtttatgccttaccagtgtaacatgaatcatgtgaaagtgttgttggaaccagatgccttttccagaatgagcctaacaggaatttttgacatgaacatgcaaatctggaagatcctgaggtatgatgatacgagatcgagggtacgcgcatgcgaatgcggaggcaagcatgccaggttccagccggtgtgtgtagatgtgactgaagatctcagaccggatcatttggttattgcccgcactggagcagagttcggatccagtggagaagaaactgactaaggtgagtattgggaaaactttggggtgggattttcagatggacagattgagtaaaaatttgttttttctgtcttgcagctgtcatgagtggaaacgcttcttttaaggggggagtcttcagcccttatctgacagggcgtctcccatcctgggcaggagttcgtcagaatgttatgggatctactgtggatggaagacccgtccaacccgccaattcttcaacgctgacctatgctactttaagttcttcacctttggacgcagctgcagctgccgccgccgcttctgttgccgctaacactgtgcttggaatgggttactatggaagcatcatggctaattccacttcctctaataacccttctaccctgactcaggacaagttacttgtccttttggcccagctggaggctttgacccaacgtctgggtgaactttctcagcaggtggtcgagttgcgagtacaaactgagtctgctgtcggcacggcaaagtctaaataaaaaaatcccagaatcaatgaataaataaacaagcttgttgttgatttaaaatcaagtgtttttatttcatttttcgcgcacggtatgccctagaccaccgatctctatcattgagaactcggtggattttttccaggatcctatagaggtgggattgaatgtttagatacatgggcattaggccgtctttggggtggagatagctccattgaagggattcatgctccggggtagtgttgtaaatcacccagtcataacaaggtcgcagtgcatggtgttgcacaatatcttttagaagtaggctgattgccacagataagcccttggtgtaggtgtttacaaaccggttgagctgggatgggtgcattcggggtgaaattatgtgcattttggattggatttttaagttggcaatattgccgccaagatcccgtcttgggttcatgttatgaaggaccaccaagacggtgtatccggtacatttaggaaatttatcgtgcagcttggatggaaaagcgtggaaaaatttggagacacccttgtgtcctccaagattttccatgcactcatccatgataatagcaatggggccgtgggcagcggcgcgggcaaacacgttccgtgggtctgacacatcatagttatgttcctgagttaaatcatcataagccattttaatgaatttggggcggagagtaccagattggggtatgaatgttccttcgggccccggagcatagttcccctcacagatttgcatttcccaagctttcagttccgagggtggaatcatgtccacctggggggctatgaaaaacaccgtttctggggcgggggtgattaattgtgatgatagcaaatttctgagcaattgagatttgccacatccggtggggccataaatgattccgattacgggttgcaggtggtagtttagggaacggcaactgccgtcttctcgaagcaagggggccacctcgttcatcatttcccttacatgcatattttcccgcaccaaatccattaggaggcgctctcctcctagtgatagaagttcttgtagtgaggaaaagtttttcagcggtttcagaccgtcagccatgggcattttggagagagtttgctgcaaaagttctagtctgttccacagttcagtgatgtgttctatggcatctcgatccagcagacctcctcgtttcgcgggtttggacggctcctggaatagggtatgagacgatgggcgtccagcgctgccagggttcggtccttccagggtctcagtgttcgagtcagggttgtttccgtcacagtgaaggggtgtgcgcctgcttgggcgcttgccagggtgcgcttcagactcatcctgctggtcgaaaacttctgtcgcttggcgccctgtatgtcggccaagtagcagtttaccatgagttcgtagttgagcgcctcggctgcgtggcctttggcgcggagcttacctttggaagttttcttgcataccgggcagtataggcatttcagcgcatacaacttgggcgcaaggaaaacggattctggggagtatgcatctgcgccgcaggaggcgcaaacagtttcacattccaccagccaggttaaatccggttcattggggtcaaaaacaagttttccgccatattttttgatgcgtttcttacctttggtctccatgagttcgtgtcctcgttgagtgacaaacaggctgtccgtgtccccgtagactgattttacaggcctcttctccagtggagtgcctcggtcttcttcgtacaggaactctgaccactctgatacaaaggcgcgcgtccaggccagcacaaaggaggctatgtgggaggggtagcgatcgttgtcaaccagggggtccaccttttccaaagtatgcaaacacatgtcaccctcttcaacatccaggaatgtgattggcttgtaggtgtatttcacgtgacctggggtccccgctgggggggtataaaagggggcggttctttgctcttcctcactgtcttccggatcgctgtccaggaacgtcagctgttggggtaggtattccctctcgaaggcgggcatgacctctgcactcaggttgtcagtttctaagaacgaggaggatttgatattgacagtgccggttgagatgcctttcatgaggttttcgtccatctggtcagaaaacacaatttttttattgtcaagtttggtggcaaatgatccatacagggcgttggataaaagtttggcaatggatcgcatggtttggttcttttccttgtccgcgcgctctttggcggcgatgttgagttggacatactcgcgtgccaggcacttccattcggggaagatagttgttaattcatctggcacgattctcacttgccaccctcgattatgcaaggtaattaaatccacactggtggccacctcgcctcgaaggggttcattggtccaacagagcctacctcctttcctagaacagaaagggggaagtgggtctagcataagttcatcgggagggtctgcatccatggtaaagattcccggaagtaaatccttatcaaaatagctgatgggagtggggtcatctaaggccatttgccattctcgagctgccagtgcgcgctcatatgggttaaggggactgccccatggcatgggatgggtgagtgcagaggcatacatgccacagatgtcatagacgtagatgggatcctcaaagatgcctatgtaggttggatagcatcgcccccctctgatacttgctcgcacatagtcatatagttcatgtgatggcgctagcagccccggacccaagttggtgcgattgggtttttctgttctgtagacgatctggcgaaagatggcgtgagaattggaagagatggtgggtctttgaaaaatgttgaaatgggcatgaggtagacctacagagtctctgacaaagtgggcataagattcttgaagcttggttaccagttcggcggtgacaagtacgtctagggcgcagtagtcaagtgtttcttgaatgatgtcataacctggttggtttttcttttcccacagttcgcggttgagaaggtattcttcgcgatccttccagtactcttctagcggaaacccgtctttgtctgcacggtaagatcctagcatgtagaactgattaactgccttgtaagggcagcagcccttctctacgggtagagagtatgcttgagcagcttttcgtagcgaagcgtgagtaagggcaaaggtgtctctgaccatgactttgaggaattggtatttgaagtcgatgtcgtcacaggctccctgttcccagagttggaagtctacccgtttcttgtaggcggggttgggcaaagcgaaagtaacatcattgaagagaatcttgccggccctgggcatgaaattgcgagtgatgcgaaaaggctgtggtacttccgctcggttattgataacctgggcagctaggacgatctcgtcgaaaccgttgatgttgtgtcctacgatgtataattctatgaaacgcggcgtgcctctgacgtgaggtagcttactgagctcatcaaaggttaggtctgtggggtcagataaggcgtagtgttcgagagcccattcgtgcaggtgaggattcgctttaaggaaggaggaccagaggtccactgccagtgctgtttgtaactggtcccggtactgacgaaaatgccgtccgactgccattttttctggggtgacgcaatagaaggtttgggggtcctgccgccagcgatcccacttgagttttatggcgaggtcataggcgatgttgacgagccgctggtctccagagagtttcatgaccagcatgaaggggattagctgcttgccaaaggaccccatccaggtgtaggtttccacatcgtaggtgagaaagagcctttctgtgcgaggatgagagccaatcgggaagaactggatctcctgccaccagttggaggaatggctgttgatgtgatggaagtagaactccctgcgacgcgccgagcattcatgcttgtgcttgtacagacggccgcagtagtcgcagcgttgcacgggttgtatctcgtgaatgagttgtacctggcttcccttgacgagaaatttcagtgggaagccgaggcctggcgattgtatctcgtgctttactatgttgtctgcatcggcctgttcatcttctgtctcgatggtggtcatgctgacgagccctcgcgggaggcaagtccagacctcggcgcggcaggggcggagctcgaggacgagagcgcgcaggctggagctgtccagggtcctgagacgctgcggactcaggttagtaggcagtgtcaggagattaacttgcatgatcttttggagggcgtgcgggaggttcagatagtacttgatctcaacgggtccgttggtggagatgtcgatggcttgcagggttccgtgtcccttgggcgctaccaccgtgcccttgtttttcattttggacggcggtggctctgttgcttcttgcatgtttagaagcggtgtcgagggcgcgcaccgggcggcaggggcggctcgggacccggcggcatggctggcagtggtacgtcggcgccgcgcgcgggtaggttctggtactgcgccctgagaagactcgcatgcgcgacgacgcggcggttgacatcctggatctgacgcctctgggtgaaagctaccggccccgtgagcttgaacctgaaagagagttcaacagaatcaatctcggtatcgttgacggcggcttgcctaaggatttcttgcacgtcaccagagttgtcctggtaggcgatctccgccatgaactgctcgatctcttcctcttgaagatctccgcggcccgctctctcgacggtggccgcgaggtcgttggagatgcgcccaatgagttgagagaatgcattcatgcccgcctcgttccagacgcggctgtagaccacggcccccacgggatctctcgcgcgcatgaccacctgggcgaggttgagctccacgtggcgggtgaagaccgcatagttgcataggcgctggaaaaggtagttgagtgtggtggcgatgtgctcggtgacgaagaaatacatgatccatcgtctcagcggcatctcgctgacatcgcccagagcttccaagcgctccatggcctcgtagaagtccacggcaaaattaaaaaactgggagtttcgcgcggacacggtcaactcctcttccagaagacggataagttcggcgatggtggtgcgcacctcgcgctcgaaagcccctgggatttcttcctcaatctcttcttcttccactaacatctcttcctcttcaggtggggctgcaggaggagggggaacgcggcgacgccggcggcgcacgggcagacggtcgatgaatctttcaatgacctctccgcggcggcggcgcatggtttcagtgacggcgcggccgttctcgcgcggtcgcagagtaaaaacaccgccgcgcatctccttaaagtggtgactgggaggttctccgtttgggagggagagggcgctgattatacattttattaattggcccgtagggactgcacgcagagatctgatcgtgtcaagatccacgggatctgaaaacctttcgacgaaagcgtctaaccagtcacagtcacaaggtaggctgagtacggcttcttgtgggcgggggtggttatgtgttcggtctgggtcttctgtttcttcttcatctcgggaaggtgagacgatgctgctggtgatgaaattaaagtaggcagttctaagacggcggatggtggcgaggagcaccaggtctttgggtccggcttgctggatacgcaggcgattggccattccccaagcattatcctgacatctagcaagatctttgtagtagtcttgcatgagccgttctacgggcacttcttcctcacccgttctgccatgcatacgtgtgagtccaaatccgcgcattggttgtaccagtgccaagtcagctacgactctttcggcgaggatggcttgctgtacttgggtaagggtggcttgaaagtcatcaaaatccacaaagcggtggtaagctcctgtattaatggtgtaagcacagttggccatgactgaccagttaactgtctggtgaccagggcgcacgagctcggtgtatttaaggcgcgaataggcgcgggtgtcaaagatgtaatcgttgcaggtgcgcaccagatactggtaccctataagaaaatgcggcggtggttggcggtagagaggccatcgttctgtagctggagcgccaggggcgaggtcttccaacataaggcggtgatagccgtagatgtacctggacatccaggtgattcctgcggcggtagtagaagcccgaggaaactcgcgtacgcggttccaaatgttgcgtagcggcatgaagtagttcattgtaggcacggtttgaccagtgaggcgcgcgcagtcattgatgctctatagacacggagaaaatgaaagcgttcagcgactcgactccgtagcctggaggaacgtgaacgggttgggtcgcggtgtaccccggttcgagacttgtactcgagccggccggagccgcggctaacgtggtattggcactcccgtctcgacccagcctacaaaaatccaggatacggaatcgagtcgttttgctggtttccgaatggcagggaagtgagtcctattttttttttttgccgctcagatgcatcccgtgctgcgacagatgcgcccccaacaacagcccccctcgcagcagcagcagcagcaatcacaaaaggctgtccctgcaactactgcaactgccgccgtgagcggtgcgggacagcccgcctatgatctggacttggaagagggcgaaggactggcacgtctaggtgcgccttcacccgagcggcatccgcgagttcaactgaaaaaagattctcgcgaggcgtatgtgccccaacagaacctatttagagacagaagcggcgaggagccggaggagatgcgagcttcccgctttaacgcgggtcgtgagctgcgtcacggtttggaccgaagacgagtgttgcgggacgaggatttcgaagttgatgaaatgacagggatcagtcctgccagggcacacgtggctgcagccaaccttgtatcggcttacgagcagacagtaaaggaagagcgtaacttccaaaagtcttttaataatcatgtgcgaaccctgattgcccgcgaagaagttacccttggtttgatgcatttgtgggatttgatggaagctatcattcagaaccctactagcaaacctctgaccgcccagctgtttctggtggtgcaacacagcagagacaatgaggctttcagagaggcgctgctgaacatcaccgaacccgaggggagatggttgtatgatcttatcaacattctacagagtatcatagtgcaggagcggagcctgggcctggccgagaaggtggctgccatcaattactcggttttgagcttgggaaaatattacgctcgcaaaatctacaagactccatacgttcccatagacaaggaggtgaagatagatgggttctacatgcgcatgacgctcaaggtcttgaccctgagcgatgatcttggggtgtatcgcaatgacagaatgcatcgcgcggttagcgccagcaggaggcgcgagttaagcgacagggaactgatgcacagtttgcaaagagctctgactggagctggaaccgagggtgagaattacttcgacatgggagctgacttgcagtggcagcctagtcgcagggctctgagcgccgcgacggcaggatgtgagcttccttacatagaagaggcggatgaaggcgaggaggaagagggcgagtacttggaagactgatggcacaacccgtgttttttgctagatggaacagcaagcaccggatcccgcaatgcgggcggcgctgcagagccagccgtccggcattaactcctcggacgattggacccaggccatgcaacgtatcatggcgttgacgactcgcaaccccgaagcctttagacagcaaccccaggccaaccgtctatcggccatcatggaagctgtagtgccttcccgctctaatcccactcatgagaaggtcctggccatcgtgaacgcgttggtggagaacaaagctattcgtccagatgaggccggactggtatacaacgctctcttagaacgcgtggctcgctacaacagtagcaatgtgcaaaccaatttggaccgtatgataacagatgtacgcgaagccgtgtctcagcgcgaaaggttccagcgtgatgccaacctgggttcgctggtggcgttaaatgctttcttgagtactcagcctgctaatgtgccgcgtggtcaacaggattatactaactttttaagtgctttgagactgatggtatcagaagtacctcagagcgaagtgtatcagtccggtcctgattacttctttcagactagcagacagggcttgcagacggtaaatctgagccaagcttttaaaaacctttaaaggtttgtggggagtgcatgccccggtaggagaaagagcaaccgtgtctagcttgttaactccgaactcccgcctattattactgttggtagctcctttcaccgacagcggtagcatcgaccgtaattcctatttgggttacctactaaacctgtatcgcgaagccatagggcaaagtcaggtggacgagcagacctatcaagaaattacccaagtcagtcgcgctttgggacaggaagacactggcagtttggaagccactctgaacttcttgcttaccaatcggtctcaaaagatccctcctcaatatgctcttactgcggaggaggagaggatccttagatatgtgcagcagagcgtgggattgtttctgatgcaagagggggcaactccgactgcagcactggacatgacagcgcgaaatatggagcccagcatgtatgccagtaaccgacctttcattaacaaactgctggactacttgcacagagctgccgctatgaactctgattatttcaccaatgccatcttaaacccgcactggctgcccccacctggtttctacacgggcgaatatgacatgcccgaccctaatgacggatttctgtgggacgacgtggacagcgatgttttttcacctctttctgatcatcgcacgtggaaaaaggaaggcggcgatagaatgcattcttctgcatcgctgtccggggtcatgggtgctaccgcggctgagcccgagtctgcaagtccttttcctagtctacccttttctctacacagtgtacgtagcagcgaagtgggtagaataagtcgcccgagtttaatgggcgaagaggagtatctaaacgattccttgctcagaccggcaagagaaaaaaatttcccaaacaatggaatagaaagtttggtggataaaatgagtagatggaagacttatgctcaggatcacagagacgagcctgggatcatggggattacaagtagagcgagccgtagacgccagcgccatgacagacagaggggtcttgtgtgggacgatgaggattcggccgatgatagcagcgtgctggacttgggtgggagaggaaggggcaacccgtttgctcatttgcgccctcgcttgggtggtatgttgtaaaaaaaaataaaaaaaaaactcaccaaggccatggcgacgagcgtacgttcgttcttctttattatctgtgtctagtataatgaggcgagtcgtgctaggcggagcggtggtgtatccggagggtcctcctccttcgtacgagagcgtgatgcagcagcagcaggcgacggcggtgatgcaatccccactggaggctccctttgtgcctccgcgatacctggcacctacggagggcagaaacagcattcgttattcggaactggcacctcagtacgataccaccaggttgtatctggtggacaacaagtcggcggacattgcttctctgaactatcagaatgaccacagcaacttcttgaccacggtggtgcaaaacaatgactttacccctacggaagccagcacccagaccattaactttgatgaacgatcgcggtggggcggtcagctaaagaccatcatgcatactaacatgccaaacgtgaacgagtatatgtttagtaacaagttcaaagcgcgtgtgatggtgtccagaaaacctcccgacggtgctgcagttggggatacttatgatcacaagcaggatattttgaaatatgagtggttcgagtttactttgccagaaggcaacttttcagttactatgactattgatttgatgaacaatgccatcatagataattacttgaaagtgggtagacagaatggagtgcttgaaagtgacattggtgttaagttcgacaccaggaacttcaagctgggatgggatcccgaaaccaagttgatcatgcctggagtgtatacgtatgaagccttccatcctgacattgtcttactgcctggctgcggagtggattttaccgagagtcgtttgagcaaccttcttggtatcagaaaaaaacagccatttcaagagggttttaagattttgtatgaagatttagaaggtggtaatattccggccctcttggatgtagatgcctatgagaacagtaagaaagaacaaaaagccaaaatagaagctgctacagctgctgcagaagctaaggcaaacatagttgccagcgactctacaagggttgctaacgctggagaggtcagaggagacaattttgcgccaacacctgttccgactgcagaatcattattggccgatgtgtctgaaggaacggacgtgaaactcactattcaacctgtagaaaaagatagtaagaatagaagctataatgtgttggaagacaaaatcaacacagcctatcgcagttggtatctttcgtacaattatggcgatcccgaaaaaggagtgcgttcctggacattgctcaccacctcagatgtcacctgcggagcagagcaggtctactggtcgcttccagacatgatgaaggatcctgtcactttccgctccactagacaagtcagtaactaccctgtggtgggtgcagagcttatgcccgtcttctcaaagagcttctacaacgaacaagctgtgtactcccagcagctccgccagtccacctcgcttacgcacgtcttcaaccgctttcctgagaaccagattttaatccgtccgccggcgcccaccattaccaccgtcagtgaaaacgttcctgctctcacagatcacgggaccctgccgttgcgcagcagtatccggggagtccaacgtgtgaccgttactgacgccagacgccgcacctgtccctacgtgtacaaggcactgggcatagtcgcaccgcgcgtcctttcaagccgcactttctaaaaaaaaaaaaaatgtccattcttatctcgcccagtaataacaccggttggggtctgcgcgctccaagcaagatgtacggaggcgcacgcaaacgttctacccaacatcctgtccgtgttcgcggacattttcgcgctccatggggcgccctcaagggccgcactcgcgttcgaaccaccgtcgatgatgtaatcgatcaggtggttgccgacgcccgtaattatactcctactgcgcctacatctactgtggatgcagttattgacagtgtagtggctgacgctcgcaactatgctcgacgtaagagccggcgaaggcgcattgccagacgccaccgagctaccactgccatgcgagccgcaagagctctgctacgaagagctagacgcgtggggcgaagagccatgcttagggcggccagacgtgcagcttcgggcgccagcgccggcaggtcccgcaggcaagcagccgctgtcgcagcggcgactattgccgacatggcccaatcgcgaagaggcaatgtatactgggtgcgtgacgctgccaccggtcaacgtgtacccgtgcgcacccgtccccctcgcacttagaagatactgagcagtctccgatgttgtgtcccagcggcgaggatgtccaagcgcaaatacaaggaagaaatgctgcaggttatcgcacctgaagtctacggccaaccgttgaaggatgaaaaaaaaccccgcaaaatcaagcgggttaaaaaggacaaaaaagaagaggaagatggcgatgatgggctggcggagtttgtgcgcgagtttgccccacggcgacgcgtgcaatggcgtgggcgcaaagttcgacatgtgttgagacctggaacttcggtggtctttacacccggcgagcgttcaagcgctacttttaagcgttcctatgatgaggtgtacggggatgatgatattcttgagcaggcggctgaccgattaggcgagtttgcttatggcaagcgtagtagaataacttccaaggatgagacagtgtcgatacccttggatcatggaaatcccacccctagtcttaaaccggtcactttgcagcaagtgttacccgtaactccgcgaacaggtgttaaacgcgaaggtgaagatttgtatcccactatgcaactgatggtacccaaacgccagaagttggaggacgttttggagaaagtaaaagtggatccagatattcaacctgaggttaaagtgagacccattaagcaggtagcgcctggtctgggggtacaaactgtagacattaagattcccactgaaagtatggaagtgcaaactgaacccgcaaagcctactgccacctccactgaagtgcaaacggatccatggatgcccatgcctattacaactgacgccgccggtcccactcgaagatcccgacgaaagtacggtccagcaagtctgttgatgcccaattatgttgtacacccatctattattcctactcctggttaccgaggcactcgctactatcgcagccgaaacagtacctcccgccgtcgccgcaagacacctgcaaatcgcagtcgtcgccgtagacgcacaagcaaaccgactcccggcgccctggtgcggcaagtgtaccgcaatggtagtgcggaacctttgacactgccgcgtgcgcgttaccatccgagtatcatcacttaatcaatgttgccgctgcctccttgcagatatggccctcacttgtcgccttcgcgttcccatcactggttaccgaggaagaaactcgcgccgtagaagagggatgttgggacgcggaatgcgacgctacaggcgacggcgtgctatccgcaagcaattgcggggtggttttttaccagccttaattccaattatcgctgctgcaattggcgcgataccaggcatagcttccgtggcggttcaggcctcgcaacgacattgacattggaaaaaaacgtataaataaaaaaaaaaaaatacaatggactctgacactcctggtcctgtgactatgttttcttagagatggaagacatcaatttttcatccttggctccgcgacacggcacgaagccgtacatgggcacctggagcgacatcggcacgagccaactgaacgggggcgccttcaattggagcagtatctggagcgggcttaaaaattttggctcaaccataaaaacatacgggaacaaagcttggaacagcagtacaggacaggcgcttagaaataaacttaaagaccagaacttccaacaaaaagtagtcgatgggatagcttccggcatcaatggagtggtagatttggctaaccaggctgtgcagaaaaagataaacagtcgtttggacccgccgccagcaaccccaggtgaaatgcaagtggaggaagaaattcctccgccagaaaaacgaggcgacaagcgtccgcgtcccgatttggaagagacgctggtgacgcgcgtagatgaaccgccttcttatgaggaagcaacgaagcttggaatgcccaccactagaccgatagccccaatggccaccggggtgatgaaaccttctcagttgcatcgacccgtcaccttggatttgccccctccccctgctgctactgctgtacccgcttctaagcctgtcgctgccccgaaaccagtcgccgtagccaggtcacgtcccgggggcgctcctcgtccaaatgcgcactggcaaaatactctgaacagcatcgtgggtctaggcgtgcaaagtgtaaaacgccgtcgctgcttttaattaaatatggagtagcgcttaacttgcctatctgtgtatatgtgtcattacacgccgtcacagcagcagaggaaaaaaggaagaggtcgtgcgtcgacgctgagttactttcaagatggccaccccatcgatgctgccccaatgggcatacatgcacatcgccggacaggatgcttcggagtacctgagtccgggtctggtgcagttcgcccgcgccacagacacctacttcaatctgggaaataagtttagaaatcccaccgtagcgccgacccacgatgtgaccaccgaccgtagccagcggctcatgttgcgcttcgtgcccgttgaccgggaggacaatacatactcttacaaagtgcggtacaccctggccgtgggcgacaacagagtgctggatatggccagcacgttctttgacattaggggtgtgttggacagaggtcccagtttcaaaccctattctggtacggcttacaactccctggctcctaaaggcgctccaaatacatctcagtggattgcagaaggtgtaaaaaatacaactggtgaggaacacgtaacagaagaggaaaccaatactactacttacacttttggcaatgctcctgtaaaagctgaagctgaaattacaaaagaaggactcccagtaggtttggaagtttcagatgaagaaagtaaaccgatttatgctgataaaacatatcagccagaacctcagctgggagatgaaacttggactgaccttgatggaaaaaccgaaaagtatggaggcagggctctcaaacccgatactaagatgaaaccatgctacgggtcctttgccaaacctactaatgtgaaaggcggtcaggcaaaacaaaaaacaacggagcagccaaatcagaaagtcgaatatgatatcgacatggagttttttgatgcggcatcgcagaaaacaaacttaagtcctaaaattgtcatgtatgcagaaaatgtaaatttggaaactccagacactcatgtagtgtacaaacctggaacagaagacacaagttccgaagctaatttgggacaacaatctatgcccaacagacccaactacattggcttcagagataactttattggacttatgtactataacagtactggtaacatgggggtgctggctggtcaagcgtctcagttaaatgcagtggttgacttgcaggacagaaacacagaactttcttaccaactcttgcttgactctctgggcgacagaaccagatactttagcatgtggaatcaggctgtggacagttatgatcctgatgtacgtgttattgaaaatcatggtgtggaagatgaacttcccaactactgttttccactggacggcataggtgttccaacaaccagttacaaatcaatagttccaaatggagacaatgcgcctaattggaaggaacctgaagtaaatggaacaagtgagatcggacagggtaatttgtttgccatggaaattaaccttcaagccaatctatggcgaagtttcctttattccaatgtggctctatatctcccagactcgtacaaatacaccccgtccaatgtcactcttccagaaaacaaaaacacctacgactacatgaacgggcgggtggtgccgccatctctagtagacacctatgtgaacattggtgccaggtggtctctggatgccatggacaatgtcaacccattcaaccaccaccgtaacgctggcttgcgttaccgatccatgcttctgggtaacggacgttatgtgcctttccacatacaagtgcctcaaaaattcttcgctgttaaaaacctgctgcttctcccaggctcctacacttatgagtggaactttaggaaggatgtgaacatggttctacagagttccctcggtaacgacctgcgggtagatggcgccagcatcagtttcacgagcatcaacctctatgctacttttttccccatggctcacaacaccgcttccacccttgaagccatgctgcggaatgacaccaatgatcagtcattcaacgactacctatctgcagctaacatgctctaccccattcctgccaatgcaaccaatattcccatttccattccttctcgcaactgggcggctttcagaggctggtcatttaccagactgaaaaccaaagaaactccctctttggggtctggatttgacccctactttgtctattctggttctattccctacctggatggtaccttctacctgaaccacacttttaagaaggtttccatcatgtttgactcttcagtgagctggcctggaaatgacaggttactatctcctaacgaatttgaaataaagcgcactgtggatggcgaaggctacaacgtagcccaatgcaacatgaccaaagactggttcttggtacagatgctcgccaactacaacatcggctatcagggcttctacattccagaaggatacaaagatcgcatgtattcatttttcagaaacttccagcccatgagcaggcaggtggttgatgaggtcaattacaaagacttcaaggccgtcgccataccctaccaacacaacaactctggctttgtgggttacatggctccgaccatgcgccaaggtcaaccctatcccgctaactatccctatccactcattggaacaactgccgtaaatagtgttacgcagaaaaagttcttgtgtgacagaaccatgtggcgcataccgttctcgagcaacttcatgtctatgggggcccttacagacttgggacagaatatgctctatgccaactcagctcatgctctggacatgacctttgaggtggatcccatggatgagcccaccctgctttatcttctcttcgaagttttcgacgtggtcagagtgcatcagccacaccgcggcatcatcgaggcagtctacctgcgtacaccgttctcggccggtaacgctaccacgtaagaagcttcttgcttcttgcaaatagcagctgcaaccatggcctgcggatcccaaaacggctccagcgagcaagagctcagagccattgtccaagacctgggttgcggaccctattttttgggaacctacgataagcgcttcccggggttcatggcccccgataagctcgcctgtgccattgtaaatacggccggacgtgagacggggggagagcactggttggctttcggttggaacccacgttctaacacctgctacctttttgatccttttggattctcggatgatcgtctcaaacagatttaccagtttgaatatgagggtctcctgcgccgcagcgctcttgctaccaaggaccgctgtattacgctggaaaaatctacccagaccgtgcagggtccccgttctgccgcctgcggacttttctgctgcatgttccttcacgcctttgtgcactggcctgaccgtcccatggacggaaaccccaccatgaaattgctaactggagtgccaaacaacatgcttcattctcctaaagtccagcccaccctgtgtgacaatcaaaaagcactctaccattttcttaatacccattcgccttattttcgctcccatcgtacacacatcgaaagggccactgcgttcgaccgtatggatgttcaataatgactcatgtaaacaacgtgttcaataaacatcactttatttttttacatgtatcaaggctctgcattacttatttatttacaagtcgaatgggttctgacgagaatcagaatgacccgcaggcagtgatacgttgcggaactgatacttgggttgccacttgaattcgggaatcaccaacttgggaaccggtatatcgggcaggatgtcactccacagctttctggtcagctgcaaagctccaagcaggtcaggagccgaaatcttgaaatcacaattaggaccagtgctttgagcgcgagagttgcggtacaccggattgcagcactgaaacaccatcagcgacggatgtctcacgcttgccagcacggtgggatctgcaatcatgcccacatccagatcttcagcattggcaatgctgaacggggtcatcttgcaggtctgcctacccatggcgggcacccaattaggcttgtggttgcaatcgcagtgcagggggatcagtatcatcttggcctgatcctgtctgattcctggatacacggctctcatgaaagcatcatattgcttgaaagcctgctgggctttactaccctcggtataaaacatcccgcaggacctgctcgaaaactggttagctgcacagccggcatcattcacacagcagcgggcgtcattgttagctatttgcaccacacttctgccccagcggttttgggtgattttggttcgctcgggattctcctttaaggctcgttgtccgttctcgctggccacatccatctcgataatctgctccttctgaatcataatattgccatgcaggcacttcagcttgccctcataatcattgcagccatgaggccacaacgcacagcctgtacattcccaattatggtgggcgatctgagaaaaagaatgtatcattccctgcagaaatcttcccatcatcgtgctcagtgtcttgtgactagtgaaagttaactggatgcctcggtgctcctcgtttacgtactggtgacagatgcgcttgtattgttcgtgttgctcaggcattagtttaaaagaggttctaagttcgttatccagcctgtacttctccatcagcagacacatcacttccatgcctttctcccaagcagacaccaggggcaagctaatcggattcttaacagtgcaggcagcagctcctttagccagagggtcatctttagcgatcttctcaatgcttcttttgccatccttctcaacgatgcgcacgggcgggtagctgaaacccactgctacaagttgcgcctcttctctttcttcttcgctgtcttgactgatgtcttgcatggggatatgtttggtcttccttggcttctttttggggggtatcggaggaggaggactgtcgctccgttccggagacagggaggattgtgacgtttcgctcaccattaccaactgactgtcggtagaagaacctgaccccacacggcgacaggtgtttctcttcgggggcagaggtggaggcgattgcgaagggctgcggtccgacctggaaggcggatgactggcagaaccccttccgcgttcgggggtgtgctccctgtggcggtcgcttaactgatttccttcgcggctggccattgtgttctcctaggcagagaaacaacagacatggaaactcagccattgctgtcaacatcgccacgagtgccatcacatctcgtcctcagcgacgaggaaaaggagcagagcttaagcattccaccgcccagtcctgccaccacctctaccctagaagataaggaggtcgacgcatctcatgacatgcagaataaaaaagcgaaagagtctgagacagacatcgagcaagacccgggctatgtgacaccggtggaacacgaggaagagttgaaacgctttctagagagagaggatgaaaactgcccaaaacaacgagcagataactatcaccaagatgctggaaatagggatcagaacaccgactacctcatagggcttgacggggaagacgcgctccttaaacatctagcaagacagtcgctcatagtcaaggatgcattattggacagaactgaagtgcccatcagtgtggaagagctcagccgcgcctacgagcttaacctcttttcacctcgtactccccccaaacgtcagccaaacggcacctgcgagccaaatcctcgcttaaacttttatccagcttttgctgtgccagaagtactggctacctatcacatcttttttaaaaatcaaaaaattccagtctcctgccgcgctaatcgcacccgcgccgatgccctactcaatctgggacctggttcacgcttacctgatatagcttccttggaagaggttccaaagatcttcgagggtctgggcaataatgagactcgggccgcaaatgctctgcaaaagggagaaaatggcatggatgagcatcacagcgttctggtggaattggaaggcgataatgccagactcgcagtactcaagcgaagcatcgaggtcacacacttcgcatatcccgctgtcaacctgccccctaaagtcatgacggcggtcatggaccagttactcattaagcgcgcaagtcccctttcagaagacatgcatgacccagatgcctgtgatgagggtaaaccagtggtcagtgatgagcagctaacccgatggctgggcaccgactctcccagggatttggaagagcgtcgcaagcttatgatggccgtggtgctggttaccgtagaactagagtgtctccgacgtttctttaccgattcagaaaccttgcgcaaactcgaagagaatctgcactacacttttagacacggctttgtgcggcaggcatgcaagatatctaacgtggaactcaccaacctggtttcctacatgggtattctgcatgagaatcgcctaggacaaagcgtgctgcacagcaccctgaagggggaagcccgccgtgattacatccgcgattgtgtctatctgtacctgtgccacacgtggcaaaccggcatgggtgtatggcagcaatgtttagaagaacagaacttgaaagagcttgacaagctcttacagaaatctcttaaggttctgtggacagggttcgacgagcgcaccgtcgcttccgacctggcagacctcatcttcccagagcgtctcagggttactttgcgaaacggattgcctgactttatgagccagagcatgcttaacaattttcgctctttcatcctggaacgctccggtatcctgcccgccacctgctgcgcactgccctccgactttgtgcctctcacctaccgcgagtgccccccgccgctatggagtcactgctacctgttccgtctggccaactatctctcctaccactcggatgtgatcgaggatgtgagcggagacggcttgctggagtgtcactgccgctgcaatctgtgcacgccccaccggtccctagcttgcaacccccagttgatgagcgaaacccagataataggcacctttgaattgcaaggccccagcagccaaggcgatgggtcttctcctgggcaaagtttaaaactgaccccgggactgtggacctccgcctacttgcgcaagtttgctccggaagattaccacccctatgaaatcaagttctatgaggaccaatcacagcctccaaaggccgaactttcggcctgcgtcatcacccagggggcaattctggcccaattgcaagccatccaaaaatcccgccaagaatttctactgaaaaagggtaagggggtctaccttgacccccagaccggcgaggaactcaacacaaggttccctcaggatgtcccaacgacgagaaaacaagaagttgaaggtgcagccgccgcccccagaagatatggaggaagattgggacagtcaggcagaggaggcggaggaggacagtctggaggacagtctggaggaagacagtttggaggaggaaaacgaggaggcagaggaggtggaagaagtaaccgccgacaaacagttatcctcggctgcggagacaagcaacagcgctaccatctccgctccgagtcgaggaacccggcggcgtcccagcagtagatgggacgagaccggacgcttcccgaacccaaccagcgcttccaagaccggtaagaaggatcggcagggatacaagtcctggcgggggcataagaatgccatcatctcctgcttgcatgagtgcgggggcaacatatccttcacgcggcgctacttgctattccaccatggggtgaactttccgcgcaatgttttgcattactaccgtcacctccacagcccctactatagccagcaaatcccggcagtctcgacagataaagacagcggcggcgacctccaacagaaaaccagcagcggcagttagaaaatacacaacaagtgcagcaacaggaggattaaagattacagccaacgagccagcgcaaacccgagagttaagaaatcggatctttccaaccctgtatgccatcttccagcagagtcggggtcaagagcaggaactgaaaataaaaaaccgatctctgcgttcgctcaccagaagttgtttgtatcacaagagcgaagatcaacttcagcgcactctcgaggacgccgaggctctcttcaacaagtactgcgcgctgactcttaaagagtaggcagcgaccgcgcttattcaaaaaaggcgggaattacatcatcctcgacatgagtaaagaaattcccacgccttacatgtggagttatcaaccccaaatgggattggcggcaggcgcctcccaggactactccacccgcatgaattggctcagcgccgggccttctatgatttctcgagttaatgatatacgcgcctaccgaaaccaaatacttttggaacagtcagctcttaccaccacgccccgccaacaccttaatcccagaaattggcccgccgccctagtgtaccaggaaagtcccgctcccaccactgtattacttcctcgagacgcccaggccgaagtccaaatgactaatgcaggtgcgcagttagctggcggctccaccctatgtcgtcacaggcctcggcataatataaaacgcctgatgatcagaggccgaggtatccagctcaacgacgagtcggtgagctctccgcttggtctacgaccagacggaatctttcagattgccggctgcgggagatcttccttcacccctcgtcaggctgttctgactttggaaagttcgtcttcgcaaccccgctcgggcggaatcgggaccgttcaatttgtggaggagtttactccctctgtctacttcaaccccttctccggatctcctgggcattacccggacgagttcataccgaacttcgacgcgattagcgagtcagtggacggctacgattgatgtctggtgacgcggctgagctatctcggctgcgacatctagaccactgccgccgctttcgctgctttgcccgggaactcattgagttcatctacttcgaactccccaaggatcaccctcaaggtccggcccacggagtgcggatttctatcgaaggcaaaatagactctcgcctgcaacgaattttctcccagcggcccgtgctgatcgagcgagaccagggaaacaccacggtttccatctactgcatttgtaatcaccccggattgcatgaaagcctttgctgtcttatgtgtactgagtttaataaaaactgaattaagactctcctacggactgccgcttcttcaacccggattttacaaccagaagaacgaaacttttcctgtcgtccaggactctgttaacttcacctttcctactcacaaactagaagctcaacgactacaccgcttttccagaagcattttccctactaatactactttcaaaaccggaggtgagctccaaggtcttcctacagaaaacccttgggtggaagcgggccttgtagtgctaggaattcttgcgggtgggcttgtgattattctttgctacctatacacaccttgcttcactttcttagtggtgttgtggtattggtttaaaaaatggggcccatactagtcttgcttgttttactttcgcttttggaaccgggttctgccaattacgatccatgtctagacttcgacccagaaaactgcacacttacttttgcacccgacacaagccgcatctgtggagttcatcgcctctcttacgaacttggcccccaacgacaaaaatttacctgcatggtgggaatcaaccccatagttatcacccagcaaagtggagatactaagggttgcattcactgctcctgcgattccatcgagtgcacctacaccctgctgaagaccctatgcggcctaagagacctgctaccaatgaattaaaaaatgattaataaaaaatcacttacttgaaatcagcaataaggtctctgttgaaattttctcccagcagcacctcacttccctcttcccaactctggtattctaaaccccgttcagcggcatactttctccatactttaaaggggatgtcaaattttagctcctctcctgtacccacaatcttcatgtctttcttcccagatgaccaagagagtccggctcagtgactccttcaaccctgtctacccctatgaagatgaaagcacctcccaacacccctttataaacccagggtttatttccccaaatggcttcacacaaagcccaaacggagttcttactttaaaatgtttaaccccactaacaaccacaggcggatctctacagctaaaagtgggagggggacttacagtggatgacaccaacggttttttgaaagaaaacataagtgccaccacaccactcgttaagactggtcactctataggtttaccactaggagccggattgggaacgaatgaaaataaactttgtatcaaattaggacaaggacttacattcaattcaaacaacatttgcattgatgacaatattaacaccttatggacaggagtcaaccccaccgaagccaactgtcaaatcatgaactccagtgaatctaatgattgcaaattaattctaacactagttaaaactggagcactagtcactgcatttgtttatgttataggagtatctaacaattttaatatgctaactacacacagaaatataaattttactgcagagctgtttttcgattctactggtaatttactaactagactctcatccctcaaaactccacttaatcataaatcaggacaaaacatggctactggtgccattactaatgctaaaggtttcatgcccagcacgactgcctatcctttcaatgataattctagagaaaaagaaaactacatttacggaacttgttactacacagctagtgatcgcactgcttttcccattgacatatctgtcatgcttaaccgaagagcaataaatgacgagacatcatattgtattcgtataacttggtcctggaacacaggagatgccccagaggtgcaaacctctgctacaaccctagtcacctccccatttaccttttactacatcagagaagacgactgacaaataaagtttgcgatcgctgctaatcctttctctcttcaggccaccatggtgagcaagggcgaggagctgttcaccggggtggtgcccatcctggtcgagctggacggcgacgtaaacggccacaagttcagcgtgtccggcgagggcgagggcgatgccacctacggcaagctgaccctgaagttcatctgcaccaccggcaagctgcccgtgccctggcccaccctcgtgaccaccctgacctacggcgtgcagtgcttcagccgctaccccgaccacatgaagcagcacgacttcttcaagtccgccatgcccgaaggctacgtccaggagcgcaccatcttcttcaaggacgacggcaactacaagacccgcgccgaggtgaagttcgagggcgacaccctggtgaaccgcatcgagctgaagggcatcgacttcaaggaggacggcaacatcctggggcacaagctggagtacaactacaacagccacaacgtctatatcatggccgacaagcagaagaacggcatcaaggtgaacttcaagatccgccacaacatcgaggacggcagcgtgcagctcgccgaccactaccagcagaacacccccatcggcgacggccccgtgctgctgcccgacaaccactacctgagcacccagtccgccctgagcaaagaccccaacgagaagcgcgatcacatggtcctgctggagttcgtgaccgccgccgggatcactctcggcatggacgagctgtacaagtaatctagaagttgtctcctcctgcactgactgactgatacaatcgatttctggatccgcaggcctctgctagcttgactgactgagatacagcgtaccttcagctcacagacatgataagatacattgatgagtttggacaaaccacaactagaatgcagtgaaaaaaatgctttatttgtgaaatttgtgatgctattgctttatttgtaaccattataagctgcaataaacaagttaacaacaacaattgcattcattttatgtttcaggttcagggggaggtgtgggaggttttttaaagcaagtaaaacctctacaaatgtggtcctgcaggaacttgtttatttgaaaatcaattcacaaaatccgagtagttattttgcctcccccttcccatttaacagaatacaccaatctctccccacgcacagctttaaacatttggataccattagatatagacatggttttagattccacattccaaacagtttcagagcgagccaatctggggtcagtgatagataaaaatccatcgggatagtcttttaaagcgctttcacagtccaactgctgcggatgcgactccggagtctggatcacggtcatctggaagaagaacgatgggaatcataatccgaaaacggtatcggacgattgtgtctcatcaaacccacaagcagccgctgtctgcgtcgctccgtgcgactgctgtttatgggatcagggtccacagtgtcctgaagcatgattttaatagcccttaacatcaactttctggtgcgatgcgcgcagcaacgcattctgatttcactcaaatctttgcagtaggtacaacacattattacaatattgtttaataaaccataattaaaagcgctccagccaaaactcatatctgatataatcgcccctgcatgaccatcataccaaagtttaatataaattaaatgacgttccctcaaaaacacactacccacatacatgatctcttttggcatgtgcatattaacaatctgtctgtaccatggacaacgttggttaatcatgcaacccaatataaccttccggaaccacactgccaacaccgctcccccagccatgcattgaagtgaaccctgctgattacaatgacaatgaagaacccaattctctcgaccgtgaatcacttgagaatgaaaaatatctatagtggcacaacatagacataaatgcatgcatcttctcataatttttaactcctcaggatttagaaacatatcccagggaataggaagctcttgcagaacagtaaagctggcagaacaaggaagaccacgaacacaacttacactatgcatagtcatagtatcacaatctggcaacagcgggtggtcttcagtcatagaagctcgggtttcattttcctcacaacgtggtaactgggctctggtgtaagggtgatgtctggcgcatgatgtcgagcgtgcgcgcaaccttgtcataatggagttgcttcctgacattctcgtattttgtatagcaaaacgcggccctggcagaacacactcttcttcgccttctatcctgccgcttagcgtgttccgtgtgatagttcaagtacaaccacactcttaagttggtcaaaagaatgctggcttcagttgtaatcaaaactccatcgcatctaatcgttctgaggaaatcatccaagcaatgcaactggattgtgtttcaagcaggagaggagagggaagagacggaagaaccatgttaatttttattccaaacgatctcgcagtacttcaaattgtagatcgcgcagatggcatctctcgcccccactgtgttggtgaaaaagcacagctagatcaaaagaaatgcgattttcaaggtgctcaacggtggcttccagcaaagcctccacgcgcacatccaagaacaaaagaataccaaaagaaggagcattttctaactcctcaatcatcatattacattcctgcaccattcccagataattttcagctttccagccttgaattattcgtgtcagttcttgtggtaaatccaatccacacattacaaacaggtcccggagggcgccctccaccaccattcttaaacacaccctcataatgacaaaatatcttgctcctgtgtcacctgtagcgaattgagaatggcaacatcaattgacatgcccttggctctaagttcttctttaagttctagttgtaaaaactctctcatattatcaccaaactgcttagccagaagccccccgggaacaagagcaggggacgctacagtgcagtacaagcgcagacctccccaattggctccagcaaaaacaagattggaataagcatattgggaaccgccagtaatatcatcgaagttgctggaaatataatcaggcagagtttcttgtaaaaattgaataaaagaaaaatttgccaaaaaaacattcaaaacctctgggatgcaaatgcaataggttaccgcgctgcgctccaacattgttagttttgaattagtctgcaaaaataaaaaaaaaaacaagcgtcatatcatagtagcctgacgaacagatggataaatcagtctttccatcacaagacaagccacagggtctccagctcgaccctcgtaaaacctgtcatcatgattaaacaacagcaccgaaagttcctcgcggtgaccagcatgaataattcttgatgaagcatacaatccagacatgttagcatcagttaacgagaaaaaacagccaacatagcctttgggtataattatgcttaatcgtaagtatagcaaagccacccctcgcggatacaaagtaaaaggcacaggagaataaaaaatataattatttctctgctgctgttcaggcaacgtcgcccccggtccctctaaatacacatacaaagcctcatcagccatggcttaccagacaaagtacagcgggcacacaaagcacaagctctaaagtgactctccaacctctccacaatatatatatacacaagccctaaactgacgtaatgggagtaaagtgtaaaaaatcccgccaaacccaacacacaccccgaaactgcgtcaccagggaaaagtacagtttcacttccgcaatcccaacaggcgtaacttcctctttctcacggtacgtgatatcccactaacttgcaacgtcattttcccacggtcgcaccgccccttttagccgttaaccccacagccaatcaccacacgatccacactttttaaaatcacctcatttacatattggcaccattccatctataaggtatattatatagataggcgcgccctctcttaaggtagcatcgggatcgagtccctgagagaacatcctcaatcccgatctatccttagatccgaggaatatcgaaatcagttacgctagggataacagggtaatatagcatcccctcggattgctatctaccggctcgtcagctatgatctctcgatttcgatcaagaaatctcattggttaccttgggctatcgaaaccagtcaagtcagctacttggcgagatcgacttgtctgagtttcgactacgctcagaattgcgtcagcgcctatcgccaggtattactccaatcccgaatatccgagcctgagagaacatcctcaatcccgatctatccttagatccgaggaatatcgaaatcgtttaaatcttttcttgatggtaaatcattcgaatataagaatggagagacgaatggggaaacgacaaagatgacattctttggtccttctggtgaggttctcaagtttttggttaatcctgtcaacaacttatatcgtatggggctgacttcaggtgctacatttgaagagataaattgcactgaaatctagtaatattttatctgattaataagatgatcttcttgagatcgttttggtctgcgcgtaatctcttgctctgaaaacgaaaaaaccgccttgcagggcggtttttcgaaggttctctgagctaccaactctttgaaccgaggtaactggcttggcagagcgcagtcaccaaaacttgtcctttcagtttagccttaaccggcgcatgacttcaagactaactctgctaaatcaattaccagtggctgctgccagtggtgcttttgcatgtctttccgggttggactcaagacgatagttaccggataaggcgcagcggtcggactgaacggggggttcgtgcatacagtccagcttggagcgaactgcctacccggaactgagtgtcaggcgtggaatgagacaaacgcggccataacagcggaatgacaccggtaaaccgaaaggcaggaacaggagagcgcacgagggagccgccagggggaaacgcctggtatctttatagtcctgtcgggtttcgccaccactgatttgagcgtcagatttcgtgatgcttgtcaggggggcggagcctatggaaaaacggctttgccgcggccctctcacttccctgttaagtatcttcctggcatcttccaggaaatctccgccccgttcgtaagccatttccgctcgccgcagtcgaacgaccgagcgtagcgagtcagtgagcgaggaagcggaatatatcctgtatcacatattctgctgacgcaccggtgcggccttttttctcctgccacatgaagcacttcactgacaccctcatcagtgccaacatagtaagccagtatacactccgctaatttaaacgtggtgtaccgagaacgatcctctcagtgcgatctcgacgatcagtggtattccgacatatcgttgcttggcagtcagccagtcgatcctagcttgggacccaggaagtccaatcgtcagatattgtactcagcctggtcacggcagcgtaccgatctcgtaactataacggtcctaaggtagcgaactagatattgatagtctgatcggtcaacgtataatcgagtcctagcttttgcaaacatctatcaagagacaggatcagcaggaggctttcgcatgattgaacaagatggattgcacgcaggttctccggcggcttgggtggagaggctattcggctatgactgggcacaacagacaatcggctgctctgatgccgccgtgttccggctgtcagcgcaggggcgtccggttctttttgtcaagaccgacctgtccggtgccctgaatgaactgcaagacgaggcagcgcggctatcgtggctggcgacgacgggcgttccttgcgcggctgtgctcgacgttgtcactgaagcgggaagggactggctgctattgggcgaagtgccggggcaggatctcctgtcatctcaccttgctcctgccgagaaagtatccatcatggctgatgcaatgcggcggctgcatacgcttgatccggctacctgcccattcgaccaccaagcgaaacatcgcatcgagcgagcacgtactcggatggaagccggtcttgtcgatcaggatgatctggacgaagagcatcaggggctcgcgccagccgaactgttcgccaggctcaaggcgtctatgcccgacggcgaggatctcgtcgtgacccacggcgatgcctgcttgccgaatatcatggtggaaaatggccgcttttctggattcatcgactgtggccgtctgggtgtggcggaccgctatcaggacatagcgttggctacccgtgatattgctgaagagcttggcggcgaatgggctgaccgcttccttgtgctttacggtatcgccgcgcccgattcgcagcgcatcgccttctatcgccttcttgacgagttcttctgaccgattctaggtgcattggcgcagaaaaaaatgcctgatgcgacgctgcgcgtcttatactcccacatatgccagattcagcaacggatacggcttccccaacttgcccacttccatacgtgtcctccttaccagaaatttatccttaaggtccgtaactataacggtcctaaggtagcgaatcgacctagctctatcgaatctccctcgtttcgagcttacgcgaactagcctctggcgatagcatccgaggggcaggcatctatgtcgggtgcggagaaagaggtaatgtcaagttcgatctgattgcttggcataaagtccgatggttcgagtagactcagttcaacctctctcttaaggtagc

SEQ ID NO: 36 - DNA, 31 bp, Artificial Sequence
  Branched splice acceptor (bSA)
tgctaatcttcctttctctcttcaggccgcc

SEQ ID NO: 37 - DNA, 1090 bp, Artificial Sequence
  GFP Transgene Cassette
gcgatcgctgctaatcctttctctcttcaggccaccatggtgagcaagggcgaggagctgttcaccggggtggtgcccatcctggtcgagctggacggcgacgtaaacggccacaagttcagcgtgtccggcgagggcgagggcgatgccacctacggcaagctgaccctgaagttcatctgcaccaccggcaagctgcccgtgccctggcccaccctcgtgaccaccctgacctacggcgtgcagtgcttcagccgctaccccgaccacatgaagcagcacgacttcttcaagtccgccatgcccgaaggctacgtccaggagcgcaccatcttcttcaaggacgacggcaactacaagacccgcgccgaggtgaagttcgagggcgacaccctggtgaaccgcatcgagctgaagggcatcgacttcaaggaggacggcaacatcctggggcacaagctggagtacaactacaacagccacaacgtctatatcatggccgacaagcagaagaacggcatcaaggtgaacttcaagatccgccacaacatcgaggacggcagcgtgcagctcgccgaccactaccagcagaacacccccatcggcgacggccccgtgctgctgcccgacaaccactacctgagcacccagtccgccctgagcaaagaccccaacgagaagcgcgatcacatggtcctgctggagttcgtgaccgccgccgggatcactctcggcatggacgagctgtacaagtaatctagaagttgtctcctcctgcactgactgactgatacaatcgatttctggatccgcaggcctctgctagcttgactgactgagatacagcgtaccttcagctcacagacatgataagatacattgatgagtttggacaaaccacaactagaatgcagtgaaaaaaatgctttatttgtgaaatttgtgatgctattgctttatttgtaaccattataagctgcaataaacaagttaacaacaacaattgcattcattttatgtttcaggttcagggggaggtgtgggaggttttttaaagcaagtaaaacctctacaaatgtggtcctgcagg

SEQ ID NO: 38 - DNA, 33421 bp, Artificial Sequence
  NG-62 Virus genome
cgcgcctatctatataatataccttatagatggaatggtgccaatatgtaaatgaggtgattttaaaaagtgtggatcgtgtggtgattggctgtggggttaacggctaaaaggggcggtgcgaccgtgggaaaatgacgttttgtgggggtggagtttttttgcaagttgtcgcgggaaatgtgacgcataaaaaggcttttttctcacggaactacttagttttcccacggtatttaacaggaaatgaggtagttttgaccggatgcaagtgaaaattgttgattttcgcgcgaaaactgaatgaggaagtgtttttctgaataatgtggtatttatggcagggtggagtatttgttcagggccaggtagactttgacccattacgtggaggtttcgattaccgtgttttttacctgaatttccgcgtaccgtgtcaaagtcttctgtttttacgtaggtgtcagctgatcgctagggtatttatacctcagggtttgtgtcaagaggccactcttgagtgccagcgagaagagttttctcctctgcgccggcagtttaataataaaaaaatgagagatttgcgatttctgcctcaggaaataatctctgctgagactggaaatgaaatattggagcttgtggtgcacgccctgatgggagacgatccggagccacctgtgcagctttttgagcctcctacgcttcaggaactgtatgatttagaggtagagggatcggaggattctaatgaggaagctgtaaatggcttttttaccgattctatgcttttagctgctaatgaagggttagaattagatccgcctttggacacttttgatactccaggggtaattgtggaaagcggtacaggtgtaagaaaattacctgatttgagttccgtggactgtgatttgcactgctatgaagacgggtttcctccgagtgatgaggaggaccatgaaaaggagcagtccatgcagactgcagcgggtgagggagtgaaggctgccaatgttggttttcagttggattgcccggagcttcctggacatggctgtaagtcttgtgaatttcacaggaaaaatactggagtaaaggaactgttatgttcgctttgttatatgagaacgcactgccactttatttacagtaagtgtgtttaagttaaaatttaaaggaatatgctgtttttcacatgtatattgagtgtgagttttgtgcttcttattataggtcctgtgtctgatgctgatgaatcaccatctcctgattctactacctcacctcctgagattcaagcacctgttcctgtggacgtgcgcaagcccattcctgtgaagcttaagcctgggaaacgtccagcagtggaaaaacttgaggacttgttacagggtggggacggacctttggacttgagtacacggaaacgtccaagacaataagtgttccatatccgtgtttacttaaggtgacgtcaatatttgtgtgacagtgcaatgtaataaaaatatgttaactgttcactggtttttattgctttttgggcggggactcaggtatataagtagaagcagacctgtgtggttagctcataggagctggctttcatccatggaggtttgggccattttggaagaccttaggaagactaggcaactgttagagaacgcttcggacggagtctccggtttttggagattctggttcgctagtgaattagctagggtagtttttaggataaaacaggactataaacaagaatttgaaaagttgttggtagattgcccaggactttttgaagctcttaatttgggccatcaggttcactttaaagaaaaagttttatcagttttagacttttcaaccccaggtagaactgctgctgctgtggcttttcttacttttatattagataaatggatcccgcagactcatttcagcaggggatacgttttggatttcatagccacagcattgtggagaacatggaaggttcgcaagatgaggacaatcttaggttactggccagtgcagcctttgggtgtagcgggaatcctgaggcatccaccggtcatgccagcggttctggaggaggaacagcaagaggacaacccgagagccggcctggaccctccagtggaggaggcggagtagctgacttgtctcctgaactgcaacgggtgcttactggatctacgtccactggacgggataggggcgttaagagggagagggcatctagtggtactgatgctagatctgagttggctttaagtttaatgagtcgcagacgtcctgaaaccatttggtggcatgaggttcagaaagagggaagggatgaagtttctgtattgcaggagaaatattcactggaacaggtgaaaacatgttggttggagcctgaggatgattgggaggtggccattaaaaattatgccaagatagctttgaggcctgataaacagtataagattactagacggattaatatccggaatgcttgttacatatctggaaatggggctgaggtggtaatagatactcaagacaaggcagttattagatgctgcatgatggatatgtggcctggggtagtcggtatggaagcagtaacttttgtaaatgttaagtttaggggagatggttataatggaatagtgtttatggccaataccaaacttatattgcatggttgtagcttttttggtttcaacaatacctgtgtagatgcctggggacaggttagtgtacggggatgtagtttctatgcgtgttggattgccacagctggcagaaccaagagtcaattgtctctgaagaaatgcatatttcaaagatgtaacctgggcattctgaatgaaggcgaagcaagggtccgccactgcgcttctacagatactggatgttttattttgattaagggaaatgccagcgtaaagcataacatgatttgcggtgcttccgatgagaggccttatcaaatgctcacttgtgctggtgggcattgtaatatgctggctactgtgcatattgtttcccatcaacgcaaaaaatggcctgtttttgatcacaatgtgatgacgaagtgtaccatgcatgcaggtgggcgtagaggaatgtttatgccttaccagtgtaacatgaatcatgtgaaagtgttgttggaaccagatgccttttccagaatgagcctaacaggaatttttgacatgaacatgcaaatctggaagatcctgaggtatgatgatacgagatcgagggtacgcgcatgcgaatgcggaggcaagcatgccaggttccagccggtgtgtgtagatgtgactgaagatctcagaccggatcatttggttattgcccgcactggagcagagttcggatccagtggagaagaaactgactaaggtgagtattgggaaaactttggggtgggattttcagatggacagattgagtaaaaatttgttttttctgtcttgcagctgtcatgagtggaaacgcttcttttaaggggggagtcttcagcccttatctgacagggcgtctcccatcctgggcaggagttcgtcagaatgttatgggatctactgtggatggaagacccgtccaacccgccaattcttcaacgctgacctatgctactttaagttcttcacctttggacgcagctgcagctgccgccgccgcttctgttgccgctaacactgtgcttggaatgggttactatggaagcatcatggctaattccacttcctctaataacccttctaccctgactcaggacaagttacttgtccttttggcccagctggaggctttgacccaacgtctgggtgaactttctcagcaggtggtcgagttgcgagtacaaactgagtctgctgtcggcacggcaaagtctaaataaaaaaatcccagaatcaatgaataaataaacaagcttgttgttgatttaaaatcaagtgtttttatttcatttttcgcgcacggtatgccctagaccaccgatctctatcattgagaactcggtggattttttccaggatcctatagaggtgggattgaatgtttagatacatgggcattaggccgtctttggggtggagatagctccattgaagggattcatgctccggggtagtgttgtaaatcacccagtcataacaaggtcgcagtgcatggtgttgcacaatatcttttagaagtaggctgattgccacagataagcccttggtgtaggtgtttacaaaccggttgagctgggatgggtgcattcggggtgaaattatgtgcattttggattggatttttaagttggcaatattgccgccaagatcccgtcttgggttcatgttatgaaggaccaccaagacggtgtatccggtacatttaggaaatttatcgtgcagcttggatggaaaagcgtggaaaaatttggagacacccttgtgtcctccaagattttccatgcactcatccatgataatagcaatggggccgtgggcagcggcgcgggcaaacacgttccgtgggtctgacacatcatagttatgttcctgagttaaatcatcataagccattttaatgaatttggggcggagagtaccagattggggtatgaatgttccttcgggccccggagcatagttcccctcacagatttgcatttcccaagctttcagttccgagggtggaatcatgtccacctggggggctatgaaaaacaccgtttctggggcgggggtgattaattgtgatgatagcaaatttctgagcaattgagatttgccacatccggtggggccataaatgattccgattacgggttgcaggtggtagtttagggaacggcaactgccgtcttctcgaagcaagggggccacctcgttcatcatttcccttacatgcatattttcccgcaccaaatccattaggaggcgctctcctcctagtgatagaagttcttgtagtgaggaaaagtttttcagcggtttcagaccgtcagccatgggcattttggagagagtttgctgcaaaagttctagtctgttccacagttcagtgatgtgttctatggcatctcgatccagcagacctcctcgtttcgcgggtttggacggctcctggaatagggtatgagacgatgggcgtccagcgctgccagggttcggtccttccagggtctcagtgttcgagtcagggttgtttccgtcacagtgaaggggtgtgcgcctgcttgggcgcttgccagggtgcgcttcagactcatcctgctggtcgaaaacttctgtcgcttggcgccctgtatgtcggccaagtagcagtttaccatgagttcgtagttgagcgcctcggctgcgtggcctttggcgcggagcttacctttggaagttttcttgcataccgggcagtataggcatttcagcgcatacaacttgggcgcaaggaaaacggattctggggagtatgcatctgcgccgcaggaggcgcaaacagtttcacattccaccagccaggttaaatccggttcattggggtcaaaaacaagttttccgccatattttttgatgcgtttcttacctttggtctccatgagttcgtgtcctcgttgagtgacaaacaggctgtccgtgtccccgtagactgattttacaggcctcttctccagtggagtgcctcggtcttcttcgtacaggaactctgaccactctgatacaaaggcgcgcgtccaggccagcacaaaggaggctatgtgggaggggtagcgatcgttgtcaaccagggggtccaccttttccaaagtatgcaaacacatgtcaccctcttcaacatccaggaatgtgattggcttgtaggtgtatttcacgtgacctggggtccccgctgggggggtataaaagggggcggttctttgctcttcctcactgtcttccggatcgctgtccaggaacgtcagctgttggggtaggtattccctctcgaaggcgggcatgacctctgcactcaggttgtcagtttctaagaacgaggaggatttgatattgacagtgccggttgagatgcctttcatgaggttttcgtccatctggtcagaaaacacaatttttttattgtcaagtttggtggcaaatgatccatacagggcgttggataaaagtttggcaatggatcgcatggtttggttcttttccttgtccgcgcgctctttggcggcgatgttgagttggacatactcgcgtgccaggcacttccattcggggaagatagttgttaattcatctggcacgattctcacttgccaccctcgattatgcaaggtaattaaatccacactggtggccacctcgcctcgaaggggttcattggtccaacagagcctacctcctttcctagaacagaaagggggaagtgggtctagcataagttcatcgggagggtctgcatccatggtaaagattcccggaagtaaatccttatcaaaatagctgatgggagtggggtcatctaaggccatttgccattctcgagctgccagtgcgcgctcatatgggttaaggggactgccccatggcatgggatgggtgagtgcagaggcatacatgccacagatgtcatagacgtagatgggatcctcaaagatgcctatgtaggttggatagcatcgcccccctctgatacttgctcgcacatagtcatatagttcatgtgatggcgctagcagccccggacccaagttggtgcgattgggtttttctgttctgtagacgatctggcgaaagatggcgtgagaattggaagagatggtgggtctttgaaaaatgttgaaatgggcatgaggtagacctacagagtctctgacaaagtgggcataagattcttgaagcttggttaccagttcggcggtgacaagtacgtctagggcgcagtagtcaagtgtttcttgaatgatgtcataacctggttggtttttcttttcccacagttcgcggttgagaaggtattcttcgcgatccttccagtactcttctagcggaaacccgtctttgtctgcacggtaagatcctagcatgtagaactgattaactgccttgtaagggcagcagcccttctctacgggtagagagtatgcttgagcagcttttcgtagcgaagcgtgagtaagggcaaaggtgtctctgaccatgactttgaggaattggtatttgaagtcgatgtcgtcacaggctccctgttcccagagttggaagtctacccgtttcttgtaggcggggttgggcaaagcgaaagtaacatcattgaagagaatcttgccggccctgggcatgaaattgcgagtgatgcgaaaaggctgtggtacttccgctcggttattgataacctgggcagctaggacgatctcgtcgaaaccgttgatgttgtgtcctacgatgtataattctatgaaacgcggcgtgcctctgacgtgaggtagcttactgagctcatcaaaggttaggtctgtggggtcagataaggcgtagtgttcgagagcccattcgtgcaggtgaggattcgctttaaggaaggaggaccagaggtccactgccagtgctgtttgtaactggtcccggtactgacgaaaatgccgtccgactgccattttttctggggtgacgcaatagaaggtttgggggtcctgccgccagcgatcccacttgagttttatggcgaggtcataggcgatgttgacgagccgctggtctccagagagtttcatgaccagcatgaaggggattagctgcttgccaaaggaccccatccaggtgtaggtttccacatcgtaggtgagaaagagcctttctgtgcgaggatgagagccaatcgggaagaactggatctcctgccaccagttggaggaatggctgttgatgtgatggaagtagaactccctgcgacgcgccgagcattcatgcttgtgcttgtacagacggccgcagtagtcgcagcgttgcacgggttgtatctcgtgaatgagttgtacctggcttcccttgacgagaaatttcagtgggaagccgaggcctggcgattgtatctcgtgctttactatgttgtctgcatcggcctgttcatcttctgtctcgatggtggtcatgctgacgagccctcgcgggaggcaagtccagacctcggcgcggcaggggcggagctcgaggacgagagcgcgcaggctggagctgtccagggtcctgagacgctgcggactcaggttagtaggcagtgtcaggagattaacttgcatgatcttttggagggcgtgcgggaggttcagatagtacttgatctcaacgggtccgttggtggagatgtcgatggcttgcagggttccgtgtcccttgggcgctaccaccgtgcccttgtttttcattttggacggcggtggctctgttgcttcttgcatgtttagaagcggtgtcgagggcgcgcaccgggcggcaggggcggctcgggacccggcggcatggctggcagtggtacgtcggcgccgcgcgcgggtaggttctggtactgcgccctgagaagactcgcatgcgcgacgacgcggcggttgacatcctggatctgacgcctctgggtgaaagctaccggccccgtgagcttgaacctgaaagagagttcaacagaatcaatctcggtatcgttgacggcggcttgcctaaggatttcttgcacgtcaccagagttgtcctggtaggcgatctccgccatgaactgctcgatctcttcctcttgaagatctccgcggcccgctctctcgacggtggccgcgaggtcgttggagatgcgcccaatgagttgagagaatgcattcatgcccgcctcgttccagacgcggctgtagaccacggcccccacgggatctctcgcgcgcatgaccacctgggcgaggttgagctccacgtggcgggtgaagaccgcatagttgcataggcgctggaaaaggtagttgagtgtggtggcgatgtgctcggtgacgaagaaatacatgatccatcgtctcagcggcatctcgctgacatcgcccagagcttccaagcgctccatggcctcgtagaagtccacggcaaaattaaaaaactgggagtttcgcgcggacacggtcaactcctcttccagaagacggataagttcggcgatggtggtgcgcacctcgcgctcgaaagcccctgggatttcttcctcaatctcttcttcttccactaacatctcttcctcttcaggtggggctgcaggaggagggggaacgcggcgacgccggcggcgcacgggcagacggtcgatgaatctttcaatgacctctccgcggcggcggcgcatggtttcagtgacggcgcggccgttctcgcgcggtcgcagagtaaaaacaccgccgcgcatctccttaaagtggtgactgggaggttctccgtttgggagggagagggcgctgattatacattttattaattggcccgtagggactgcacgcagagatctgatcgtgtcaagatccacgggatctgaaaacctttcgacgaaagcgtctaaccagtcacagtcacaaggtaggctgagtacggcttcttgtgggcgggggtggttatgtgttcggtctgggtcttctgtttcttcttcatctcgggaaggtgagacgatgctgctggtgatgaaattaaagtaggcagttctaagacggcggatggtggcgaggagcaccaggtctttgggtccggcttgctggatacgcaggcgattggccattccccaagcattatcctgacatctagcaagatctttgtagtagtcttgcatgagccgttctacgggcacttcttcctcacccgttctgccatgcatacgtgtgagtccaaatccgcgcattggttgtaccagtgccaagtcagctacgactctttcggcgaggatggcttgctgtacttgggtaagggtggcttgaaagtcatcaaaatccacaaagcggtggtaagctcctgtattaatggtgtaagcacagttggccatgactgaccagttaactgtctggtgaccagggcgcacgagctcggtgtatttaaggcgcgaataggcgcgggtgtcaaagatgtaatcgttgcaggtgcgcaccagatactggtaccctataagaaaatgcggcggtggttggcggtagagaggccatcgttctgtagctggagcgccaggggcgaggtcttccaacataaggcggtgatagccgtagatgtacctggacatccaggtgattcctgcggcggtagtagaagcccgaggaaactcgcgtacgcggttccaaatgttgcgtagcggcatgaagtagttcattgtaggcacggtttgaccagtgaggcgcgcgcagtcattgatgctctatagacacggagaaaatgaaagcgttcagcgactcgactccgtagcctggaggaacgtgaacgggttgggtcgcggtgtaccccggttcgagacttgtactcgagccggccggagccgcggctaacgtggtattggcactcccgtctcgacccagcctacaaaaatccaggatacggaatcgagtcgttttgctggtttccgaatggcagggaagtgagtcctattttttttttttgccgctcagatgcatcccgtgctgcgacagatgcgcccccaacaacagcccccctcgcagcagcagcagcagcaatcacaaaaggctgtccctgcaactactgcaactgccgccgtgagcggtgcgggacagcccgcctatgatctggacttggaagagggcgaaggactggcacgtctaggtgcgccttcacccgagcggcatccgcgagttcaactgaaaaaagattctcgcgaggcgtatgtgccccaacagaacctatttagagacagaagcggcgaggagccggaggagatgcgagcttcccgctttaacgcgggtcgtgagctgcgtcacggtttggaccgaagacgagtgttgcgggacgaggatttcgaagttgatgaaatgacagggatcagtcctgccagggcacacgtggctgcagccaaccttgtatcggcttacgagcagacagtaaaggaagagcgtaacttccaaaagtcttttaataatcatgtgcgaaccctgattgcccgcgaagaagttacccttggtttgatgcatttgtgggatttgatggaagctatcattcagaaccctactagcaaacctctgaccgcccagctgtttctggtggtgcaacacagcagagacaatgaggctttcagagaggcgctgctgaacatcaccgaacccgaggggagatggttgtatgatcttatcaacattctacagagtatcatagtgcaggagcggagcctgggcctggccgagaaggtggctgccatcaattactcggttttgagcttgggaaaatattacgctcgcaaaatctacaagactccatacgttcccatagacaaggaggtgaagatagatgggttctacatgcgcatgacgctcaaggtcttgaccctgagcgatgatcttggggtgtatcgcaatgacagaatgcatcgcgcggttagcgccagcaggaggcgcgagttaagcgacagggaactgatgcacagtttgcaaagagctctgactggagctggaaccgagggtgagaattacttcgacatgggagctgacttgcagtggcagcctagtcgcagggctctgagcgccgcgacggcaggatgtgagcttccttacatagaagaggcggatgaaggcgaggaggaagagggcgagtacttggaagactgatggcacaacccgtgttttttgctagatggaacagcaagcaccggatcccgcaatgcgggcggcgctgcagagccagccgtccggcattaactcctcggacgattggacccaggccatgcaacgtatcatggcgttgacgactcgcaaccccgaagcctttagacagcaaccccaggccaaccgtctatcggccatcatggaagctgtagtgccttcccgctctaatcccactcatgagaaggtcctggccatcgtgaacgcgttggtggagaacaaagctattcgtccagatgaggccggactggtatacaacgctctcttagaacgcgtggctcgctacaacagtagcaatgtgcaaaccaatttggaccgtatgataacagatgtacgcgaagccgtgtctcagcgcgaaaggttccagcgtgatgccaacctgggttcgctggtggcgttaaatgctttcttgagtactcagcctgctaatgtgccgcgtggtcaacaggattatactaactttttaagtgctttgagactgatggtatcagaagtacctcagagcgaagtgtatcagtccggtcctgattacttctttcagactagcagacagggcttgcagacggtaaatctgagccaagcttttaaaaacctttaaaggtttgtggggagtgcatgccccggtaggagaaagagcaaccgtgtctagcttgttaactccgaactcccgcctattattactgttggtagctcctttcaccgacagcggtagcatcgaccgtaattcctatttgggttacctactaaacctgtatcgcgaagccatagggcaaagtcaggtggacgagcagacctatcaagaaattacccaagtcagtcgcgctttgggacaggaagacactggcagtttggaagccactctgaacttcttgcttaccaatcggtctcaaaagatccctcctcaatatgctcttactgcggaggaggagaggatccttagatatgtgcagcagagcgtgggattgtttctgatgcaagagggggcaactccgactgcagcactggacatgacagcgcgaaatatggagcccagcatgtatgccagtaaccgacctttcattaacaaactgctggactacttgcacagagctgccgctatgaactctgattatttcaccaatgccatcttaaacccgcactggctgcccccacctggtttctacacgggcgaatatgacatgcccgaccctaatgacggatttctgtgggacgacgtggacagcgatgttttttcacctctttctgatcatcgcacgtggaaaaaggaaggcggcgatagaatgcattcttctgcatcgctgtccggggtcatgggtgctaccgcggctgagcccgagtctgcaagtccttttcctagtctacccttttctctacacagtgtacgtagcagcgaagtgggtagaataagtcgcccgagtttaatgggcgaagaggagtatctaaacgattccttgctcagaccggcaagagaaaaaaatttcccaaacaatggaatagaaagtttggtggataaaatgagtagatggaagacttatgctcaggatcacagagacgagcctgggatcatggggattacaagtagagcgagccgtagacgccagcgccatgacagacagaggggtcttgtgtgggacgatgaggattcggccgatgatagcagcgtgctggacttgggtgggagaggaaggggcaacccgtttgctcatttgcgccctcgcttgggtggtatgttgtaaaaaaaaataaaaaaaaaactcaccaaggccatggcgacgagcgtacgttcgttcttctttattatctgtgtctagtataatgaggcgagtcgtgctaggcggagcggtggtgtatccggagggtcctcctccttcgtacgagagcgtgatgcagcagcagcaggcgacggcggtgatgcaatccccactggaggctccctttgtgcctccgcgatacctggcacctacggagggcagaaacagcattcgttattcggaactggcacctcagtacgataccaccaggttgtatctggtggacaacaagtcggcggacattgcttctctgaactatcagaatgaccacagcaacttcttgaccacggtggtgcaaaacaatgactttacccctacggaagccagcacccagaccattaactttgatgaacgatcgcggtggggcggtcagctaaagaccatcatgcatactaacatgccaaacgtgaacgagtatatgtttagtaacaagttcaaagcgcgtgtgatggtgtccagaaaacctcccgacggtgctgcagttggggatacttatgatcacaagcaggatattttgaaatatgagtggttcgagtttactttgccagaaggcaacttttcagttactatgactattgatttgatgaacaatgccatcatagataattacttgaaagtgggtagacagaatggagtgcttgaaagtgacattggtgttaagttcgacaccaggaacttcaagctgggatgggatcccgaaaccaagttgatcatgcctggagtgtatacgtatgaagccttccatcctgacattgtcttactgcctggctgcggagtggattttaccgagagtcgtttgagcaaccttcttggtatcagaaaaaaacagccatttcaagagggttttaagattttgtatgaagatttagaaggtggtaatattccggccctcttggatgtagatgcctatgagaacagtaagaaagaacaaaaagccaaaatagaagctgctacagctgctgcagaagctaaggcaaacatagttgccagcgactctacaagggttgctaacgctggagaggtcagaggagacaattttgcgccaacacctgttccgactgcagaatcattattggccgatgtgtctgaaggaacggacgtgaaactcactattcaacctgtagaaaaagatagtaagaatagaagctataatgtgttggaagacaaaatcaacacagcctatcgcagttggtatctttcgtacaattatggcgatcccgaaaaaggagtgcgttcctggacattgctcaccacctcagatgtcacctgcggagcagagcaggtctactggtcgcttccagacatgatgaaggatcctgtcactttccgctccactagacaagtcagtaactaccctgtggtgggtgcagagcttatgcccgtcttctcaaagagcttctacaacgaacaagctgtgtactcccagcagctccgccagtccacctcgcttacgcacgtcttcaaccgctttcctgagaaccagattttaatccgtccgccggcgcccaccattaccaccgtcagtgaaaacgttcctgctctcacagatcacgggaccctgccgttgcgcagcagtatccggggagtccaacgtgtgaccgttactgacgccagacgccgcacctgtccctacgtgtacaaggcactgggcatagtcgcaccgcgcgtcctttcaagccgcactttctaaaaaaaaaaaaaatgtccattcttatctcgcccagtaataacaccggttggggtctgcgcgctccaagcaagatgtacggaggcgcacgcaaacgttctacccaacatcctgtccgtgttcgcggacattttcgcgctccatggggcgccctcaagggccgcactcgcgttcgaaccaccgtcgatgatgtaatcgatcaggtggttgccgacgcccgtaattatactcctactgcgcctacatctactgtggatgcagttattgacagtgtagtggctgacgctcgcaactatgctcgacgtaagagccggcgaaggcgcattgccagacgccaccgagctaccactgccatgcgagccgcaagagctctgctacgaagagctagacgcgtggggcgaagagccatgcttagggcggccagacgtgcagcttcgggcgccagcgccggcaggtcccgcaggcaagcagccgctgtcgcagcggcgactattgccgacatggcccaatcgcgaagaggcaatgtatactgggtgcgtgacgctgccaccggtcaacgtgtacccgtgcgcacccgtccccctcgcacttagaagatactgagcagtctccgatgttgtgtcccagcggcgaggatgtccaagcgcaaatacaaggaagaaatgctgcaggttatcgcacctgaagtctacggccaaccgttgaaggatgaaaaaaaaccccgcaaaatcaagcgggttaaaaaggacaaaaaagaagaggaagatggcgatgatgggctggcggagtttgtgcgcgagtttgccccacggcgacgcgtgcaatggcgtgggcgcaaagttcgacatgtgttgagacctggaacttcggtggtctttacacccggcgagcgttcaagcgctacttttaagcgttcctatgatgaggtgtacggggatgatgatattcttgagcaggcggctgaccgattaggcgagtttgcttatggcaagcgtagtagaataacttccaaggatgagacagtgtcgatacccttggatcatggaaatcccacccctagtcttaaaccggtcactttgcagcaagtgttacccgtaactccgcgaacaggtgttaaacgcgaaggtgaagatttgtatcccactatgcaactgatggtacccaaacgccagaagttggaggacgttttggagaaagtaaaagtggatccagatattcaacctgaggttaaagtgagacccattaagcaggtagcgcctggtctgggggtacaaactgtagacattaagattcccactgaaagtatggaagtgcaaactgaacccgcaaagcctactgccacctccactgaagtgcaaacggatccatggatgcccatgcctattacaactgacgccgccggtcccactcgaagatcccgacgaaagtacggtccagcaagtctgttgatgcccaattatgttgtacacccatctattattcctactcctggttaccgaggcactcgctactatcgcagccgaaacagtacctcccgccgtcgccgcaagacacctgcaaatcgcagtcgtcgccgtagacgcacaagcaaaccgactcccggcgccctggtgcggcaagtgtaccgcaatggtagtgcggaacctttgacactgccgcgtgcgcgttaccatccgagtatcatcacttaatcaatgttgccgctgcctccttgcagatatggccctcacttgtcgccttcgcgttcccatcactggttaccgaggaagaaactcgcgccgtagaagagggatgttgggacgcggaatgcgacgctacaggcgacggcgtgctatccgcaagcaattgcggggtggttttttaccagccttaattccaattatcgctgctgcaattggcgcgataccaggcatagcttccgtggcggttcaggcctcgcaacgacattgacattggaaaaaaacgtataaataaaaaaaaaaaaatacaatggactctgacactcctggtcctgtgactatgttttcttagagatggaagacatcaatttttcatccttggctccgcgacacggcacgaagccgtacatgggcacctggagcgacatcggcacgagccaactgaacgggggcgccttcaattggagcagtatctggagcgggcttaaaaattttggctcaaccataaaaacatacgggaacaaagcttggaacagcagtacaggacaggcgcttagaaataaacttaaagaccagaacttccaacaaaaagtagtcgatgggatagcttccggcatcaatggagtggtagatttggctaaccaggctgtgcagaaaaagataaacagtcgtttggacccgccgccagcaaccccaggtgaaatgcaagtggaggaagaaattcctccgccagaaaaacgaggcgacaagcgtccgcgtcccgatttggaagagacgctggtgacgcgcgtagatgaaccgccttcttatgaggaagcaacgaagcttggaatgcccaccactagaccgatagccccaatggccaccggggtgatgaaaccttctcagttgcatcgacccgtcaccttggatttgccccctccccctgctgctactgctgtacccgcttctaagcctgtcgctgccccgaaaccagtcgccgtagccaggtcacgtcccgggggcgctcctcgtccaaatgcgcactggcaaaatactctgaacagcatcgtgggtctaggcgtgcaaagtgtaaaacgccgtcgctgcttttaattaaatatggagtagcgcttaacttgcctatctgtgtatatgtgtcattacacgccgtcacagcagcagaggaaaaaaggaagaggtcgtgcgtcgacgctgagttactttcaagatggccaccccatcgatgctgccccaatgggcatacatgcacatcgccggacaggatgcttcggagtacctgagtccgggtctggtgcagttcgcccgcgccacagacacctacttcaatctgggaaataagtttagaaatcccaccgtagcgccgacccacgatgtgaccaccgaccgtagccagcggctcatgttgcgcttcgtgcccgttgaccgggaggacaatacatactcttacaaagtgcggtacaccctggccgtgggcgacaacagagtgctggatatggccagcacgttctttgacattaggggtgtgttggacagaggtcccagtttcaaaccctattctggtacggcttacaactccctggctcctaaaggcgctccaaatacatctcagtggattgcagaaggtgtaaaaaatacaactggtgaggaacacgtaacagaagaggaaaccaatactactacttacacttttggcaatgctcctgtaaaagctgaagctgaaattacaaaagaaggactcccagtaggtttggaagtttcagatgaagaaagtaaaccgatttatgctgataaaacatatcagccagaacctcagctgggagatgaaacttggactgaccttgatggaaaaaccgaaaagtatggaggcagggctctcaaacccgatactaagatgaaaccatgctacgggtcctttgccaaacctactaatgtgaaaggcggtcaggcaaaacaaaaaacaacggagcagccaaatcagaaagtcgaatatgatatcgacatggagttttttgatgcggcatcgcagaaaacaaacttaagtcctaaaattgtcatgtatgcagaaaatgtaaatttggaaactccagacactcatgtagtgtacaaacctggaacagaagacacaagttccgaagctaatttgggacaacaatctatgcccaacagacccaactacattggcttcagagataactttattggacttatgtactataacagtactggtaacatgggggtgctggctggtcaagcgtctcagttaaatgcagtggttgacttgcaggacagaaacacagaactttcttaccaactcttgcttgactctctgggcgacagaaccagatactttagcatgtggaatcaggctgtggacagttatgatcctgatgtacgtgttattgaaaatcatggtgtggaagatgaacttcccaactactgttttccactggacggcataggtgttccaacaaccagttacaaatcaatagttccaaatggagacaatgcgcctaattggaaggaacctgaagtaaatggaacaagtgagatcggacagggtaatttgtttgccatggaaattaaccttcaagccaatctatggcgaagtttcctttattccaatgtggctctatatctcccagactcgtacaaatacaccccgtccaatgtcactcttccagaaaacaaaaacacctacgactacatgaacgggcgggtggtgccgccatctctagtagacacctatgtgaacattggtgccaggtggtctctggatgccatggacaatgtcaacccattcaaccaccaccgtaacgctggcttgcgttaccgatccatgcttctgggtaacggacgttatgtgcctttccacatacaagtgcctcaaaaattcttcgctgttaaaaacctgctgcttctcccaggctcctacacttatgagtggaactttaggaaggatgtgaacatggttctacagagttccctcggtaacgacctgcgggtagatggcgccagcatcagtttcacgagcatcaacctctatgctacttttttccccatggctcacaacaccgcttccacccttgaagccatgctgcggaatgacaccaatgatcagtcattcaacgactacctatctgcagctaacatgctctaccccattcctgccaatgcaaccaatattcccatttccattccttctcgcaactgggcggctttcagaggctggtcatttaccagactgaaaaccaaagaaactccctctttggggtctggatttgacccctactttgtctattctggttctattccctacctggatggtaccttctacctgaaccacacttttaagaaggtttccatcatgtttgactcttcagtgagctggcctggaaatgacaggttactatctcctaacgaatttgaaataaagcgcactgtggatggcgaaggctacaacgtagcccaatgcaacatgaccaaagactggttcttggtacagatgctcgccaactacaacatcggctatcagggcttctacattccagaaggatacaaagatcgcatgtattcatttttcagaaacttccagcccatgagcaggcaggtggttgatgaggtcaattacaaagacttcaaggccgtcgccataccctaccaacacaacaactctggctttgtgggttacatggctccgaccatgcgccaaggtcaaccctatcccgctaactatccctatccactcattggaacaactgccgtaaatagtgttacgcagaaaaagttcttgtgtgacagaaccatgtggcgcataccgttctcgagcaacttcatgtctatgggggcccttacagacttgggacagaatatgctctatgccaactcagctcatgctctggacatgacctttgaggtggatcccatggatgagcccaccctgctttatcttctcttcgaagttttcgacgtggtcagagtgcatcagccacaccgcggcatcatcgaggcagtctacctgcgtacaccgttctcggccggtaacgctaccacgtaagaagcttcttgcttcttgcaaatagcagctgcaaccatggcctgcggatcccaaaacggctccagcgagcaagagctcagagccattgtccaagacctgggttgcggaccctattttttgggaacctacgataagcgcttcccggggttcatggcccccgataagctcgcctgtgccattgtaaatacggccggacgtgagacggggggagagcactggttggctttcggttggaacccacgttctaacacctgctacctttttgatccttttggattctcggatgatcgtctcaaacagatttaccagtttgaatatgagggtctcctgcgccgcagcgctcttgctaccaaggaccgctgtattacgctggaaaaatctacccagaccgtgcagggtccccgttctgccgcctgcggacttttctgctgcatgttccttcacgcctttgtgcactggcctgaccgtcccatggacggaaaccccaccatgaaattgctaactggagtgccaaacaacatgcttcattctcctaaagtccagcccaccctgtgtgacaatcaaaaagcactctaccattttcttaatacccattcgccttattttcgctcccatcgtacacacatcgaaagggccactgcgttcgaccgtatggatgttcaataatgactcatgtaaacaacgtgttcaataaacatcactttatttttttacatgtatcaaggctctgcattacttatttatttacaagtcgaatgggttctgacgagaatcagaatgacccgcaggcagtgatacgttgcggaactgatacttgggttgccacttgaattcgggaatcaccaacttgggaaccggtatatcgggcaggatgtcactccacagctttctggtcagctgcaaagctccaagcaggtcaggagccgaaatcttgaaatcacaattaggaccagtgctttgagcgcgagagttgcggtacaccggattgcagcactgaaacaccatcagcgacggatgtctcacgcttgccagcacggtgggatctgcaatcatgcccacatccagatcttcagcattggcaatgctgaacggggtcatcttgcaggtctgcctacccatggcgggcacccaattaggcttgtggttgcaatcgcagtgcagggggatcagtatcatcttggcctgatcctgtctgattcctggatacacggctctcatgaaagcatcatattgcttgaaagcctgctgggctttactaccctcggtataaaacatcccgcaggacctgctcgaaaactggttagctgcacagccggcatcattcacacagcagcgggcgtcattgttagctatttgcaccacacttctgccccagcggttttgggtgattttggttcgctcgggattctcctttaaggctcgttgtccgttctcgctggccacatccatctcgataatctgctccttctgaatcataatattgccatgcaggcacttcagcttgccctcataatcattgcagccatgaggccacaacgcacagcctgtacattcccaattatggtgggcgatctgagaaaaagaatgtatcattccctgcagaaatcttcccatcatcgtgctcagtgtcttgtgactagtgaaagttaactggatgcctcggtgctcctcgtttacgtactggtgacagatgcgcttgtattgttcgtgttgctcaggcattagtttaaaagaggttctaagttcgttatccagcctgtacttctccatcagcagacacatcacttccatgcctttctcccaagcagacaccaggggcaagctaatcggattcttaacagtgcaggcagcagctcctttagccagagggtcatctttagcgatcttctcaatgcttcttttgccatccttctcaacgatgcgcacgggcgggtagctgaaacccactgctacaagttgcgcctcttctctttcttcttcgctgtcttgactgatgtcttgcatggggatatgtttggtcttccttggcttctttttggggggtatcggaggaggaggactgtcgctccgttccggagacagggaggattgtgacgtttcgctcaccattaccaactgactgtcggtagaagaacctgaccccacacggcgacaggtgtttctcttcgggggcagaggtggaggcgattgcgaagggctgcggtccgacctggaaggcggatgactggcagaaccccttccgcgttcgggggtgtgctccctgtggcggtcgcttaactgatttccttcgcggctggccattgtgttctcctaggcagagaaacaacagacatggaaactcagccattgctgtcaacatcgccacgagtgccatcacatctcgtcctcagcgacgaggaaaaggagcagagcttaagcattccaccgcccagtcctgccaccacctctaccctagaagataaggaggtcgacgcatctcatgacatgcagaataaaaaagcgaaagagtctgagacagacatcgagcaagacccgggctatgtgacaccggtggaacacgaggaagagttgaaacgctttctagagagagaggatgaaaactgcccaaaacaacgagcagataactatcaccaagatgctggaaatagggatcagaacaccgactacctcatagggcttgacggggaagacgcgctccttaaacatctagcaagacagtcgctcatagtcaaggatgcattattggacagaactgaagtgcccatcagtgtggaagagctcagccgcgcctacgagcttaacctcttttcacctcgtactccccccaaacgtcagccaaacggcacctgcgagccaaatcctcgcttaaacttttatccagcttttgctgtgccagaagtactggctacctatcacatcttttttaaaaatcaaaaaattccagtctcctgccgcgctaatcgcacccgcgccgatgccctactcaatctgggacctggttcacgcttacctgatatagcttccttggaagaggttccaaagatcttcgagggtctgggcaataatgagactcgggccgcaaatgctctgcaaaagggagaaaatggcatggatgagcatcacagcgttctggtggaattggaaggcgataatgccagactcgcagtactcaagcgaagcatcgaggtcacacacttcgcatatcccgctgtcaacctgccccctaaagtcatgacggcggtcatggaccagttactcattaagcgcgcaagtcccctttcagaagacatgcatgacccagatgcctgtgatgagggtaaaccagtggtcagtgatgagcagctaacccgatggctgggcaccgactctcccagggatttggaagagcgtcgcaagcttatgatggccgtggtgctggttaccgtagaactagagtgtctccgacgtttctttaccgattcagaaaccttgcgcaaactcgaagagaatctgcactacacttttagacacggctttgtgcggcaggcatgcaagatatctaacgtggaactcaccaacctggtttcctacatgggtattctgcatgagaatcgcctaggacaaagcgtgctgcacagcaccctgaagggggaagcccgccgtgattacatccgcgattgtgtctatctgtacctgtgccacacgtggcaaaccggcatgggtgtatggcagcaatgtttagaagaacagaacttgaaagagcttgacaagctcttacagaaatctcttaaggttctgtggacagggttcgacgagcgcaccgtcgcttccgacctggcagacctcatcttcccagagcgtctcagggttactttgcgaaacggattgcctgactttatgagccagagcatgcttaacaattttcgctctttcatcctggaacgctccggtatcctgcccgccacctgctgcgcactgccctccgactttgtgcctctcacctaccgcgagtgccccccgccgctatggagtcactgctacctgttccgtctggccaactatctctcctaccactcggatgtgatcgaggatgtgagcggagacggcttgctggagtgtcactgccgctgcaatctgtgcacgccccaccggtccctagcttgcaacccccagttgatgagcgaaacccagataataggcacctttgaattgcaaggccccagcagccaaggcgatgggtcttctcctgggcaaagtttaaaactgaccccgggactgtggacctccgcctacttgcgcaagtttgctccggaagattaccacccctatgaaatcaagttctatgaggaccaatcacagcctccaaaggccgaactttcggcctgcgtcatcacccagggggcaattctggcccaattgcaagccatccaaaaatcccgccaagaatttctactgaaaaagggtaagggggtctaccttgacccccagaccggcgaggaactcaacacaaggttccctcaggatgtcccaacgacgagaaaacaagaagttgaaggtgcagccgccgcccccagaagatatggaggaagattgggacagtcaggcagaggaggcggaggaggacagtctggaggacagtctggaggaagacagtttggaggaggaaaacgaggaggcagaggaggtggaagaagtaaccgccgacaaacagttatcctcggctgcggagacaagcaacagcgctaccatctccgctccgagtcgaggaacccggcggcgtcccagcagtagatgggacgagaccggacgcttcccgaacccaaccagcgcttccaagaccggtaagaaggatcggcagggatacaagtcctggcgggggcataagaatgccatcatctcctgcttgcatgagtgcgggggcaacatatccttcacgcggcgctacttgctattccaccatggggtgaactttccgcgcaatgttttgcattactaccgtcacctccacagcccctactatagccagcaaatcccggcagtctcgacagataaagacagcggcggcgacctccaacagaaaaccagcagcggcagttagaaaatacacaacaagtgcagcaacaggaggattaaagattacagccaacgagccagcgcaaacccgagagttaagaaatcggatctttccaaccctgtatgccatcttccagcagagtcggggtcaagagcaggaactgaaaataaaaaaccgatctctgcgttcgctcaccagaagttgtttgtatcacaagagcgaagatcaacttcagcgcactctcgaggacgccgaggctctcttcaacaagtactgcgcgctgactcttaaagagtaggcagcgaccgcgcttattcaaaaaaggcgggaattacatcatcctcgacatgagtaaagaaattcccacgccttacatgtggagttatcaaccccaaatgggattggcggcaggcgcctcccaggactactccacccgcatgaattggctcagcgccgggccttctatgatttctcgagttaatgatatacgcgcctaccgaaaccaaatacttttggaacagtcagctcttaccaccacgccccgccaacaccttaatcccagaaattggcccgccgccctagtgtaccaggaaagtcccgctcccaccactgtattacttcctcgagacgcccaggccgaagtccaaatgactaatgcaggtgcgcagttagctggcggctccaccctatgtcgtcacaggcctcggcataatataaaacgcctgatgatcagaggccgaggtatccagctcaacgacgagtcggtgagctctccgcttggtctacgaccagacggaatctttcagattgccggctgcgggagatcttccttcacccctcgtcaggctgttctgactttggaaagttcgtcttcgcaaccccgctcgggcggaatcgggaccgttcaatttgtggaggagtttactccctctgtctacttcaaccccttctccggatctcctgggcattacccggacgagttcataccgaacttcgacgcgattagcgagtcagtggacggctacgattgatgtctggtgacgcggctgagctatctcggctgcgacatctagaccactgccgccgctttcgctgctttgcccgggaactcattgagttcatctacttcgaactccccaaggatcaccctcaaggtccggcccacggagtgcggatttctatcgaaggcaaaatagactctcgcctgcaacgaattttctcccagcggcccgtgctgatcgagcgagaccagggaaacaccacggtttccatctactgcatttgtaatcaccccggattgcatgaaagcctttgctgtcttatgtgtactgagtttaataaaaactgaattaagactctcctacggactgccgcttcttcaacccggattttacaaccagaagaacgaaacttttcctgtcgtccaggactctgttaacttcacctttcctactcacaaactagaagctcaacgactacaccgcttttccagaagcattttccctactaatactactttcaaaaccggaggtgagctccaaggtcttcctacagaaaacccttgggtggaagcgggccttgtagtgctaggaattcttgcgggtgggcttgtgattattctttgctacctatacacaccttgcttcactttcttagtggtgttgtggtattggtttaaaaaatggggcccatactagtcttgcttgttttactttcgcttttggaaccgggttctgccaattacgatccatgtctagacttcgacccagaaaactgcacacttacttttgcacccgacacaagccgcatctgtggagttcatcgcctctcttacgaacttggcccccaacgacaaaaatttacctgcatggtgggaatcaaccccatagttatcacccagcaaagtggagatactaagggttgcattcactgctcctgcgattccatcgagtgcacctacaccctgctgaagaccctatgcggcctaagagacctgctaccaatgaattaaaaaatgattaataaaaaatcacttacttgaaatcagcaataaggtctctgttgaaattttctcccagcagcacctcacttccctcttcccaactctggtattctaaaccccgttcagcggcatactttctccatactttaaaggggatgtcaaattttagctcctctcctgtacccacaatcttcatgtctttcttcccagatgaccaagagagtccggctcagtgactccttcaaccctgtctacccctatgaagatgaaagcacctcccaacacccctttataaacccagggtttatttccccaaatggcttcacacaaagcccaaacggagttcttactttaaaatgtttaaccccactaacaaccacaggcggatctctacagctaaaagtgggagggggacttacagtggatgacaccaacggttttttgaaagaaaacataagtgccaccacaccactcgttaagactggtcactctataggtttaccactaggagccggattgggaacgaatgaaaataaactttgtatcaaattaggacaaggacttacattcaattcaaacaacatttgcattgatgacaatattaacaccttatggacaggagtcaaccccaccgaagccaactgtcaaatcatgaactccagtgaatctaatgattgcaaattaattctaacactagttaaaactggagcactagtcactgcatttgtttatgttataggagtatctaacaattttaatatgctaactacacacagaaatataaattttactgcagagctgtttttcgattctactggtaatttactaactagactctcatccctcaaaactccacttaatcataaatcaggacaaaacatggctactggtgccattactaatgctaaaggtttcatgcccagcacgactgcctatcctttcaatgataattctagagaaaaagaaaactacatttacggaacttgttactacacagctagtgatcgcactgcttttcccattgacatatctgtcatgcttaaccgaagagcaataaatgacgagacatcatattgtattcgtataacttggtcctggaacacaggagatgccccagaggtgcaaacctctgctacaaccctagtcacctccccatttaccttttactacatcagagaagacgactgacaaataaagtttgcgatcgctgctaatcctttctctcttcaggccaccatggtgagcaagggcgaggagctgttcaccggggtggtgcccatcctggtcgagctggacggcgacgtaaacggccacaagttcagcgtgtccggcgagggcgagggcgatgccacctacggcaagctgaccctgaagttcatctgcaccaccggcaagctgcccgtgccctggcccaccctcgtgaccaccctgacctacggcgtgcagtgcttcagccgctaccccgaccacatgaagcagcacgacttcttcaagtccgccatgcccgaaggctacgtccaggagcgcaccatcttcttcaaggacgacggcaactacaagacccgcgccgaggtgaagttcgagggcgacaccctggtgaaccgcatcgagctgaagggcatcgacttcaaggaggacggcaacatcctggggcacaagctggagtacaactacaacagccacaacgtctatatcatggccgacaagcagaagaacggcatcaaggtgaacttcaagatccgccacaacatcgaggacggcagcgtgcagctcgccgaccactaccagcagaacacccccatcggcgacggccccgtgctgctgcccgacaaccactacctgagcacccagtccgccctgagcaaagaccccaacgagaagcgcgatcacatggtcctgctggagttcgtgaccgccgccgggatcactctcggcatggacgagctgtacaagtaatctagaagttgtctcctcctgcactgactgactgatacaatcgatttctggatccgcaggcctctgctagcttgactgactgagatacagcgtaccttcagctcacagacatgataagatacattgatgagtttggacaaaccacaactagaatgcagtgaaaaaaatgctttatttgtgaaatttgtgatgctattgctttatttgtaaccattataagctgcaataaacaagttaacaacaacaattgcattcattttatgtttcaggttcagggggaggtgtgggaggttttttaaagcaagtaaaacctctacaaatgtggtcctgcaggaacttgtttatttgaaaatcaattcacaaaatccgagtagttattttgcctcccccttcccatttaacagaatacaccaatctctccccacgcacagctttaaacatttggataccattagatatagacatggttttagattccacattccaaacagtttcagagcgagccaatctggggtcagtgatagataaaaatccatcgggatagtcttttaaagcgctttcacagtccaactgctgcggatgcgactccggagtctggatcacggtcatctggaagaagaacgatgggaatcataatccgaaaacggtatcggacgattgtgtctcatcaaacccacaagcagccgctgtctgcgtcgctccgtgcgactgctgtttatgggatcagggtccacagtgtcctgaagcatgattttaatagcccttaacatcaactttctggtgcgatgcgcgcagcaacgcattctgatttcactcaaatctttgcagtaggtacaacacattattacaatattgtttaataaaccataattaaaagcgctccagccaaaactcatatctgatataatcgcccctgcatgaccatcataccaaagtttaatataaattaaatgacgttccctcaaaaacacactacccacatacatgatctcttttggcatgtgcatattaacaatctgtctgtaccatggacaacgttggttaatcatgcaacccaatataaccttccggaaccacactgccaacaccgctcccccagccatgcattgaagtgaaccctgctgattacaatgacaatgaagaacccaattctctcgaccgtgaatcacttgagaatgaaaaatatctatagtggcacaacatagacataaatgcatgcatcttctcataatttttaactcctcaggatttagaaacatatcccagggaataggaagctcttgcagaacagtaaagctggcagaacaaggaagaccacgaacacaacttacactatgcatagtcatagtatcacaatctggcaacagcgggtggtcttcagtcatagaagctcgggtttcattttcctcacaacgtggtaactgggctctggtgtaagggtgatgtctggcgcatgatgtcgagcgtgcgcgcaaccttgtcataatggagttgcttcctgacattctcgtattttgtatagcaaaacgcggccctggcagaacacactcttcttcgccttctatcctgccgcttagcgtgttccgtgtgatagttcaagtacaaccacactcttaagttggtcaaaagaatgctggcttcagttgtaatcaaaactccatcgcatctaatcgttctgaggaaatcatccaagcaatgcaactggattgtgtttcaagcaggagaggagagggaagagacggaagaaccatgttaatttttattccaaacgatctcgcagtacttcaaattgtagatcgcgcagatggcatctctcgcccccactgtgttggtgaaaaagcacagctagatcaaaagaaatgcgattttcaaggtgctcaacggtggcttccagcaaagcctccacgcgcacatccaagaacaaaagaataccaaaagaaggagcattttctaactcctcaatcatcatattacattcctgcaccattcccagataattttcagctttccagccttgaattattcgtgtcagttcttgtggtaaatccaatccacacattacaaacaggtcccggagggcgccctccaccaccattcttaaacacaccctcataatgacaaaatatcttgctcctgtgtcacctgtagcgaattgagaatggcaacatcaattgacatgcccttggctctaagttcttctttaagttctagttgtaaaaactctctcatattatcaccaaactgcttagccagaagccccccgggaacaagagcaggggacgctacagtgcagtacaagcgcagacctccccaattggctccagcaaaaacaagattggaataagcatattgggaaccgccagtaatatcatcgaagttgctggaaatataatcaggcagagtttcttgtaaaaattgaataaaagaaaaatttgccaaaaaaacattcaaaacctctgggatgcaaatgcaataggttaccgcgctgcgctccaacattgttagttttgaattagtctgcaaaaataaaaaaaaaaacaagcgtcatatcatagtagcctgacgaacagatggataaatcagtctttccatcacaagacaagccacagggtctccagctcgaccctcgtaaaacctgtcatcatgattaaacaacagcaccgaaagttcctcgcggtgaccagcatgaataattcttgatgaagcatacaatccagacatgttagcatcagttaacgagaaaaaacagccaacatagcctttgggtataattatgcttaatcgtaagtatagcaaagccacccctcgcggatacaaagtaaaaggcacaggagaataaaaaatataattatttctctgctgctgttcaggcaacgtcgcccccggtccctctaaatacacatacaaagcctcatcagccatggcttaccagacaaagtacagcgggcacacaaagcacaagctctaaagtgactctccaacctctccacaatatatatatacacaagccctaaactgacgtaatgggagtaaagtgtaaaaaatcccgccaaacccaacacacaccccgaaactgcgtcaccagggaaaagtacagtttcacttccgcaatcccaacaggcgtaacttcctctttctcacggtacgtgatatcccactaacttgcaacgtcattttcccacggtcgcaccgccccttttagccgttaaccccacagccaatcaccacacgatccacactttttaaaatcacctcatttacatattggcaccattccatctataaggtatattatatagatagg

SEQ ID NO: 39 - DNA, 54 bp, Artificial Sequence
  primer 350
tatgcgatcgctgctaatcctttctctcttcaggccaccatggtgagcaagggc

SEQ ID NO: 40 - DNA, 46 bp, Artificial Sequence
  primer 323
ctgaagagagaaactacctgcaggaccacatttgtagaggttttac

SEQ ID NO: 41 - DNA, 22 bp, Artificial Sequence
  Restriction site
caaaacgtcgtgagacagtttg

SEQ ID NO: 42 - DNA, 27 bp, Artificial Sequence
  Restriction site
taactataacggtcctaaggtagcgaa

SEQ ID NO: 43 - DNA, 18 bp, Artificial Sequence
  Restriction site
tagggataacagggtaat